European Patent Application EP 4 285 914 A2, published December 6, 2023. Title: Oncolytic Virotherapy and Immunotherapy. Applicant: Bayor College of Medicine. Application EP. The sequence listing filed with the application follows.

SEQUENCE LISTING (131 sequences)

SEQ ID NO: 1 - protein, 446 aa, synthetic construct
QVQLQESGPGLVKPSETLSLTCTVSGGSISSSSYYWGWIRQPPGKGLEWIGSIYYSGSTYYNPSLKSRVTISVDTSKNQFSLKLSSVTAADTAVYYCARYAPDSSGYLVAFDIWGQGTMVTVSSGGGGSGGGGSGGGGSQTVVTQEPSFSVSPGGTVTLTCGLSSGSVSTGYYPSWYQQTPGQAPRTLIYSTNSRSSGVPDRFSGSILGNKAALTITGAQADDESDYYCVLYMGSGISVFGGGTKLTVLGSEPKSCDKTHTCPTRFWVLVVVGGVLACYSLLVTVAFIIFWVRSKRSRLLHSDYMNMTPRRPGPTRKHYQPYAPPRDFAAYRSRVKFSRSADAPAYQQGQNQLYNELNLGRREEYDVLDKRRGRDPEMGGKPQRRKNPQEGLYNELQKDKMAEAYSEIGMKGERRRGKGHDGLYQGLSTATKDTYDALHMQALPPR

SEQ ID NO: 2 - protein, 444 aa, synthetic construct
QVQLQQWGAGLLKPSETLSLTCAVYGGSFSGYYWSWIRQPPGKGLEWIGEINHSGSTNYNPSLKSRVTISVDTSKNQFSLKLSSVTTADTAVYYCARMGINSGGYLYGMDVWGQGTTVTVSSGGGGSGGGGSGGGGSQTVVTQEPSFSVSPGGTVTLTCGLSSGSVSTSYYPSWYQQIPGQAPRTLIYTTNIRSSGVPDRFGGSILGNKAALTITGAQAEDESDYYCMLYMGSGIWVFGGGTKLTVLGSEPKSCDKTHTCPTRFWVLVVVGGVLACYSLLVTVAFIIFWVRSKRSRLLHSDYMNMTPRRPGPTRKHYQPYAPPRDFAAYRSRVKFSRSADAPAYQQGQNQLYNELNLGRREEYDVLDKRRGRDPEMGGKPQRRKNPQEGLYNELQKDKMAEAYSEIGMKGERRRGKGHDGLYQGLSTATKDTYDALHMQALPPR

SEQ ID NO: 3 - protein, 445 aa, synthetic construct
QVQLVESGPGLVKPSGTLSLTCAVSGGSISSSNWWSWVRQPPGKGLEWIGEIYHSGSTNYNPSLKSRVTISVDTSKNQFSLKLSSVTAADTAVYYCARMGANSGGYLYGMDVWGQGTTVTVSSGGGGSGGGGSGGGGSQTVVTQEPSFSVSPGGTVTLTCGLSSGSVSTSYYPSWYQQTPGQAPRTLIYSTNTRSSGVPDRFSGSILGNKAALTITGAQADDESDYYCVLYMGSGIWVFGGGTKLTVLGSEPKSCDKTHTCPTRFWVLVVVGGVLACYSLLVTVAFIIFWVRSKRSRLLHSDYMNMTPRRPGPTRKHYQPYAPPRDFAAYRSRVKFSRSADAPAYQQGQNQLYNELNLGRREEYDVLDKRRGRDPEMGGKPQRRKNPQEGLYNELQKDKMAEAYSEIGMKGERRRGKGHDGLYQGLSTATKDTYDALHMQALPPR

SEQ ID NO: 4 - protein, 439 aa, synthetic construct
QLVQSGTEVKKPGASVRVSCKSSGYTFTSYYIHWVRQAPGQGLEWMAIINPGNGDTNYAQRFQGRVTMTRDTSTSTVYMELRSLRSDDTAVYFCAREIASYSGSYYDYWGQGTLVTVSSGGGGSGGGGSGGGGSQAVVLQEPSLSVSPGGTVTLTCGLSSGSVSTGHYASWYQQTPGQAPRTLFYNTNTRSSGVPDRFSGSIVGNKAALTITGAQADDESDYYCVLYVGDGIWVFGGGTKLTVLEPKSCDKTHTCPTRFWVLVVVGGVLACYSLLVTVAFIIFWVRSKRSRLLHSDYMNMTPRRPGPTRKHYQPYAPPRDFAAYRSRVKFSRSADAPAYQQGQNQLYNELNLGRREEYDVLDKRRGRDPEMGGKPQRRKNPQEGLYNELQKDKMAEAYSEIGMKGERRRGKGHDGLYQGLSTATKDTYDALHMQALPPR

SEQ ID NO: 5 - protein, 27 aa, synthetic construct
FWVLVVVGGVLACYSLLVTVAFIIFWV

SEQ ID NO: 6 - protein, 41 aa, synthetic construct
RSKRSRLLHSDYMNMTPRRPGPTRKHYQPYAPPRDFAAYRS

SEQ ID NO: 7 - protein, 113 aa, synthetic construct
RVKFSRSADAPAYQQGQNQLYNELNLGRREEYDVLDKRRGRDPEMGGKPQRRKNPQEGLYNELQKDKMAEAYSEIGMKGERRRGKGHDGLYQGLSTATKDTYDALHMQALPPR

SEQ ID NO: 8 - protein, 14 aa, synthetic construct
EPKSCDKTHTCPTR

SEQ ID NO: 9 - protein, 14 aa, synthetic construct
GLSSGSVSTGYYPS

SEQ ID NO: 10 - protein, 7 aa, synthetic construct
STNSRSS

SEQ ID NO: 11 - protein, 10 aa, synthetic construct
VLYMGSGISV

SEQ ID NO: 12 - protein, 7 aa, synthetic construct
SSSYYWG

SEQ ID NO: 13 - protein, 16 aa, synthetic construct
SIYYSGSTYYNPSLKS

SEQ ID NO: 14 - protein, 14 aa, synthetic construct
YAPDSSGYLVAFDI

SEQ ID NO: 15 - protein, 112 aa, synthetic construct
QTVVTQEPSFSVSPGGTVTLTCGLSSGSVSTGYYPSWYQQTPGQAPRTLIYSTNSRSSGVPDRFSGSILGNKAALTITGAQADDESDYYCVLYMGSGISVFGGGTKLTVLGS

SEQ ID NO: 16 - protein, 124 aa, synthetic construct
QVQLQESGPGLVKPSETLSLTCTVSGGSISSSSYYWGWIRQPPGKGLEWIGSIYYSGSTYYNPSLKSRVTISVDTSKNQFSLKLSSVTAADTAVYYCARYAPDSSGYLVAFDIWGQGTMVTVSS

SEQ ID NO: 17 - protein, 14 aa, synthetic construct
GLSSGSVSTSYYPS

SEQ ID NO: 18 - protein, 7 aa, synthetic construct
TTNIRSS

SEQ ID NO: 19 - protein, 10 aa, synthetic construct
MLYMGSGIWV

SEQ ID NO: 20 - protein, 6 aa, synthetic construct
SGYYWS

SEQ ID NO: 21 - protein, 16 aa, synthetic construct
EINHSGSTNYNPSLKS

SEQ ID NO: 22 - protein, 14 aa, synthetic construct
MGINSGGYLYGMDV

SEQ ID NO: 23 - protein, 112 aa, synthetic construct
QTVVTQEPSFSVSPGGTVTLTCGLSSGSVSTSYYPSWYQQIPGQAPRTLIYTTNIRSSGVPDRFGGSILGNKAALTITGAQAEDESDYYCMLYMGSGIWVFGGGTKLTVLGS

SEQ ID NO: 24 - protein, 122 aa, synthetic construct
QVQLQQWGAGLLKPSETLSLTCAVYGGSFSGYYWSWIRQPPGKGLEWIGEINHSGSTNYNPSLKSRVTISVDTSKNQFSLKLSSVTTADTAVYYCARMGINSGGYLYGMDVWGQGTTVTVSS

SEQ ID NO: 25 - protein, 14 aa, synthetic construct
GLSSGSVSTSYYPS

SEQ ID NO: 26 - protein, 7 aa, synthetic construct
STNTRSS

SEQ ID NO: 27 - protein, 10 aa, synthetic construct
VLYMGSGIWV

SEQ ID NO: 28 - protein, 6 aa, synthetic construct
SSNWWS

SEQ ID NO: 29 - protein, 16 aa, synthetic construct
EIYHSGSTNYNPSLKS

SEQ ID NO: 30 - protein, 14 aa, synthetic construct
MGANSGGYLYGMDV

SEQ ID NO: 31 - protein, 112 aa, synthetic construct
QTVVTQEPSFSVSPGGTVTLTCGLSSGSVSTSYYPSWYQQTPGQAPRTLIYSTNTRSSGVPDRFSGSILGNKAALTITGAQADDESDYYCVLYMGSGIWVFGGGTKLTVLGS

SEQ ID NO: 32 - protein, 123 aa, synthetic construct
QVQLVESGPGLVKPSGTLSLTCAVSGGSISSSNWWSWVRQPPGKGLEWIGEIYHSGSTNYNPSLKSRVTISVDTSKNQFSLKLSSVTAADTAVYYCARMGANSGGYLYGMDVWGQGTTVTVSS

SEQ ID NO: 33 - protein, 14 aa, synthetic construct
GLSSGSVSTGHYAS

SEQ ID NO: 34 - protein, 7 aa, synthetic construct
NTNTRSS

SEQ ID NO: 35 - protein, 10 aa, synthetic construct
VLYVGDGIWV

SEQ ID NO: 36 - protein, 10 aa, synthetic construct
SYYIHWVRQA

SEQ ID NO: 37 - protein, 17 aa, synthetic construct
IINPGNGDTNYAQRFQG

SEQ ID NO: 38 - protein, 12 aa, synthetic construct
EIASYSGSYYDY

SEQ ID NO: 39 - protein, 110 aa, synthetic construct
QAVVLQEPSLSVSPGGTVTLTCGLSSGSVSTGHYASWYQQTPGQAPRTLFYNTNTRSSGVPDRFSGSIVGNKAALTITGAQADDESDYYCVLYVGDGIWVFGGGTKLTVL

SEQ ID NO: 40 - protein, 121 aa, synthetic construct
EVQLVQSGTEVKKPGASVRVSCKSSGYTFTSYYIHWVRQAPGQGLEWMAIINPGNGDTNYAQRFQGRVTMTRDTSTSTVYMELRSLRSDDTAVYFCAREIASYSGSYYDYWGQGTLVTVSS

SEQ ID NO: 41 - protein, 536 aa, synthetic construct
MGHQQLVISWFSLVFLASPLVAIWELKKDVYVVELDWYPDAPGEMVVLTCDTPEEDGITWTLDQSSEVLGSGKTLTIQVKEFGDAGQYTCHKGGEVLSHSLLLLHKKEDGIWSTDILKDQKEPKNKTFLRCEAKNYSGRFTCWWLTTISTDLTFSVKSSRGSSDPQGVTCGAATLSAERVRGDNKEYEYSVECQEDSACPAAEESLPIEVMVDAVHKLKYENYTSSFFIRDIIKPDPPKNLQLKPLKNSRQVEVSWEYPDTWSTPHSYFSLTFCVQVQGKSKREKKDRVFTDKTSATVICRKNASISVRAQDRYYSSSWSEWASVPCSVPGVGVPGVGARNLPVATPDPGMFPCLHHSQNLLRAVSNMLQKARQTLEFYPCTSEEIDHEDITKDKTSTVEACLPLELTKNESCLNSRETSFITNGSCLASRKTSFMMALCLSSIYEDLKMYQVEFKTMNAKLLMDPKRQIFLDQNMLAVIDELMQALNFNSETVPQKSSLEEPDFYKTKIKLCILLHAFRIRAVTIDRVMSYLNAS

SEQ ID NO: 42 - protein, 376 aa, synthetic construct
MASYPGHQHASAFDQAARSRGHSNRRTALRPRRQQEATEVRPEQKMPTLLRVYIDGPHGMGKTTTTQLLVALGSRDDIVYVPEPMTYWRVLGASETIANIYTTQHRLDQGEISAGDAAVVMTSAQITMGMPYAVTDAVLAPHIGGEAGSSHAPPPALTLIFDRHPIAALLCYPAARYLMGSMTPQAVLAFVALIPPTLPGTNIVLGALPEDRHIDRLAKRQRPGERLDLAMLAAIRRVYGLLANTVRYLQGGGSWREDWGQLSGTAVPPQGAEPQSNAGPRPHIGDTLFTLFRAPELLAPNGDLYNVFAWALDVLAKRLRPMHVFILDYDQSPAGCRDALLQLTSGMIQTHVTTPGSIPTICDLARTFAREMGEAN

SEQ ID NO: 43 - protein, 481 aa, synthetic construct
EVQLVQSGAEVKKPGASVKVSCKASGGTFSSYAISWVRQAPGQGLEWMGRIIPILGIANYAQKFQGRVTITADKSTSTAYMELSSLRSEDTAVYYCARSGHGYSYGAFDYWGQGTLVTVSSGGGGSGGGGSGGGGSQSVLTQPPSVSGAPGQRVTISCTGSSSNIGAGYDVHWYQQLPGTAPKLLIYGNSNRPSGVPDRFSGSKSGTSASLAITGLQAEDEADYYCQSYDSSLSGSYVVFGGGTKLTVLEAKSCDKTHTCPPCPAPELLGGPSVFLFPPKPKDTLMISRTPEVTCVVVDVSHEDPEVKFNWYVDGVEVHNAKTKPREEQYNSTYRVVSVLTVLHQDWLNGKEYKCKVSNKALPAPIEKTISKAKGQPREPQVYTLPPSRDELTKNQVSLTCLVKGFYPSDIAVEWESNGQPENNYKTTPPVLDSDGSFFLYSKLTVDKSRWQQGNVFSCSVMHEALHNHYTQKSLSLSPGK

SEQ ID NO: 44 - protein, 14 aa, synthetic construct
TGSSSNIGAGYDVH

SEQ ID NO: 45 - protein, 7 aa, synthetic construct
GNSNRPS

SEQ ID NO: 46 - protein, 13 aa, synthetic construct
QSYDSSLSGSYVV

SEQ ID NO: 47 - protein, 5 aa, synthetic construct
SYAIS

SEQ ID NO: 48 - protein, 17 aa, synthetic construct
RIIPILGIANYAQKFQG

SEQ ID NO: 49 - protein, 12 aa, synthetic construct
SGHGYSYGAFDY

SEQ ID NO: 50 - protein, 113 aa, synthetic construct
QSVLTQPPSVSGAPGQRVTISCTGSSSNIGAGYDVHWYQQLPGTAPKLLIYGNSNRPSGVPDRFSGSKSGTSASLAITGLQAEDEADYYCQSYDSSLSGSYVVFGGGTKLTVL

SEQ ID NO: 51 - protein, 121 aa, synthetic construct
EVQLVQSGAEVKKPGASVKVSCKASGGTFSSYAISWVRQAPGQGLEWMGRIIPILGIANYAQKFQGRVTITADKSTSTAYMELSSLRSEDTAVYYCARSGHGYSYGAFDYWGQGTLVTVSS

SEQ ID NO: 52 - protein, 473 aa, synthetic construct
EVQLVESGGGLVQPGGSLRLSCAASGFTFSDSWIHWVRQAPGKGLEWVAWISPYGGSTYYADSVKGRFTISADTSKNTAYLQMNSLRAEDTAVYYCARRHWPGGFDYWGQGTLVTVSAGGGGSGGGGSGGGGSDIQMTQSPSSLSASVGDRVTITCRASQDVSTAVAWYQQKPGKAPKLLIYSASFLYSGVPSRFSGSGSGTDFTLTISSLQPEDFATYYCQQYLYHPATFGQGTKVEIKREAKSCDKTHTCPPCPAPELLGGPSVFLFPPKPKDTLMISRTPEVTCVVVDVSHEDPEVKFNWYVDGVEVHNAKTKPREEQYNSTYRVVSVLTVLHQDWLNGKEYKCKVSNKALPAPIEKTISKAKGQPREPQVYTLPPSRDELTKNQVSLTCLVKGFYPSDIAVEWESNGQPENNYKTTPPVLDSDGSFFLYSKLTVDKSRWQQGNVFSCSVMHEALHNHYTQKSLSLSPGK

SEQ ID NO: 53 - protein, 6 aa, synthetic construct
QDVSTA

SEQ ID NO: 54 - skipped

SEQ ID NO: 55 - protein, 9 aa, synthetic construct
QQYLYHPAT

SEQ ID NO: 56 - protein, 8 aa, synthetic construct
GFTFSDSW

SEQ ID NO: 57 - protein, 8 aa, synthetic construct
ISPYGGST

SEQ ID NO: 58 - protein, 11 aa, synthetic construct
ARRHWPGGFDY

SEQ ID NO: 59 - protein, 107 aa, synthetic construct [sequence omitted]

SEQ ID NO: 60 - protein, 117 aa, synthetic construct
EVQLVESGGGLVQPGGSLRLSCAASGFTFSDSWIHWVRQAPGKGLEWVAWISPYGGSTYYADSVKGRFTISADTSKNTAYLQMNSLRAEDTAVYYCARRHWPGGFDYWGQGTLVTVS

SEQ ID NO: 61 - protein, 10 aa, synthetic construct
KSCDKTHTCP

SEQ ID NO: 62 - protein, 113 aa, synthetic construct
PCPAPELLGGPSVFLFPPKPKDTLMISRTPEVTCVVVDVSHEDPEVKFNWYVDGVEVHNAKTKPREEQYNSTYRVVSVLTVLHQDWLNGKEYKCKVSNKALPAPIEKTISKAK

SEQ ID NO: 63 - protein, 107 aa, synthetic construct
GQPREPQVYTLPPSRDELTKNQVSLTCLVKGFYPSDIAVEWESNGQPENNYKTTPPVLDSDGSFFLYSKLTVDKSRWQQGNVFSCSVMHEALHNHYTQKSLSLSPGK

SEQ ID NO: 64 - protein, 487 aa, synthetic construct
EIVLTQSPATLSLSPGERATLSCSASSSINYIYWLQQKPGQAPRILIYLTSNLASGVPARFSGSGSGTDFTLTISSLEPEDFAVYYCLQWSSNPLTFGGGTKVEIKRGGGGSGGGGSGGGGSGGGGSEVQLVESGGGLVKPGGSLRLSCAASGFTFSSYDMSWVRQAPGKGLEWVSTISSGGSYTYYLDSIKGRFTISRDNAKNSLYLQMNSLRAEDTAVYYCARQGLDYWGRGTLVTVSSGGGGGSDIKLQQSGAELARPGASVKMSCKTSGYTFTRYTMHWVKQRPGQGLEWIGYINPSRGYTNYNQKFKDKATLTTDKSSSTAYMQLSSLTSEDSAVYYCARYYDDHYCLDYWGQGTTLTVSSGGGGSGGGGSGGGGSDIQLTQSPAIMSASPGEKVTMTCRASSSVSYMNWYQQKSGTSPKRWIYDTSKVASGVPYRFSGSGSGTSYSLTISSMEAEDAATYYCQQWSSNPLTFGAGTKLELK

SEQ ID NO: 65 - protein, 241 aa, synthetic construct
EIVLTQSPATLSLSPGERATLSCSASSSINYIYWLQQKPGQAPRILIYLTSNLASGVPARFSGSGSGTDFTLTISSLEPEDFAVYYCLQWSSNPLTFGGGTKVEIKRGGGGSGGGGSGGGGSGGGGSEVQLVESGGGLVKPGGSLRLSCAASGFTFSSYDMSWVRQAPGKGLEWVSTISSGGSYTYYLDSIKGRFTISRDNAKNSLYLQMNSLRAEDTAVYYCARQGLDYWGRGTLVTVSS

SEQ ID NO: 66 - protein, 5 aa, synthetic construct
SSINY

SEQ ID NO: 67 - skipped

SEQ ID NO: 68 - protein, 9 aa, synthetic construct
LQWSSNPLT

SEQ ID NO: 69 - protein, 8 aa, synthetic construct
GFTFSSYD

SEQ ID NO: 70 - protein, 8 aa, synthetic construct
ISSGGSYT

SEQ ID NO: 71 - protein, 7 aa, synthetic construct
ARQGLDY

SEQ ID NO: 72 - protein, 106 aa, synthetic construct
EIVLTQSPATLSLSPGERATLSCSASSSINYIYWLQQKPGQAPRILIYLTSNLASGVPARFSGSGSGTDFTLTISSLEPEDFAVYYCLQWSSNPLTFGGGTKVEIK

SEQ ID NO: 73 - protein, 114 aa, synthetic construct
EVQLVESGGGLVKPGGSLRLSCAASGFTFSSYDMSWVRQAPGKGLEWVSTISSGGSYTYYLDSIKGRFTISRDNAKNSLYLQMNSLRAEDTAVYYCARQGLDYWGRGTLVTVSS

SEQ ID NO: 74 - protein, 240 aa, synthetic construct
DIKLQQSGAELARPGASVKMSCKTSGYTFTRYTMHWVKQRPGQGLEWIGYINPSRGYTNYNQKFKDKATLTTDKSSSTAYMQLSSLTSEDSAVYYCARYYDDHYCLDYWGQGTTLTVSSGGGGSGGGGSGGGGSDIQLTQSPAIMSASPGEKVTMTCRASSSVSYMNWYQQKSGTSPKRWIYDTSKVASGVPYRFSGSGSGTSYSLTISSMEAEDAATYYCQQWSSNPLTFGAGTKLELK

SEQ ID NO: 75 - protein, 5 aa, synthetic construct
SSVSY

SEQ ID NO: 76 - skipped

SEQ ID NO: 77 - protein, 9 aa, synthetic construct
QQWSSNPLT

SEQ ID NO: 78 - protein, 8 aa, synthetic construct
GYTFTRYT

SEQ ID NO: 79 - protein, 8 aa, synthetic construct
INPSRGYT

SEQ ID NO: 80 - protein, 12 aa, synthetic construct
ARYYDDHYCLDY

SEQ ID NO: 81 - protein, 106 aa, synthetic construct
DIQLTQSPAIMSASPGEKVTMTCRASSSVSYMNWYQQKSGTSPKRWIYDTSKVASGVPYRFSGSGSGTSYSLTISSMEAEDAATYYCQQWSSNPLTFGAGTKLELK

SEQ ID NO: 82 - protein, 119 aa, synthetic construct
DIKLQQSGAELARPGASVKMSCKTSGYTFTRYTMHWVKQRPGQGLEWIGYINPSRGYTNYNQKFKDKATLTTDKSSSTAYMQLSSLTSEDSAVYYCARYYDDHYCLDYWGQGTTLTVSS

SEQ ID NO: 83 - protein, 488 aa, synthetic construct
EVQLQQSGPELKKPGETVKISCKASGYPFTNYGMNWVKQAPGQGLKWMGWINTSTGESTFADDFKGRFDFSLETSANTAYLQINNLKSEDMATYFCARWEVYHGYVPYWGQGTTVTVSSGGGGSGGGGSGGGGSDIQLTQSHKFLSTSVGDRVSITCKASQDVYNAVAWYQQKPGQSPKLLIYSASSRYTGVPSRFTGSGSGPDFTFTISSVQAEDLAVYFCQQHFRTPFTFGSGTKLEIKALGGGGSDIKLQQSGAELARPGASVKMSCKTSGYTFTRYTMHWVKQRPGQGLEWIGYINPSRGYTNYNQKFKDKATLTTDKSSSTAYMQLSSLTSEDSAVYYCARYYDDHYCLDYWGQGTTLTVSSGGGGSGGGGSGGGGSDIQLTQSPAIMSASPGEKVTMTCRASSSVSYMNWYQQKSGTSPKRWIYDTSKVASGVPYRFSGSGSGTSYSLTISSMEAEDAATYYCQQWSSNPLTFGAGTKLELK

SEQ ID NO: 84 - protein, 241 aa, synthetic construct
EVQLQQSGPELKKPGETVKISCKASGYPFTNYGMNWVKQAPGQGLKWMGWINTSTGESTFADDFKGRFDFSLETSANTAYLQINNLKSEDMATYFCARWEVYHGYVPYWGQGTTVTVSSGGGGSGGGGSGGGGSDIQLTQSHKFLSTSVGDRVSITCKASQDVYNAVAWYQQKPGQSPKLLIYSASSRYTGVPSRFTGSGSGPDFTFTISSVQAEDLAVYFCQQHFRTPFTFGSGTKLEIK

SEQ ID NO: 85 - protein, 6 aa, synthetic construct
QDVYNA

SEQ ID NO: 86 - skipped

SEQ ID NO: 87 - protein, 9 aa, synthetic construct
QQHFRTPFT

SEQ ID NO: 88 - protein, 8 aa, synthetic construct
GYPFTNYG

SEQ ID NO: 89 - protein, 8 aa, synthetic construct
INTSTGES

SEQ ID NO: 90 - protein, 12 aa, synthetic construct
ARWEVYHGYVPY

SEQ ID NO: 91 - protein, 107 aa, synthetic construct
DIQLTQSHKFLSTSVGDRVSITCKASQDVYNAVAWYQQKPGQSPKLLIYSASSRYTGVPSRFTGSGSGPDFTFTISSVQAEDLAVYFCQQHFRTPFTFGSGTKLEIK

SEQ ID NO: 92 - protein, 119 aa, synthetic construct
EVQLQQSGPELKKPGETVKISCKASGYPFTNYGMNWVKQAPGQGLKWMGWINTSTGESTFADDFKGRFDFSLETSANTAYLQINNLKSEDMATYFCARWEVYHGYVPYWGQGTTVTVSS

SEQ ID NO: 93 - protein, 488 aa, synthetic construct
DIQMTQTTSSLSASLGDRVTISCRASQDISKYLNWYQQKPDGTVKLLIYHTSRLHSGVPSRFSGSGSGTDYSLTISNLEQEDIATYFCQQGNTLPYTFGGGTKLEITGGGGSGGGGSGGGGSEVKLQESGPGLVAPSQSLSVTCTVSGVSLPDYGVSWIRQPPRKGLEWLGVIWGSETTYYNSALKSRLTIIKDNSKSQVFLKMNSLQTDDTAIYYCAKHYYYGGSYAMDYWGQGTSVTVSSGGGGGSDIKLQQSGAELARPGASVKMSCKTSGYTFTRYTMHWVKQRPGQGLEWIGYINPSRGYTNYNQKFKDKATLTTDKSSSTAYMQLSSLTSEDSAVYYCARYYDDHYCLDYWGQGTTLTVSSGGGGSGGGGSGGGGSDIQLTQSPAIMSASPGEKVTMTCRASSSVSYMNWYQQKSGTSPKRWIYDTSKVASGVPYRFSGSGSGTSYSLTISSMEAEDAATYYCQQWSSNPLTFGAGTKLELK

SEQ ID NO: 94 - protein, 242 aa, synthetic construct
DIQMTQTTSSLSASLGDRVTISCRASQDISKYLNWYQQKPDGTVKLLIYHTSRLHSGVPSRFSGSGSGTDYSLTISNLEQEDIATYFCQQGNTLPYTFGGGTKLEITGGGGSGGGGSGGGGSEVKLQESGPGLVAPSQSLSVTCTVSGVSLPDYGVSWIRQPPRKGLEWLGVIWGSETTYYNSALKSRLTIIKDNSKSQVFLKMNSLQTDDTAIYYCAKHYYYGGSYAMDYWGQGTSVTVSS

SEQ ID NO: 95 - protein, 6 aa, synthetic construct
QDISKY

SEQ ID NO: 96 - skipped

SEQ ID NO: 97 - protein, 9 aa, synthetic construct
QQGNTLPYT

SEQ ID NO: 98 - protein, 8 aa, synthetic construct
GVSLPDYG

SEQ ID NO: 99 - protein, 7 aa, synthetic construct
IWGSETT

SEQ ID NO: 100 - protein, 14 aa, synthetic construct
AKHYYYGGSYAMDY

SEQ ID NO: 101 - protein, 107 aa, synthetic construct
DIQMTQTTSSLSASLGDRVTISCRASQDISKYLNWYQQKPDGTVKLLIYHTSRLHSGVPSRFSGSGSGTDYSLTISNLEQEDIATYFCQQGNTLPYTFGGGTKLEIT

SEQ ID NO: 102 - protein, 120 aa, synthetic construct
EVKLQESGPGLVAPSQSLSVTCTVSGVSLPDYGVSWIRQPPRKGLEWLGVIWGSETTYYNSALKSRLTIIKDNSKSQVFLKMNSLQTDDTAIYYCAKHYYYGGSYAMDYWGQGTSVTVSS

SEQ ID NO: 103 - protein, 1014 aa, synthetic construct
EIVLTQSPATLSLSPGERATLSCSASSSINYIYWLQQKPGQAPRILIYLTSNLASGVPARFSGSGSGTDFTLTISSLEPEDFAVYYCLQWSSNPLTFGGGTKVEIKRGGGGSGGGGSGGGGSGGGGSEVQLVESGGGLVKPGGSLRLSCAASGFTFSSYDMSWVRQAPGKGLEWVSTISSGGSYTYYLDSIKGRFTISRDNAKNSLYLQMNSLRAEDTAVYYCARQGLDYWGRGTLVTVSSGGGGGSDIKLQQSGAELARPGASVKMSCKTSGYTFTRYTMHWVKQRPGQGLEWIGYINPSRGYTNYNQKFKDKATLTTDKSSSTAYMQLSSLTSEDSAVYYCARYYDDHYCLDYWGQGTTLTVSSGGGGSGGGGSGGGGSDIQLTQSPAIMSASPGEKVTMTCRASSSVSYMNWYQQKSGTSPKRWIYDTSKVASGVPYRFSGSGSGTSYSLTISSMEAEDAATYYCQQWSSNPLTFGAGTKLELKSEGRGSLLTCGDVEENPGPSMDWIWRILFLVGAATGAHSEVQLQQSGPELKKPGETVKISCKASGYPFTNYGMNWVKQAPGQGLKWMGWINTSTGESTFADDFKGRFDFSLETSANTAYLQINNLKSEDMATYFCARWEVYHGYVPYWGQGTTVTVSSGGGGSGGGGSGGGGSDIQLTQSHKFLSTSVGDRVSITCKASQDVYNAVAWYQQKPGQSPKLLIYSASSRYTGVPSRFTGSGSGPDFTFTISSVQAEDLAVYFCQQHFRTPFTFGSGTKLEIKALGGGGSDIKLQQSGAELARPGASVKMSCKTSGYTFTRYTMHWVKQRPGQGLEWIGYINPSRGYTNYNQKFKDKATLTTDKSSSTAYMQLSSLTSEDSAVYYCARYYDDHYCLDYWGQGTTLTVSSGGGGSGGGGSGGGGSDIQLTQSPAIMSASPGEKVTMTCRASSSVSYMNWYQQKSGTSPKRWIYDTSKVASGVPYRFSGSGSGTSYSLTISSMEAEDAATYYCQQWSSNPLTFGAGTKLELK

SEQ ID NO: 104 - protein, 281 aa, synthetic construct
MRHIICHGGVITEEMAASLLDQLIEEVLADNLPPPSHFEPPTLHELYDLDVTAPEDPNEEAVSQIFPESVMLAVQEGIDLFTFPPAPGSPEPPHLSRQPEQPEQRALGPVSMPNLVPEVIDPPSDDEDEEGEEFVLDYVEHPGHGCRSCHYHRRNTGDPDIMCSLCYMRTCGMFVYSPVSEPEPEPEPEPEPARPTRRPKLVPAILRRPTSPVSRECNSSTDSCDSGPSNTPPEIHPVVPLCPIKPVAVRVGGRRQAVECIEDLLNESGQPLDLSCKRPRP

SEQ ID NO: 105 - protein, 8 aa, synthetic construct
LTCHEACF

SEQ ID NO: 106 - protein, 19 aa, synthetic construct
MDWIWRILFLVGAATGAHS

SEQ ID NO: 107 - protein, 20 aa, synthetic construct
MEAPAQLLFLLLLWLPDTTG

SEQ ID NO: 108 - protein, 22 aa, synthetic construct
MGHQQLVISWFSLVFLASPLVA

SEQ ID NO: 109 - protein, 5 aa, synthetic construct
GGGGS

SEQ ID NO: 110 - protein, 10 aa, synthetic construct
GGGGSGGGGS

SEQ ID NO: 111 - protein, 15 aa, synthetic construct
GGGGSGGGGSGGGGS

SEQ ID NO: 112 - protein, 20 aa, synthetic construct
GGGGSGGGGSGGGGSGGGGS

SEQ ID NO: 113 - protein, 9 aa, synthetic construct
YPYDVPDYA

SEQ ID NO: 114 - protein, 29 aa, synthetic construct
YPYDVPDYAGYPYDVPDYAGYPYDVPDYA

SEQ ID NO: 115 - protein, 18 aa, synthetic construct
EGRGSLLTCGDVEENPGP

SEQ ID NO: 116 - protein, 7 aa, synthetic construct
  VARIANT 1: note = X is V or I
  VARIANT 3: note = X is S or E
XEXNPGP

SEQ ID NO: 117 - DNA, 3750 bp, synthetic construct
  source 1..3750: mol_type = other DNA
aagttcagatcaaggtcaggaacagatggaacagctgaatatgggccaaacaggatatctgtggtaagcagttcctgccccggctcagggccaagaacagatggaacagctgaatatgggccaaacaggatatctgtggtaagcagttcctgccccggctcagggccaagaacagatggtccccagatgcggtccagccctcagcagtttctagagaaccatcagatgtttccagggtgccccaaggacctgaaatgaccctgtgccttatttgaactaaccaatcagttcgcttctcgcttctgttcgcgcgcttctgctccccgagctcaataaaagagcccacaacccctcactcggcgcgccagtcctccgattgactgagtcgcccgggtacccgtgtatccaataaaccctcttgcagttgcatccgacttgtggtctcgctgttccttgggagggtctcctctgagtgattgactacccgtcagcgggggtctttcatttgggggctcgtccgggatcgggagacccctgcccagggaccaccgacccaccaccgggaggtaagctggccagcaacttatctgtgtctgtccgattgtctagtgtctatgactgattttatgcgcctgcgtcggtactagttagctaactagctctgtatctggcggacccgtggtggaactgacgagttcggaacacccggccgcaaccctgggagacgtcccagggacttcgggggccgtttttgtggcccgacctgagtcctaaaatcccgatcgtttaggactctttggtgcaccccccttagaggagggatatgtggttctggtaggagacgagaacctaaaacagttcccgcctccgtctgaatttttgctttcggtttgggaccgaagccgcgccgcgcgtcttgtctgctgcagcatcgttctgtgttgtctctgtctgactgtgtttctgtatttgtctgaaaatatgggcccgggctagcctgttaccactcccttaagtttgaccttaggtcactggaaagatgtcgagcggatcgctcacaaccagtcggtagatgtcaagaagagacgttgggttaccttctgctctgcagaatggccaacctttaacgtcggatggccgcgagacggcacctttaaccgagacctcatcacccaggttaagatcaaggtcttttcacctggcccgcatggacacccagaccaggtcccctacatcgtgacctgggaagccttggcttttgacccccctccctgggtcaagccctttgtacaccctaagcctccgcctcctcttcctccatccgccccgtctctcccccttgaacctcctcgttcgaccccgcctcgatcctccctttatccagccctcactccttctctaggcgcccccatatggccatatgagatcttatatggggcacccccgccccttgtaaacttccctgaccctgacatgacaagagttactaacagcccctctctccaagctcacttacaggctctctacttagtccagcacgaagtctggagacctctggcggcagcctaccaagaacaactggaccgaccggtggtacctcacccttaccgagtcggcgacacagtgtgggtccgccgacaccagactaagaacctagaacctcgctggaaaggaccttacacagtcctgctgaccacccccaccgccctcaaagtagacggcatcgcagcttggatacacgccgcccacgtgaaggctgccgaccccgggggtggaccatgactcgagccatggattggatctggcgcatcctgtttctcgtgggagctgccacaggcgcccattctcaggttcagctgcaagagtctggccctggcctggtcaagcctagcgaaacactgagcctgacctgtaccgtgtctggcggcagcatcagcagcagctcttactactggggctggatcagacagcctcctggcaaaggcctggaatggatcggctccatctactacagcggcagcacctactacaaccccagcctgaagtccagagtgaccatcagcgtggacaccagcaagaaccagttctccctgaagctgagcagcgtgacagccgccgatacagccgtgtactactgtgccagatacgcccctgatagcagcggctacctggtggcctttgatatctggggccagggcacaatggtcaccgtttctagcggaggcggaggttctggtggcggaggaagtggcggcggaggatctcagacagtggtcacacaagagcccagcttctccgtgtctcctggcggaacagtgaccctgacatgtggccttagctctggctctgtgtccaccggctactaccccagctggtatcagcagacacctggacaggcccctcggacactgatctacagcaccaacagcagatccagcggcgtgcccgatagattcagcggctctatcctgggcaacaaggccgcactgacaatcacaggcgctcaggccgatgacgagagcgactactactgcgtgctgtacatgggcagcggcatctccgtttttggcggaggcacaaagctgaccgtgctgggatccgaaccaaagagttgcgacaaaacacacacctgccctacgcgtttttgggtgctcgtggtggtgggtggcgtgctcgcttgctactcacttctggtgaccgtagcgtttatcattttttgggtcaggagcaagcgatcccgcctattgcacagcgactacatgaacatgaccccccggcgccccgggccaacccggaagcactaccagccatatgcgcctccccgcgatttcgcagcgtatcggtcccgggtcaaattttcacggtccgctgacgccccggcctatcaacagggccagaatcagctgtataatgaattaaacctcggtagacgcgaggagtacgacgtcctcgacaagagaagggggcgcgacccagagatgggaggcaaaccgcagcgcaggaagaatccacaggagggcctgtacaacgaattacagaaggacaagatggcagaggcctacagcgagataggaatgaagggtgaaaggcgtcgtggaaagggccacgatgggctttaccagggcctaagtactgccacaaaagatacgtatgacgcgctgcatatgcaagccctcccccccaggtaagcatgcaacctcgatccggattagtccaatttgttaaagacaggatatcagtggtccaggctctagttttgactcaacaatatcaccagctgaagcctatagagtacgagccatagataaaataaaagattttatttagtctccagaaaaaggggggaatgaaagaccccacctgtaggtttggcaagctagcttaagtaacgccattttgcaaggcatggaaaaatacataactgagaatagagaagttcagatcaaggtcaggaacagatggaacagctgaatatgggccaaacaggatatctgtggtaagcagttcctgccccggctcagggccaagaacagatggaacagctgaatatgggccaaacaggatatctgtggtaagcagttcctgccccggctcagggccaagaacagatggtccccagatgcggtccagccctcagcagtttctagagaaccatcagatgtttccagggtgccccaaggacctgaaatgaccctgtgccttatttgaactaaccaatcagttcgcttctcgcttctgttcgcgcgcttc

SEQ ID NO: 118 - DNA, 3744 bp, synthetic construct
  source 1..3744: mol_type = other DNA
aagttcagatcaaggtcaggaacagatggaacagctgaatatgggccaaacaggatatctgtggtaagcagttcctgccccggctcagggccaagaacagatggaacagctgaatatgggccaaacaggatatctgtggtaagcagttcctgccccggctcagggccaagaacagatggtccccagatgcggtccagccctcagcagtttctagagaaccatcagatgtttccagggtgccccaaggacctgaaatgaccctgtgccttatttgaactaaccaatcagttcgcttctcgcttctgttcgcgcgcttctgctccccgagctcaataaaagagcccacaacccctcactcggcgcgccagtcctccgattgactgagtcgcccgggtacccgtgtatccaataaaccctcttgcagttgcatccgacttgtggtctcgctgttccttgggagggtctcctctgagtgattgactacccgtcagcgggggtctttcatttgggggctcgtccgggatcgggagacccctgcccagggaccaccgacccaccaccgggaggtaagctggccagcaacttatctgtgtctgtccgattgtctagtgtctatgactgattttatgcgcctgcgtcggtactagttagctaactagctctgtatctggcggacccgtggtggaactgacgagttcggaacacccggccgcaaccctgggagacgtcccagggacttcgggggccgtttttgtggcccgacctgagtcctaaaatcccgatcgtttaggactctttggtgcaccccccttagaggagggatatgtggttctggtaggagacgagaacctaaaacagttcccgcctccgtctgaatttttgctttcggtttgggaccgaagccgcgccgcgcgtcttgtctgctgcagcatcgttctgtgttgtctctgtctgactgtgtttctgtatttgtctgaaaatatgggcccgggctagcctgttaccactcccttaagtttgaccttaggtcactggaaagatgtcgagcggatcgctcacaaccagtcggtagatgtcaagaagagacgttgggttaccttctgctctgcagaatggccaacctttaacgtcggatggccgcgagacggcacctttaaccgagacctcatcacccaggttaagatcaaggtcttttcacctggcccgcatggacacccagaccaggtcccctacatcgtgacctgggaagccttggcttttgacccccctccctgggtcaagccctttgtacaccctaagcctccgcctcctcttcctccatccgccccgtctctcccccttgaacctcctcgttcgaccccgcctcgatcctccctttatccagccctcactccttctctaggcgcccccatatggccatatgagatcttatatggggcacccccgccccttgtaaacttccctgaccctgacatgacaagagttactaacagcccctctctccaagctcacttacaggctctctacttagtccagcacgaagtctggagacctctggcggcagcctaccaagaacaactggaccgaccggtggtacctcacccttaccgagtcggcgacacagtgtgggtccgccgacaccagactaagaacctagaacctcgctggaaaggaccttacacagtcctgctgaccacccccaccgccctcaaagtagacggcatcgcagcttggatacacgccgcccacgtgaaggctgccgaccccgggggtggaccatgactcgagccatggattggatctggcgcatcctgtttctcgtgggagctgccacaggcgcccattctcaggttcagctgcaacagtggggagccggactgctgaagcctagcgaaacactgagcctgacctgtgccgtgtacggcggcagctttagcggctactactggtcctggatcagacagcctcctggcaaaggcctggaatggatcggcgagatcaatcacagcggcagcaccaactacaaccccagcctgaagtccagagtgaccatcagcgtggacaccagcaagaaccagttctccctgaagctgagcagcgtgaccacagccgataccgccgtgtactactgtgcccggatgggcatcaatagcggcggctacctgtacggcatggatgtgtggggacagggcaccaccgtgacagtttctagcggaggcggaggttctggtggcggaggaagtggcggcggaggatctcagacagtggtcacacaagagcccagcttctccgtgtctcctggcggaacagtgaccctgacatgtggccttagcagcggctctgtgtccaccagctactaccctagctggtatcagcagatccccggacaggcccctcggacactgatctacaccaccaacatcagatccagcggcgtgcccgatagattcggcggatctatcctgggcaacaaggccgcactgacaatcacaggtgcccaggccgaggacgagtccgactactactgcatgctgtacatgggcagcggcatctgggttttcggcggaggcacaaagctgaccgttctgggatccgaaccaaagagttgcgacaaaacacacacctgccctacgcgtttttgggtgctcgtggtggtgggtggcgtgctcgcttgctactcacttctggtgaccgtagcgtttatcattttttgggtcaggagcaagcgatcccgcctattgcacagcgactacatgaacatgaccccccggcgccccgggccaacccggaagcactaccagccatatgcgcctccccgcgatttcgcagcgtatcggtcccgggtcaaattttcacggtccgctgacgccccggcctatcaacagggccagaatcagctgtataatgaattaaacctcggtagacgcgaggagtacgacgtcctcgacaagagaagggggcgcgacccagagatgggaggcaaaccgcagcgcaggaagaatccacaggagggcctgtacaacgaattacagaaggacaagatggcagaggcctacagcgagataggaatgaagggtgaaaggcgtcgtggaaagggccacgatgggctttaccagggcctaagtactgccacaaaagatacgtatgacgcgctgcatatgcaagccctcccccccaggtaagcatgcaacctcgatccggattagtccaatttgttaaagacaggatatcagtggtccaggctctagttttgactcaacaatatcaccagctgaagcctatagagtacgagccatagataaaataaaagattttatttagtctccagaaaaaggggggaatgaaagaccccacctgtaggtttggcaagctagcttaagtaacgccattttgcaaggcatggaaaaatacataactgagaatagagaagttcagatcaaggtcaggaacagatggaacagctgaatatgggccaaacaggatatctgtggtaagcagttcctgccccggctcagggccaagaacagatggaacagctgaatatgggccaaacaggatatctgtggtaagcagttcctgccccggctcagggccaagaacagatggtccccagatgcggtccagccctcagcagtttctagagaaccatcagatgtttccagggtgccccaaggacctgaaatgaccctgtgccttatttgaactaaccaatcagttcgcttctcgcttctgttcgcgcgcttc

SEQ ID NO: 119 - DNA, 3747 bp, synthetic construct
  source 1..3747: mol_type = other DNA
aagttcagatcaaggtcaggaacagatggaacagctgaatatgggccaaacaggatatctgtggtaagcagttcctgccccggctcagggccaagaacagatggaacagctgaatatgggccaaacaggatatctgtggtaagcagttcctgccccggctcagggccaagaacagatggtccccagatgcggtccagccctcagcagtttctagagaaccatcagatgtttccagggtgccccaaggacctgaaatgaccctgtgccttatttgaactaaccaatcagttcgcttctcgcttctgttcgcgcgcttctgctccccgagctcaataaaagagcccacaacccctcactcggcgcgccagtcctccgattgactgagtcgcccgggtacccgtgtatccaataaaccctcttgcagttgcatccgacttgtggtctcgctgttccttgggagggtctcctctgagtgattgactacccgtcagcgggggtctttcatttgggggctcgtccgggatcgggagacccctgcccagggaccaccgacccaccaccgggaggtaagctggccagcaacttatctgtgtctgtccgattgtctagtgtctatgactgattttatgcgcctgcgtcggtactagttagctaactagctctgtatctggcggacccgtggtggaactgacgagttcggaacacccggccgcaaccctgggagacgtcccagggacttcgggggccgtttttgtggcccgacctgagtcctaaaatcccgatcgtttaggactctttggtgcaccccccttagaggagggatatgtggttctggtaggagacgagaacctaaaacagttcccgcctccgtctgaatttttgctttcggtttgggaccgaagccgcgccgcgcgtcttgtctgctgcagcatcgttctgtgttgtctctgtctgactgtgtttctgtatttgtctgaaaatatgggcccgggctagcctgttaccactcccttaagtttgaccttaggtcactggaaagatgtcgagcggatcgctcacaaccagtcggtagatgtcaagaagagacgttgggttaccttctgctctgcagaatggccaacctttaacgtcggatggccgcgagacggcacctttaaccgagacctcatcacccaggttaagatcaaggtcttttcacctggcccgcatggacacccagaccaggtcccctacatcgtgacctgggaagccttggcttttgacccccctccctgggtcaagccctttgtacaccctaagcctccgcctcctcttcctccatccgccccgtctctcccccttgaacctcctcgttcgaccccgcctcgatcctccctttatccagccctcactccttctctaggcgcccccatatggccatatgagatcttatatggggcacccccgccccttgtaaacttccctgaccctgacatgacaagagttactaacagcccctctctccaagctcacttacaggctctctacttagtccagcacgaagtctggagacctctggcggcagcctaccaagaacaactggaccgaccggtggtacctcacccttaccgagtcggcgacacagtgtgggtccgccgacaccagactaagaacctagaacctcgctggaaaggaccttacacagtcctgctgaccacccccaccgccctcaaagtagacggcatcgcagcttggatacacgccgcccacgtgaaggctgccgaccccgggggtggaccatgactcgagccatggattggatctggcgcatcctgtttctcgtgggagctgccacaggcgcccattctcaggttcagctggtggaatctggccctggcctggttaagcctagcggcacactgtctctgacctgtgctgtgtctggcggcagcatcagcagcagcaattggtggtcttgggtccgacagcctcctggcaaaggcctggaatggatcggcgagatctaccacagcggcagcaccaactacaaccccagcctgaagtccagagtgaccatcagcgtggacaccagcaagaaccagttctccctgaagctgagcagcgtgacagccgccgatacagccgtgtactactgtgccagaatgggagccaatagcggcggctacctgtacggcatggatgtgtggggacagggcaccaccgtgacagtttctagcggaggcggaggttctggtggcggaggaagtggcggcggaggatctcagacagtggtcacacaagagcccagcttctccgtgtctcctggcggaacagtgaccctgacatgtggccttagcagcggctctgtgtctaccagctactacccctcctggtatcagcagacccctggacaggctccccggacactgatctactccaccaacaccagatccagcggcgtgcccgatagattctccggctctatcctgggcaacaaggccgcactgacaatcacaggcgctcaggccgatgacgagagcgactactactgcgtgctgtacatgggcagcggcatctgggttttcggcggaggcacaaagctgaccgttctgggatccgaaccaaagagttgcgacaaaacacacacctgccctacgcgtttttgggtgctcgtggtggtgggtggcgtgctcgcttgctactcacttctggtgaccgtagcgtttatcattttttgggtcaggagcaagcgatcccgcctattgcacagcgactacatgaacatgaccccccggcgccccgggccaacccggaagcactaccagccatatgcgcctccccgcgatttcgcagcgtatcggtcccgggtcaaattttcacggtccgctgacgccccggcctatcaacagggccagaatcagctgtataatgaattaaacctcggtagacgcgaggagtacgacgtcctcgacaagagaagggggcgcgacccagagatgggaggcaaaccgcagcgcaggaagaatccacaggagggcctgtacaacgaattacagaaggacaagatggcagaggcctacagcgagataggaatgaagggtgaaaggcgtcgtggaaagggccacgatgggctttaccagggcctaagtactgccacaaaagatacgtatgacgcgctgcatatgcaagccctcccccccaggtaagcatgcaacctcgatccggattagtccaatttgttaaagacaggatatcagtggtccaggctctagttttgactcaacaatatcaccagctgaagcctatagagtacgagccatagataaaataaaagattttatttagtctccagaaaaaggggggaatgaaagaccccacctgtaggtttggcaagctagcttaagtaacgccattttgcaaggcatggaaaaatacataactgagaatagagaagttcagatcaaggtcaggaacagatggaacagctgaatatgggccaaacaggatatctgtggtaagcagttcctgccccggctcagggccaagaacagatggaacagctgaatatgggccaaacaggatatctgtggtaagcagttcctgccccggctcagggccaagaacagatggtccccagatgcggtccagccctcagcagtttctagagaaccatcagatgtttccagggtgccccaaggacctgaaatgaccctgtgccttatttgaactaaccaatcagttcgcttctcgcttctgttcgcgcgcttc

SEQ ID NO: 120 - DNA, 30590 bp, synthetic construct
  source 1..30590: mol_type = other DNA
aaacatcatcaataatataccttattttggattgaagccaatatgataatgagggggtggagtttgtgacgtggcgcggggcgtgggaacggggcgggtgacgtagtagtgtggcggaagtgtgatgttgcaagtgtggcggaacacatgtaagcgacggatgtggcaaaagtgacgtttttggtgtgcgccggtgtacacaggaagtgacaattttcgcgcggttttaggcggatgttgtagtaaatttgggcgtaaccgagtaagatttggccattttcgcgggaaaactgaataagaggaagtgaaatctgaataattttgtgttactcatagcgcgtaatatttgtctagggccgcggggactttgaccgtttacgtggagactcgcccaggtgtttttctcaggtgttttccgcgttccgggtcaaagttggcgttttgatatcaagcttatcgataccgtaaacaagtctttaattcaagcaagactttaacaagttaaaaggagcttatgggtaggaagtagtgttatgatgtatgggcataaagggttttaatgggatagtgaaaatgtctataataatacttaaatggctgcccaatcacctacaggattgatgtaaacatggaaaaggtcaaaaacttgggtcactaaaatagatgattaatggagaggatgaggttgatagttaaatgtagataagtggtcttattctcaataaaaatgtgaacataaggcgagtttctacaaagatggacaggactcattcatgaaacagcaaaaactggacatttgttctaatctttgaagagtatgaaaaattcctattttaaaggtaaaacagtaactcacaggaaataccaacccaacataaaatcagaaacaatagtctaaagtaataaaaatcaaacgtttgcacgatcaaattatgaatgaaattcactactaaaattcacactgattttgtttcatccacagtgtcaatgttgtgatgcatttcaattgtgtgacacaggcagactgtggatcaaaagtggtttctggtgcgacttactctcttgagtatacctgcagtcccctttcttaagtgtgttaaaaaaaaagggggatttcttcaattcgccaatactctagctctccatgtgctttctaggaaacaagtgttaacccaccttatttgtcaaacctagctccaaaggacttttgactccccacaaaccgatgtagctcaagagagggtatctgtcaccagtatgtatagtgaaaaaagtatcccaagtcccaacagcaattcctaaaaggagtttatttaaaaaaccacacacacctgtaaaataagtatatatcctccaaggtgactagttttaaaaaaacagtattggctttgatgtaaagtactagtgaatatgttagaaaaatctcactgtaaccaagtgaaatgaaagcaagtatggtttgcagagattcaaagaaaatataagaaaacctactgttgccactaaaaagaatcatatattaaatatactcacacaatagctcttcagtctgataaaatctacagtcataggaatggatctatcactatttctattcagtgctttgatgtaatccagcaggtcagcaaagaatttatagccccccttgagcacacagagggctacaatgtgatggcctcccatctccttcatcacatctcgagcaagacgttcagtcctacagaaataaaatcaggaatttaatagaaagtttcatacattaaactttataacaaacacctcttagtcattaaacttccacaccaacctgggcaatatagtgagaccccatgcctgcaaaaaaaaaaaaattagccaggcatggtagcatgtacctgtagtcccagctacttgagaggtgaggtgggaaaatcactttagtgcaggatgttgaggctggagtgaactgtgattgtgccactgcactccagcctggacaatagagcaagaccttgtctcaaaaaaatgcattaaaaattttttttaaatcttccacgtatcacatcctttgccctcatgtttcataaggtaaaaaatttgataccttcaaaaaaaccaagcataccactatcataattttttttaaatgcaaataaaaacaagataccattttcacctatcagactggcaggttctgattaaatgaaattttctggataatatacaatattaagagagactgtagaaactgggccagtggctcatgcctgtaatcccagcactttgggaggctgggtaacatggcgaaccctgtttctacaaaataaaaatattagctgggagtggtggcgcacacctatagtcccagctactcaggaggctgaggtggaaggatcgcttgaacccaggaggttgagactgcagtgaactgtgatcattctgctgcactgcaccccagcctgggcaacagagaccttgtctcaaaaaaaaaaaaaaaagagacaaattgtgaagagaaaggtactctcatataacatcaggagtataaaatgattcaacttcttagaggaaaatttggcaataccaaaatattcaataaactctttccccttgacccagaaattccacttgaataaagctgaacaagtaccaaacatgtaaaagaatgtttcttctagtacagtcggtaagaacaaaatagtgtctatcaatagtggactggttaaatcagttatggtatctccataagacagaatgctatgcaacctttaaaatatattagatagctctagacacactaatattaaaagtgtccaataacatttaaaactatactcatacgttaaaatataaatgtatatatgtacttttgcatatagtatacatgcataggccagtgcttgagaagaaatgtgtacagaaggctgaaaggagagaactttagtcttcttgtttatggcctccatagttagaatattttataacacaaatattttgatattataattttaaaataaaaacacagaatagccagacatacaatgcaagcattcaataccaggtaaggtttttcactgtaattgacttaacagaaaattttcaagctagatgtgcataataataaaaatctgaccttgccttcatgtgattcagccccagtccattaccctgtttaggactgagaaatgcaagactctggctagagttccttcttccatctcccttcaatgtttactttgttctggtccctacagagtcccactataccacaactgatactaagtaattagtaaggccctcctcttttatttttaataaagaagattttagaaagcatcagttatttaataagttggcctagtttatgttcaaatagcaagtactcagaacagctgctgatgtttgaaattaacacaagaaaaagtaaaaaacctcattttaagatcttacttacctgtccataattagtccatgaggaataaacaccctttccaaatcctcagcataatgattaggtatgcaaaataaatcaaggtcataacctggttcatcatcactaatctgaaaaagaaatatagctgtttcaatgagagcattacaggatacaaacatttgattggattaagatgttaaaaaataaccttagtctatcagagaaatttaggtgtaagatgatattagtaactgttaactttgtaggtatgataatgaattatgtaagaaaacaacaggccgggcgggttggttcacacgtgtaatcccagcactttgggaggctgaggcaggcagactgcctgagctcaggagttcgagaccagcctgggcaacacggtgaaatcccgtctctactaaaaatacaaaaaaattagccgggtgtggtgacacatgcctgtagtcccagctacttgggaggctgaggcaggagaatcacttgaacctgggaggtgaaggttgcagtgagccaagatggcaccacttcactccagcctgggaaacagagcaagactctgtctctgagctgagatggcaccacttcactccagcctgggaaacagagcaagactctgtctcaaaaaaaacaaaacacacaaacaaaaaaacaggctgggcgcggtggctcacgcctgtaatcccagcactttgggaggccgaggcgggtggatcacctgaggtcaggagttccagaccagccttgtcaacatggtgaaacctccccccgccgtctctactaaaaatacaaaaattagccaggcgtggtggcaggagcctgtaatcccagctacttgggaggctgaggcaggagaatcgcttgtacccagaaggcagaggttgcactgagctgagatggcaccattgcactccagcctgggggacaagagcgagatttcgtctttaaaaaacaaaaacaaaacaaaaaaccatgtaactatatgtcttagtcatcttagtcaagaatgtagaagtaaagtgataagatatggaatttcctttaggtcacaaagagaaaaagaaaaattttaaagagctaagacaaacgcagcaaaatctttatatttaataatattctaaacatgggtgatgaacatacgggtattcattatactattctctccacttttgagtatgtttgaaaatttagtaaaacaagttttaacacactgtagtctaacaagataaaatatcacactgaacaggaaaaactggcatggtgtggtggctcacacttgtaatcccagtgctttgggaggctgagacaggagagttgcttgaggccaggagttcaagaccgacatggggaatgtagcaagaccccgtccctacaaaaaactttgtaaaaatttgccaggtatggtggtgcatacctgtagtcccagctactcgggaggcggaggcagaaggaatcacttgagcccaggagtttgaggctgcagtgagctacgatcataccacagcactccagcgtggacaacagagtaagaccctatctcaaaaacaaaacaaaacaaaacaaacaaaaaaaaccacaagaaaaactgctggctgatgcagcggctcatgcctgtaatcccagtattttgggaggcccaggtgggcgtatcacctgaggtcaggagttagagaccagcctggccaacatggtgaaaccccatctctactaaaaatacaaaattagccaggcatgtggcacgcgcctgtagtcccagttactgggaggctgaagcaggaggatcacctgagcccgggaggtggaggttgcagtgagccgagatcacaccactgcactccagcctgggtgacacagcaataccctacctcaaaataaaaaagaaaaagaaaagaaaagttgctgtccccgctaccccaatcccaaatccaaacagcctctctcatctcacagtaagggggaaaaatcacccaaaaaagctaagtgatcttttgaaaacccaaactcttagaagtctaagattattatagtcaactcatgaagtgtcatcataaaagatactctaatattatttaagtagaaccacatattggttgtcttggtatgtctagcccctggcatacaaaatatttaataacactgatatggtacctgtgatgtgaaaatgtactatgagtacagctttataaatactatatatgtacctatatacagaaaaaaatacaacaaaatcataaaagcacttatctttgaaagaggagttacagcaattttatttagttctttattgctttgctatatattctaaatttttttcaatgaatatatatcacttttaaaaaaattcaatggtctttcttataaattatctttggcagcatgcgtttttatatatacatataaaatgtatgggaaatttttaaaggatacattaaattaaagcaaaatatacaaacaaaaaatcagaatacaaaaagataaaaagattgggaagggagggagggagtaaggaggaagggtgggtgggtatagagaaatataccaaataatggtaagaagtggggtcttgacactttctacactttttttaaataaaaaaaatttttttctctctcttttttttttttagagacgaagtctcgctatgttgcccaggctggtcttgaactcctgggatcaagagatcctcctgcctcagcctcccaaggtgcttggattacaggtgtgagccaccacgcctggtcactttctacactttaatatatatattttttcattttcaatgtcatttttattagttaatttataatacccattcaccattatattcaaagtctatttgaagaaataaaccagaaagaatgaaatactctagctcacatgctattcaatactaaattacctttcaaatcacattcaagaagctgatgatttaagctttggcggtttccaataaatattggtcaaaccataattaaatctcaatatatcagttagtacctattgagcatctccttttacaacctaagcattgtattaggtgcttaaatacaagcagcttgacttttaatacatttaaaaatacatatttaagacttaaaatcttatttatggaattcagttatattttgaggtttccagtgctgagaaatttgaggtttgtgctgtctttcagtccccaaagctcagttctgagttctcagactttggtggaacttcatgtattgtcaggttggcccgtaatacctgtgggacaacttcagcccctgtgcacatggccaggaggctggttgcaaacattttcaggtaggtggaccaggacatgcccctggtcatggccaggtggaggcatagtgctatacagcaggcagaagtcaatattgatttgtttttaaagaaacatgtactactttcataagcagaaaaaatttctattcttgggggaaaagattatgccagatcctctaggattaaatgctgatgcatctgctaaaccttcacatatcagaacatatttactatagaaagaatgaaaatgggacatttgtgtgtcacctatgtgaacattccaaaaatattttacaacaactaagtattttataaattttatgaactgaaatttagttcaagttctaggaaaatacaaaccttgctagatattataaaaatgatacaatatatattcatttcaggctcatcagaatatatctgttatcacttgacaagaatgaaaatgcaccattttgtagtgctttaaaatcaggaagatccagagtactaaaaatgacttcttccttgaagcttactcaccaacttcctcccagttactcactgcttctgccacaagcataaactaggacccagccagaactcccttgaaatatacacttgcaacgattactgcatctatcaaaatggttcagtgcctggctacaggttctgcagatcgactaagaatttgaaaagtcttgtttatttcaaaggaagcccatgtgaattctgcccagagttcatcccagatatgcagtctaagaatacagacagatcagcagagatgtattctaaaacaggaattctggcaatataacaaattgatttccaatcaaaacagatttacataccatacttatgtcaagaagttgttttgttttattgcatcctagattttatttttttgatttatggtttactttaagcataaaaaatttgtcaatacaactcttcccaaaaggcataaacaaaaattcataaaacttgcatcacttgagatacttcaggtatgaattcacaactttgttacaacttactatatatatgcacacatatatatatatttgggtatattgggggggttctaatttaagaaatgcataattggctatagacagacagttgtctggaatgaaaatcaatacttttgctataatcgattactgaaataattttactttccagtaaaactggcattataattttttttaatttttaaaacttcataattttttgccagactgacccatgtaaacatacaaattactaataattatgcacgtcacatctgtaataatggccttcatgtaaacatttttgtggtttacacataaaatctctaattacaaagctatattatctaaaattacagtaagcaagaaaattaatccaagctaagacaatacttgcaacatcaattcatcatctgtgacaaggactgcttaagtctctttgtggttaaaaaggaaaaaaaaaaaaaagacatgttggccagatgcggtggctcacacctgtaatcccagcactttgggaggctgaggtgggcggatcacccctggcctgcccaacatggtgaaaccccgtctctactaaaaacacaaaaattagctgggcgtggtggcgggcgcctgtaattccagctactcgggaggctgaggcaggagaattgctagaacccaggaggcagagattgcagtgagctgagattgcaccattgcactacagtctgggcaacaaaagtgaaactccatcttaaaaaaaaaaagacaatgttcgtgggtccaaacaagacttaatggaagtgagtctaaaaatgagctatgtgggccaggcgtagtggctcccacctgtaatcccagcactttgggaggccgaagcaggcagatcatgaggtcaggagatggagaccatcctggccaacacggtgaaatcctgtctctacaaaaattagctgggcgtggtggtgcctgcctgtaatcccagctactcagaaggctcaggcaggagaatcgcttgaaccagggagtcggtggctagagtgagccgagatttgcatcactgcactcctgcctggtgacagagcaagactccatctcaaaaaaaacaaacaaaaataaaagataaaaatgagctatgtgaattaaaagaggtataacaatagataaaccatattttatttaattcctagtaatgagtaatatttccaaacttctggaatgggcagaaattgctagttggcatatttttaccttttatattcagatacattaaaattctcaaaaaaaaacacctcaaagcagatgatccgccatctccttggataatttgtgttaactcaggataacagaaaaccaaaattatgagttactgatgcaatattcctaaatgtaaaaataattaaagctaatagtagattcatcttccaatttcatatcagtcttacaaataaactacatatataacttgcttgccttcccttctgagggataaagctgttagaagaattaaaatcagcattcttgactattcaaccaagggagggataaattattactcattctagggacatgggctcataactactacatgtgtaaggacatgaatttacccaatattacaatttttccttttattagtgtgtacagtggaagaatagacatgttcactctggacaaaaaaaaaattatacttatcagttatcagaagcacaatgctgaagacagtagttccataacaatttgaagtatgtgatcgaactagtagattatcttagtagtagtgaattattgtaaatgttagtaatttggcagccactgggcagaaaaataagaattgaggctcaatattgatattaatggtggtgattgacacataaattttatcaagtctacacaatataaaattacagaaaggtagaagagtataccagtacaacttcaacatatcttcactacaagggagtaaaatgacatggcctagttactatctaatgaactgcagaaaactaaaagaaaactccaaggcaactcttctctgctgatctggttggtccttttcctaccttttgcaatacccagatacaaacaatggatagaaaacaaagtagacttgtagtatgcaggtcacagtgctaaattcacagaaagaaacccctgaactgaactgctctatttcctggtggtcacaaagagtaattctggtttacacctacagattgatgtcaatctacaccctgttgataacagtgtggccaaggacaaaaaaaaggtgctccgttttaccaattctgtaaaaaattattggcagggtaagctcggctagggcaggattacatttctaggactaccatccccgaaatttagaagatattatatccacataaagcatatctttcacattaatttgcaaaaatctaaaagctttttcttagctcaagtgtgtccaagtttaccctggcagtttaaaacgatagttacaagcagcatgggttgtatcagacacatttgagggccaatttcatgtaagtgatattgggcaagttacttcaactatctgtgcctccaaggtcatactagtgtttatttacctaaagggtacctgttatgtaactttagggtgtttacattagataatgcctgcaaaatatttacttcaacgcctaaaacatagttaagtattcaataaatacctactattgtcactactaacttaaaagtttagagattaagagcagaatctggggtgagacaaacttaggttcaaatcctagtattgttgggtaatcttgggcaagttacttaacctctctgatttgtgtaatttaaaaaattagttaatatacataacagggcttagaagagtatctagcacatagcaccatttaagcatttgttattgctaacatgcaaacaatttaagggaaagaaattttttaaaaaggaagagggatttgcaaactaaaaacaatgagtatcttatgttcaaagaaaactaacaaacagccagctctagcaataattaaattcactatatactggggcaggcatcacaccccaaagctaaaagcgtctacctaggccaggcacggtggctcatgcctgtaatcccagcactttgggaagcagaggcgggcagatcgcttgagctcaggagttcaagaccagcctggacaacatggcaaaacaccatctctacaaaaaatacaaatattaggccgggcgcagtggctcacgcctgtaatcccagcactttgggaggccaaggcgggtggatcacctgagatcaggagttcgagagtagcctggccaacatggtgaaacctcgtctctattaaaaatacaaaaaattagccaggcatggtggcaggcgcctgtaatcccagctactcagggggatgaggtaggagaatcgcttgaacccgggaggcagaggttgcactgagccgagatcatgccactgtactccagcccgggcaacaagagcgaaactccatctcaaaaaataaataaataaataaataaaataaagtacaaatattagccagggatggtggtgcgcacctgtagtcccagctacttgggaggctgaagtgggagaatcccctgagcctggggagaatcacccgagcccgggaagtcgaggctgcagtgagcagtgattgtgccactgcactccatcctaggtgacagagtgagaccctgtctcaaaaaaaagaaattggcagaattaagtaagttgatgtttagagatgaaaaatcaacattttttcctcagcaactgaataaaaacaacagccactaccatttttttgagtacctatttgtagcctattttttaactggtattactcgagagagagagagctaggttcgagacagagctccttctcttaataactgtatgacctagggtatgtctgttagcctctctgaggcttcaaaggttcctcatctgtaaaatggtaataatcataccattgctacagggctgttttgaagactaattaggactatgtaagtaaacatgatgatggctattattactgttccccgccaggggccatgcaagggttgctgattcacatagactgtcttataatcctctcaataactccaagaggtagccagcacctcagatatacataaaatgacttaagcccagagaggtgaagtaagttgcccacagccacacaactagtaaatagcccaaacaagctggattcccagttagactccgttaatagcactgctctttaccttaagtcattacaatgcctaatatgaaatagaatcgcttctttcttagggttcaagtggttaattatttaatgtattcattcaacaaaccatcatcgaggacctcttacaagccaagtactgtgctaagtgctagagttacggcggtgattcctgcccttaaaaagttttagtgggagaaacaacaggtaaccaggtcattgccaaaacaacaaaaataatcataataaagcaggctaaagcatatttaactggccggggttttgactattttagcaagcatgatcagaacggttgaggagggaggccagcagcttggccggttcaacaaacaagaaaaaaccagtgagggtggagctaagataccagaggctgattacggttaagaatgttcttgaaggtaaggaccagattctcattttctatatcctggggcatcggtcagcatggaatctggattctagcacatgtgaatttcggcttgaaatgacctaatgccttttccctagttccttcgtgtgtcaaatacgcatggttaccgctaccagagctgtagtggggcttcaatgaggccatgagcatctccataaagatgaactacagtgtgtgcaaaactaaaggcaaaacctggtccccacacgccctcccaggtggtcgctttccgtgccgaggcccctccagaggtgccccgagaacctcaccatcgcaccccaaacttccagggaagggcctctcccgagaaagcccccacgcccccaccccgcgccatcattcccgaatctgccctcggcccctccccgcagcacgctcgcaggcggcacatgtcaaccaaaacgccatttccaccttctcttcccacacgcagtcctcttttcccagggctcccccgaggagggacccaccccaaaccccgccattccgtcctccctgccgccctcgcgtgacgtaaagccgaacccgggaaactggccgcccccgcctgcggggttccctgggcccggccgctctagaactagtggatcccaattgaaggcctggtctaaatgactccaaaatcaccacttaattcaagagactgatttccctgagtcaggccccttaaagcagctatttcaatgggacagggaaacaaccctaggatctggattagaatcacttgggggctgccacacccccagggctctgatcctgcccttctcccacacgcacattcacatactgctgcagtgaccttccatttctaatgggttcctgggccatctgtcaggtatagggaatggaaaaggggttggggaggctctgcttcagaaagtttgtgtcaggggctcccagagcctccacagatagatagcaggggtccccaccctaccatggcagctataaatgtgatcaacatttattggcctaggatacagcagttagcaaaatgcctgatgtagttcccactccgtggaggttgcaggctagctctttcctaatgagctttacagcagaagctgttttatcgttaagtgccccacagagacactttaccaggaggctgggagagttctccagatttgggagaggcgcagagacagtgtgtgagccgagccctgtctcagcaatccacctggaggagctagagtatcctcctccctttaccattcagaccgagagaaaaagcccagcttgtgtgcaccctcgtggggttaaggcgagctgttcctggtttaaagcctttcagtatttgttttgatgtaaggctctgtggtttgggggggaacatctgtaaacattattagttgatttggggtttgtctttgatggtttctatctgcaattatcgtcatgtatatttaagtgtctgttatagaaaacccacacccactgtcctgtaaacttttctcagtgtccagactttctgtaatcacattttaattgccacctcgtatttcacctctacatttgaaatctggcgtctgtttcaagccagtgtgttttttcttcgttctgtaataaacagccaggagaaaagtgcctctatgtttttatttttcaagggagtattcagtacctacaaacccaagtcaggaagcctgctagtggctttggttctttcagaggctgctcgatgccttgtgtgtcagaaagaaagattcagcagttttgcatcatggcaaagaagcctgttattttggggctcagcccctcattttatagaggatgaaacagagggggatgggaggtcacaaagacaactgccccgggagcaggtgtgggggagacttgccctgagggtctagacgctctgcaccaccgtcctgtctcccttgctgaagaccacacatgcccttctttgaccagaccctgccacctgataggccaggacctggtaggcgggtacccaggtttcatggatggaaccacatctccccaaaagtggggaggtagctactgggatgcacgcctcccgccatgtgctataggagagcagctgaagcaacagttgggatcagatgtagtcacaattgaatgcatcatcacatttatccctctaagtggctgggagagttgatatcctcatccctaaggtacaaaatgttccaatttgatcagtggctttcaggagctgagaaaggcatgtgctctgaggcagagctgttatgtcccgcagagcctaaaaatgctctaagaacatgctccctgccaaaattctcaatggctgtgacaagggacaacgatcgaccaatgggggtggaagcagacctccgcagtccaggggccagagctaggacagaggggtcggagaaagagtcattttcccaacactccagctcttggccagtcctcacacagtcccctcctgcttcctgctgagagagatatcctcataggtctgggtaaagtccttcagtcagctttcattccctgtcaccaactttgtctctgttctccctgcccgtctcaggcagcactcctcaggaaacctctccaagagccagcctcactgcagcgcccactattgtccctctgcctcaagtgtcccatccatgccaggccccaggcaggctgcagctttccctcagggccacaccaaagcacttgggctcagctgtgctgtccccctccatcactgagctcaggggcagcaggggtggggtgccaggaggcccattcacccttctctggctctgtgttggacccacctgcccagccactgctgcttagaacctacccgctgggaaaatgaagccctcccggaggggccacctcaacctgagagcctcacggatcacagttgtccccactcagctctgccagccctcagagacccatagataaaagctgagcttggctcgcagagctggttccatcttccattcccagagggttcaacttcctaccccaaccacacagggaacctcaaggctgagccagtgtgggctgcagtgcagaccagcttcctggacacgtcctgccacctgaccccaggctggcctcactgcccctggcactcctgaccctatcctcattcctcctggcagtgcgtgttctgccattccgctttcccttagctgtcctctcactgtactgtcagcttctccttttccaggtgccccccaggggctttccacatgaccctgtcaccccacagcccatccagcaccaattccagctctctgccacccttcaaaggagtgacagtgccctgcttcacctcccactcacccctcaacccagagcaatctggctccagtcttgcctccttccccctaagtactctagtcacagttccaaattcctcctggtcataaagccaaatgaagcttcctggtcctcagcggacttgccacttcagcagtactggactctctcctcccagaaacctgtttccccttggctcctggagcccacactctgctggaatccttctgcctctctggcctgtagcctggccctctctcccaacctgaggtccattctctcctgctcctccacaagatgttgctccttccattacttcctccctctcaaccaaagctccttcattagctctttatcttctggtttcttcccctgggcagacgaatggattcaagagcctgtggcccagcagcccagcactccaggatctcagcacttcagcatcccagtaccctagcatctcaataccccagcaccccagcaccatagtattccagcaccccattgtccaagcatctcagcactccagcatcccagcaccccaacactccagcagcccagaatctcagcaccctagcactgcagcatctcaggaccccagcacttcagcatcccagcacactagtactccagcatctcggcaccccagcacctaggcatcccaacacccagcaccccagcacttaagcatcccaccactacagtatctcaacactccagcaccccagcaccatagtgttccagcaccccagcatcccaacaccccagcacttaagcatcccaacacctcggcatcccaacaccccagcactgcagcatctcagcaccttagcatcccagtgccctagcatctcaatgctccagcacaccagtactacagtattccagcaccccagcactccagcatctcagcactgcagcactgcagcactccagcatcccaaaatcccagcatcccaacaccccagcagaccagcagaccagcatctcagcaccgcagcatccaaggactatcccagcatcccagcaacccagcacctcagcatcccaacaccccagcatttcagcatggcaacaccccagtaccccagcacttcagcaccccagtatcccagcatctcagcgacccagtatcacaaaacctcagcatcctagcaccccagcaccccagcaccttagcaccttagcatcccagcatctcagcgcctcagcatcttgatattctggctgaggtcagcgtggtgtatctagtcagggtcctaactttcacttcgcagggaaatgctgctggactgggtctcatgttgggctgaagctctctagaccccttgaagacagcataaaagagcttggagacgctgggtgtcccccatggaagagttcactctcatcctgctttgacaacagccttctctggggtccctcacgggcccctctttcttactgcaagtttgtctctgagaagactgtgatgcagaagtcactcagctgcctgtggctcctgaagagctgaaggtggaggcctgtaggcctccctatgagaggcgcagaaaaaaccatgattgctagtggggaggtgctccctctacaacccactccataatctgcccccgcccagctctgaggccagccccaggggaaaatgccagatccccagggaggtgtgtgagacctcaggggctccctcctcccttacagcaggctcaggcccctgggggcctcagggccaaggtctgtgggtaagctactatctctcacttgtcctctagccacaaaagccagggagatctggcaatggacatgaggttctgaagaagcacatatgactggcttcctaatgcgtggttgttcagtgattcaataaacacgcatgggccaggcatggggaaatagacaaacatgatccccaacctctcccagagtgaactgggagggaggagtgttcatccctcaggattacaccagagaaacaaaccagcaggagatatatatggttttggggggtcaagaaagaggaaaaacctggcaaggcaagtccaaaatcataggacaggctgtcaggaagggcagcctggaacctctcaagcaggagctgatgctgcagtccacaggcagaatttcttcttcctcggggaaatctcagctttgttcttaaggcctttcaactgattggctgaggtctgccccttcccccacattctccaggataatcttccttacttaaagtcaactattaatcacagctacaaaatcccttcacagctacacatagatcagtgtttgattgacgaacagcccctacagcctagccaagttgacacataaaactaaccatcacagggggacaaatgatgtaaacacatcaacaaataaaacagtaacaagttaaggtctatggaaaaaacacagaaggggcagagagaaagaaagcaagaaggagagtcccagtttgctagggcttgtgggaagtggggagcagttctctttagctaggatatttgggaaaggcatatctgaaggagtgatatttgagcttagattaaaagatgggaaggagcaagccatgcaaagagctaggatgttccaagcagagacggaacagcaagtgcaaatgtcaggaggaatagaaggaggctggtgggtggggtccagtgagcaagaggagggcaggcaggagaggggatggggaggtgggcaggcccagaccacccagggccctggagactatcctgatccaacaagggaagccttgagtcacttcagtgtccatgtggagaatggacctcagactgaatgagggaggcagtaaggagggcctctacctccagggcttcgccctgtggactgcgcatagacatctccaactcagaaagtctgaaccaaactttccatagttcccccaagtctgggcatcctcctactcagtgaaaggcagccatcacacctccctgccctgctcccggatgccccaaatcctcttggtctccaagtccagaacctgagacttgtccttgatgtttgtctttccctcaccctttctgtattctgggaagatgggtttttttcccccagatgaatctgtaaaacttctgtgatcacaataaaaattctggcagtattattttctggaacatgacaaagtgattcaaaattatttatctggaagactacaaaacaagaatagccaggaaatttctaaaaagaaagaagaaggaggaggagaaagaaggaggaggaaaaggaggagaagaagaaaagaaaaagaaccaagaaagggttctagctctaccaaatattaaaacatatcatgaagctatttaaaacaatatggttgtggatactgaaaaagatgtgaataaagtggaaggaaaataaatagaaatgcacatggggattgagactgtgaaaaaggcagcatctcacatcagtgagggatgttcaacacctggtgttgggaaaactggctagtcatttaaaccaaacaactgggtcctctacctcactcctgacattaagatacatttagatgattcaaagagtaagacagaaaaaataacacgtgaaaacactatcagaaaacaacgtgggccaggtgtggtgggtcacgcctgtaatcccagcactttgggaggccgaggcagacagatcacctgaggtggggagttcaagaccagcctgaccaacatggtgaaatcctgtctctactaaaaatacaaaattagctgagcgtggtggcgcatgcctgtaatcccagctactcaggaggccgaggcaggagaatcacttgaacctgggaggcagaggttgtggtgagccgagatcacgccattgcactccagcctgggcaacaagagtgaaaatccatctaaaaaaaaaaaaaaaagccaaggtggatatttttatagtatcagggtagatcaagcttctccaatcatgacatgaaacccagaaaccataaaagaaaagaatgataaaattgcccacgtaaagtaaaaagcttgcacacagaaaaacaccatacaggttacaagatgagcagcaaaatcagagaaaaaacattgcaattcaggacacacagaggctattgttcctaatatttaaaaataaaagtagtggattgtctacaaaaagatgaagacaagaatttcagaaaaccaaatactgcatgttttcacttacaagtggaagctaaacactgagtacacgtgtacacaaagaatggaaccataggccaggcaccgtggctcacgcctgtaatcccagtactttgcgaggccgaagcgggcggatcacctgaggtgaggagttcgagaccatcctggccaacatggtgaaacccagtctctactaaaaatacaaaaattagccgggcgtggtggtgggtgcctgtaatcccagctactcgggaggctgcggcagtagaatcgcttgaaccctggaggtggaccttgcagtgagccgagatcgcaccactgcactccagcctgggcaacagagtgagactccatctcaaaaaaaaaaaaaaggaatagaacaatagacactggggcctacttgagggaggagggtgaggatcaaaaacctgcctatcaggtactatgcttattacctgggtggtgaaataatctgtacaccaaaccccagtgacatgcaatttaccgatgtaacaaacctgcccatgtacccgctgaacctaaaataaaagttggaaaaaaatatagaaattttctttgtaatagccaaaaactgcaaacagcccaggtgtctattagtagaatgcataaacaaactcgggcatgttcatacaatgtaaaactactcatcaataaaaagtgatacttctcagcaatgaaaagaaactagctactgataccagctacaacatggatggatttcaagtgctttatgatgagagcaagaagccagacacaaaagtgtctatatatatatacagtatatatacgtatatatacacatatatacagtatatatatacatatacatgtatatatatactgtatatatactgtatatatatacacagtatatatatacatatatacagtgtatatatactgtgtatatatacatgtatatatactgtgtatatatacatgtatatatactgtgtatatatacatgtatatatactgtgtatatatacatgtatatatatgtatactgtatatatactgtatatatatatacacatatatacagtatatatatacagtatatactgtatatatacagtatatacgtgtatatatacatatatacagtatatatgtaaatatacatatatacagtatatatgtaaatatacatatatacatgtatatatatacactatatatatacatatatagtgtatatatacatatatacatgtatatatttactatatgattccatttatataaagtgccaaaacagtcaaaaataatctatgtggaaaaaatcaacaaagggatcccccgggctgcaggaattcgatggcgcgccgacgtcgcatgcagttagggataacagggtaatacgaccatggcatgtcctctagactcgagcggccgcaataaaatatctttattttcattacatctgtgtgttggttttttgtgtgaatcgtaactaacatacgctctccatcaaaacaaaacgaaacaaaacaaactagcaaaataggctgtccccagtgcaagtgcaggtgccagaacatttctctatcgaaggatctgcgatcgctccggtgcccgtcagtgggcagagcgcacatcgcccacagtccccgagaagttggggggaggggtcggcaattgaaccggtgcctagagaaggtggcgcggggtaaactgggaaagtgatgtcgtgtactggctccgcctttttcccgagggtgggggagaaccgtatataagtgcagtagtcgccgtgaacgttctttttcgcaacgggtttgccgccagaacacagctgaagcttcgaggggctcgcatctctccttcacgcgcccgccgccctacctgaggccgccatccacgccggttgagtcgcgttctgccgcctcccgcctgtggtgcctcctgaactgcgtccgccgtctaggtaagtttaaagctcaggtcgagaccgggcctttgtccggcgctcccttggagcctacctagactcagccggctctccacgctttgcctgaccctgcttgctcaactctacgtctttgtttcgttttctgttctgcgccgttacagatccaagctgtgaccggcgcctacgtaagtgatatctactagatttatcaaaaagagtgttgacttgtgagcgctcacaattgatacttagattcatcgagagggacacgtcgactactaaccttcttctctttcctacagctgagatcaccggcgaaggagggccaccatgggtcaccagcagttggtcatctcttggttttccctggtttttctggcatctcccctcgtggccatatgggaactgaagaaagatgtttatgtcgtagaattggattggtatccggatgcccctggagaaatggtggtcctcacctgtgacacccctgaagaagatggtatcacctggaccttggaccagagcagtgaggtcttaggctctggcaaaaccctgaccatccaagtcaaagagtttggagatgctggccagtacacctgtcacaaaggaggcgaggttctaagccattcgctcctgctgcttcacaaaaaggaagatggaatttggtccactgatattttaaaggaccagaaagaacccaaaaataagacctttctaagatgcgaggccaagaattattctggacgtttcacctgctggtggctgacgacaatcagtactgatttgacattcagtgtcaaaagcagcagaggctcttctgacccccaaggggtgacgtgcggagctgctacactctctgcagagagagtcagaggggacaacaaggagtatgagtactcagtggagtgccaggaggacagtgcctgcccagctgctgaggagagtctgcccattgaggtcatggtggatgccgttcacaagctcaagtatgaaaactacaccagcagcttcttcatcagggacatcatcaaacctgacccacccaagaacttgcagctgaagccattaaagaattctcggcaggtggaggtcagctgggagtaccctgacacctggagtactccacattcctacttctccctgacattctgcgttcaggtccagggcaagagcaagagagaaaagaaagatagagtcttcacggacaagacctcagccacggtcatctgccgcaaaaatgccagcattagcgtgcgggcccaggaccgctactatagctcatcttggagcgaatgggcatctgtgccctgcagtgttcctggagtaggggtacctggggtgggcgccagaaacctccccgtggccactccagacccaggaatgttcccatgccttcaccactcccaaaacctgctgagggccgtcagcaacatgctccagaaggccagacaaactctagaattttacccttgcacttctgaagagattgatcatgaagatatcacaaaagataaaaccagcacagtggaggcctgtttaccattggaattaaccaagaatgagagttgcctaaattccagagagacctctttcataactaatgggagttgcctggcctccagaaagacctcttttatgatggccctgtgccttagtagtatttatgaagacttgaagatgtaccaggtggagttcaagaccatgaatgcaaagctgctgatggatcctaagaggcagatctttctagatcaaaacatgctggcagttattgatgagctgatgcaggccctgaatttcaacagtgagactgtgccacaaaaatcctcccttgaagaaccggatttttataaaactaaaatcaagctctgcatacttcttcatgctttcagaattcgggcagtgactattgatagagtgatgagctatctgaatgcttcctaaaaagcgaggtccctccaaaccgttgtcatttttataaaactttgaaatgaggaaactttgataggatgtggattaagaactagggaggggctagctcgacatgataagatacattgatgagtttggacaaaccacaactagaatgcagtgaaaaaaatgctttatttgtgaaatttgtgatgctattgctttatttgtgaaatttgtgatgctattgctttatttgtaaccattataagctgcaataaacaagttaacaacaacaattgcattcattttatgtttcaggttcagggggaggtgtgggaggttttttaaagcaagtaaaacctctacaaatgtggtagatccatttattagctaggagtttcagaaaagggggcctgagtggccccttttttcaacttaattaacctgcagggcctgaaataacctctgaaagaggaacttggttaggtaccttctgaggctgaaagaaccagctgtggaatgtgtgtcagttagggtgtggaaagtccccaggctccccagcaggcagaagtatgcaaagcatgcatctcaattagtcagcaaccaggtgtggaaagtccccaggctccccagcaggcagaagtatgcaaagcatgcatctcaattagtcagcaaccatagtcccactagtttcatcaccaccgccacccccccgcccccccgccatctgaaagggttctaggggatttgcaacctctctcgtgtgtttcttctttccgagaagcgccgccacacgagaaagctggccgcgaaagtcgtgctggaatcacttccaacgaaaccccaggcatagatgggaaagggtgaagaacacgttgtcatggctaccgtttccccggtcacggaataaacgctctctaggatccggaagtagttccgccgcgacctctctaaaaggatggatgtgttctctgcttacattcattggacgttttcccttagaggccaaggccgcccaggcaaaggggcggtcccacgcgtgaggggcccgcggagccatttgattggagaaaagctgcaaaccctgaccaatcggaaggagccacgcttcgggcatcggtcaccgcacctggacagctccgattggtggacttccgccccccctcacgaatcctcattgggtgccgtgggtgcgtggtgcggcgcgattggtgggttcatgtttcccgtcccccgcccgcgagaagtgggggtgaaaagcggcccgacctgcttggggtgtagtgggcggaccgcgcggctggaggtgtgaggatccgaacccaggggtggggggtggaggcggctcctgcgatcgaaggggacttgagactcaccggtcgcacgtcatgaatctagaaccatggcttcgtaccccggccatcagcacgcgtctgcgttcgaccaggctgcgcgttctcgcggccatagcaaccgacgtacggcgttgcgccctcgccggcagcaagaagccacggaagtccgcccggagcagaaaatgcccacgctactgcgggtttatatagacggtccccacgggatggggaaaaccaccaccacgcaactgctggtggccctgggttcgcgcgacgatatcgtctacgtacccgagccgatgacttactggcgggtgctgggggcttccgagacaatcgcgaacatctacaccacacaacaccgccttgaccagggtgagatatcggccggggacgcggcggtggtaatgacaagcgcccagataacaatgggcatgccttatgccgtgaccgacgccgttctggctcctcatatcgggggggaggctgggagctcacatgccccgcccccggccctcaccctcatcttcgaccgccatcccatcgccgccctcctgtgctacccggccgcgcgataccttatgggcagcatgaccccccaggccgtgctggcgttcgtggccctcatcccgccgaccttgcccggcacaaacatcgtgttgggggcccttccggaggacagacacatcgaccgcctggccaaacgccagcgccccggcgagcggcttgacctggctatgctggccgcgattcgccgcgtttacgggctgcttgccaatacggtgcggtatctgcagggcggcgggtcgtggcgggaggattggggacagctttcggggacggccgtgccgccccagggtgccgagccccagagcaacgcgggcccacgaccccatatcggggacacgttatttaccctgtttcgggcccccgagttgctggcccccaacggcgacctgtacaacgtgtttgcctgggccttggacgtcttggccaaacgcctccgtcccatgcacgtctttatcctggattacgaccaatcgcccgccggctgccgggacgccctgctgcaacttacctccgggatgatccagacccacgtcaccaccccaggctccataccgacgatctgcgacctggcgcgcacgtttgcccgggagatgggggaggctaactgagtataccctaggattatccctaatacctgccaccccactcttaatcagtggtggaagaacggtctcagaactgtttgtttcaattggccatttaagtttagtagtaaaagactggttaatgataacaatgcatcgtaaaaccttcagaaggaaaggagaatgttttgtggaccactttggttttcttttttgcgtgtggcagttttaagttattagtttttaaaatcagtactttttaatggaaacaacttgaccaaaaatttgtcacagaattttgagacccattaaaaaagttaaatgagaaacctgtgtgttcctttggtcaacaccgagacatttaggtgaaagacatctaattctggttttacgaatctggaaacttcttgaaaatgtaattcttgagttaacacttctgggtggagaatagggttgttttccccccacataattggaaggggaaggaatatcatttaaagctatgggagggtttctttgattacaacactggagagaaatgcagcatgttgctgattgcctgtcactaaaacaggccaaaaactgagtccttgggttgcatagaaagctgcctgcaggcgttacataacttacggtaaatggcccgcctggctgaccgcccaacgacccccgcccattgacgtcaataatgacgtatgttcccatagtaacgccaatagggactttccattgacgtcaatgggtggagtatttacggtaaactgcccacttggcagtacatcaagtgtatcatatgccaagtacgccccctattgacgtcaatgacggtaaatggcccgcctggcattatgcccagtacatgaccttatgggactttcctacttggcagtacatctacgtattagtcatcgctattaccatgatgatgcggttttggcagtacatcaatgggcgtggatagcggtttgactcacggggatttccaagtctccaccccattgacgtcaatgggagtttgttttgactagttaccggcggaaacggtctcgggttgagaggtcacccgagggacaggcagctgctgaaccaataggaccggcgcacagggcggatgctgcccctcattggcggccgttgagagtgaccaagagccaatgagtcagcccggggggcgtagcagtgacgtaagttgcggaggaggccgcttcgaatcggcagcggccagcttggtggcatggaccaatcagcgtcctccaacgaggagcgccttcgccaatcggaggcctccacgacggggctggggggagggtatataagccgagtcggcggcggcgcgctccacacgggccgagaccacagcgacgggagcgtctgcctctgcggggccgagaggtaagcgccgcggcctgccctttccaggccaactcggagcccgtctcgtggctccgcctgatcgggggctcctgtcgccctcagatcggtcggaacgccgtcgcgctccgggactacaagcctgttgctgggcccggagactgccgaaggaccgctgagcactgtcctcagcgccggcaccatggattggatctggcggatcctgttccttgtgggagctgccacaggcgcccattctgaagttcagctggttcagtctggcgccgaagtgaagaaacctggcgcctctgtgaaggtgtcctgcaaagcttctggcggcaccttcagcagctacgccatctcttgggttcgacaggcccctggacaaggcctggaatggatgggcagaatcatccccatcctgggaatcgccaactacgcccagaaattccagggcagagtgaccatcaccgccgacaagagcacaagcaccgcctacatggaactgagcagcctgagaagcgaggacaccgccgtgtactactgtgccagaagcggccacggctacagctacggcgcctttgattattggggccagggcaccctggtcaccgtttctagcggaggcggaggtagtggtggcggaggttcaggcggcggaggatctcaatctgtgctgacacagcctccaagcgtgtcaggtgctcctggccagagagtgacaatcagctgtacaggcagcagcagcaacatcggagccggctatgacgtgcactggtatcagcagctgcctggcacagcccctaaactgctgatctacggcaacagcaacagacccagcggcgtgcccgatagattttccggctctaagagcggcacaagcgccagcctggctattactggactgcaggccgaggacgaggccgactactactgtcagagctacgacagcagcctgtccggcagctacgttgtgtttggcggcggaacaaagctgaccgtgctggaagccaagagctgcgacaagacccacacctgtcctccatgtcctgctccagaactgctcggcggaccttccgtgttcctgtttcctccaaagcctaaggacaccctgatgatcagcagaacccctgaagtgacctgcgtggtggtggatgtgtcccacgaggacccagaagtgaagttcaattggtacgtggacggcgtggaagtgcacaacgccaagaccaagcctagagaggaacagtacaacagcacctacagagtggtgtccgtgctgacagtgctgcaccaggattggctgaacggcaaagagtacaagtgcaaggtgtccaacaaggccctgcctgctcctatcgagaaaaccatcagcaaggccaagggccagcctagggaaccccaggtttacacactgccacctagcagggacgagctgaccaagaatcaggtgtccctgacctgcctggtcaagggcttctacccttccgatatcgccgtggaatgggagagcaatggccagccagagaacaactacaagacaacccctcctgtgctggacagcgacggctcattcttcctgtactccaagctgactgtggacaagagccggtggcagcagggcaatgtgttcagctgtagcgtgatgcacgaggccctgcacaaccactacacacagaagtccctgtctctgagccccggaaaaggtggcggtggctcttacccttacgacgtgccagattacgccggctatccctacgatgtgcctgactatgctggctacccctatgacgtccccgactacgcttaactagctacggaattccggctagctggccagacatgataagatacattgatgagtttggacaaaccacaactagaatgcagtgaaaaaaatgctttatttgtgaaatttgtgatgctattgctttatttgtaaccattataagctgcaataaacaagttaacaacaacaattgcattcattttatgtttcaggttcagggggaggtgtgggaggttttttaaagcaagtaaaacctctacaaatgtggtatggaaatgttaattaactagccatgaccaaaatcccttaacgtgagttttcgttccactgagcgtcagaccccgtagaaaagatcaaaggatcttcttgagatcctttttttctgcgcgtaatctgctgcttgcaaacaaaaaaaccaccgctaccagcggtggtttgtttgccggatcaagagctaccaactctttttccgaaggtaactggcttcagcagagcgcagataccaaatactgttcttctagtgtagccgtagttaggccaccacttcaagaactctgtagcaccgcctacatacctcgctctgctaatcctgttaccagtggctgctgccagtggcgataagtcgtgtcttaccgggttggactcaagacgatagttaccggataaggcgcagcggtcgggctgaacggggggttcgtgcacacagcccagcttggagcgaacgacctacaccgaactgagatacctacagcgtgagctatgagaaagcgccacgcttcccgaagggagaaaggcggacaggtatccggtaagcggcagggtcggaacaggagagcgcacgagggagcttccagggggaaacgcctggtatctttatagtcctgtcgggtttcgccacctctgacttgagcgtcgatttttgtgatgctcgtcaggggggcggagcctatggaaaaacgccagcaacgcggcctttttacggttcctggccttttgctggccttttgctcagggttcgaaatcgataagcttggatccggagagctcccaacgcgtcggctagctagtagggataacagggtaataagcgtcgacggcgcgcccctaggggccggccttaattaaatcaagcttatcgataccgtcgaacctcgagggggggcatcactccgccctaaaacctacgtcacccgccccgttcccacgccccgcgccacgtcacaaactccaccccctcattatcatattggcttcaatccaaaataaggtatattattgatgatgttt

SEQ ID NO: 121 - DNA, 30881 bp, synthetic construct
  source 1..30881: mol_type = other DNA
aaacatcatcaataatataccttattttggattgaagccaatatgataatgagggggtggagtttgtgacgtggcgcggggcgtgggaacggggcgggtgacgtaggttttagggcggagtaacttgtatgtgttgggaattgtagttttcttaaaatgggaagtgacgtaacgtgggaaaacggaagtgacgatttgaggaagttgtgggttttttggctttcgtttctgggcgtaggttcgcgtgcggttttctgggtgttttttgtggactttaaccgttacgtcattttttagtcctatatatactcgctctgcacttggcccttttttacactgtgactgattgagctggtgccgtgtcgagtggtgtttttttaataggttttcttttttactggtaggcgcgccgtcgacgcttattaccctgttatccctactagctagccgacgcgttgggagctctccggatccaagcttatcgatttcgaacccaaatggatctaccacatttgtagaggttttacttgctttaaaaaacctcccacacctccccctgaacctgaaacataaaatgaatgcaattgttgttgttaacttgtttattgcagcttataatggttacaaataaagcaatagcatcacaaatttcacaaataaagcaatagcatcacaaatttcacaaataaagcatttttttcactgcattctagttgtggtttgtccaaactcatcaatgtatcttatcatgtcgagctagctagtcaggacttcagttccagctttgtgccggctccgaaggtcagcgggttgctagaccattgctgacagtaatatgtggcggcatcctcggcttccatagagctgattgtcaggctgtagctggtgccagatccagatccgctgaatctgtagggcacgccggaggccactttgcttgtgtcgtagatccaccgcttggggcttgtgccagacttctgctgataccagttcatgtaggacacgctgctgctggctctgcatgtcatggtcactttctcgcctggggaagcgctcatgatggcggggctttgtgtcagctgaatatcggagccaccaccaccgcttccaccaccacctgaaccgcctccgccactagaaactgtcagggttgtgccctggccccagtaatccagacagtagtggtcgtcgtagtaccgggcacaatagtacacagcgctatcttcagaggtcaggctggacagctgcatgtaggcggtagagctgctcttgtcggtggtcagtgtggccttgtccttgaacttctggttgtaattggtgtagccccggctggggttgatgtagccgatccattccagtccttggccaggcctctgcttgacccagtgcatggtgtaccgggtgaatgtgtagccgctggtcttgcaggacatcttcacagaggcgccaggtctagccagttcggcgccagactgttgcagcttgatatcggatccgccacctccgccagatgacactgtgaccagtgttcctctgccccagtagtcgaggccctgtctggcgcaataatacacggcggtgtcctcggctctcagggagttcatctgcaggtacaggctgttcttggcgttgtcccggctgatggtgaatctgcccttgatgctgtccaggtagtaggtgtagctgccgccgctgctgattgtggacacccattcaaggcctttgccaggagcctgtcggacccagctcatatcgtagctgctgaaggtgaagccggaagcggcacagctcagtctcagagagccgccaggtttcacaagtccgccgcctgattccaccagctgcacttcagatccaccaccgccactacctccgcctccgcttcctccgccgccagatcctccgccacctctcttgatttccaccttggtgcctccgccaaatgtcaggggattgctggaccactgcaggcagtagtacacggcgaagtcctcaggttccaggctgcttatggtcagggtgaaatcggtgccgctgccagagccagaaaatctggcaggcactccgctggccagattgctggtcaggtagatcaggattctaggggcctgtccgggcttctgctgcagccagtagatgtagttgatggagctgctggcgctacagctcagggtagctctctcgccagggctcagagacagtgtggctggagactgtgtcagcacgatctcgccggtggtatcaggcagccaaagcagcagcaggaacagcagctgagcaggggcttccatggtggccctccttcgccggtgatctcagctgtaggaaagagaagaaggttagtagtcgacgtgtccctctcgatgaatctaagtatcaattgtgagcgctcacaagtcaacactctttttgataaatctagtagatatcacttacgtaggcgccggtcacagcttggatctgtaacggcgcagaacagaaaacgaaacaaagacgtagagttgagcaagcagggtcaggcaaagcgtggagagccggctgagtctaggtaggctccaagggagcgccggacaaaggcccggtctcgacctgagctttaaacttacctagacggcggacgcagttcaggaggcaccacaggcgggaggcggcagaacgcgactcaaccggcgtggatggcggcctcaggtagggcggcgggcgcgtgaaggagagatgcgagcccctcgaagcttcagctgtgttctggcggcaaacccgttgcgaaaaagaacgttcacggcgactactgcacttatatacggttctcccccaccctcgggaaaaaggcggagccagtacacgacatcactttcccagtttaccccgcgccaccttctctaggcaccggttcaattgccgacccctccccccaacttctcggggactgtgggcgatgtgcgctctgcccactgacgggcaccggagcgatcgcagatccttcgatagagaaatgttctggcacctgcacttgcactggggacagcctattttgctagtttgttttgtttcgttttgttttgatggagagcgtatgttagttacgattcacacaaaaaaccaacacacagatgtaatgaaaataaagatattttattgcggccgctcgagtctagaggacatgccatggtcgtattaccctgttatccctaactgcatgcgacgtcggcgcgccatcgaattcctgcagcccgggggatccctttgttgattttttccacatagattatttttgactgttttggcactttatataaatggaatcatatagtaaatatatacatgtatatatgtatatatacactatatatgtatatatatagtgtatatatatacatgtatatatgtatatttacatatatactgtatatatgtatatttacatatatactgtatatatgtatatatacacgtatatactgtatatatacagtatatactgtatatatatactgtatatatgtgtatatatatatacagtatatatacagtatacatatatatacatgtatatatacacagtatatatacatgtatatatacacagtatatatacatgtatatatacacagtatatatacatgtatatatacacagtatatatacactgtatatatgtatatatatactgtgtatatatatacagtatatatacagtatatatatacatgtatatgtatatatatactgtatatatgtgtatatatacgtatatatactgtatatatatatagacacttttgtgtctggcttcttgctctcatcataaagcacttgaaatccatccatgttgtagctggtatcagtagctagtttcttttcattgctgagaagtatcactttttattgatgagtagttttacattgtatgaacatgcccgagtttgtttatgcattctactaatagacacctgggctgtttgcagtttttggctattacaaagaaaatttctatatttttttccaacttttattttaggttcagcgggtacatgggcaggtttgttacatcggtaaattgcatgtcactggggtttggtgtacagattatttcaccacccaggtaataagcatagtacctgataggcaggtttttgatcctcaccctcctccctcaagtaggccccagtgtctattgttctattccttttttttttttttgagatggagtctcactctgttgcccaggctggagtgcagtggtgcgatctcggctcactgcaaggtccacctccagggttcaagcgattctactgccgcagcctcccgagtagctgggattacaggcacccaccaccacgcccggctaatttttgtatttttagtagagactgggtttcaccatgttggccaggatggtctcgaactcctcacctcaggtgatccgcccgcttcggcctcgcaaagtactgggattacaggcgtgagccacggtgcctggcctatggttccattctttgtgtacacgtgtactcagtgtttagcttccacttgtaagtgaaaacatgcagtatttggttttctgaaattcttgtcttcatctttttgtagacaatccactacttttatttttaaatattaggaacaatagcctctgtgtgtcctgaattgcaatgttttttctctgattttgctgctcatcttgtaacctgtatggtgtttttctgtgtgcaagctttttactttacgtgggcaattttatcattcttttcttttatggtttctgggtttcatgtcatgattggagaagcttgatctaccctgatactataaaaatatccaccttggcttttttttttttttttagatggattttcactcttgttgcccaggctggagtgcaatggcgtgatctcggctcaccacaacctctgcctcccaggttcaagtgattctcctgcctcggcctcctgagtagctgggattacaggcatgcgccaccacgctcagctaattttgtatttttagtagagacaggatttcaccatgttggtcaggctggtcttgaactccccacctcaggtgatctgtctgcctcggcctcccaaagtgctgggattacaggcgtgacccaccacacctggcccacgttgttttctgatagtgttttcacgtgttattttttctgtcttactctttgaatcatctaaatgtatcttaatgtcaggagtgaggtagaggacccagttgtttggtttaaatgactagccagttttcccaacaccaggtgttgaacatccctcactgatgtgagatgctgcctttttcacagtctcaatccccatgtgcatttctatttattttccttccactttattcacatctttttcagtatccacaaccatattgttttaaatagcttcatgatatgttttaatatttggtagagctagaaccctttcttggttctttttcttttcttcttctcctccttttcctcctccttctttctcctcctccttcttctttctttttagaaatttcctggctattcttgttttgtagtcttccagataaataattttgaatcactttgtcatgttccagaaaataatactgccagaatttttattgtgatcacagaagttttacagattcatctgggggaaaaaaacccatcttcccagaatacagaaagggtgagggaaagacaaacatcaaggacaagtctcaggttctggacttggagaccaagaggatttggggcatccgggagcagggcagggaggtgtgatggctgcctttcactgagtaggaggatgcccagacttgggggaactatggaaagtttggttcagactttctgagttggagatgtctatgcgcagtccacagggcgaagccctggaggtagaggccctccttactgcctccctcattcagtctgaggtccattctccacatggacactgaagtgactcaaggcttcccttgttggatcaggatagtctccagggccctgggtggtctgggcctgcccacctccccatcccctctcctgcctgccctcctcttgctcactggaccccacccaccagcctccttctattcctcctgacatttgcacttgctgttccgtctctgcttggaacatcctagctctttgcatggcttgctccttcccatcttttaatctaagctcaaatatcactccttcagatatgcctttcccaaatatcctagctaaagagaactgctccccacttcccacaagccctagcaaactgggactctccttcttgctttctttctctctgccccttctgtgttttttccatagaccttaacttgttactgttttatttgttgatgtgtttacatcatttgtccccctgtgatggttagttttatgtgtcaacttggctaggctgtaggggctgttcgtcaatcaaacactgatctatgtgtagctgtgaagggattttgtagctgtgattaatagttgactttaagtaaggaagattatcctggagaatgtgggggaaggggcagacctcagccaatcagttgaaaggccttaagaacaaagctgagatttccccgaggaagaagaaattctgcctgtggactgcagcatcagctcctgcttgagaggttccaggctgcccttcctgacagcctgtcctatgattttggacttgccttgccaggtttttcctctttcttgaccccccaaaaccatatatatctcctgctggtttgtttctctggtgtaatcctgagggatgaacactcctccctcccagttcactctgggagaggttggggatcatgtttgtctatttccccatgcctggcccatgcgtgtttattgaatcactgaacaaccacgcattaggaagccagtcatatgtgcttcttcagaacctcatgtccattgccagatctccctggcttttgtggctagaggacaagtgagagatagtagcttacccacagaccttggccctgaggcccccaggggcctgagcctgctgtaagggaggagggagcccctgaggtctcacacacctccctggggatctggcattttcccctggggctggcctcagagctgggcgggggcagattatggagtgggttgtagagggagcacctccccactagcaatcatggttttttctgcgcctctcatagggaggcctacaggcctccaccttcagctcttcaggagccacaggcagctgagtgacttctgcatcacagtcttctcagagacaaacttgcagtaagaaagaggggcccgtgagggaccccagagaaggctgttgtcaaagcaggatgagagtgaactcttccatgggggacacccagcgtctccaagctcttttatgctgtcttcaaggggtctagagagcttcagcccaacatgagacccagtccagcagcatttccctgcgaagtgaaagttaggaccctgactagatacaccacgctgacctcagccagaatatcaagatgctgaggcgctgagatgctgggatgctaaggtgctaaggtgctggggtgctggggtgctaggatgctgaggttttgtgatactgggtcgctgagatgctgggatactggggtgctgaagtgctggggtactggggtgttgccatgctgaaatgctggggtgttgggatgctgaggtgctgggttgctgggatgctgggatagtccttggatgctgcggtgctgagatgctggtctgctggtctgctggggtgttgggatgctgggattttgggatgctggagtgctgcagtgctgcagtgctgagatgctggagtgctggggtgctggaatactgtagtactggtgtgctggagcattgagatgctagggcactgggatgctaaggtgctgagatgctgcagtgctggggtgttgggatgccgaggtgttgggatgcttaagtgctggggtgttgggatgctggggtgctggaacactatggtgctggggtgctggagtgttgagatactgtagtggtgggatgcttaagtgctggggtgctgggtgttgggatgcctaggtgctggggtgccgagatgctggagtactagtgtgctgggatgctgaagtgctggggtcctgagatgctgcagtgctagggtgctgagattctgggctgctggagtgttggggtgctgggatgctggagtgctgagatgcttggacaatggggtgctggaatactatggtgctggggtgctggggtattgagatgctagggtactgggatgctgaagtgctgagatcctggagtgctgggctgctgggccacaggctcttgaatccattcgtctgcccaggggaagaaaccagaagataaagagctaatgaaggagctttggttgagagggaggaagtaatggaaggagcaacatcttgtggaggagcaggagagaatggacctcaggttgggagagagggccaggctacaggccagagaggcagaaggattccagcagagtgtgggctccaggagccaaggggaaacaggtttctgggaggagagagtccagtactgctgaagtggcaagtccgctgaggaccaggaagcttcatttggctttatgaccaggaggaatttggaactgtgactagagtacttagggggaaggaggcaagactggagccagattgctctgggttgaggggtgagtgggaggtgaagcagggcactgtcactcctttgaagggtggcagagagctggaattggtgctggatgggctgtggggtgacagggtcatgtggaaagcccctggggggcacctggaaaaggagaagctgacagtacagtgagaggacagctaagggaaagcggaatggcagaacacgcactgccaggaggaatgaggatagggtcaggagtgccaggggcagtgaggccagcctggggtcaggtggcaggacgtgtccaggaagctggtctgcactgcagcccacactggctcagccttgaggttccctgtgtggttggggtaggaagttgaaccctctgggaatggaagatggaaccagctctgcgagccaagctcagcttttatctatgggtctctgagggctggcagagctgagtggggacaactgtgatccgtgaggctctcaggttgaggtggcccctccgggagggcttcattttcccagcgggtaggttctaagcagcagtggctgggcaggtgggtccaacacagagccagagaagggtgaatgggcctcctggcaccccacccctgctgcccctgagctcagtgatggagggggacagcacagctgagcccaagtgctttggtgtggccctgagggaaagctgcagcctgcctggggcctggcatggatgggacacttgaggcagagggacaatagtgggcgctgcagtgaggctggctcttggagaggtttcctgaggagtgctgcctgagacgggcagggagaacagagacaaagttggtgacagggaatgaaagctgactgaaggactttacccagacctatgaggatatctctctcagcaggaagcaggaggggactgtgtgaggactggccaagagctggagtgttgggaaaatgactctttctccgacccctctgtcctagctctggcccctggactgcggaggtctgcttccacccccattggtcgatcgttgtcccttgtcacagccattgagaattttggcagggagcatgttcttagagcatttttaggctctgcgggacataacagctctgcctcagagcacatgcctttctcagctcctgaaagccactgatcaaattggaacattttgtaccttagggatgaggatatcaactctcccagccacttagagggataaatgtgatgatgcattcaattgtgactacatctgatcccaactgttgcttcagctgctctcctatagcacatggcgggaggcgtgcatcccagtagctacctccccacttttggggagatgtggttccatccatgaaacctgggtacccgcctaccaggtcctggcctatcaggtggcagggtctggtcaaagaagggcatgtgtggtcttcagcaagggagacaggacggtggtgcagagcgtctagaccctcagggcaagtctcccccacacctgctcccggggcagttgtctttgtgacctcccatccccctctgtttcatcctctataaaatgaggggctgagccccaaaataacaggcttctttgccatgatgcaaaactgctgaatctttctttctgacacacaaggcatcgagcagcctctgaaagaaccaaagccactagcaggcttcctgacttgggtttgtaggtactgaatactcccttgaaaaataaaaacatagaggcacttttctcctggctgtttattacagaacgaagaaaaaacacactggcttgaaacagacgccagatttcaaatgtagaggtgaaatacgaggtggcaattaaaatgtgattacagaaagtctggacactgagaaaagtttacaggacagtgggtgtgggttttctataacagacacttaaatatacatgacgataattgcagatagaaaccatcaaagacaaaccccaaatcaactaataatgtttacagatgttcccccccaaaccacagagccttacatcaaaacaaatactgaaaggctttaaaccaggaacagctcgccttaaccccacgagggtgcacacaagctgggctttttctctcggtctgaatggtaaagggaggaggatactctagctcctccaggtggattgctgagacagggctcggctcacacactgtctctgcgcctctcccaaatctggagaactctcccagcctcctggtaaagtgtctctgtggggcacttaacgataaaacagcttctgctgtaaagctcattaggaaagagctagcggagactgaaaggttcgcaaaagagattaagaatcacacaaggcaataggatttttagtgaacatagaaataaatggccaagtggttttctatttggcatttgtcaacttgcacaacaactcttggtcatatccacattgctcattgcattaaaaccataagcgactcagccacctagcttaacaaggtatcactggagcaaacaacacggtctgcatatttgtaacattgtataataaacacaaaacaatgcatagtaaacacaactctactgaaacaaaagccgtcgctttatttacaaagtcacaaaatgaagtataaatacttctgtcattaatgtttaggaaaaccatttacaaaattttcaaatatgtacacgtagcttgaaaaatcaccagctttccattttgtcacaggtagagagagggataagcatgggctgacaacaccactcaaattgtaacgggagacaactgcgggtatggatcgacaccacttcctagagtgatgtcaccatgggggtttctatgggcatcctgctcagatttaaagtgccccagcatcctgggtgacttgcccagaattctgggctgtggcattttgagcagcagcatgctgttccaaaatgtcgtcgatcagcctcaagttgcacacccagtcttcatctgggctcacacaggagcctttcaagagagcttcaatgaaatctacctcattgcagtcaggtgacgaaatcagatcatttagtgggggttggggctggcgcaaaaagtcggcaggtggcagctcagggggaatatccgttctgtcgaacggacctgggaactggctggcagcaacggcagaagcagcagcagcggtggcagcagcagccacatagcttggtggctcgatgccctgtatggggctcaggggactaaagctggccataccctgctggaggaacttggtggtgtttgctacaggcaccgggccctgtaccgggctctgcctgaggctctggctgcccagcaggctgaagctggggttgttggccaggggcacttgtgttcccatcgcagcgggcacttgtgcctcccaatcagatggcctctgaaggcaggcctggccagaaggtgagtgctgctgaacgctattatccacttggctgaggggtgttttccccgaaactgctgtggtcacagctgctgccgctgtgacccatgcagcattgttgaacgcagtgggcattcttggcacactaggccgtctgagctggtggggactcaaggactgggtgcccagggagctgggacagaacccaggcaggggcacttctggtggggtggccttggggctctgcatatgctggcagacagagtcaagtctgcccaggggagtctggcctgagtgtgagaggatgggacactgggggctggaggtgaaaattccttgccgcttccccagagttggtgagatcactcccatgccctcgcagctctggtgcctggtgagtgggatcattcctggactcagattgttctgaagaagcccagttctgggtggcatcaagtgcttgctagatggggggcttgccttgatccggctacacttggaggtgacttgttcttggacggctacatacagaaagagagaagtggggatgagttccaaaggcatcctcgacttcggctgtggccaccggagggtagctcctggcccaacacggacttctcacctcccgcccttggctctctactgagctcccccctgctccccaattcctcgccattcccctcatttctctgccctcagcctggactgcagttcttctgggaagctgccccaactccctaggtctgtgctcaccaagagcagatcacactggactgaaatgccagctgatttgtctcttcaagaaaattggaagctcctggaggtcagggtccatgtctgcttttacactcagtgctctgtatgcaggcctggcactgcccaccctttgacaggtggtgcatattttgtagaaggaaggaaggggccaggtggggtgggctgggctggtggcgggagctagctcagcctcttagattctctacccgatggatgtgacctgggacagcaagtgagtgtggtgagtgagtgcagacggtgctttgttcccctcttgtctcatagcctagatggcctctgagcccagatctggggctcagacaacatttgttcaactgaacggtaatgggtttcctttctgaaggctgaaatctgggagctgacattctggactccctgagttctgaagagcctggggatggagagacacggagcagaagatggaaggtagagtcccaggtgcctaagatggggaatacatctcccctcattgtcatgagagtccactctagctgatatctactgtggccaatatctaccggtacttttttggggtggacactgagtcatgcagcagtcttatggtttacccaaggtcaggtaggggagacagtgcagtcagagcacaagcccagtgtgtctgacccacccaagaatccatgctcgtatctacaaaaatgattttttctcttgtaatggtgcctaggttcttttattatcatggcatgtgtatgtttttcaactaggttacaatctggccttataaggttaacctcctggaggccaccagccttcctgaaacttgtctgtgctgtccctgcaactggagtgtgcctgatgtggcactccagcctggacaagtgggacacagactccgctgttatcaggcccaaagatgtcttccataagaccagaagagcaatggtgtagaggtgtcatgggctacaataaagatgctgacctcctgtctgagggcaagcagcctcttctggccctcagacaaatgctgagtgttcccaagactaccctcggcctggtccaatctcatcccactggtgcgtaagggttgctgaactcatgacttcttggctagcctgcaacctccacggagtgggaactacatcaggcattttgctaactgctgtatcctaggccaataaatgttgatcacatttatagctgccatggtagggtggggacccctgctatctatctgtggaggctctgggagcccctgacacaaactttctgaagcagagcctccccaaccccttttccattccctatacctgacagatggcccaggaacccattagaaatggaaggtcactgcagcagtatgtgaatgtgcgtgtgggagaagggcaggatcagagccctgggggtgtggcagcccccaagtgattctaatccagatcctagggttgtttccctgtcccattgaaatagctgctttaaggggcctgactcagggaaatcagtctcttgaattaagtggtgattttggagtcatttagaccaggccttcaattgggatccactagttctagagcggccgggcccagggaaccccgcaggcgggggcggccagtttcccgggttcggctttacgtcacgcgagggcggcagggaggacggaatggcggggtttggggtgggtccctcctcgggggagccctgggaaaagaggactgcgtgtgggaagagaaggtggaaatggcgttttggttgacatgtgccgcctgcgagcgtgctgcggggaggggccgagggcagattcgggaatgatggcgcggggtgggggcgtgggggctttctcgggagaggcccttccctggaagtttggggtgcgatggtgaggttctcggggcacctctggaggggcctcggcacggaaagcgaccacctgggagggcgtgtggggaccaggttttgcctttagttttgcacacactgtagttcatctttatggagatgctcatggcctcattgaagccccactacagctctggtagcggtaaccatgcgtatttgacacacgaaggaactagggaaaaggcattaggtcatttcaagccgaaattcacatgtgctagaatccagattccatgctgaccgatgccccaggatatagaaaatgagaatctggtccttaccttcaagaacattcttaaccgtaatcagcctctggtatcttagctccaccctcactggttttttcttgtttgttgaaccggccaagctgctggcctccctcctcaaccgttctgatcatgcttgctaaaatagtcaaaaccccggccagttaaatatgctttagcctgctttattatgattatttttgttgttttggcaatgacctggttacctgttgtttctcccactaaaactttttaagggcaggaatcaccgccgtaactctagcacttagcacagtacttggcttgtaagaggtcctcgatgatggtttgttgaatgaatacattaaataattaaccacttgaaccctaagaaagaagcgattctatttcatattaggcattgtaatgacttaaggtaaagagcagtgctattaacggagtctaactgggaatccagcttgtttgggctatttactagttgtgtggctgtgggcaacttacttcacctctctgggcttaagtcattttatgtatatctgaggtgctggctacctcttggagttattgagaggattataagacagtctatgtgaatcagcaacccttgcatggcccctggcggggaacagtaataatagccatcatcatgtttacttacatagtcctaattagtcttcaaaacagccctgtagcaatggtatgattattaccattttacagatgaggaacctttgaagcctcagagaggctaacagacataccctaggtcatacagttattaagagaaggagctctgtctcgaacctagctctctctctctcgagtaataccagttaaaaaataggctacaaataggtactcaaaaaaatggtagtggctgttgtttttattcagttgctgaggaaaaaatgttgatttttcatctctaaacatcaacttacttaattctgccaatttcttttttttgagacagggtctcactctgtcacctaggatggagtgcagtggcacaatcactgctcactgcagcctcgacttcccgggctcgggtgattctccccaggctcaggggattctcccacttcagcctcccaagtagctgggactacaggtgcgcaccaccatccctggctaatatttgtactttattttatttatttatttatttattttttgagatggagtttcgctcttgttgcccgggctggagtacagtggcatgatctcggctcagtgcaacctctgcctcccgggttcaagcgattctcctacctcatccccctgagtagctgggattacaggcgcctgccaccatgcctggctaattttttgtatttttaatagagacgaggtttcaccatgttggccaggctactctcgaactcctgatctcaggtgatccacccgccttggcctcccaaagtgctgggattacaggcgtgagccactgcgcccggcctaatatttgtattttttgtagagatggtgttttgccatgttgtccaggctggtcttgaactcctgagctcaagcgatctgcccgcctctgcttcccaaagtgctgggattacaggcatgagccaccgtgcctggcctaggtagacgcttttagctttggggtgtgatgcctgccccagtatatagtgaatttaattattgctagagctggctgtttgttagttttctttgaacataagatactcattgtttttagtttgcaaatccctcttcctttttaaaaaatttctttcccttaaattgtttgcatgttagcaataacaaatgcttaaatggtgctatgtgctagatactcttctaagccctgttatgtatattaactaattttttaaattacacaaatcagagaggttaagtaacttgcccaagattacccaacaatactaggatttgaacctaagtttgtctcaccccagattctgctcttaatctctaaacttttaagttagtagtgacaatagtaggtatttattgaatacttaactatgttttaggcgttgaagtaaatattttgcaggcattatctaatgtaaacaccctaaagttacataacaggtaccctttaggtaaataaacactagtatgaccttggaggcacagatagttgaagtaacttgcccaatatcacttacatgaaattggccctcaaatgtgtctgatacaacccatgctgcttgtaactatcgttttaaactgccagggtaaacttggacacacttgagctaagaaaaagcttttagatttttgcaaattaatgtgaaagatatgctttatgtggatataatatcttctaaatttcggggatggtagtcctagaaatgtaatcctgccctagccgagcttaccctgccaataattttttacagaattggtaaaacggagcaccttttttttgtccttggccacactgttatcaacagggtgtagattgacatcaatctgtaggtgtaaaccagaattactctttgtgaccaccaggaaatagagcagttcagttcaggggtttctttctgtgaatttagcactgtgacctgcatactacaagtctactttgttttctatccattgtttgtatctgggtattgcaaaaggtaggaaaaggaccaaccagatcagcagagaagagttgccttggagttttcttttagttttctgcagttcattagatagtaactaggccatgtcattttactcccttgtagtgaagatatgttgaagttgtactggtatactcttctacctttctgtaattttatattgtgtagacttgataaaatttatgtgtcaatcaccaccattaatatcaatattgagcctcaattcttatttttctgcccagtggctgccaaattactaacatttacaataattcactactactaagataatctactagttcgatcacatacttcaaattgttatggaactactgtcttcagcattgtgcttctgataactgataagtataattttttttttgtccagagtgaacatgtctattcttccactgtacacactaataaaaggaaaaattgtaatattgggtaaattcatgtccttacacatgtagtagttatgagcccatgtccctagaatgagtaataatttatccctcccttggttgaatagtcaagaatgctgattttaattcttctaacagctttatccctcagaagggaaggcaagcaagttatatatgtagtttatttgtaagactgatatgaaattggaagatgaatctactattagctttaattatttttacatttaggaatattgcatcagtaactcataattttggttttctgttatcctgagttaacacaaattatccaaggagatggcggatcatctgctttgaggtgtttttttttgagaattttaatgtatctgaatataaaaggtaaaaatatgccaactagcaatttctgcccattccagaagtttggaaatattactcattactaggaattaaataaaatatggtttatctattgttatacctcttttaattcacatagctcatttttatcttttatttttgtttgttttttttgagatggagtcttgctctgtcaccaggcaggagtgcagtgatgcaaatctcggctcactctagccaccgactccctggttcaagcgattctcctgcctgagccttctgagtagctgggattacaggcaggcaccaccacgcccagctaatttttgtagagacaggatttcaccgtgttggccaggatggtctccatctcctgacctcatgatctgcctgcttcggcctcccaaagtgctgggattacaggtgggagccactacgcctggcccacatagctcatttttagactcacttccattaagtcttgtttggacccacgaacattgtctttttttttttaagatggagtttcacttttgttgcccagactgtagtgcaatggtgcaatctcagctcactgcaatctctgcctcctgggttctagcaattctcctgcctcagcctcccgagtagctggaattacaggcgcccgccaccacgcccagctaatttttgtgtttttagtagagacggggtttcaccatgttgggcaggccaggggtgatccgcccacctcagcctcccaaagtgctgggattacaggtgtgagccaccgcatctggccaacatgtcttttttttttttttcctttttaaccacaaagagacttaagcagtccttgtcacagatgatgaattgatgttgcaagtattgtcttagcttggattaattttcttgcttactgtaattttagataatatagctttgtaattagagattttatgtgtaaaccacaaaaatgtttacatgaaggccattattacagatgtgacgtgcataattattagtaatttgtatgtttacatgggtcagtctggcaaaaaattatgaagttttaaaaattaaaaaaaattataatgccagttttactggaaagtaaaattatttcagtaatcgattatagcaaaagtattgattttcattccagacaaaagtcagaatgaaaggtaatttctcaatactctttcagattaataaaagtacctgtagcgatttttatcattcacaagtatatcacaagtaagttagaatttgagaactgtgttctagatctctgaggagatgcagtcagatttctgaactgtctcagcaaatggtaagtaacttagagctagtaattaataacctgtcctttgatttctgattcagccaagaatggccatatttgggaaaggcagatctggagagtaaccacgttttcattcatttaccacttctaggcccctccagagctctcagatattttggggttgagcccttccccaaagccatacaggaccttttttttgtgatctgttctagccatttttatgttgggtgcttgttatggactgagcatttatgtcctcccacaccccccccataccttttttgaagtcctaacccccagtgtgatggtatttggagacagggcctttggaaggtaattacagttagaagaagtcgggagggttgggcccaggtctgattggattagtgcccttatatgaaaagacaccaggacgggcgcagtggctcacacctgtaatcccagcactttgggaggccaaggtgggtggatcacgaggtcaggagtttgagaccagcctggccaatgtagtgaaacaccatctctactaaaaatacaaaaattagctgggtgtggtagcgggctcctgtcatccaagctactcgggagggtgaggcatgagaatcacttgaacccgggagttggaggttgcagtgagcccagattgtgccactgtactccagcctgggtgacagagtgagactctgtctcaaaaaagaaaaaaaaaaaaaaagagacaccagagagcttgttagaagaggtcatgtgagcacacagttagaagaccttcaagccaaagaagaggcctgagattgaaacctaccttgcaggtaccttaattttggacttcccagcctccaaaactgtgagaaataagtttctgttaagtcactcagtctgtggtattttgttatggcagcctgagcaggtagttgttctttcagaaggtgttgataataaccacatgcaacaccaagtcacaaataataaaacagatgtaacttatattcatacagaaagttgggcactgccattgccttgttggtttacacggctgtgctagttcagtagcagaaaggtgctggtctcctttactcagtttacaatctaggcagtagaatgtaatcactgctttaaacttgatactgcttagggagagaatcattggtgctgggtaactttgggttctaggtttactttttgtgtatatataactgtttttggtaaatcacaagtttctgggcttgtcgaattagattttgttacagattatgagctttattatgctatacagttagttgtatgtatatatgcctttcccactagattttaagctttttttttttttttttttttgtgacggagtcttgctcttgtcgcccaggctgaagtggagtgcagtggcacaatctcggctcactgcagcctccacctcctaggttcaagcgattctcctgcctcggcctcccaagtaactgggactacaggcacgtgccaccacacccggctaatttttgtattttttgtagagacagggtttcgccatgttggctaggctggtcttgaacttctggcctcaggtgatccacccgcctcagcctcccaaagtgctgggatttacaggcatgagccaccacgcccagctatagctctttaagggttgtaaatttataatcattcttttactctcctgcaaattctgttgcacactgccttaatcaaggtagatgctgaatgcatttttgtataattgaatatgttgcaatccccaactctctccaactgttcctgtcaaagcagccactggattgttaactaatccatattagatggggttaattaatatcagatgggacaagtaagggctaataagattataggccaccaagtagatttctgtctagctcttatagagattgagtttattggacctgtttgataggaagttttggtgtttgggatgattaaaactgaagttcctatttattgaattatacctatttatattatttcatatcagtggtccacatgcaagtgaggcttctgagacagagtttgagttctctcttcaactaccataacacttaacctgtatctttttttttttttttttttttagacaggagtctcgctctgtcactcaggctggagtgtagtggtatgatctcggctcactgtaacctctgcctcctggattcaagcagttctccatgtctcagcctccctagtagctgggattacaggcctgtgccaccatgcctggctaattttttttttgtatttttagtagagacggggttttaccacgttggccaggctggtctcgaactcttgacctcgagcgatcaacttgccttggcctcccaaagtgctgggattacaggcatgagccacagcgcccagccgtctttttttttaaatagcaatttaacactgttcacagttactcatgtacatgtcatgccatctattacactgtaagttctgtgagggtagctgtatcaaatttatctaactctctctagtatgcatgacatagtaagtattcaataaatatttgcatattagtgataaggatacaggttctgaatagtgggtccttaccatttaagaattagtatttgatggccgggcggggtggctcacgcctgtaatcccagcactttgggaggctgaggcgggcggatcatgagatcaggagatcgagaccatcctggctaacatggtgaaatcccgtctttacaaaaaaaatacaaaagaattaaccaagtgtggtggtgggtgcctgtagtcccagctactgctttgtgaggctgaggcaggcagatcacctgaggtgggaaattcaagaccagcctgaccaacatggagaaaccccatctctactaaaaatacaaaattagccgggcgtggtggcgcatgtctgtaatcccagctactcgggaggctgaggcaggagaatggcgtgaacccgggaggcggagcttgcagtgagccaggatcgcgccactgcactccagcctgggcgacagagcgagactccgtctcaaaaaaaaaaaaaaaaaaaaaattagtatttgatatttgatcattaaatatgaattaagaggacttagactttttgttaaatgtcaagctgggaaaagttgtcatttaaatgaattgcctcttatttaatttcgtctgatgatacattttgtttttattttgtaaaaaattattttttttctttttggagacagggtcttgctctgttgcccaggctggtcacaaactcctgacctcaagcaatcctcctgccttagcctcccaaaatgctgggattacaggcgtgacgacctcgcccggccttgtattatgatacattttgaacaactacaagtagacttggtataatgaacctgcacgtacccattgccaagttctgacaactgtctgtctatagccaattatgcatttcttaaattagaacccccccaatatacccaaatatatatatatgtgtgcatatatatagtaagttgtaacaaagttgtgaattcatacctgaagtatctcaagtgatgcaagttttatgaatttttgtttatgccttttgggaagagttgtattgacaaattttttatgcttaaagtaaaccataaatcaaaaaaataaaatctaggatgcaataaaacaaaacaacttcttgacataagtatggtatgtaaatctgttttgattggaaatcaatttgttatattgccagaattcctgttttagaatacatctctgctgatctgtctgtattcttagactgcatatctgggatgaactctgggcagaattcacatgggcttcctttgaaataaacaagacttttcaaattcttagtcgatctgcagaacctgtagccaggcactgaaccattttgatagatgcagtaatcgttgcaagtgtatatttcaagggagttctggctgggtcctagtttatgcttgtggcagaagcagtgagtaactgggaggaagttggtgagtaagcttcaaggaagaagtcatttttagtactctggatcttcctgattttaaagcactacaaaatggtgcattttcattcttgtcaagtgataacagatatattctgatgagcctgaaatgaatatatattgtatcatttttataatatctagcaaggtttgtattttcctagaacttgaactaaatttcagttcataaaatttataaaatacttagttgttgtaaaatatttttggaatgttcacataggtgacacacaaatgtcccattttcattctttctatagtaaatatgttctgatatgtgaaggtttagcagatgcatcagcatttaatcctagaggatctggcataatcttttcccccaagaatagaaattttttctgcttatgaaagtagtacatgtttctttaaaaacaaatcaatattgacttctgcctgctgtatagcactatgcctccacctggccatgaccaggggcatgtcctggtccacctacctgaaaatgtttgcaaccagcctcctggccatgtgcacaggggctgaagttgtcccacaggtattacgggccaacctgacaatacatgaagttccaccaaagtctgagaactcagaactgagctttggggactgaaagacagcacaaacctcaaatttctcagcactggaaacctcaaaatataactgaattccataaataagattttaagtcttaaatatgtatttttaaatgtattaaaagtcaagctgcttgtatttaagcacctaatacaatgcttaggttgtaaaaggagatgctcaataggtactaactgatatattgagatttaattatggtttgaccaatatttattggaaaccgccaaagcttaaatcatcagcttcttgaatgtgatttgaaaggtaatttagtattgaatagcatgtgagctagagtatttcattctttctggtttatttcttcaaatagactttgaatataatggtgaatgggtattataaattaactaataaaaatgacattgaaaatgaaaaaatatatatattaaagtgtagaaagtgaccaggcgtggtggctcacacctgtaatccaagcaccttgggaggctgaggcaggaggatctcttgatcccaggagttcaagaccagcctgggcaacatagcgagacttcgtctctaaaaaaaaaaaagagagagaaaaaaattttttttatttaaaaaaagtgtagaaagtgtcaagaccccacttcttaccattatttggtatatttctctatacccacccacccttcctccttactccctccctcccttcccaatctttttatctttttgtattctgattttttgtttgtatattttgctttaatttaatgtatcctttaaaaatttcccatacattttatatgtatatataaaaacgcatgctgccaaagataatttataagaaagaccattgaatttttttaaaagtgatatatattcattgaaaaaaatttagaatatatagcaaagcaataaagaactaaataaaattgctgtaactcctctttcaaagataagtgcttttatgattttgttgtatttttttctgtatataggtacatatatagtatttataaagctgtactcatagtacattttcacatcacaggtaccatatcagtgttattaaatattttgtatgccaggggctagacataccaagacaaccaatatgtggttctacttaaataatattagagtatcttttatgatgacacttcatgagttgactataataatcttagacttctaagagtttgggttttcaaaagatcacttagcttttttgggtgatttttcccccttactgtgagatgagagaggctgtttggatttgggattggggtagcggggacagcaacttttcttttctttttcttttttattttgaggtagggtattgctgtgtcacccaggctggagtgcagtggtgtgatctcggctcactgcaacctccacctcccgggctcaggtgatcctcctgcttcagcctcccagtaactgggactacaggcgcgtgccacatgcctggctaattttgtatttttagtagagatggggtttcaccatgttggccaggctggtctctaactcctgacctcaggtgatacgcccacctgggcctcccaaaatactgggattacaggcatgagccgctgcatcagccagcagtttttcttgtggttttttttgtttgttttgttttgttttgtttttgagatagggtcttactctgttgtccacgctggagtgctgtggtatgatcgtagctcactgcagcctcaaactcctgggctcaagtgattccttctgcctccgcctcccgagtagctgggactacaggtatgcaccaccatacctggcaaatttttacaaagttttttgtagggacggggtcttgctacattccccatgtcggtcttgaactcctggcctcaagcaactctcctgtctcagcctcccaaagcactgggattacaagtgtgagccaccacaccatgccagtttttcctgttcagtgtgatattttatcttgttagactacagtgtgttaaaacttgttttactaaattttcaaacatactcaaaagtggagagaatagtataatgaatacccgtatgttcatcacccatgtttagaatattattaaatataaagattttgctgcgtttgtcttagctctttaaaatttttctttttctctttgtgacctaaaggaaattccatatcttatcactttacttctacattcttgactaagatgactaagacatatagttacatggttttttgttttgtttttgttttttaaagacgaaatctcgctcttgtcccccaggctggagtgcaatggtgccatctcagctcagtgcaacctctgccttctgggtacaagcgattctcctgcctcagcctcccaagtagctgggattacaggctcctgccaccacgcctggctaatttttgtatttttagtagagacggcggggggaggtttcaccatgttgacaaggctggtctggaactcctgacctcaggtgatccacccgcctcggcctcccaaagtgctgggattacaggcgtgagccaccgcgcccagcctgtttttttgtttgtgtgttttgttttttttgagacagagtcttgctctgtttcccaggctggagtgaagtggtgccatctcagctcagagacagagtcttgctctgtttcccaggctggagtgaagtggtgccatcttggctcactgcaaccttcacctcccaggttcaagtgattctcctgcctcagcctcccaagtagctgggactacaggcatgtgtcaccacacccggctaatttttttgtatttttagtagagacgggatttcaccgtgttgcccaggctggtctcgaactcctgagctcaggcagtctgcctgcctcagcctcccaaagtgctgggattacacgtgtgaaccaacccgcccggcctgttgttttcttacataattcattatcatacctacaaagttaacagttactaatatcatcttacacctaaatttctctgatagactaaggttattttttaacatcttaatccaatcaaatgtttgtatcctgtaatgctctcattgaaacagctatatttctttttcagattagtgatgatgaaccaggttatgaccttgatttattttgcatacctaatcattatgctgaggatttggaaagggtgtttattcctcatggactaattatggacaggtaagtaagatcttaaaatgaggttttttactttttcttgtgttaatttcaaacatcagcagctgttctgagtacttgctatttgaacataaactaggccaacttattaaataactgatgctttctaaaatcttctttattaaaaataaaagaggagggccttactaattacttagtatcagttgtggtatagtgggactctgtagggaccagaacaaagtaaacattgaagggagatggaagaaggaactctagccagagtcttgcatttctcagtcctaaacagggtaatggactggggctgaatcacatgaaggcaaggtcagatttttattattatgcacatctagcttgaaaattttctgttaagtcaattacagtgaaaaaccttacctggtattgaatgcttgcattgtatgtctggctattctgtgtttttattttaaaattataatatcaaaatatttgtgttataaaatattctaactatggaggccataaacaagaagactaaagttctctcctttcagccttctgtacacatttcttctcaagcactggcctatgcatgtatactatatgcaaaagtacatatatacatttatattttaacgtatgagtatagttttaaatgttattggacacttttaatattagtgtgtctagagctatctaatatattttaaaggttgcatagcattctgtcttatggagataccataactgatttaaccagtccactattgatagacactattttgttcttaccgactgtactagaagaaacattcttttacatgtttggtacttgttcagctttattcaagtggaatttctgggtcaaggggaaagagtttattgaatattttggtattgccaaattttcctctaagaagttgaatcattttatactcctgatgttatatgagagtacctttctcttcacaatttgtctcttttttttttttttttgagacaaggtctctgttgcccaggctggggtgcagtgcagcagaatgatcacagttcactgcagtctcaacctcctgggttcaagcgatccttccacctcagcctcctgagtagctgggactataggtgtgcgccaccactcccagctaatatttttattttgtagaaacagggttcgccatgttacccagcctcccaaagtgctgggattacaggcatgagccactggcccagtttctacagtctctcttaatattgtatattatccagaaaatttcatttaatcagaacctgccagtctgataggtgaaaatggtatcttgtttttatttgcatttaaaaaaaattatgatagtggtatgcttggtttttttgaaggtatcaaattttttaccttatgaaacatgagggcaaaggatgtgatacgtggaagatttaaaaaaaatttttaatgcatttttttgagacaaggtcttgctctattgtccaggctggagtgcagtggcacaatcacagttcactccagcctcaacatcctgcactaaagtgattttcccacctcacctctcaagtagctgggactacaggtacatgctaccatgcctggctaatttttttttttttgcaggcatggggtctcactatattgcccaggttggtgtggaagtttaatgactaagaggtgtttgttataaagtttaatgtatgaaactttctattaaattcctgattttatttctgtaggactgaacgtcttgctcgagatgtgatgaaggagatgggaggccatcacattgtagccctctgtgtgctcaaggggggctataaattctttgctgacctgctggattacatcaaagcactgaatagaaatagtgatagatccattcctatgactgtagattttatcagactgaagagctattgtgtgagtatatttaatatatgattctttttagtggcaacagtaggttttcttatattttctttgaatctctgcaaaccatacttgctttcatttcacttggttacagtgagatttttctaacatattcactagtactttacatcaaagccaatactgtttttttaaaactagtcaccttggaggatatatacttattttacaggtgtgtgtggttttttaaataaactccttttaggaattgctgttgggacttgggatacttttttcactatacatactggtgacagataccctctcttgagctacatcggtttgtggggagtcaaaagtcctttggagctaggtttgacaaataaggtgggttaacacttgtttcctagaaagcacatggagagctagagtattggcgaattgaagaaatccccctttttttttaacacacttaagaaaggggactgcaggtatactcaagagagtaagtcgcaccagaaaccacttttgatccacagtctgcctgtgtcacacaattgaaatgcatcacaacattgacactgtggatgaaacaaaatcagtgtgaattttagtagtgaatttcattcataatttgatcgtgcaaacgtttgatttttattactttagactattgtttctgattttatgttgggttggtatttcctgtgagttactgttttacctttaaaataggaatttttcatactcttcaaagattagaacaaatgtccagtttttgctgtttcatgaatgagtcctgtccatctttgtagaaactcgccttatgttcacatttttattgagaataagaccacttatctacatttaactatcaacctcatcctctccattaatcatctattttagtgacccaagtttttgaccttttccatgtttacatcaatcctgtaggtgattgggcagccatttaagtattattatagacattttcactatcccattaaaaccctttatgcccatacatcataacactacttcctacccataagctccttttaacttgttaaagtcttgcttgaattaaagacttgtttacggtatcgataagcttgatatcaaaacgccaactttgacccggaacgcggaaaacacctgagaaaaacacctgggcgagtctccacgtaaacggtcaaagtccccgcggccctagacaaatattacgcgctatgagtaacacaaaattattcagatttcacttcctcttattcagttttcccgcgaaaatggccaaatcttactcggttacgcccaaatttactacaacatccgcctaaaaccgcgcgaaaattgtcacttcctgtgtacaccggcgcacaccaaaaacgtcacttttgccacatccgtcgcttacatgtgttccgccacacttgcaacatcacacttccgccacactactacgtcacccgccccgttcccacgccccgcgccacgtcacaaactccaccccctcattatcatattggcttcaatccaaaataaggtatattattgatgatgttt

SEQ ID NO: 122 - DNA, 30924 bp, synthetic construct
  source 1..30924: mol_type = other DNA
aaacatcatcaataatataccttattttggattgaagccaatatgataatgagggggtggagtttgtgacgtggcgcggggcgtgggaacggggcgggtgacgtaggttttagggcggagtaacttgtatgtgttgggaattgtagttttcttaaaatgggaagtgacgtaacgtgggaaaacggaagtgacgatttgaggaagttgtgggttttttggctttcgtttctgggcgtaggttcgcgtgcggttttctgggtgttttttgtggactttaaccgttacgtcattttttagtcctatatatactcgctctgcacttggcccttttttacactgtgactgattgagctggtgccgtgtcgagtggtgtttttttaataggttttcttttttactggtaggcgcgccgtcgacgcgacaactgtcttattaccctgttatccctaccttaattaagctagccgacgcgttggccaggagctcagatctccggatccaagcttatcgatttcgaacccaaatggatctaccacatttgtagaggttttacttgctttaaaaaacctcccacacctccccctgaacctgaaacataaaatgaatgcaattgttgttgttaacttgtttattgcagcttataatggttacaaataaagcaatagcatcacaaatttcacaaataaagcaatagcatcacaaatttcacaaataaagcatttttttcactgcattctagttgtggtttgtccaaactcatcaatgtatcttatcatgtcgagctagctagtcaggacttcagttccagctttgtgccggctccgaaggtcagcgggttgctagaccattgctgacagtaatatgtggcggcatcctcggcttccatagagctgattgtcaggctgtagctggtgccagatccagatccgctgaatctgtagggcacgccggaggccactttgcttgtgtcgtagatccaccgcttggggcttgtgccagacttctgctgataccagttcatgtaggacacgctgctgctggctctgcatgtcatggtcactttctcgcctggggaagcgctcatgatggcggggctttgtgtcagctgaatatcggagccaccaccaccgcttccaccaccacctgaaccgcctccgccactagaaactgtcagggttgtgccctggccccagtaatccagacagtagtggtcgtcgtagtaccgggcacaatagtacacagcgctatcttcagaggtcaggctggacagctgcatgtaggcggtagagctgctcttgtcggtggtcagtgtggccttgtccttgaacttctggttgtaattggtgtagccccggctggggttgatgtagccgatccattccagtccttggccaggcctctgcttgacccagtgcatggtgtaccgggtgaatgtgtagccgctggtcttgcaggacatcttcacagaggcgccaggtctagccagttcggcgccagactgttgcagcttgatatcggatccaccgccaccaagggctttgatttccagcttggtgccgctgccgaaggtgaaaggggttctgaagtgctgctgacaaaagtacacggccagatcctcggcctgcacgctgctgatggtaaaggtgaagtcagggccagagccagagccggtgaatctagagggcacgcctgtgtatctgctgctggcgctgtagatcagcagcttaggagactggccaggcttctgctgataccaggccacggcgttgtacacgtcctggctggctttacaggtgatggacactctgtcgcccacgctggtgctcagaaacttgtggctctgggtcagctgaatatcagatcctccgccgcctgaacctccgcctccgcttcctccgccaccagaagagactgtcacggttgtgccctggccccaatatggcacgtagccgtggtacacttcccatctggcacaaaagtaggtggccatgtcctcggacttcaggttgttgatctgcaggtaggcggtgttggcgctggtttccaggctgaagtcgaatctgcccttgaaatcgtcggcgaaggtgctctcgccggtgctggtattgatccagcccatccatttcaggccctgtccaggggcctgcttgacccagttcatgccgtagttggtgaaggggtagccgctggccttgcaggagatcttcactgtctcgccaggtttcttcagctcggggccagactgctgcagctgaacttcagaatgggcgcctgtggcggctcccacaagaaacaggatgcgccagatccagtccatggtggccctccttcgccggtgatctcagctgtaggaaagagaagaaggttagtagtcgacgtgtccctctcgatgaatctaagtatcaattgtgagcgctcacaagtcaacactctttttgataaatctagtagatatcacttacgtaggcgccggtcacagcttggatctgtaacggcgcagaacagaaaacgaaacaaagacgtagagttgagcaagcagggtcaggcaaagcgtggagagccggctgagtctaggtaggctccaagggagcgccggacaaaggcccggtctcgacctgagctttaaacttacctagacggcggacgcagttcaggaggcaccacaggcgggaggcggcagaacgcgactcaaccggcgtggatggcggcctcaggtagggcggcgggcgcgtgaaggagagatgcgagcccctcgaagcttcagctgtgttctggcggcaaacccgttgcgaaaaagaacgttcacggcgactactgcacttatatacggttctcccccaccctcgggaaaaaggcggagccagtacacgacatcactttcccagtttaccccgcgccaccttctctaggcaccggttcaattgccgacccctccccccaacttctcggggactgtgggcgatgtgcgctctgcccactgacgggcaccggagcgatcgcagatccttcgatagagaaatgttctggcacctgcacttgcactggggacagcctattttgctagtttgttttgtttcgttttgttttgatggagagcgtatgttagttacgattcacacaaaaaaccaacacacagatgtaatgaaaataaagatattttattgcggccgctcgagtctagaggtatacatgccatggtccgcggtattaccctgttatccctaagacaactgtcctgcatgcgacgtcggcgcgccatcgaattcctgcagcccgggggatccctttgttgattttttccacatagattatttttgactgttttggcactttatataaatggaatcatatagtaaatatatacatgtatatatgtatatatacactatatatgtatatatatagtgtatatatatacatgtatatatgtatatttacatatatactgtatatatgtatatttacatatatactgtatatatgtatatatacacgtatatactgtatatatacagtatatactgtatatatatactgtatatatgtgtatatatatatacagtatatatacagtatacatatatatacatgtatatatacacagtatatatacatgtatatatacacagtatatatacatgtatatatacacagtatatatacatgtatatatacacagtatatatacactgtatatatgtatatatatactgtgtatatatatacagtatatatacagtatatatatacatgtatatgtatatatatactgtatatatgtgtatatatacgtatatatactgtatatatatatagacacttttgtgtctggcttcttgctctcatcataaagcacttgaaatccatccatgttgtagctggtatcagtagctagtttcttttcattgctgagaagtatcactttttattgatgagtagttttacattgtatgaacatgcccgagtttgtttatgcattctactaatagacacctgggctgtttgcagtttttggctattacaaagaaaatttctatatttttttccaacttttattttaggttcagcgggtacatgggcaggtttgttacatcggtaaattgcatgtcactggggtttggtgtacagattatttcaccacccaggtaataagcatagtacctgataggcaggtttttgatcctcaccctcctccctcaagtaggccccagtgtctattgttctattccttttttttttttttgagatggagtctcactctgttgcccaggctggagtgcagtggtgcgatctcggctcactgcaaggtccacctccagggttcaagcgattctactgccgcagcctcccgagtagctgggattacaggcacccaccaccacgcccggctaatttttgtatttttagtagagactgggtttcaccatgttggccaggatggtctcgaactcctcacctcaggtgatccgcccgcttcggcctcgcaaagtactgggattacaggcgtgagccacggtgcctggcctatggttccattctttgtgtacacgtgtactcagtgtttagcttccacttgtaagtgaaaacatgcagtatttggttttctgaaattcttgtcttcatctttttgtagacaatccactacttttatttttaaatattaggaacaatagcctctgtgtgtcctgaattgcaatgttttttctctgattttgctgctcatcttgtaacctgtatggtgtttttctgtgtgcaagctttttactttacgtgggcaattttatcattcttttcttttatggtttctgggtttcatgtcatgattggagaagcttgatctaccctgatactataaaaatatccaccttggcttttttttttttttttagatggattttcactcttgttgcccaggctggagtgcaatggcgtgatctcggctcaccacaacctctgcctcccaggttcaagtgattctcctgcctcggcctcctgagtagctgggattacaggcatgcgccaccacgctcagctaattttgtatttttagtagagacaggatttcaccatgttggtcaggctggtcttgaactccccacctcaggtgatctgtctgcctcggcctcccaaagtgctgggattacaggcgtgacccaccacacctggcccacgttgttttctgatagtgttttcacgtgttattttttctgtcttactctttgaatcatctaaatgtatcttaatgtcaggagtgaggtagaggacccagttgtttggtttaaatgactagccagttttcccaacaccaggtgttgaacatccctcactgatgtgagatgctgcctttttcacagtctcaatccccatgtgcatttctatttattttccttccactttattcacatctttttcagtatccacaaccatattgttttaaatagcttcatgatatgttttaatatttggtagagctagaaccctttcttggttctttttcttttcttcttctcctccttttcctcctccttctttctcctcctccttcttctttctttttagaaatttcctggctattcttgttttgtagtcttccagataaataattttgaatcactttgtcatgttccagaaaataatactgccagaatttttattgtgatcacagaagttttacagattcatctgggggaaaaaaacccatcttcccagaatacagaaagggtgagggaaagacaaacatcaaggacaagtctcaggttctggacttggagaccaagaggatttggggcatccgggagcagggcagggaggtgtgatggctgcctttcactgagtaggaggatgcccagacttgggggaactatggaaagtttggttcagactttctgagttggagatgtctatgcgcagtccacagggcgaagccctggaggtagaggccctccttactgcctccctcattcagtctgaggtccattctccacatggacactgaagtgactcaaggcttcccttgttggatcaggatagtctccagggccctgggtggtctgggcctgcccacctccccatcccctctcctgcctgccctcctcttgctcactggaccccacccaccagcctccttctattcctcctgacatttgcacttgctgttccgtctctgcttggaacatcctagctctttgcatggcttgctccttcccatcttttaatctaagctcaaatatcactccttcagatatgcctttcccaaatatcctagctaaagagaactgctccccacttcccacaagccctagcaaactgggactctccttcttgctttctttctctctgccccttctgtgttttttccatagaccttaacttgttactgttttatttgttgatgtgtttacatcatttgtccccctgtgatggttagttttatgtgtcaacttggctaggctgtaggggctgttcgtcaatcaaacactgatctatgtgtagctgtgaagggattttgtagctgtgattaatagttgactttaagtaaggaagattatcctggagaatgtgggggaaggggcagacctcagccaatcagttgaaaggccttaagaacaaagctgagatttccccgaggaagaagaaattctgcctgtggactgcagcatcagctcctgcttgagaggttccaggctgcccttcctgacagcctgtcctatgattttggacttgccttgccaggtttttcctctttcttgaccccccaaaaccatatatatctcctgctggtttgtttctctggtgtaatcctgagggatgaacactcctccctcccagttcactctgggagaggttggggatcatgtttgtctatttccccatgcctggcccatgcgtgtttattgaatcactgaacaaccacgcattaggaagccagtcatatgtgcttcttcagaacctcatgtccattgccagatctccctggcttttgtggctagaggacaagtgagagatagtagcttacccacagaccttggccctgaggcccccaggggcctgagcctgctgtaagggaggagggagcccctgaggtctcacacacctccctggggatctggcattttcccctggggctggcctcagagctgggcgggggcagattatggagtgggttgtagagggagcacctccccactagcaatcatggttttttctgcgcctctcatagggaggcctacaggcctccaccttcagctcttcaggagccacaggcagctgagtgacttctgcatcacagtcttctcagagacaaacttgcagtaagaaagaggggcccgtgagggaccccagagaaggctgttgtcaaagcaggatgagagtgaactcttccatgggggacacccagcgtctccaagctcttttatgctgtcttcaaggggtctagagagcttcagcccaacatgagacccagtccagcagcatttccctgcgaagtgaaagttaggaccctgactagatacaccacgctgacctcagccagaatatcaagatgctgaggcgctgagatgctgggatgctaaggtgctaaggtgctggggtgctggggtgctaggatgctgaggttttgtgatactgggtcgctgagatgctgggatactggggtgctgaagtgctggggtactggggtgttgccatgctgaaatgctggggtgttgggatgctgaggtgctgggttgctgggatgctgggatagtccttggatgctgcggtgctgagatgctggtctgctggtctgctggggtgttgggatgctgggattttgggatgctggagtgctgcagtgctgcagtgctgagatgctggagtgctggggtgctggaatactgtagtactggtgtgctggagcattgagatgctagggcactgggatgctaaggtgctgagatgctgcagtgctggggtgttgggatgccgaggtgttgggatgcttaagtgctggggtgttgggatgctggggtgctggaacactatggtgctggggtgctggagtgttgagatactgtagtggtgggatgcttaagtgctggggtgctgggtgttgggatgcctaggtgctggggtgccgagatgctggagtactagtgtgctgggatgctgaagtgctggggtcctgagatgctgcagtgctagggtgctgagattctgggctgctggagtgttggggtgctgggatgctggagtgctgagatgcttggacaatggggtgctggaatactatggtgctggggtgctggggtattgagatgctagggtactgggatgctgaagtgctgagatcctggagtgctgggctgctgggccacaggctcttgaatccattcgtctgcccaggggaagaaaccagaagataaagagctaatgaaggagctttggttgagagggaggaagtaatggaaggagcaacatcttgtggaggagcaggagagaatggacctcaggttgggagagagggccaggctacaggccagagaggcagaaggattccagcagagtgtgggctccaggagccaaggggaaacaggtttctgggaggagagagtccagtactgctgaagtggcaagtccgctgaggaccaggaagcttcatttggctttatgaccaggaggaatttggaactgtgactagagtacttagggggaaggaggcaagactggagccagattgctctgggttgaggggtgagtgggaggtgaagcagggcactgtcactcctttgaagggtggcagagagctggaattggtgctggatgggctgtggggtgacagggtcatgtggaaagcccctggggggcacctggaaaaggagaagctgacagtacagtgagaggacagctaagggaaagcggaatggcagaacacgcactgccaggaggaatgaggatagggtcaggagtgccaggggcagtgaggccagcctggggtcaggtggcaggacgtgtccaggaagctggtctgcactgcagcccacactggctcagccttgaggttccctgtgtggttggggtaggaagttgaaccctctgggaatggaagatggaaccagctctgcgagccaagctcagcttttatctatgggtctctgagggctggcagagctgagtggggacaactgtgatccgtgaggctctcaggttgaggtggcccctccgggagggcttcattttcccagcgggtaggttctaagcagcagtggctgggcaggtgggtccaacacagagccagagaagggtgaatgggcctcctggcaccccacccctgctgcccctgagctcagtgatggagggggacagcacagctgagcccaagtgctttggtgtggccctgagggaaagctgcagcctgcctggggcctggcatggatgggacacttgaggcagagggacaatagtgggcgctgcagtgaggctggctcttggagaggtttcctgaggagtgctgcctgagacgggcagggagaacagagacaaagttggtgacagggaatgaaagctgactgaaggactttacccagacctatgaggatatctctctcagcaggaagcaggaggggactgtgtgaggactggccaagagctggagtgttgggaaaatgactctttctccgacccctctgtcctagctctggcccctggactgcggaggtctgcttccacccccattggtcgatcgttgtcccttgtcacagccattgagaattttggcagggagcatgttcttagagcatttttaggctctgcgggacataacagctctgcctcagagcacatgcctttctcagctcctgaaagccactgatcaaattggaacattttgtaccttagggatgaggatatcaactctcccagccacttagagggataaatgtgatgatgcattcaattgtgactacatctgatcccaactgttgcttcagctgctctcctatagcacatggcgggaggcgtgcatcccagtagctacctccccacttttggggagatgtggttccatccatgaaacctgggtacccgcctaccaggtcctggcctatcaggtggcagggtctggtcaaagaagggcatgtgtggtcttcagcaagggagacaggacggtggtgcagagcgtctagaccctcagggcaagtctcccccacacctgctcccggggcagttgtctttgtgacctcccatccccctctgtttcatcctctataaaatgaggggctgagccccaaaataacaggcttctttgccatgatgcaaaactgctgaatctttctttctgacacacaaggcatcgagcagcctctgaaagaaccaaagccactagcaggcttcctgacttgggtttgtaggtactgaatactcccttgaaaaataaaaacatagaggcacttttctcctggctgtttattacagaacgaagaaaaaacacactggcttgaaacagacgccagatttcaaatgtagaggtgaaatacgaggtggcaattaaaatgtgattacagaaagtctggacactgagaaaagtttacaggacagtgggtgtgggttttctataacagacacttaaatatacatgacgataattgcagatagaaaccatcaaagacaaaccccaaatcaactaataatgtttacagatgttcccccccaaaccacagagccttacatcaaaacaaatactgaaaggctttaaaccaggaacagctcgccttaaccccacgagggtgcacacaagctgggctttttctctcggtctgaatggtaaagggaggaggatactctagctcctccaggtggattgctgagacagggctcggctcacacactgtctctgcgcctctcccaaatctggagaactctcccagcctcctggtaaagtgtctctgtggggcacttaacgataaaacagcttctgctgtaaagctcattaggaaagagctagcggagactgaaaggttcgcaaaagagattaagaatcacacaaggcaataggatttttagtgaacatagaaataaatggccaagtggttttctatttggcatttgtcaacttgcacaacaactcttggtcatatccacattgctcattgcattaaaaccataagcgactcagccacctagcttaacaaggtatcactggagcaaacaacacggtctgcatatttgtaacattgtataataaacacaaaacaatgcatagtaaacacaactctactgaaacaaaagccgtcgctttatttacaaagtcacaaaatgaagtataaatacttctgtcattaatgtttaggaaaaccatttacaaaattttcaaatatgtacacgtagcttgaaaaatcaccagctttccattttgtcacaggtagagagagggataagcatgggctgacaacaccactcaaattgtaacgggagacaactgcgggtatggatcgacaccacttcctagagtgatgtcaccatgggggtttctatgggcatcctgctcagatttaaagtgccccagcatcctgggtgacttgcccagaattctgggctgtggcattttgagcagcagcatgctgttccaaaatgtcgtcgatcagcctcaagttgcacacccagtcttcatctgggctcacacaggagcctttcaagagagcttcaatgaaatctacctcattgcagtcaggtgacgaaatcagatcatttagtgggggttggggctggcgcaaaaagtcggcaggtggcagctcagggggaatatccgttctgtcgaacggacctgggaactggctggcagcaacggcagaagcagcagcagcggtggcagcagcagccacatagcttggtggctcgatgccctgtatggggctcaggggactaaagctggccataccctgctggaggaacttggtggtgtttgctacaggcaccgggccctgtaccgggctctgcctgaggctctggctgcccagcaggctgaagctggggttgttggccaggggcacttgtgttcccatcgcagcgggcacttgtgcctcccaatcagatggcctctgaaggcaggcctggccagaaggtgagtgctgctgaacgctattatccacttggctgaggggtgttttccccgaaactgctgtggtcacagctgctgccgctgtgacccatgcagcattgttgaacgcagtgggcattcttggcacactaggccgtctgagctggtggggactcaaggactgggtgcccagggagctgggacagaacccaggcaggggcacttctggtggggtggccttggggctctgcatatgctggcagacagagtcaagtctgcccaggggagtctggcctgagtgtgagaggatgggacactgggggctggaggtgaaaattccttgccgcttccccagagttggtgagatcactcccatgccctcgcagctctggtgcctggtgagtgggatcattcctggactcagattgttctgaagaagcccagttctgggtggcatcaagtgcttgctagatggggggcttgccttgatccggctacacttggaggtgacttgttcttggacggctacatacagaaagagagaagtggggatgagttccaaaggcatcctcgacttcggctgtggccaccggagggtagctcctggcccaacacggacttctcacctcccgcccttggctctctactgagctcccccctgctccccaattcctcgccattcccctcatttctctgccctcagcctggactgcagttcttctgggaagctgccccaactccctaggtctgtgctcaccaagagcagatcacactggactgaaatgccagctgatttgtctcttcaagaaaattggaagctcctggaggtcagggtccatgtctgcttttacactcagtgctctgtatgcaggcctggcactgcccaccctttgacaggtggtgcatattttgtagaaggaaggaaggggccaggtggggtgggctgggctggtggcgggagctagctcagcctcttagattctctacccgatggatgtgacctgggacagcaagtgagtgtggtgagtgagtgcagacggtgctttgttcccctcttgtctcatagcctagatggcctctgagcccagatctggggctcagacaacatttgttcaactgaacggtaatgggtttcctttctgaaggctgaaatctgggagctgacattctggactccctgagttctgaagagcctggggatggagagacacggagcagaagatggaaggtagagtcccaggtgcctaagatggggaatacatctcccctcattgtcatgagagtccactctagctgatatctactgtggccaatatctaccggtacttttttggggtggacactgagtcatgcagcagtcttatggtttacccaaggtcaggtaggggagacagtgcagtcagagcacaagcccagtgtgtctgacccacccaagaatccatgctcgtatctacaaaaatgattttttctcttgtaatggtgcctaggttcttttattatcatggcatgtgtatgtttttcaactaggttacaatctggccttataaggttaacctcctggaggccaccagccttcctgaaacttgtctgtgctgtccctgcaactggagtgtgcctgatgtggcactccagcctggacaagtgggacacagactccgctgttatcaggcccaaagatgtcttccataagaccagaagagcaatggtgtagaggtgtcatgggctacaataaagatgctgacctcctgtctgagggcaagcagcctcttctggccctcagacaaatgctgagtgttcccaagactaccctcggcctggtccaatctcatcccactggtgcgtaagggttgctgaactcatgacttcttggctagcctgcaacctccacggagtgggaactacatcaggcattttgctaactgctgtatcctaggccaataaatgttgatcacatttatagctgccatggtagggtggggacccctgctatctatctgtggaggctctgggagcccctgacacaaactttctgaagcagagcctccccaaccccttttccattccctatacctgacagatggcccaggaacccattagaaatggaaggtcactgcagcagtatgtgaatgtgcgtgtgggagaagggcaggatcagagccctgggggtgtggcagcccccaagtgattctaatccagatcctagggttgtttccctgtcccattgaaatagctgctttaaggggcctgactcagggaaatcagtctcttgaattaagtggtgattttggagtcatttagaccaggccttcaattgggatccactagttctagagcggccgggcccagggaaccccgcaggcgggggcggccagtttcccgggttcggctttacgtcacgcgagggcggcagggaggacggaatggcggggtttggggtgggtccctcctcgggggagccctgggaaaagaggactgcgtgtgggaagagaaggtggaaatggcgttttggttgacatgtgccgcctgcgagcgtgctgcggggaggggccgagggcagattcgggaatgatggcgcggggtgggggcgtgggggctttctcgggagaggcccttccctggaagtttggggtgcgatggtgaggttctcggggcacctctggaggggcctcggcacggaaagcgaccacctgggagggcgtgtggggaccaggttttgcctttagttttgcacacactgtagttcatctttatggagatgctcatggcctcattgaagccccactacagctctggtagcggtaaccatgcgtatttgacacacgaaggaactagggaaaaggcattaggtcatttcaagccgaaattcacatgtgctagaatccagattccatgctgaccgatgccccaggatatagaaaatgagaatctggtccttaccttcaagaacattcttaaccgtaatcagcctctggtatcttagctccaccctcactggttttttcttgtttgttgaaccggccaagctgctggcctccctcctcaaccgttctgatcatgcttgctaaaatagtcaaaaccccggccagttaaatatgctttagcctgctttattatgattatttttgttgttttggcaatgacctggttacctgttgtttctcccactaaaactttttaagggcaggaatcaccgccgtaactctagcacttagcacagtacttggcttgtaagaggtcctcgatgatggtttgttgaatgaatacattaaataattaaccacttgaaccctaagaaagaagcgattctatttcatattaggcattgtaatgacttaaggtaaagagcagtgctattaacggagtctaactgggaatccagcttgtttgggctatttactagttgtgtggctgtgggcaacttacttcacctctctgggcttaagtcattttatgtatatctgaggtgctggctacctcttggagttattgagaggattataagacagtctatgtgaatcagcaacccttgcatggcccctggcggggaacagtaataatagccatcatcatgtttacttacatagtcctaattagtcttcaaaacagccctgtagcaatggtatgattattaccattttacagatgaggaacctttgaagcctcagagaggctaacagacataccctaggtcatacagttattaagagaaggagctctgtctcgaacctagctctctctctctcgagtaataccagttaaaaaataggctacaaataggtactcaaaaaaatggtagtggctgttgtttttattcagttgctgaggaaaaaatgttgatttttcatctctaaacatcaacttacttaattctgccaatttcttttttttgagacagggtctcactctgtcacctaggatggagtgcagtggcacaatcactgctcactgcagcctcgacttcccgggctcgggtgattctccccaggctcaggggattctcccacttcagcctcccaagtagctgggactacaggtgcgcaccaccatccctggctaatatttgtactttattttatttatttatttatttattttttgagatggagtttcgctcttgttgcccgggctggagtacagtggcatgatctcggctcagtgcaacctctgcctcccgggttcaagcgattctcctacctcatccccctgagtagctgggattacaggcgcctgccaccatgcctggctaattttttgtatttttaatagagacgaggtttcaccatgttggccaggctactctcgaactcctgatctcaggtgatccacccgccttggcctcccaaagtgctgggattacaggcgtgagccactgcgcccggcctaatatttgtattttttgtagagatggtgttttgccatgttgtccaggctggtcttgaactcctgagctcaagcgatctgcccgcctctgcttcccaaagtgctgggattacaggcatgagccaccgtgcctggcctaggtagacgcttttagctttggggtgtgatgcctgccccagtatatagtgaatttaattattgctagagctggctgtttgttagttttctttgaacataagatactcattgtttttagtttgcaaatccctcttcctttttaaaaaatttctttcccttaaattgtttgcatgttagcaataacaaatgcttaaatggtgctatgtgctagatactcttctaagccctgttatgtatattaactaattttttaaattacacaaatcagagaggttaagtaacttgcccaagattacccaacaatactaggatttgaacctaagtttgtctcaccccagattctgctcttaatctctaaacttttaagttagtagtgacaatagtaggtatttattgaatacttaactatgttttaggcgttgaagtaaatattttgcaggcattatctaatgtaaacaccctaaagttacataacaggtaccctttaggtaaataaacactagtatgaccttggaggcacagatagttgaagtaacttgcccaatatcacttacatgaaattggccctcaaatgtgtctgatacaacccatgctgcttgtaactatcgttttaaactgccagggtaaacttggacacacttgagctaagaaaaagcttttagatttttgcaaattaatgtgaaagatatgctttatgtggatataatatcttctaaatttcggggatggtagtcctagaaatgtaatcctgccctagccgagcttaccctgccaataattttttacagaattggtaaaacggagcaccttttttttgtccttggccacactgttatcaacagggtgtagattgacatcaatctgtaggtgtaaaccagaattactctttgtgaccaccaggaaatagagcagttcagttcaggggtttctttctgtgaatttagcactgtgacctgcatactacaagtctactttgttttctatccattgtttgtatctgggtattgcaaaaggtaggaaaaggaccaaccagatcagcagagaagagttgccttggagttttcttttagttttctgcagttcattagatagtaactaggccatgtcattttactcccttgtagtgaagatatgttgaagttgtactggtatactcttctacctttctgtaattttatattgtgtagacttgataaaatttatgtgtcaatcaccaccattaatatcaatattgagcctcaattcttatttttctgcccagtggctgccaaattactaacatttacaataattcactactactaagataatctactagttcgatcacatacttcaaattgttatggaactactgtcttcagcattgtgcttctgataactgataagtataattttttttttgtccagagtgaacatgtctattcttccactgtacacactaataaaaggaaaaattgtaatattgggtaaattcatgtccttacacatgtagtagttatgagcccatgtccctagaatgagtaataatttatccctcccttggttgaatagtcaagaatgctgattttaattcttctaacagctttatccctcagaagggaaggcaagcaagttatatatgtagtttatttgtaagactgatatgaaattggaagatgaatctactattagctttaattatttttacatttaggaatattgcatcagtaactcataattttggttttctgttatcctgagttaacacaaattatccaaggagatggcggatcatctgctttgaggtgtttttttttgagaattttaatgtatctgaatataaaaggtaaaaatatgccaactagcaatttctgcccattccagaagtttggaaatattactcattactaggaattaaataaaatatggtttatctattgttatacctcttttaattcacatagctcatttttatcttttatttttgtttgttttttttgagatggagtcttgctctgtcaccaggcaggagtgcagtgatgcaaatctcggctcactctagccaccgactccctggttcaagcgattctcctgcctgagccttctgagtagctgggattacaggcaggcaccaccacgcccagctaatttttgtagagacaggatttcaccgtgttggccaggatggtctccatctcctgacctcatgatctgcctgcttcggcctcccaaagtgctgggattacaggtgggagccactacgcctggcccacatagctcatttttagactcacttccattaagtcttgtttggacccacgaacattgtctttttttttttaagatggagtttcacttttgttgcccagactgtagtgcaatggtgcaatctcagctcactgcaatctctgcctcctgggttctagcaattctcctgcctcagcctcccgagtagctggaattacaggcgcccgccaccacgcccagctaatttttgtgtttttagtagagacggggtttcaccatgttgggcaggccaggggtgatccgcccacctcagcctcccaaagtgctgggattacaggtgtgagccaccgcatctggccaacatgtcttttttttttttttcctttttaaccacaaagagacttaagcagtccttgtcacagatgatgaattgatgttgcaagtattgtcttagcttggattaattttcttgcttactgtaattttagataatatagctttgtaattagagattttatgtgtaaaccacaaaaatgtttacatgaaggccattattacagatgtgacgtgcataattattagtaatttgtatgtttacatgggtcagtctggcaaaaaattatgaagttttaaaaattaaaaaaaattataatgccagttttactggaaagtaaaattatttcagtaatcgattatagcaaaagtattgattttcattccagacaaaagtcagaatgaaaggtaatttctcaatactctttcagattaataaaagtacctgtagcgatttttatcattcacaagtatatcacaagtaagttagaatttgagaactgtgttctagatctctgaggagatgcagtcagatttctgaactgtctcagcaaatggtaagtaacttagagctagtaattaataacctgtcctttgatttctgattcagccaagaatggccatatttgggaaaggcagatctggagagtaaccacgttttcattcatttaccacttctaggcccctccagagctctcagatattttggggttgagcccttccccaaagccatacaggaccttttttttgtgatctgttctagccatttttatgttgggtgcttgttatggactgagcatttatgtcctcccacaccccccccataccttttttgaagtcctaacccccagtgtgatggtatttggagacagggcctttggaaggtaattacagttagaagaagtcgggagggttgggcccaggtctgattggattagtgcccttatatgaaaagacaccaggacgggcgcagtggctcacacctgtaatcccagcactttgggaggccaaggtgggtggatcacgaggtcaggagtttgagaccagcctggccaatgtagtgaaacaccatctctactaaaaatacaaaaattagctgggtgtggtagcgggctcctgtcatccaagctactcgggagggtgaggcatgagaatcacttgaacccgggagttggaggttgcagtgagcccagattgtgccactgtactccagcctgggtgacagagtgagactctgtctcaaaaaagaaaaaaaaaaaaaaagagacaccagagagcttgttagaagaggtcatgtgagcacacagttagaagaccttcaagccaaagaagaggcctgagattgaaacctaccttgcaggtaccttaattttggacttcccagcctccaaaactgtgagaaataagtttctgttaagtcactcagtctgtggtattttgttatggcagcctgagcaggtagttgttctttcagaaggtgttgataataaccacatgcaacaccaagtcacaaataataaaacagatgtaacttatattcatacagaaagttgggcactgccattgccttgttggtttacacggctgtgctagttcagtagcagaaaggtgctggtctcctttactcagtttacaatctaggcagtagaatgtaatcactgctttaaacttgatactgcttagggagagaatcattggtgctgggtaactttgggttctaggtttactttttgtgtatatataactgtttttggtaaatcacaagtttctgggcttgtcgaattagattttgttacagattatgagctttattatgctatacagttagttgtatgtatatatgcctttcccactagattttaagctttttttttttttttttttttgtgacggagtcttgctcttgtcgcccaggctgaagtggagtgcagtggcacaatctcggctcactgcagcctccacctcctaggttcaagcgattctcctgcctcggcctcccaagtaactgggactacaggcacgtgccaccacacccggctaatttttgtattttttgtagagacagggtttcgccatgttggctaggctggtcttgaacttctggcctcaggtgatccacccgcctcagcctcccaaagtgctgggatttacaggcatgagccaccacgcccagctatagctctttaagggttgtaaatttataatcattcttttactctcctgcaaattctgttgcacactgccttaatcaaggtagatgctgaatgcatttttgtataattgaatatgttgcaatccccaactctctccaactgttcctgtcaaagcagccactggattgttaactaatccatattagatggggttaattaatatcagatgggacaagtaagggctaataagattataggccaccaagtagatttctgtctagctcttatagagattgagtttattggacctgtttgataggaagttttggtgtttgggatgattaaaactgaagttcctatttattgaattatacctatttatattatttcatatcagtggtccacatgcaagtgaggcttctgagacagagtttgagttctctcttcaactaccataacacttaacctgtatctttttttttttttttttttttagacaggagtctcgctctgtcactcaggctggagtgtagtggtatgatctcggctcactgtaacctctgcctcctggattcaagcagttctccatgtctcagcctccctagtagctgggattacaggcctgtgccaccatgcctggctaattttttttttgtatttttagtagagacggggttttaccacgttggccaggctggtctcgaactcttgacctcgagcgatcaacttgccttggcctcccaaagtgctgggattacaggcatgagccacagcgcccagccgtctttttttttaaatagcaatttaacactgttcacagttactcatgtacatgtcatgccatctattacactgtaagttctgtgagggtagctgtatcaaatttatctaactctctctagtatgcatgacatagtaagtattcaataaatatttgcatattagtgataaggatacaggttctgaatagtgggtccttaccatttaagaattagtatttgatggccgggcggggtggctcacgcctgtaatcccagcactttgggaggctgaggcgggcggatcatgagatcaggagatcgagaccatcctggctaacatggtgaaatcccgtctttacaaaaaaaatacaaaagaattaaccaagtgtggtggtgggtgcctgtagtcccagctactgctttgtgaggctgaggcaggcagatcacctgaggtgggaaattcaagaccagcctgaccaacatggagaaaccccatctctactaaaaatacaaaattagccgggcgtggtggcgcatgtctgtaatcccagctactcgggaggctgaggcaggagaatggcgtgaacccgggaggcggagcttgcagtgagccaggatcgcgccactgcactccagcctgggcgacagagcgagactccgtctcaaaaaaaaaaaaaaaaaaaaaattagtatttgatatttgatcattaaatatgaattaagaggacttagactttttgttaaatgtcaagctgggaaaagttgtcatttaaatgaattgcctcttatttaatttcgtctgatgatacattttgtttttattttgtaaaaaattattttttttctttttggagacagggtcttgctctgttgcccaggctggtcacaaactcctgacctcaagcaatcctcctgccttagcctcccaaaatgctgggattacaggcgtgacgacctcgcccggccttgtattatgatacattttgaacaactacaagtagacttggtataatgaacctgcacgtacccattgccaagttctgacaactgtctgtctatagccaattatgcatttcttaaattagaacccccccaatatacccaaatatatatatatgtgtgcatatatatagtaagttgtaacaaagttgtgaattcatacctgaagtatctcaagtgatgcaagttttatgaatttttgtttatgccttttgggaagagttgtattgacaaattttttatgcttaaagtaaaccataaatcaaaaaaataaaatctaggatgcaataaaacaaaacaacttcttgacataagtatggtatgtaaatctgttttgattggaaatcaatttgttatattgccagaattcctgttttagaatacatctctgctgatctgtctgtattcttagactgcatatctgggatgaactctgggcagaattcacatgggcttcctttgaaataaacaagacttttcaaattcttagtcgatctgcagaacctgtagccaggcactgaaccattttgatagatgcagtaatcgttgcaagtgtatatttcaagggagttctggctgggtcctagtttatgcttgtggcagaagcagtgagtaactgggaggaagttggtgagtaagcttcaaggaagaagtcatttttagtactctggatcttcctgattttaaagcactacaaaatggtgcattttcattcttgtcaagtgataacagatatattctgatgagcctgaaatgaatatatattgtatcatttttataatatctagcaaggtttgtattttcctagaacttgaactaaatttcagttcataaaatttataaaatacttagttgttgtaaaatatttttggaatgttcacataggtgacacacaaatgtcccattttcattctttctatagtaaatatgttctgatatgtgaaggtttagcagatgcatcagcatttaatcctagaggatctggcataatcttttcccccaagaatagaaattttttctgcttatgaaagtagtacatgtttctttaaaaacaaatcaatattgacttctgcctgctgtatagcactatgcctccacctggccatgaccaggggcatgtcctggtccacctacctgaaaatgtttgcaaccagcctcctggccatgtgcacaggggctgaagttgtcccacaggtattacgggccaacctgacaatacatgaagttccaccaaagtctgagaactcagaactgagctttggggactgaaagacagcacaaacctcaaatttctcagcactggaaacctcaaaatataactgaattccataaataagattttaagtcttaaatatgtatttttaaatgtattaaaagtcaagctgcttgtatttaagcacctaatacaatgcttaggttgtaaaaggagatgctcaataggtactaactgatatattgagatttaattatggtttgaccaatatttattggaaaccgccaaagcttaaatcatcagcttcttgaatgtgatttgaaaggtaatttagtattgaatagcatgtgagctagagtatttcattctttctggtttatttcttcaaatagactttgaatataatggtgaatgggtattataaattaactaataaaaatgacattgaaaatgaaaaaatatatatattaaagtgtagaaagtgaccaggcgtggtggctcacacctgtaatccaagcaccttgggaggctgaggcaggaggatctcttgatcccaggagttcaagaccagcctgggcaacatagcgagacttcgtctctaaaaaaaaaaaagagagagaaaaaaattttttttatttaaaaaaagtgtagaaagtgtcaagaccccacttcttaccattatttggtatatttctctatacccacccacccttcctccttactccctccctcccttcccaatctttttatctttttgtattctgattttttgtttgtatattttgctttaatttaatgtatcctttaaaaatttcccatacattttatatgtatatataaaaacgcatgctgccaaagataatttataagaaagaccattgaatttttttaaaagtgatatatattcattgaaaaaaatttagaatatatagcaaagcaataaagaactaaataaaattgctgtaactcctctttcaaagataagtgcttttatgattttgttgtatttttttctgtatataggtacatatatagtatttataaagctgtactcatagtacattttcacatcacaggtaccatatcagtgttattaaatattttgtatgccaggggctagacataccaagacaaccaatatgtggttctacttaaataatattagagtatcttttatgatgacacttcatgagttgactataataatcttagacttctaagagtttgggttttcaaaagatcacttagcttttttgggtgatttttcccccttactgtgagatgagagaggctgtttggatttgggattggggtagcggggacagcaacttttcttttctttttcttttttattttgaggtagggtattgctgtgtcacccaggctggagtgcagtggtgtgatctcggctcactgcaacctccacctcccgggctcaggtgatcctcctgcttcagcctcccagtaactgggactacaggcgcgtgccacatgcctggctaattttgtatttttagtagagatggggtttcaccatgttggccaggctggtctctaactcctgacctcaggtgatacgcccacctgggcctcccaaaatactgggattacaggcatgagccgctgcatcagccagcagtttttcttgtggttttttttgtttgttttgttttgttttgtttttgagatagggtcttactctgttgtccacgctggagtgctgtggtatgatcgtagctcactgcagcctcaaactcctgggctcaagtgattccttctgcctccgcctcccgagtagctgggactacaggtatgcaccaccatacctggcaaatttttacaaagttttttgtagggacggggtcttgctacattccccatgtcggtcttgaactcctggcctcaagcaactctcctgtctcagcctcccaaagcactgggattacaagtgtgagccaccacaccatgccagtttttcctgttcagtgtgatattttatcttgttagactacagtgtgttaaaacttgttttactaaattttcaaacatactcaaaagtggagagaatagtataatgaatacccgtatgttcatcacccatgtttagaatattattaaatataaagattttgctgcgtttgtcttagctctttaaaatttttctttttctctttgtgacctaaaggaaattccatatcttatcactttacttctacattcttgactaagatgactaagacatatagttacatggttttttgttttgtttttgttttttaaagacgaaatctcgctcttgtcccccaggctggagtgcaatggtgccatctcagctcagtgcaacctctgccttctgggtacaagcgattctcctgcctcagcctcccaagtagctgggattacaggctcctgccaccacgcctggctaatttttgtatttttagtagagacggcggggggaggtttcaccatgttgacaaggctggtctggaactcctgacctcaggtgatccacccgcctcggcctcccaaagtgctgggattacaggcgtgagccaccgcgcccagcctgtttttttgtttgtgtgttttgttttttttgagacagagtcttgctctgtttcccaggctggagtgaagtggtgccatctcagctcagagacagagtcttgctctgtttcccaggctggagtgaagtggtgccatcttggctcactgcaaccttcacctcccaggttcaagtgattctcctgcctcagcctcccaagtagctgggactacaggcatgtgtcaccacacccggctaatttttttgtatttttagtagagacgggatttcaccgtgttgcccaggctggtctcgaactcctgagctcaggcagtctgcctgcctcagcctcccaaagtgctgggattacacgtgtgaaccaacccgcccggcctgttgttttcttacataattcattatcatacctacaaagttaacagttactaatatcatcttacacctaaatttctctgatagactaaggttattttttaacatcttaatccaatcaaatgtttgtatcctgtaatgctctcattgaaacagctatatttctttttcagattagtgatgatgaaccaggttatgaccttgatttattttgcatacctaatcattatgctgaggatttggaaagggtgtttattcctcatggactaattatggacaggtaagtaagatcttaaaatgaggttttttactttttcttgtgttaatttcaaacatcagcagctgttctgagtacttgctatttgaacataaactaggccaacttattaaataactgatgctttctaaaatcttctttattaaaaataaaagaggagggccttactaattacttagtatcagttgtggtatagtgggactctgtagggaccagaacaaagtaaacattgaagggagatggaagaaggaactctagccagagtcttgcatttctcagtcctaaacagggtaatggactggggctgaatcacatgaaggcaaggtcagatttttattattatgcacatctagcttgaaaattttctgttaagtcaattacagtgaaaaaccttacctggtattgaatgcttgcattgtatgtctggctattctgtgtttttattttaaaattataatatcaaaatatttgtgttataaaatattctaactatggaggccataaacaagaagactaaagttctctcctttcagccttctgtacacatttcttctcaagcactggcctatgcatgtatactatatgcaaaagtacatatatacatttatattttaacgtatgagtatagttttaaatgttattggacacttttaatattagtgtgtctagagctatctaatatattttaaaggttgcatagcattctgtcttatggagataccataactgatttaaccagtccactattgatagacactattttgttcttaccgactgtactagaagaaacattcttttacatgtttggtacttgttcagctttattcaagtggaatttctgggtcaaggggaaagagtttattgaatattttggtattgccaaattttcctctaagaagttgaatcattttatactcctgatgttatatgagagtacctttctcttcacaatttgtctcttttttttttttttttgagacaaggtctctgttgcccaggctggggtgcagtgcagcagaatgatcacagttcactgcagtctcaacctcctgggttcaagcgatccttccacctcagcctcctgagtagctgggactataggtgtgcgccaccactcccagctaatatttttattttgtagaaacagggttcgccatgttacccagcctcccaaagtgctgggattacaggcatgagccactggcccagtttctacagtctctcttaatattgtatattatccagaaaatttcatttaatcagaacctgccagtctgataggtgaaaatggtatcttgtttttatttgcatttaaaaaaaattatgatagtggtatgcttggtttttttgaaggtatcaaattttttaccttatgaaacatgagggcaaaggatgtgatacgtggaagatttaaaaaaaatttttaatgcatttttttgagacaaggtcttgctctattgtccaggctggagtgcagtggcacaatcacagttcactccagcctcaacatcctgcactaaagtgattttcccacctcacctctcaagtagctgggactacaggtacatgctaccatgcctggctaatttttttttttttgcaggcatggggtctcactatattgcccaggttggtgtggaagtttaatgactaagaggtgtttgttataaagtttaatgtatgaaactttctattaaattcctgattttatttctgtaggactgaacgtcttgctcgagatgtgatgaaggagatgggaggccatcacattgtagccctctgtgtgctcaaggggggctataaattctttgctgacctgctggattacatcaaagcactgaatagaaatagtgatagatccattcctatgactgtagattttatcagactgaagagctattgtgtgagtatatttaatatatgattctttttagtggcaacagtaggttttcttatattttctttgaatctctgcaaaccatacttgctttcatttcacttggttacagtgagatttttctaacatattcactagtactttacatcaaagccaatactgtttttttaaaactagtcaccttggaggatatatacttattttacaggtgtgtgtggttttttaaataaactccttttaggaattgctgttgggacttgggatacttttttcactatacatactggtgacagataccctctcttgagctacatcggtttgtggggagtcaaaagtcctttggagctaggtttgacaaataaggtgggttaacacttgtttcctagaaagcacatggagagctagagtattggcgaattgaagaaatccccctttttttttaacacacttaagaaaggggactgcaggtatactcaagagagtaagtcgcaccagaaaccacttttgatccacagtctgcctgtgtcacacaattgaaatgcatcacaacattgacactgtggatgaaacaaaatcagtgtgaattttagtagtgaatttcattcataatttgatcgtgcaaacgtttgatttttattactttagactattgtttctgattttatgttgggttggtatttcctgtgagttactgttttacctttaaaataggaatttttcatactcttcaaagattagaacaaatgtccagtttttgctgtttcatgaatgagtcctgtccatctttgtagaaactcgccttatgttcacatttttattgagaataagaccacttatctacatttaactatcaacctcatcctctccattaatcatctattttagtgacccaagtttttgaccttttccatgtttacatcaatcctgtaggtgattgggcagccatttaagtattattatagacattttcactatcccattaaaaccctttatgcccatacatcataacactacttcctacccataagctccttttaacttgttaaagtcttgcttgaattaaagacttgtttacggtatcgataagcttgatatcaaaacgccaactttgacccggaacgcggaaaacacctgagaaaaacacctgggcgagtctccacgtaaacggtcaaagtccccgcggccctagacaaatattacgcgctatgagtaacacaaaattattcagatttcacttcctcttattcagttttcccgcgaaaatggccaaatcttactcggttacgcccaaatttactacaacatccgcctaaaaccgcgcgaaaattgtcacttcctgtgtacaccggcgcacaccaaaaacgtcacttttgccacatccgtcgcttacatgtgttccgccacacttgcaacatcacacttccgccacactactacgtcacccgccccgttcccacgccccgcgccacgtcacaaactccaccccctcattatcatattggcttcaatccaaaataaggtatattattgatgatgttt

SEQ ID NO: 123 - DNA, 30881 bp, synthetic construct
  source 1..30881: mol_type = other DNA
aaacatcatcaataatataccttattttggattgaagccaatatgataatgagggggtggagtttgtgacgtggcgcggggcgtgggaacggggcgggtgacgtaggttttagggcggagtaacttgtatgtgttgggaattgtagttttcttaaaatgggaagtgacgtaacgtgggaaaacggaagtgacgatttgaggaagttgtgggttttttggctttcgtttctgggcgtaggttcgcgtgcggttttctgggtgttttttgtggactttaaccgttacgtcattttttagtcctatatatactcgctctgcacttggcccttttttacactgtgactgattgagctggtgccgtgtcgagtggtgtttttttaataggttttcttttttactggtaggcgcgccgtcgacgcttattaccctgttatccctactagctagccgacgcgttgggagctctccggatccaagcttatcgatttcgaacccaaatggatctaccacatttgtagaggttttacttgctttaaaaaacctcccacacctccccctgaacctgaaacataaaatgaatgcaattgttgttgttaacttgtttattgcagcttataatggttacaaataaagcaatagcatcacaaatttcacaaataaagcaatagcatcacaaatttcacaaataaagcatttttttcactgcattctagttgtggtttgtccaaactcatcaatgtatcttatcatgtcgagctagctagtcaggacttcagttccagctttgtgccggctccgaaggtcagcgggttgctagaccattgctgacagtaatatgtggcggcatcctcggcttccatagagctgattgtcaggctgtagctggtgccagatccagatccgctgaatctgtagggcacgccggaggccactttgcttgtgtcgtagatccaccgcttggggcttgtgccagacttctgctgataccagttcatgtaggacacgctgctgctggctctgcatgtcatggtcactttctcgcctggggaagcgctcatgatggcggggctttgtgtcagctgaatatcggagccaccaccaccgcttccaccaccacctgaaccgcctccgccactagaaactgtcagggttgtgccctggccccagtaatccagacagtagtggtcgtcgtagtaccgggcacaatagtacacagcgctatcttcagaggtcaggctggacagctgcatgtaggcggtagagctgctcttgtcggtggtcagtgtggccttgtccttgaacttctggttgtaattggtgtagccccggctggggttgatgtagccgatccattccagtccttggccaggcctctgcttgacccagtgcatggtgtaccgggtgaatgtgtagccgctggtcttgcaggacatcttcacagaggcgccaggtctagccagttcggcgccagactgttgcagcttgatatcggatccaccacctccgccagaagaaactgtcacgctggtgccctggccccaatagtccatagcgtagctgccgccgtagtagtagtgcttggcgcaatagtagatggcggtgtcgtcggtctgcaggctgttcatcttcaggaacacctggctcttggagttgtccttgatgatggtcagccgggacttcagggcgctgttgtagtaggttgtctcgctgccccagatcactcccagccattccaggcctttccgaggaggctgtctgatccaggacacgccataatcaggcagggacactccgctgacggtacaggtcacgctcagagattgagatggggccaccaggccagggccagactcttgcagtttcacttcagatcctccgccaccagaacctccgcctccgcttcctccgccgcctgtgatttccagcttggtgcctccgccaaaggtgtaaggcagggtgttgccttgctggcagaagtaggtagcgatatcctcttgttccaggttgctgattgtcaggctgtagtcggtgccagagccgctgccagaaaatctgcttggcacgccgctgtgcagtctgctggtgtggtagatcagcagcttcacggtgccgtcgggtttctgctgataccagttcaggtacttgctgatgtcctggctggctctacagctgatggtcactctatcgcccagagaggcagacaggctgctggtggtctgggtcatctgaatatcgctgtgggcgcctgtggcagctcccacaaggaacaggatgcgccagatccaatccatggtggccctccttcgccggtgatctcagctgtaggaaagagaagaaggttagtagtcgacgtgtccctctcgatgaatctaagtatcaattgtgagcgctcacaagtcaacactctttttgataaatctagtagatatcacttacgtaggcgccggtcacagcttggatctgtaacggcgcagaacagaaaacgaaacaaagacgtagagttgagcaagcagggtcaggcaaagcgtggagagccggctgagtctaggtaggctccaagggagcgccggacaaaggcccggtctcgacctgagctttaaacttacctagacggcggacgcagttcaggaggcaccacaggcgggaggcggcagaacgcgactcaaccggcgtggatggcggcctcaggtagggcggcgggcgcgtgaaggagagatgcgagcccctcgaagcttcagctgtgttctggcggcaaacccgttgcgaaaaagaacgttcacggcgactactgcacttatatacggttctcccccaccctcgggaaaaaggcggagccagtacacgacatcactttcccagtttaccccgcgccaccttctctaggcaccggttcaattgccgacccctccccccaacttctcggggactgtgggcgatgtgcgctctgcccactgacgggcaccggagcgatcgcagatccttcgatagagaaatgttctggcacctgcacttgcactggggacagcctattttgctagtttgttttgtttcgttttgttttgatggagagcgtatgttagttacgattcacacaaaaaaccaacacacagatgtaatgaaaataaagatattttattgcggccgctcgagtctagaggacatgccatggtcgtattaccctgttatccctaactgcatgcgacgtcggcgcgccatcgaattcctgcagcccgggggatccctttgttgattttttccacatagattatttttgactgttttggcactttatataaatggaatcatatagtaaatatatacatgtatatatgtatatatacactatatatgtatatatatagtgtatatatatacatgtatatatgtatatttacatatatactgtatatatgtatatttacatatatactgtatatatgtatatatacacgtatatactgtatatatacagtatatactgtatatatatactgtatatatgtgtatatatatatacagtatatatacagtatacatatatatacatgtatatatacacagtatatatacatgtatatatacacagtatatatacatgtatatatacacagtatatatacatgtatatatacacagtatatatacactgtatatatgtatatatatactgtgtatatatatacagtatatatacagtatatatatacatgtatatgtatatatatactgtatatatgtgtatatatacgtatatatactgtatatatatatagacacttttgtgtctggcttcttgctctcatcataaagcacttgaaatccatccatgttgtagctggtatcagtagctagtttcttttcattgctgagaagtatcactttttattgatgagtagttttacattgtatgaacatgcccgagtttgtttatgcattctactaatagacacctgggctgtttgcagtttttggctattacaaagaaaatttctatatttttttccaacttttattttaggttcagcgggtacatgggcaggtttgttacatcggtaaattgcatgtcactggggtttggtgtacagattatttcaccacccaggtaataagcatagtacctgataggcaggtttttgatcctcaccctcctccctcaagtaggccccagtgtctattgttctattccttttttttttttttgagatggagtctcactctgttgcccaggctggagtgcagtggtgcgatctcggctcactgcaaggtccacctccagggttcaagcgattctactgccgcagcctcccgagtagctgggattacaggcacccaccaccacgcccggctaatttttgtatttttagtagagactgggtttcaccatgttggccaggatggtctcgaactcctcacctcaggtgatccgcccgcttcggcctcgcaaagtactgggattacaggcgtgagccacggtgcctggcctatggttccattctttgtgtacacgtgtactcagtgtttagcttccacttgtaagtgaaaacatgcagtatttggttttctgaaattcttgtcttcatctttttgtagacaatccactacttttatttttaaatattaggaacaatagcctctgtgtgtcctgaattgcaatgttttttctctgattttgctgctcatcttgtaacctgtatggtgtttttctgtgtgcaagctttttactttacgtgggcaattttatcattcttttcttttatggtttctgggtttcatgtcatgattggagaagcttgatctaccctgatactataaaaatatccaccttggcttttttttttttttttagatggattttcactcttgttgcccaggctggagtgcaatggcgtgatctcggctcaccacaacctctgcctcccaggttcaagtgattctcctgcctcggcctcctgagtagctgggattacaggcatgcgccaccacgctcagctaattttgtatttttagtagagacaggatttcaccatgttggtcaggctggtcttgaactccccacctcaggtgatctgtctgcctcggcctcccaaagtgctgggattacaggcgtgacccaccacacctggcccacgttgttttctgatagtgttttcacgtgttattttttctgtcttactctttgaatcatctaaatgtatcttaatgtcaggagtgaggtagaggacccagttgtttggtttaaatgactagccagttttcccaacaccaggtgttgaacatccctcactgatgtgagatgctgcctttttcacagtctcaatccccatgtgcatttctatttattttccttccactttattcacatctttttcagtatccacaaccatattgttttaaatagcttcatgatatgttttaatatttggtagagctagaaccctttcttggttctttttcttttcttcttctcctccttttcctcctccttctttctcctcctccttcttctttctttttagaaatttcctggctattcttgttttgtagtcttccagataaataattttgaatcactttgtcatgttccagaaaataatactgccagaatttttattgtgatcacagaagttttacagattcatctgggggaaaaaaacccatcttcccagaatacagaaagggtgagggaaagacaaacatcaaggacaagtctcaggttctggacttggagaccaagaggatttggggcatccgggagcagggcagggaggtgtgatggctgcctttcactgagtaggaggatgcccagacttgggggaactatggaaagtttggttcagactttctgagttggagatgtctatgcgcagtccacagggcgaagccctggaggtagaggccctccttactgcctccctcattcagtctgaggtccattctccacatggacactgaagtgactcaaggcttcccttgttggatcaggatagtctccagggccctgggtggtctgggcctgcccacctccccatcccctctcctgcctgccctcctcttgctcactggaccccacccaccagcctccttctattcctcctgacatttgcacttgctgttccgtctctgcttggaacatcctagctctttgcatggcttgctccttcccatcttttaatctaagctcaaatatcactccttcagatatgcctttcccaaatatcctagctaaagagaactgctccccacttcccacaagccctagcaaactgggactctccttcttgctttctttctctctgccccttctgtgttttttccatagaccttaacttgttactgttttatttgttgatgtgtttacatcatttgtccccctgtgatggttagttttatgtgtcaacttggctaggctgtaggggctgttcgtcaatcaaacactgatctatgtgtagctgtgaagggattttgtagctgtgattaatagttgactttaagtaaggaagattatcctggagaatgtgggggaaggggcagacctcagccaatcagttgaaaggccttaagaacaaagctgagatttccccgaggaagaagaaattctgcctgtggactgcagcatcagctcctgcttgagaggttccaggctgcccttcctgacagcctgtcctatgattttggacttgccttgccaggtttttcctctttcttgaccccccaaaaccatatatatctcctgctggtttgtttctctggtgtaatcctgagggatgaacactcctccctcccagttcactctgggagaggttggggatcatgtttgtctatttccccatgcctggcccatgcgtgtttattgaatcactgaacaaccacgcattaggaagccagtcatatgtgcttcttcagaacctcatgtccattgccagatctccctggcttttgtggctagaggacaagtgagagatagtagcttacccacagaccttggccctgaggcccccaggggcctgagcctgctgtaagggaggagggagcccctgaggtctcacacacctccctggggatctggcattttcccctggggctggcctcagagctgggcgggggcagattatggagtgggttgtagagggagcacctccccactagcaatcatggttttttctgcgcctctcatagggaggcctacaggcctccaccttcagctcttcaggagccacaggcagctgagtgacttctgcatcacagtcttctcagagacaaacttgcagtaagaaagaggggcccgtgagggaccccagagaaggctgttgtcaaagcaggatgagagtgaactcttccatgggggacacccagcgtctccaagctcttttatgctgtcttcaaggggtctagagagcttcagcccaacatgagacccagtccagcagcatttccctgcgaagtgaaagttaggaccctgactagatacaccacgctgacctcagccagaatatcaagatgctgaggcgctgagatgctgggatgctaaggtgctaaggtgctggggtgctggggtgctaggatgctgaggttttgtgatactgggtcgctgagatgctgggatactggggtgctgaagtgctggggtactggggtgttgccatgctgaaatgctggggtgttgggatgctgaggtgctgggttgctgggatgctgggatagtccttggatgctgcggtgctgagatgctggtctgctggtctgctggggtgttgggatgctgggattttgggatgctggagtgctgcagtgctgcagtgctgagatgctggagtgctggggtgctggaatactgtagtactggtgtgctggagcattgagatgctagggcactgggatgctaaggtgctgagatgctgcagtgctggggtgttgggatgccgaggtgttgggatgcttaagtgctggggtgttgggatgctggggtgctggaacactatggtgctggggtgctggagtgttgagatactgtagtggtgggatgcttaagtgctggggtgctgggtgttgggatgcctaggtgctggggtgccgagatgctggagtactagtgtgctgggatgctgaagtgctggggtcctgagatgctgcagtgctagggtgctgagattctgggctgctggagtgttggggtgctgggatgctggagtgctgagatgcttggacaatggggtgctggaatactatggtgctggggtgctggggtattgagatgctagggtactgggatgctgaagtgctgagatcctggagtgctgggctgctgggccacaggctcttgaatccattcgtctgcccaggggaagaaaccagaagataaagagctaatgaaggagctttggttgagagggaggaagtaatggaaggagcaacatcttgtggaggagcaggagagaatggacctcaggttgggagagagggccaggctacaggccagagaggcagaaggattccagcagagtgtgggctccaggagccaaggggaaacaggtttctgggaggagagagtccagtactgctgaagtggcaagtccgctgaggaccaggaagcttcatttggctttatgaccaggaggaatttggaactgtgactagagtacttagggggaaggaggcaagactggagccagattgctctgggttgaggggtgagtgggaggtgaagcagggcactgtcactcctttgaagggtggcagagagctggaattggtgctggatgggctgtggggtgacagggtcatgtggaaagcccctggggggcacctggaaaaggagaagctgacagtacagtgagaggacagctaagggaaagcggaatggcagaacacgcactgccaggaggaatgaggatagggtcaggagtgccaggggcagtgaggccagcctggggtcaggtggcaggacgtgtccaggaagctggtctgcactgcagcccacactggctcagccttgaggttccctgtgtggttggggtaggaagttgaaccctctgggaatggaagatggaaccagctctgcgagccaagctcagcttttatctatgggtctctgagggctggcagagctgagtggggacaactgtgatccgtgaggctctcaggttgaggtggcccctccgggagggcttcattttcccagcgggtaggttctaagcagcagtggctgggcaggtgggtccaacacagagccagagaagggtgaatgggcctcctggcaccccacccctgctgcccctgagctcagtgatggagggggacagcacagctgagcccaagtgctttggtgtggccctgagggaaagctgcagcctgcctggggcctggcatggatgggacacttgaggcagagggacaatagtgggcgctgcagtgaggctggctcttggagaggtttcctgaggagtgctgcctgagacgggcagggagaacagagacaaagttggtgacagggaatgaaagctgactgaaggactttacccagacctatgaggatatctctctcagcaggaagcaggaggggactgtgtgaggactggccaagagctggagtgttgggaaaatgactctttctccgacccctctgtcctagctctggcccctggactgcggaggtctgcttccacccccattggtcgatcgttgtcccttgtcacagccattgagaattttggcagggagcatgttcttagagcatttttaggctctgcgggacataacagctctgcctcagagcacatgcctttctcagctcctgaaagccactgatcaaattggaacattttgtaccttagggatgaggatatcaactctcccagccacttagagggataaatgtgatgatgcattcaattgtgactacatctgatcccaactgttgcttcagctgctctcctatagcacatggcgggaggcgtgcatcccagtagctacctccccacttttggggagatgtggttccatccatgaaacctgggtacccgcctaccaggtcctggcctatcaggtggcagggtctggtcaaagaagggcatgtgtggtcttcagcaagggagacaggacggtggtgcagagcgtctagaccctcagggcaagtctcccccacacctgctcccggggcagttgtctttgtgacctcccatccccctctgtttcatcctctataaaatgaggggctgagccccaaaataacaggcttctttgccatgatgcaaaactgctgaatctttctttctgacacacaaggcatcgagcagcctctgaaagaaccaaagccactagcaggcttcctgacttgggtttgtaggtactgaatactcccttgaaaaataaaaacatagaggcacttttctcctggctgtttattacagaacgaagaaaaaacacactggcttgaaacagacgccagatttcaaatgtagaggtgaaatacgaggtggcaattaaaatgtgattacagaaagtctggacactgagaaaagtttacaggacagtgggtgtgggttttctataacagacacttaaatatacatgacgataattgcagatagaaaccatcaaagacaaaccccaaatcaactaataatgtttacagatgttcccccccaaaccacagagccttacatcaaaacaaatactgaaaggctttaaaccaggaacagctcgccttaaccccacgagggtgcacacaagctgggctttttctctcggtctgaatggtaaagggaggaggatactctagctcctccaggtggattgctgagacagggctcggctcacacactgtctctgcgcctctcccaaatctggagaactctcccagcctcctggtaaagtgtctctgtggggcacttaacgataaaacagcttctgctgtaaagctcattaggaaagagctagcggagactgaaaggttcgcaaaagagattaagaatcacacaaggcaataggatttttagtgaacatagaaataaatggccaagtggttttctatttggcatttgtcaacttgcacaacaactcttggtcatatccacattgctcattgcattaaaaccataagcgactcagccacctagcttaacaaggtatcactggagcaaacaacacggtctgcatatttgtaacattgtataataaacacaaaacaatgcatagtaaacacaactctactgaaacaaaagccgtcgctttatttacaaagtcacaaaatgaagtataaatacttctgtcattaatgtttaggaaaaccatttacaaaattttcaaatatgtacacgtagcttgaaaaatcaccagctttccattttgtcacaggtagagagagggataagcatgggctgacaacaccactcaaattgtaacgggagacaactgcgggtatggatcgacaccacttcctagagtgatgtcaccatgggggtttctatgggcatcctgctcagatttaaagtgccccagcatcctgggtgacttgcccagaattctgggctgtggcattttgagcagcagcatgctgttccaaaatgtcgtcgatcagcctcaagttgcacacccagtcttcatctgggctcacacaggagcctttcaagagagcttcaatgaaatctacctcattgcagtcaggtgacgaaatcagatcatttagtgggggttggggctggcgcaaaaagtcggcaggtggcagctcagggggaatatccgttctgtcgaacggacctgggaactggctggcagcaacggcagaagcagcagcagcggtggcagcagcagccacatagcttggtggctcgatgccctgtatggggctcaggggactaaagctggccataccctgctggaggaacttggtggtgtttgctacaggcaccgggccctgtaccgggctctgcctgaggctctggctgcccagcaggctgaagctggggttgttggccaggggcacttgtgttcccatcgcagcgggcacttgtgcctcccaatcagatggcctctgaaggcaggcctggccagaaggtgagtgctgctgaacgctattatccacttggctgaggggtgttttccccgaaactgctgtggtcacagctgctgccgctgtgacccatgcagcattgttgaacgcagtgggcattcttggcacactaggccgtctgagctggtggggactcaaggactgggtgcccagggagctgggacagaacccaggcaggggcacttctggtggggtggccttggggctctgcatatgctggcagacagagtcaagtctgcccaggggagtctggcctgagtgtgagaggatgggacactgggggctggaggtgaaaattccttgccgcttccccagagttggtgagatcactcccatgccctcgcagctctggtgcctggtgagtgggatcattcctggactcagattgttctgaagaagcccagttctgggtggcatcaagtgcttgctagatggggggcttgccttgatccggctacacttggaggtgacttgttcttggacggctacatacagaaagagagaagtggggatgagttccaaaggcatcctcgacttcggctgtggccaccggagggtagctcctggcccaacacggacttctcacctcccgcccttggctctctactgagctcccccctgctccccaattcctcgccattcccctcatttctctgccctcagcctggactgcagttcttctgggaagctgccccaactccctaggtctgtgctcaccaagagcagatcacactggactgaaatgccagctgatttgtctcttcaagaaaattggaagctcctggaggtcagggtccatgtctgcttttacactcagtgctctgtatgcaggcctggcactgcccaccctttgacaggtggtgcatattttgtagaaggaaggaaggggccaggtggggtgggctgggctggtggcgggagctagctcagcctcttagattctctacccgatggatgtgacctgggacagcaagtgagtgtggtgagtgagtgcagacggtgctttgttcccctcttgtctcatagcctagatggcctctgagcccagatctggggctcagacaacatttgttcaactgaacggtaatgggtttcctttctgaaggctgaaatctgggagctgacattctggactccctgagttctgaagagcctggggatggagagacacggagcagaagatggaaggtagagtcccaggtgcctaagatggggaatacatctcccctcattgtcatgagagtccactctagctgatatctactgtggccaatatctaccggtacttttttggggtggacactgagtcatgcagcagtcttatggtttacccaaggtcaggtaggggagacagtgcagtcagagcacaagcccagtgtgtctgacccacccaagaatccatgctcgtatctacaaaaatgattttttctcttgtaatggtgcctaggttcttttattatcatggcatgtgtatgtttttcaactaggttacaatctggccttataaggttaacctcctggaggccaccagccttcctgaaacttgtctgtgctgtccctgcaactggagtgtgcctgatgtggcactccagcctggacaagtgggacacagactccgctgttatcaggcccaaagatgtcttccataagaccagaagagcaatggtgtagaggtgtcatgggctacaataaagatgctgacctcctgtctgagggcaagcagcctcttctggccctcagacaaatgctgagtgttcccaagactaccctcggcctggtccaatctcatcccactggtgcgtaagggttgctgaactcatgacttcttggctagcctgcaacctccacggagtgggaactacatcaggcattttgctaactgctgtatcctaggccaataaatgttgatcacatttatagctgccatggtagggtggggacccctgctatctatctgtggaggctctgggagcccctgacacaaactttctgaagcagagcctccccaaccccttttccattccctatacctgacagatggcccaggaacccattagaaatggaaggtcactgcagcagtatgtgaatgtgcgtgtgggagaagggcaggatcagagccctgggggtgtggcagcccccaagtgattctaatccagatcctagggttgtttccctgtcccattgaaatagctgctttaaggggcctgactcagggaaatcagtctcttgaattaagtggtgattttggagtcatttagaccaggccttcaattgggatccactagttctagagcggccgggcccagggaaccccgcaggcgggggcggccagtttcccgggttcggctttacgtcacgcgagggcggcagggaggacggaatggcggggtttggggtgggtccctcctcgggggagccctgggaaaagaggactgcgtgtgggaagagaaggtggaaatggcgttttggttgacatgtgccgcctgcgagcgtgctgcggggaggggccgagggcagattcgggaatgatggcgcggggtgggggcgtgggggctttctcgggagaggcccttccctggaagtttggggtgcgatggtgaggttctcggggcacctctggaggggcctcggcacggaaagcgaccacctgggagggcgtgtggggaccaggttttgcctttagttttgcacacactgtagttcatctttatggagatgctcatggcctcattgaagccccactacagctctggtagcggtaaccatgcgtatttgacacacgaaggaactagggaaaaggcattaggtcatttcaagccgaaattcacatgtgctagaatccagattccatgctgaccgatgccccaggatatagaaaatgagaatctggtccttaccttcaagaacattcttaaccgtaatcagcctctggtatcttagctccaccctcactggttttttcttgtttgttgaaccggccaagctgctggcctccctcctcaaccgttctgatcatgcttgctaaaatagtcaaaaccccggccagttaaatatgctttagcctgctttattatgattatttttgttgttttggcaatgacctggttacctgttgtttctcccactaaaactttttaagggcaggaatcaccgccgtaactctagcacttagcacagtacttggcttgtaagaggtcctcgatgatggtttgttgaatgaatacattaaataattaaccacttgaaccctaagaaagaagcgattctatttcatattaggcattgtaatgacttaaggtaaagagcagtgctattaacggagtctaactgggaatccagcttgtttgggctatttactagttgtgtggctgtgggcaacttacttcacctctctgggcttaagtcattttatgtatatctgaggtgctggctacctcttggagttattgagaggattataagacagtctatgtgaatcagcaacccttgcatggcccctggcggggaacagtaataatagccatcatcatgtttacttacatagtcctaattagtcttcaaaacagccctgtagcaatggtatgattattaccattttacagatgaggaacctttgaagcctcagagaggctaacagacataccctaggtcatacagttattaagagaaggagctctgtctcgaacctagctctctctctctcgagtaataccagttaaaaaataggctacaaataggtactcaaaaaaatggtagtggctgttgtttttattcagttgctgaggaaaaaatgttgatttttcatctctaaacatcaacttacttaattctgccaatttcttttttttgagacagggtctcactctgtcacctaggatggagtgcagtggcacaatcactgctcactgcagcctcgacttcccgggctcgggtgattctccccaggctcaggggattctcccacttcagcctcccaagtagctgggactacaggtgcgcaccaccatccctggctaatatttgtactttattttatttatttatttatttattttttgagatggagtttcgctcttgttgcccgggctggagtacagtggcatgatctcggctcagtgcaacctctgcctcccgggttcaagcgattctcctacctcatccccctgagtagctgggattacaggcgcctgccaccatgcctggctaattttttgtatttttaatagagacgaggtttcaccatgttggccaggctactctcgaactcctgatctcaggtgatccacccgccttggcctcccaaagtgctgggattacaggcgtgagccactgcgcccggcctaatatttgtattttttgtagagatggtgttttgccatgttgtccaggctggtcttgaactcctgagctcaagcgatctgcccgcctctgcttcccaaagtgctgggattacaggcatgagccaccgtgcctggcctaggtagacgcttttagctttggggtgtgatgcctgccccagtatatagtgaatttaattattgctagagctggctgtttgttagttttctttgaacataagatactcattgtttttagtttgcaaatccctcttcctttttaaaaaatttctttcccttaaattgtttgcatgttagcaataacaaatgcttaaatggtgctatgtgctagatactcttctaagccctgttatgtatattaactaattttttaaattacacaaatcagagaggttaagtaacttgcccaagattacccaacaatactaggatttgaacctaagtttgtctcaccccagattctgctcttaatctctaaacttttaagttagtagtgacaatagtaggtatttattgaatacttaactatgttttaggcgttgaagtaaatattttgcaggcattatctaatgtaaacaccctaaagttacataacaggtaccctttaggtaaataaacactagtatgaccttggaggcacagatagttgaagtaacttgcccaatatcacttacatgaaattggccctcaaatgtgtctgatacaacccatgctgcttgtaactatcgttttaaactgccagggtaaacttggacacacttgagctaagaaaaagcttttagatttttgcaaattaatgtgaaagatatgctttatgtggatataatatcttctaaatttcggggatggtagtcctagaaatgtaatcctgccctagccgagcttaccctgccaataattttttacagaattggtaaaacggagcaccttttttttgtccttggccacactgttatcaacagggtgtagattgacatcaatctgtaggtgtaaaccagaattactctttgtgaccaccaggaaatagagcagttcagttcaggggtttctttctgtgaatttagcactgtgacctgcatactacaagtctactttgttttctatccattgtttgtatctgggtattgcaaaaggtaggaaaaggaccaaccagatcagcagagaagagttgccttggagttttcttttagttttctgcagttcattagatagtaactaggccatgtcattttactcccttgtagtgaagatatgttgaagttgtactggtatactcttctacctttctgtaattttatattgtgtagacttgataaaatttatgtgtcaatcaccaccattaatatcaatattgagcctcaattcttatttttctgcccagtggctgccaaattactaacatttacaataattcactactactaagataatctactagttcgatcacatacttcaaattgttatggaactactgtcttcagcattgtgcttctgataactgataagtataattttttttttgtccagagtgaacatgtctattcttccactgtacacactaataaaaggaaaaattgtaatattgggtaaattcatgtccttacacatgtagtagttatgagcccatgtccctagaatgagtaataatttatccctcccttggttgaatagtcaagaatgctgattttaattcttctaacagctttatccctcagaagggaaggcaagcaagttatatatgtagtttatttgtaagactgatatgaaattggaagatgaatctactattagctttaattatttttacatttaggaatattgcatcagtaactcataattttggttttctgttatcctgagttaacacaaattatccaaggagatggcggatcatctgctttgaggtgtttttttttgagaattttaatgtatctgaatataaaaggtaaaaatatgccaactagcaatttctgcccattccagaagtttggaaatattactcattactaggaattaaataaaatatggtttatctattgttatacctcttttaattcacatagctcatttttatcttttatttttgtttgttttttttgagatggagtcttgctctgtcaccaggcaggagtgcagtgatgcaaatctcggctcactctagccaccgactccctggttcaagcgattctcctgcctgagccttctgagtagctgggattacaggcaggcaccaccacgcccagctaatttttgtagagacaggatttcaccgtgttggccaggatggtctccatctcctgacctcatgatctgcctgcttcggcctcccaaagtgctgggattacaggtgggagccactacgcctggcccacatagctcatttttagactcacttccattaagtcttgtttggacccacgaacattgtctttttttttttaagatggagtttcacttttgttgcccagactgtagtgcaatggtgcaatctcagctcactgcaatctctgcctcctgggttctagcaattctcctgcctcagcctcccgagtagctggaattacaggcgcccgccaccacgcccagctaatttttgtgtttttagtagagacggggtttcaccatgttgggcaggccaggggtgatccgcccacctcagcctcccaaagtgctgggattacaggtgtgagccaccgcatctggccaacatgtcttttttttttttttcctttttaaccacaaagagacttaagcagtccttgtcacagatgatgaattgatgttgcaagtattgtcttagcttggattaattttcttgcttactgtaattttagataatatagctttgtaattagagattttatgtgtaaaccacaaaaatgtttacatgaaggccattattacagatgtgacgtgcataattattagtaatttgtatgtttacatgggtcagtctggcaaaaaattatgaagttttaaaaattaaaaaaaattataatgccagttttactggaaagtaaaattatttcagtaatcgattatagcaaaagtattgattttcattccagacaaaagtcagaatgaaaggtaatttctcaatactctttcagattaataaaagtacctgtagcgatttttatcattcacaagtatatcacaagtaagttagaatttgagaactgtgttctagatctctgaggagatgcagtcagatttctgaactgtctcagcaaatggtaagtaacttagagctagtaattaataacctgtcctttgatttctgattcagccaagaatggccatatttgggaaaggcagatctggagagtaaccacgttttcattcatttaccacttctaggcccctccagagctctcagatattttggggttgagcccttccccaaagccatacaggaccttttttttgtgatctgttctagccatttttatgttgggtgcttgttatggactgagcatttatgtcctcccacaccccccccataccttttttgaagtcctaacccccagtgtgatggtatttggagacagggcctttggaaggtaattacagttagaagaagtcgggagggttgggcccaggtctgattggattagtgcccttatatgaaaagacaccaggacgggcgcagtggctcacacctgtaatcccagcactttgggaggccaaggtgggtggatcacgaggtcaggagtttgagaccagcctggccaatgtagtgaaacaccatctctactaaaaatacaaaaattagctgggtgtggtagcgggctcctgtcatccaagctactcgggagggtgaggcatgagaatcacttgaacccgggagttggaggttgcagtgagcccagattgtgccactgtactccagcctgggtgacagagtgagactctgtctcaaaaaagaaaaaaaaaaaaaaagagacaccagagagcttgttagaagaggtcatgtgagcacacagttagaagaccttcaagccaaagaagaggcctgagattgaaacctaccttgcaggtaccttaattttggacttcccagcctccaaaactgtgagaaataagtttctgttaagtcactcagtctgtggtattttgttatggcagcctgagcaggtagttgttctttcagaaggtgttgataataaccacatgcaacaccaagtcacaaataataaaacagatgtaacttatattcatacagaaagttgggcactgccattgccttgttggtttacacggctgtgctagttcagtagcagaaaggtgctggtctcctttactcagtttacaatctaggcagtagaatgtaatcactgctttaaacttgatactgcttagggagagaatcattggtgctgggtaactttgggttctaggtttactttttgtgtatatataactgtttttggtaaatcacaagtttctgggcttgtcgaattagattttgttacagattatgagctttattatgctatacagttagttgtatgtatatatgcctttcccactagattttaagctttttttttttttttttttttgtgacggagtcttgctcttgtcgcccaggctgaagtggagtgcagtggcacaatctcggctcactgcagcctccacctcctaggttcaagcgattctcctgcctcggcctcccaagtaactgggactacaggcacgtgccaccacacccggctaatttttgtattttttgtagagacagggtttcgccatgttggctaggctggtcttgaacttctggcctcaggtgatccacccgcctcagcctcccaaagtgctgggatttacaggcatgagccaccacgcccagctatagctctttaagggttgtaaatttataatcattcttttactctcctgcaaattctgttgcacactgccttaatcaaggtagatgctgaatgcatttttgtataattgaatatgttgcaatccccaactctctccaactgttcctgtcaaagcagccactggattgttaactaatccatattagatggggttaattaatatcagatgggacaagtaagggctaataagattataggccaccaagtagatttctgtctagctcttatagagattgagtttattggacctgtttgataggaagttttggtgtttgggatgattaaaactgaagttcctatttattgaattatacctatttatattatttcatatcagtggtccacatgcaagtgaggcttctgagacagagtttgagttctctcttcaactaccataacacttaacctgtatctttttttttttttttttttttagacaggagtctcgctctgtcactcaggctggagtgtagtggtatgatctcggctcactgtaacctctgcctcctggattcaagcagttctccatgtctcagcctccctagtagctgggattacaggcctgtgccaccatgcctggctaattttttttttgtatttttagtagagacggggttttaccacgttggccaggctggtctcgaactcttgacctcgagcgatcaacttgccttggcctcccaaagtgctgggattacaggcatgagccacagcgcccagccgtctttttttttaaatagcaatttaacactgttcacagttactcatgtacatgtcatgccatctattacactgtaagttctgtgagggtagctgtatcaaatttatctaactctctctagtatgcatgacatagtaagtattcaataaatatttgcatattagtgataaggatacaggttctgaatagtgggtccttaccatttaagaattagtatttgatggccgggcggggtggctcacgcctgtaatcccagcactttgggaggctgaggcgggcggatcatgagatcaggagatcgagaccatcctggctaacatggtgaaatcccgtctttacaaaaaaaatacaaaagaattaaccaagtgtggtggtgggtgcctgtagtcccagctactgctttgtgaggctgaggcaggcagatcacctgaggtgggaaattcaagaccagcctgaccaacatggagaaaccccatctctactaaaaatacaaaattagccgggcgtggtggcgcatgtctgtaatcccagctactcgggaggctgaggcaggagaatggcgtgaacccgggaggcggagcttgcagtgagccaggatcgcgccactgcactccagcctgggcgacagagcgagactccgtctcaaaaaaaaaaaaaaaaaaaaaattagtatttgatatttgatcattaaatatgaattaagaggacttagactttttgttaaatgtcaagctgggaaaagttgtcatttaaatgaattgcctcttatttaatttcgtctgatgatacattttgtttttattttgtaaaaaattattttttttctttttggagacagggtcttgctctgttgcccaggctggtcacaaactcctgacctcaagcaatcctcctgccttagcctcccaaaatgctgggattacaggcgtgacgacctcgcccggccttgtattatgatacattttgaacaactacaagtagacttggtataatgaacctgcacgtacccattgccaagttctgacaactgtctgtctatagccaattatgcatttcttaaattagaacccccccaatatacccaaatatatatatatgtgtgcatatatatagtaagttgtaacaaagttgtgaattcatacctgaagtatctcaagtgatgcaagttttatgaatttttgtttatgccttttgggaagagttgtattgacaaattttttatgcttaaagtaaaccataaatcaaaaaaataaaatctaggatgcaataaaacaaaacaacttcttgacataagtatggtatgtaaatctgttttgattggaaatcaatttgttatattgccagaattcctgttttagaatacatctctgctgatctgtctgtattcttagactgcatatctgggatgaactctgggcagaattcacatgggcttcctttgaaataaacaagacttttcaaattcttagtcgatctgcagaacctgtagccaggcactgaaccattttgatagatgcagtaatcgttgcaagtgtatatttcaagggagttctggctgggtcctagtttatgcttgtggcagaagcagtgagtaactgggaggaagttggtgagtaagcttcaaggaagaagtcatttttagtactctggatcttcctgattttaaagcactacaaaatggtgcattttcattcttgtcaagtgataacagatatattctgatgagcctgaaatgaatatatattgtatcatttttataatatctagcaaggtttgtattttcctagaacttgaactaaatttcagttcataaaatttataaaatacttagttgttgtaaaatatttttggaatgttcacataggtgacacacaaatgtcccattttcattctttctatagtaaatatgttctgatatgtgaaggtttagcagatgcatcagcatttaatcctagaggatctggcataatcttttcccccaagaatagaaattttttctgcttatgaaagtagtacatgtttctttaaaaacaaatcaatattgacttctgcctgctgtatagcactatgcctccacctggccatgaccaggggcatgtcctggtccacctacctgaaaatgtttgcaaccagcctcctggccatgtgcacaggggctgaagttgtcccacaggtattacgggccaacctgacaatacatgaagttccaccaaagtctgagaactcagaactgagctttggggactgaaagacagcacaaacctcaaatttctcagcactggaaacctcaaaatataactgaattccataaataagattttaagtcttaaatatgtatttttaaatgtattaaaagtcaagctgcttgtatttaagcacctaatacaatgcttaggttgtaaaaggagatgctcaataggtactaactgatatattgagatttaattatggtttgaccaatatttattggaaaccgccaaagcttaaatcatcagcttcttgaatgtgatttgaaaggtaatttagtattgaatagcatgtgagctagagtatttcattctttctggtttatttcttcaaatagactttgaatataatggtgaatgggtattataaattaactaataaaaatgacattgaaaatgaaaaaatatatatattaaagtgtagaaagtgaccaggcgtggtggctcacacctgtaatccaagcaccttgggaggctgaggcaggaggatctcttgatcccaggagttcaagaccagcctgggcaacatagcgagacttcgtctctaaaaaaaaaaaagagagagaaaaaaattttttttatttaaaaaaagtgtagaaagtgtcaagaccccacttcttaccattatttggtatatttctctatacccacccacccttcctccttactccctccctcccttcccaatctttttatctttttgtattctgattttttgtttgtatattttgctttaatttaatgtatcctttaaaaatttcccatacattttatatgtatatataaaaacgcatgctgccaaagataatttataagaaagaccattgaatttttttaaaagtgatatatattcattgaaaaaaatttagaatatatagcaaagcaataaagaactaaataaaattgctgtaactcctctttcaaagataagtgcttttatgattttgttgtatttttttctgtatataggtacatatatagtatttataaagctgtactcatagtacattttcacatcacaggtaccatatcagtgttattaaatattttgtatgccaggggctagacataccaagacaaccaatatgtggttctacttaaataatattagagtatcttttatgatgacacttcatgagttgactataataatcttagacttctaagagtttgggttttcaaaagatcacttagcttttttgggtgatttttcccccttactgtgagatgagagaggctgtttggatttgggattggggtagcggggacagcaacttttcttttctttttcttttttattttgaggtagggtattgctgtgtcacccaggctggagtgcagtggtgtgatctcggctcactgcaacctccacctcccgggctcaggtgatcctcctgcttcagcctcccagtaactgggactacaggcgcgtgccacatgcctggctaattttgtatttttagtagagatggggtttcaccatgttggccaggctggtctctaactcctgacctcaggtgatacgcccacctgggcctcccaaaatactgggattacaggcatgagccgctgcatcagccagcagtttttcttgtggttttttttgtttgttttgttttgttttgtttttgagatagggtcttactctgttgtccacgctggagtgctgtggtatgatcgtagctcactgcagcctcaaactcctgggctcaagtgattccttctgcctccgcctcccgagtagctgggactacaggtatgcaccaccatacctggcaaatttttacaaagttttttgtagggacggggtcttgctacattccccatgtcggtcttgaactcctggcctcaagcaactctcctgtctcagcctcccaaagcactgggattacaagtgtgagccaccacaccatgccagtttttcctgttcagtgtgatattttatcttgttagactacagtgtgttaaaacttgttttactaaattttcaaacatactcaaaagtggagagaatagtataatgaatacccgtatgttcatcacccatgtttagaatattattaaatataaagattttgctgcgtttgtcttagctctttaaaatttttctttttctctttgtgacctaaaggaaattccatatcttatcactttacttctacattcttgactaagatgactaagacatatagttacatggttttttgttttgtttttgttttttaaagacgaaatctcgctcttgtcccccaggctggagtgcaatggtgccatctcagctcagtgcaacctctgccttctgggtacaagcgattctcctgcctcagcctcccaagtagctgggattacaggctcctgccaccacgcctggctaatttttgtatttttagtagagacggcggggggaggtttcaccatgttgacaaggctggtctggaactcctgacctcaggtgatccacccgcctcggcctcccaaagtgctgggattacaggcgtgagccaccgcgcccagcctgtttttttgtttgtgtgttttgttttttttgagacagagtcttgctctgtttcccaggctggagtgaagtggtgccatctcagctcagagacagagtcttgctctgtttcccaggctggagtgaagtggtgccatcttggctcactgcaaccttcacctcccaggttcaagtgattctcctgcctcagcctcccaagtagctgggactacaggcatgtgtcaccacacccggctaatttttttgtatttttagtagagacgggatttcaccgtgttgcccaggctggtctcgaactcctgagctcaggcagtctgcctgcctcagcctcccaaagtgctgggattacacgtgtgaaccaacccgcccggcctgttgttttcttacataattcattatcatacctacaaagttaacagttactaatatcatcttacacctaaatttctctgatagactaaggttattttttaacatcttaatccaatcaaatgtttgtatcctgtaatgctctcattgaaacagctatatttctttttcagattagtgatgatgaaccaggttatgaccttgatttattttgcatacctaatcattatgctgaggatttggaaagggtgtttattcctcatggactaattatggacaggtaagtaagatcttaaaatgaggttttttactttttcttgtgttaatttcaaacatcagcagctgttctgagtacttgctatttgaacataaactaggccaacttattaaataactgatgctttctaaaatcttctttattaaaaataaaagaggagggccttactaattacttagtatcagttgtggtatagtgggactctgtagggaccagaacaaagtaaacattgaagggagatggaagaaggaactctagccagagtcttgcatttctcagtcctaaacagggtaatggactggggctgaatcacatgaaggcaaggtcagatttttattattatgcacatctagcttgaaaattttctgttaagtcaattacagtgaaaaaccttacctggtattgaatgcttgcattgtatgtctggctattctgtgtttttattttaaaattataatatcaaaatatttgtgttataaaatattctaactatggaggccataaacaagaagactaaagttctctcctttcagccttctgtacacatttcttctcaagcactggcctatgcatgtatactatatgcaaaagtacatatatacatttatattttaacgtatgagtatagttttaaatgttattggacacttttaatattagtgtgtctagagctatctaatatattttaaaggttgcatagcattctgtcttatggagataccataactgatttaaccagtccactattgatagacactattttgttcttaccgactgtactagaagaaacattcttttacatgtttggtacttgttcagctttattcaagtggaatttctgggtcaaggggaaagagtttattgaatattttggtattgccaaattttcctctaagaagttgaatcattttatactcctgatgttatatgagagtacctttctcttcacaatttgtctcttttttttttttttttgagacaaggtctctgttgcccaggctggggtgcagtgcagcagaatgatcacagttcactgcagtctcaacctcctgggttcaagcgatccttccacctcagcctcctgagtagctgggactataggtgtgcgccaccactcccagctaatatttttattttgtagaaacagggttcgccatgttacccagcctcccaaagtgctgggattacaggcatgagccactggcccagtttctacagtctctcttaatattgtatattatccagaaaatttcatttaatcagaacctgccagtctgataggtgaaaatggtatcttgtttttatttgcatttaaaaaaaattatgatagtggtatgcttggtttttttgaaggtatcaaattttttaccttatgaaacatgagggcaaaggatgtgatacgtggaagatttaaaaaaaatttttaatgcatttttttgagacaaggtcttgctctattgtccaggctggagtgcagtggcacaatcacagttcactccagcctcaacatcctgcactaaagtgattttcccacctcacctctcaagtagctgggactacaggtacatgctaccatgcctggctaatttttttttttttgcaggcatggggtctcactatattgcccaggttggtgtggaagtttaatgactaagaggtgtttgttataaagtttaatgtatgaaactttctattaaattcctgattttatttctgtaggactgaacgtcttgctcgagatgtgatgaaggagatgggaggccatcacattgtagccctctgtgtgctcaaggggggctataaattctttgctgacctgctggattacatcaaagcactgaatagaaatagtgatagatccattcctatgactgtagattttatcagactgaagagctattgtgtgagtatatttaatatatgattctttttagtggcaacagtaggttttcttatattttctttgaatctctgcaaaccatacttgctttcatttcacttggttacagtgagatttttctaacatattcactagtactttacatcaaagccaatactgtttttttaaaactagtcaccttggaggatatatacttattttacaggtgtgtgtggttttttaaataaactccttttaggaattgctgttgggacttgggatacttttttcactatacatactggtgacagataccctctcttgagctacatcggtttgtggggagtcaaaagtcctttggagctaggtttgacaaataaggtgggttaacacttgtttcctagaaagcacatggagagctagagtattggcgaattgaagaaatccccctttttttttaacacacttaagaaaggggactgcaggtatactcaagagagtaagtcgcaccagaaaccacttttgatccacagtctgcctgtgtcacacaattgaaatgcatcacaacattgacactgtggatgaaacaaaatcagtgtgaattttagtagtgaatttcattcataatttgatcgtgcaaacgtttgatttttattactttagactattgtttctgattttatgttgggttggtatttcctgtgagttactgttttacctttaaaataggaatttttcatactcttcaaagattagaacaaatgtccagtttttgctgtttcatgaatgagtcctgtccatctttgtagaaactcgccttatgttcacatttttattgagaataagaccacttatctacatttaactatcaacctcatcctctccattaatcatctattttagtgacccaagtttttgaccttttccatgtttacatcaatcctgtaggtgattgggcagccatttaagtattattatagacattttcactatcccattaaaaccctttatgcccatacatcataacactacttcctacccataagctccttttaacttgttaaagtcttgcttgaattaaagacttgtttacggtatcgataagcttgatatcaaaacgccaactttgacccggaacgcggaaaacacctgagaaaaacacctgggcgagtctccacgtaaacggtcaaagtccccgcggccctagacaaatattacgcgctatgagtaacacaaaattattcagatttcacttcctcttattcagttttcccgcgaaaatggccaaatcttactcggttacgcccaaatttactacaacatccgcctaaaaccgcgcgaaaattgtcacttcctgtgtacaccggcgcacaccaaaaacgtcacttttgccacatccgtcgcttacatgtgttccgccacacttgcaacatcacacttccgccacactactacgtcacccgccccgttcccacgccccgcgccacgtcacaaactccaccccctcattatcatattggcttcaatccaaaataaggtatattattgatgatgttt

SEQ ID NO: 124 - DNA, 29539 bp, synthetic construct
  source 1..29539: mol_type = other DNA
aaacatcatcaataatataccttattttggattgaagccaatatgataatgagggggtggagtttgtgacgtggcgcggggcgtgggaacggggcgggtgacgtaggttttagggcggagtaacttgtatgtgttgggaattgtagttttcttaaaatgggaagtgacgtaacgtgggaaaacggaagtgacgatttgaggaagttgtgggttttttggctttcgtttctgggcgtaggttcgcgtgcggttttctgggtgttttttgtggactttaaccgttacgtcattttttagtcctatatatactcgctctgcacttggcccttttttacactgtgactgattgagctggtgccgtgtcgagtggtgtttttttaataggttttcttttttactggtaggcgcgccgtcgacgcgacaactgtcttattaccctgttatccctaccttaattaagctagccgacgcgttggccaggagctcagatctccggatccaagcttatcgatttcgaacccaaatggatctaccacatttgtagaggttttacttgctttaaaaaacctcccacacctccccctgaacctgaaacataaaatgaatgcaattgttgttgttaacttgtttattgcagcttataatggttacaaataaagcaatagcatcacaaatttcacaaataaagcaatagcatcacaaatttcacaaataaagcatttttttcactgcattctagttgtggtttgtccaaactcatcaatgtatcttatcatgtcgagctagctagtcaggacttcagttccagctttgtgccggctccgaaggtcagcgggttgctagaccattgctgacagtaatatgtggcggcatcctcggcttccatagagctgattgtcaggctgtagctggtgccagatccagatccgctgaatctgtagggcacgccggaggccactttgcttgtgtcgtagatccaccgcttggggcttgtgccagacttctgctgataccagttcatgtaggacacgctgctgctggctctgcatgtcatggtcactttctcgcctggggaagcgctcatgatggcggggctttgtgtcagctgaatatcggagccaccaccaccgcttccaccaccacctgaaccgcctccgccactagaaactgtcagggttgtgccctggccccagtaatccagacagtagtggtcgtcgtagtaccgggcacaatagtacacagcgctatcttcagaggtcaggctggacagctgcatgtaggcggtagagctgctcttgtcggtggtcagtgtggccttgtccttgaacttctggttgtaattggtgtagccccggctggggttgatgtagccgatccattccagtccttggccaggcctctgcttgacccagtgcatggtgtaccgggtgaatgtgtagccgctggtcttgcaggacatcttcacagaggcgccaggtctagccagttcggcgccagactgttgcagcttgatatcggatccaccgccaccaagggctttgatttccagcttggtgccgctgccgaaggtgaaaggggttctgaagtgctgctgacaaaagtacacggccagatcctcggcctgcacgctgctgatggtaaaggtgaagtcagggccagagccagagccggtgaatctagagggcacgcctgtgtatctgctgctggcgctgtagatcagcagcttaggagactggccaggcttctgctgataccaggccacggcgttgtacacgtcctggctggctttacaggtgatggacactctgtcgcccacgctggtgctcagaaacttgtggctctgggtcagctgaatatcagatcctccgccgcctgaacctccgcctccgcttcctccgccaccagaagagactgtcacggttgtgccctggccccaatatggcacgtagccgtggtacacttcccatctggcacaaaagtaggtggccatgtcctcggacttcaggttgttgatctgcaggtaggcggtgttggcgctggtttccaggctgaagtcgaatctgcccttgaaatcgtcggcgaaggtgctctcgccggtgctggtattgatccagcccatccatttcaggccctgtccaggggcctgcttgacccagttcatgccgtagttggtgaaggggtagccgctggccttgcaggagatcttcactgtctcgccaggtttcttcagctcggggccagactgctgcagctgaacttcagaatgggcgcctgtggcggctcccacaagaaacaggatgcgccagatccagtccatggaaggtccggggttctcttccacgtcgccacatgtcagcaggctgcctctgccttcggacttcagttccagctttgtgccggctccgaaggtcagcgggttgctagaccattgctgacagtaatatgtggcggcatcctcggcttccatgctggagattgtcaggctgtagctggttccgctgccgcttccggaaaatctgtagggcacgccggaggccactttgcttgtgtcgtagatccaccgcttggggcttgtgccagacttctgctgataccagttcatgtaggacacgctggagctggctctacaggtcatggtcactttctcgcctgggctagcgctcatgatggcaggagactgggtcagctgaatatcagaaccgccaccaccgcttccgccgccacctgaaccaccaccacctgaagaaactgtcagtgtggtgccctggccccagtaatccagacagtagtggtcgtcgtagtaccgggcacaatagtacacagcgctatcttcagaggtcaggctgctcagctgcatgtaggcggtagagctgctcttgtcggtggtcagagtggccttgtccttgaacttctggttgtaattggtgtagccccggctggggttgatgtagccgatccattccagtccttggccaggcctctgcttgacccagtgcatggtgtaccgggtgaatgtgtatccgctggtcttgcagctcatcttcacagaagcgccaggtctagccagctcggcgccagactgttgcagcttaatatcgctgcctccgcctccgccactagacactgtgaccagtgttcctctgccccagtagtcgaggccctgtctggcgcaataatacacggcggtgtcctcggctctcagggagttcatctgcaggtacaggctgttcttggcgttgtcccggctgatggtgaatctgcccttgatgctgtccaggtagtaggtgtagctgccgccgctgctgattgtggacacccattcaaggcctttgccaggagcctgtcggacccagctcatatcgtagctgctgaaggtgaagccgctggcggcacaagacagtctcagagatccgccaggcttaaccaggcctccgcctgattccaccagctgaacttcagatccaccaccgccggatccgccgcctccgcttcctccgccgccagatcctccgccacctctcttgatttccaccttggtgcctccgccaaatgtcaggggattgctggaccactgcaggcagtagtacacggcgaagtcctcaggttccaggctgcttatggtcagggtgaaatcggtgccgctgccagagccagaaaatctggcaggcactccgctggccagattgctggtcaggtagatcaggattctaggggcctgtccgggcttctgctgcagccagtagatgtagttgatggagctgctggcgctacagctcagtgtggctctttcgccagggctaagagacagtgtggcagggctctgtgtcagcacaatctcgccggtggtatcaggcagccacagcagcagcagaaacagcagttgagctggagcctccatggtggccctccttcgccggtgatctcagctgtaggaaagagaagaaggttagtagtcgacgtgtccctctcgatgaatctaagtatcaattgtgagcgctcacaagtcaacactctttttgataaatctagtagatatcacttacgtaggcgccggtcacagcttggatctgtaacggcgcagaacagaaaacgaaacaaagacgtagagttgagcaagcagggtcaggcaaagcgtggagagccggctgagtctaggtaggctccaagggagcgccggacaaaggcccggtctcgacctgagctttaaacttacctagacggcggacgcagttcaggaggcaccacaggcgggaggcggcagaacgcgactcaaccggcgtggatggcggcctcaggtagggcggcgggcgcgtgaaggagagatgcgagcccctcgaagcttcagctgtgttctggcggcaaacccgttgcgaaaaagaacgttcacggcgactactgcacttatatacggttctcccccaccctcgggaaaaaggcggagccagtacacgacatcactttcccagtttaccccgcgccaccttctctaggcaccggttcaattgccgacccctccccccaacttctcggggactgtgggcgatgtgcgctctgcccactgacgggcaccggagcgatcgcagatccttcgatagagaaatgttctggcacctgcacttgcactggggacagcctattttgctagtttgttttgtttcgttttgttttgatggagagcgtatgttagttacgattcacacaaaaaaccaacacacagatgtaatgaaaataaagatattttattgcggccgctcgagtctagaggtatacatgccatggtccgcggtattaccctgttatccctaagacaactgtcctgcatgcgacgtcggcgcgccatcgaattcctgcagcccgggggatccctttgttgattttttccacatagattatttttgactgttttggcactttatataaatggaatcatatagtaaatatatacatgtatatatgtatatatacactatatatgtatatatatagtgtatatatatacatgtatatatgtatatttacatatatactgtatatatgtatatttacatatatactgtatatatgtatatatacacgtatatactgtatatatacagtatatactgtatatatatactgtatatatgtgtatatatatatacagtatatatacagtatacatatatatacatgtatatatacacagtatatatacatgtatatatacacagtatatatacatgtatatatacacagtatatatacatgtatatatacacagtatatatacactgtatatatgtatatatatactgtgtatatatatacagtatatatacagtatatatatacatgtatatgtatatatatactgtatatatgtgtatatatacgtatatatactgtatatatatatagacacttttgtgtctggcttcttgctctcatcataaagcacttgaaatccatccatgttgtagctggtatcagtagctagtttcttttcattgctgagaagtatcactttttattgatgagtagttttacattgtatgaacatgcccgagtttgtttatgcattctactaatagacacctgggctgtttgcagtttttggctattacaaagaaaatttctatatttttttccaacttttattttaggttcagcgggtacatgggcaggtttgttacatcggtaaattgcatgtcactggggtttggtgtacagattatttcaccacccaggtaataagcatagtacctgataggcaggtttttgatcctcaccctcctccctcaagtaggccccagtgtctattgttctattccttttttttttttttgagatggagtctcactctgttgcccaggctggagtgcagtggtgcgatctcggctcactgcaaggtccacctccagggttcaagcgattctactgccgcagcctcccgagtagctgggattacaggcacccaccaccacgcccggctaatttttgtatttttagtagagactgggtttcaccatgttggccaggatggtctcgaactcctcacctcaggtgatccgcccgcttcggcctcgcaaagtactgggattacaggcgtgagccacggtgcctggcctatggttccattctttgtgtacacgtgtactcagtgtttagcttccacttgtaagtgaaaacatgcagtatttggttttctgaaattcttgtcttcatctttttgtagacaatccactacttttatttttaaatattaggaacaatagcctctgtgtgtcctgaattgcaatgttttttctctgattttgctgctcatcttgtaacctgtatggtgtttttctgtgtgcaagctttttactttacgtgggcaattttatcattcttttcttttatggtttctgggtttcatgtcatgattggagaagcttgatctaccctgatactataaaaatatccaccttggcttttttttttttttttagatggattttcactcttgttgcccaggctggagtgcaatggcgtgatctcggctcaccacaacctctgcctcccaggttcaagtgattctcctgcctcggcctcctgagtagctgggattacaggcatgcgccaccacgctcagctaattttgtatttttagtagagacaggatttcaccatgttggtcaggctggtcttgaactccccacctcaggtgatctgtctgcctcggcctcccaaagtgctgggattacaggcgtgacccaccacacctggcccacgttgttttctgatagtgttttcacgtgttattttttctgtcttactctttgaatcatctaaatgtatcttaatgtcaggagtgaggtagaggacccagttgtttggtttaaatgactagccagttttcccaacaccaggtgttgaacatccctcactgatgtgagatgctgcctttttcacagtctcaatccccatgtgcatttctatttattttccttccactttattcacatctttttcagtatccacaaccatattgttttaaatagcttcatgatatgttttaatatttggtagagctagaaccctttcttggttctttttcttttcttcttctcctccttttcctcctccttctttctcctcctccttcttctttctttttagaaatttcctggctattcttgttttgtagtcttccagataaataattttgaatcactttgtcatgttccagaaaataatactgccagaatttttattgtgatcacagaagttttacagattcatctgggggaaaaaaacccatcttcccagaatacagaaagggtgagggaaagacaaacatcaaggacaagtctcaggttctggacttggagaccaagaggatttggggcatccgggagcagggcagggaggtgtgatggctgcctttcactgagtaggaggatgcccagacttgggggaactatggaaagtttggttcagactttctgagttggagatgtctatgcgcagtccacagggcgaagccctggaggtagaggccctccttactgcctccctcattcagtctgaggtccattctccacatggacactgaagtgactcaaggcttcccttgttggatcaggatagtctccagggccctgggtggtctgggcctgcccacctccccatcccctctcctgcctgccctcctcttgctcactggaccccacccaccagcctccttctattcctcctgacatttgcacttgctgttccgtctctgcttggaacatcctagctctttgcatggcttgctccttcccatcttttaatctaagctcaaatatcactccttcagatatgcctttcccaaatatcctagctaaagagaactgctccccacttcccacaagccctagcaaactgggactctccttcttgctttctttctctctgccccttctgtgttttttccatagaccttaacttgttactgttttatttgttgatgtgtttacatcatttgtccccctgtgatggttagttttatgtgtcaacttggctaggctgtaggggctgttcgtcaatcaaacactgatctatgtgtagctgtgaagggattttgtagctgtgattaatagttgactttaagtaaggaagattatcctggagaatgtgggggaaggggcagacctcagccaatcagttgaaaggccttaagaacaaagctgagatttccccgaggaagaagaaattctgcctgtggactgcagcatcagctcctgcttgagaggttccaggctgcccttcctgacagcctgtcctatgattttggacttgccttgccaggtttttcctctttcttgaccccccaaaaccatatatatctcctgctggtttgtttctctggtgtaatcctgagggatgaacactcctccctcccagttcactctgggagaggttggggatcatgtttgtctatttccccatgcctggcccatgcgtgtttattgaatcactgaacaaccacgcattaggaagccagtcatatgtgcttcttcagaacctcatgtccattgccagatctccctggcttttgtggctagaggacaagtgagagatagtagcttacccacagaccttggccctgaggcccccaggggcctgagcctgctgtaagggaggagggagcccctgaggtctcacacacctccctggggatctggcattttcccctggggctggcctcagagctgggcgggggcagattatggagtgggttgtagagggagcacctccccactagcaatcatggttttttctgcgcctctcatagggaggcctacaggcctccaccttcagctcttcaggagccacaggcagctgagtgacttctgcatcacagtcttctcagagacaaacttgcagtaagaaagaggggcccgtgagggaccccagagaaggctgttgtcaaagcaggatgagagtgaactcttccatgggggacacccagcgtctccaagctcttttatgctgtcttcaaggggtctagagagcttcagcccaacatgagacccagtccagcagcatttccctgcgaagtgaaagttaggaccctgactagatacaccacgctgacctcagccagaatatcaagatgctgaggcgctgagatgctgggatgctaaggtgctaaggtgctggggtgctggggtgctaggatgctgaggttttgtgatactgggtcgctgagatgctgggatactggggtgctgaagtgctggggtactggggtgttgccatgctgaaatgctggggtgttgggatgctgaggtgctgggttgctgggatgctgggatagtccttggatgctgcggtgctgagatgctggtctgctggtctgctggggtgttgggatgctgggattttgggatgctggagtgctgcagtgctgcagtgctgagatgctggagtgctggggtgctggaatactgtagtactggtgtgctggagcattgagatgctagggcactgggatgctaaggtgctgagatgctgcagtgctggggtgttgggatgccgaggtgttgggatgcttaagtgctggggtgttgggatgctggggtgctggaacactatggtgctggggtgctggagtgttgagatactgtagtggtgggatgcttaagtgctggggtgctgggtgttgggatgcctaggtgctggggtgccgagatgctggagtactagtgtgctgggatgctgaagtgctggggtcctgagatgctgcagtgctagggtgctgagattctgggctgctggagtgttggggtgctgggatgctggagtgctgagatgcttggacaatggggtgctggaatactatggtgctggggtgctggggtattgagatgctagggtactgggatgctgaagtgctgagatcctggagtgctgggctgctgggccacaggctcttgaatccattcgtctgcccaggggaagaaaccagaagataaagagctaatgaaggagctttggttgagagggaggaagtaatggaaggagcaacatcttgtggaggagcaggagagaatggacctcaggttgggagagagggccaggctacaggccagagaggcagaaggattccagcagagtgtgggctccaggagccaaggggaaacaggtttctgggaggagagagtccagtactgctgaagtggcaagtccgctgaggaccaggaagcttcatttggctttatgaccaggaggaatttggaactgtgactagagtacttagggggaaggaggcaagactggagccagattgctctgggttgaggggtgagtgggaggtgaagcagggcactgtcactcctttgaagggtggcagagagctggaattggtgctggatgggctgtggggtgacagggtcatgtggaaagcccctggggggcacctggaaaaggagaagctgacagtacagtgagaggacagctaagggaaagcggaatggcagaacacgcactgccaggaggaatgaggatagggtcaggagtgccaggggcagtgaggccagcctggggtcaggtggcaggacgtgtccaggaagctggtctgcactgcagcccacactggctcagccttgaggttccctgtgtggttggggtaggaagttgaaccctctgggaatggaagatggaaccagctctgcgagccaagctcagcttttatctatgggtctctgagggctggcagagctgagtggggacaactgtgatccgtgaggctctcaggttgaggtggcccctccgggagggcttcattttcccagcgggtaggttctaagcagcagtggctgggcaggtgggtccaacacagagccagagaagggtgaatgggcctcctggcaccccacccctgctgcccctgagctcagtgatggagggggacagcacagctgagcccaagtgctttggtgtggccctgagggaaagctgcagcctgcctggggcctggcatggatgggacacttgaggcagagggacaatagtgggcgctgcagtgaggctggctcttggagaggtttcctgaggagtgctgcctgagacgggcagggagaacagagacaaagttggtgacagggaatgaaagctgactgaaggactttacccagacctatgaggatatctctctcagcaggaagcaggaggggactgtgtgaggactggccaagagctggagtgttgggaaaatgactctttctccgacccctctgtcctagctctggcccctggactgcggaggtctgcttccacccccattggtcgatcgttgtcccttgtcacagccattgagaattttggcagggagcatgttcttagagcatttttaggctctgcgggacataacagctctgcctcagagcacatgcctttctcagctcctgaaagccactgatcaaattggaacattttgtaccttagggatgaggatatcaactctcccagccacttagagggataaatgtgatgatgcattcaattgtgactacatctgatcccaactgttgcttcagctgctctcctatagcacatggcgggaggcgtgcatcccagtagctacctccccacttttggggagatgtggttccatccatgaaacctgggtacccgcctaccaggtcctggcctatcaggtggcagggtctggtcaaagaagggcatgtgtggtcttcagcaagggagacaggacggtggtgcagagcgtctagaccctcagggcaagtctcccccacacctgctcccggggcagttgtctttgtgacctcccatccccctctgtttcatcctctataaaatgaggggctgagccccaaaataacaggcttctttgccatgatgcaaaactgctgaatctttctttctgacacacaaggcatcgagcagcctctgaaagaaccaaagccactagcaggcttcctgacttgggtttgtaggtactgaatactcccttgaaaaataaaaacatagaggcacttttctcctggctgtttattacagaacgaagaaaaaacacactggcttgaaacagacgccagatttcaaatgtagaggtgaaatacgaggtggcaattaaaatgtgattacagaaagtctggacactgagaaaagtttacaggacagtgggtgtgggttttctataacagacacttaaatatacatgacgataattgcagatagaaaccatcaaagacaaaccccaaatcaactaataatgtttacagatgttcccccccaaaccacagagccttacatcaaaacaaatactgaaaggctttaaaccaggaacagctcgccttaaccccacgagggtgcacacaagctgggctttttctctcggtctgaatggtaaagggaggaggatactctagctcctccaggtggattgctgagacagggctcggctcacacactgtctctgcgcctctcccaaatctggagaactctcccagcctcctggtaaagtgtctctgtggggcacttaacgataaaacagcttctgctgtaaagctcattaggaaagagctagcctgcaacctccacggagtgggaactacatcaggcattttgctaactgctgtatcctaggccaataaatgttgatcacatttatagctgccatggtagggtggggacccctgctatctatctgtggaggctctgggagcccctgacacaaactttctgaagcagagcctccccaaccccttttccattccctatacctgacagatggcccaggaacccattagaaatggaaggtcactgcagcagtatgtgaatgtgcgtgtgggagaagggcaggatcagagccctgggggtgtggcagcccccaagtgattctaatccagatcctagggttgtttccctgtcccattgaaatagctgctttaaggggcctgactcagggaaatcagtctcttgaattaagtggtgattttggagtcatttagaccaggccttcaattgggatccactagttctagagcggccgggcccagggaaccccgcaggcgggggcggccagtttcccgggttcggctttacgtcacgcgagggcggcagggaggacggaatggcggggtttggggtgggtccctcctcgggggagccctgggaaaagaggactgcgtgtgggaagagaaggtggaaatggcgttttggttgacatgtgccgcctgcgagcgtgctgcggggaggggccgagggcagattcgggaatgatggcgcggggtgggggcgtgggggctttctcgggagaggcccttccctggaagtttggggtgcgatggtgaggttctcggggcacctctggaggggcctcggcacggaaagcgaccacctgggagggcgtgtggggaccaggttttgcctttagttttgcacacactgtagttcatctttatggagatgctcatggcctcattgaagccccactacagctctggtagcggtaaccatgcgtatttgacacacgaaggaactagggaaaaggcattaggtcatttcaagccgaaattcacatgtgctagaatccagattccatgctgaccgatgccccaggatatagaaaatgagaatctggtccttaccttcaagaacattcttaaccgtaatcagcctctggtatcttagctccaccctcactggttttttcttgtttgttgaaccggccaagctgctggcctccctcctcaaccgttctgatcatgcttgctaaaatagtcaaaaccccggccagttaaatatgctttagcctgctttattatgattatttttgttgttttggcaatgacctggttacctgttgtttctcccactaaaactttttaagggcaggaatcaccgccgtaactctagcacttagcacagtacttggcttgtaagaggtcctcgatgatggtttgttgaatgaatacattaaataattaaccacttgaaccctaagaaagaagcgattctatttcatattaggcattgtaatgacttaaggtaaagagcagtgctattaacggagtctaactgggaatccagcttgtttgggctatttactagttgtgtggctgtgggcaacttacttcacctctctgggcttaagtcattttatgtatatctgaggtgctggctacctcttggagttattgagaggattataagacagtctatgtgaatcagcaacccttgcatggcccctggcggggaacagtaataatagccatcatcatgtttacttacatagtcctaattagtcttcaaaacagccctgtagcaatggtatgattattaccattttacagatgaggaacctttgaagcctcagagaggctaacagacataccctaggtcatacagttattaagagaaggagctctgtctcgaacctagctctctctctctcgagtaataccagttaaaaaataggctacaaataggtactcaaaaaaatggtagtggctgttgtttttattcagttgctgaggaaaaaatgttgatttttcatctctaaacatcaacttacttaattctgccaatttcttttttttgagacagggtctcactctgtcacctaggatggagtgcagtggcacaatcactgctcactgcagcctcgacttcccgggctcgggtgattctccccaggctcaggggattctcccacttcagcctcccaagtagctgggactacaggtgcgcaccaccatccctggctaatatttgtactttattttatttatttatttatttattttttgagatggagtttcgctcttgttgcccgggctggagtacagtggcatgatctcggctcagtgcaacctctgcctcccgggttcaagcgattctcctacctcatccccctgagtagctgggattacaggcgcctgccaccatgcctggctaattttttgtatttttaatagagacgaggtttcaccatgttggccaggctactctcgaactcctgatctcaggtgatccacccgccttggcctcccaaagtgctgggattacaggcgtgagccactgcgcccggcctaatatttgtattttttgtagagatggtgttttgccatgttgtccaggctggtcttgaactcctgagctcaagcgatctgcccgcctctgcttcccaaagtgctgggattacaggcatgagccaccgtgcctggcctaggtagacgcttttagctttggggtgtgatgcctgccccagtatatagtgaatttaattattgctagagctggctgtttgttagttttctttgaacataagatactcattgtttttagtttgcaaatccctcttcctttttaaaaaatttctttcccttaaattgtttgcatgttagcaataacaaatgcttaaatggtgctatgtgctagatactcttctaagccctgttatgtatattaactaattttttaaattacacaaatcagagaggttaagtaacttgcccaagattacccaacaatactaggatttgaacctaagtttgtctcaccccagattctgctcttaatctctaaacttttaagttagtagtgacaatagtaggtatttattgaatacttaactatgttttaggcgttgaagtaaatattttgcaggcattatctaatgtaaacaccctaaagttacataacaggtaccctttaggtaaataaacactagtatgaccttggaggcacagatagttgaagtaacttgcccaatatcacttacatgaaattggccctcaaatgtgtctgatacaacccatgctgcttgtaactatcgttttaaactgccagggtaaacttggacacacttgagctaagaaaaagcttttagatttttgcaaattaatgtgaaagatatgctttatgtggatataatatcttctaaatttcggggatggtagtcctagaaatgtaatcctgccctagccgagcttaccctgccaataattttttacagaattggtaaaacggagcaccttttttttgtccttggccacactgttatcaacagggtgtagattgacatcaatctgtaggtgtaaaccagaattactctttgtgaccaccaggaaatagagcagttcagttcaggggtttctttctgtgaatttagcactgtgacctgcatactacaagtctactttgttttctatccattgtttgtatctgggtattgcaaaaggtaggaaaaggaccaaccagatcagcagagaagagttgccttggagttttcttttagttttctgcagttcattagatagtaactaggccatgtcattttactcccttgtagtgaagatatgttgaagttgtactggtatactcttctacctttctgtaattttatattgtgtagacttgataaaatttatgtgtcaatcaccaccattaatatcaatattgagcctcaattcttatttttctgcccagtggctgccaaattactaacatttacaataattcactactactaagataatctactagttcgatcacatacttcaaattgttatggaactactgtcttcagcattgtgcttctgataactgataagtataattttttttttgtccagagtgaacatgtctattcttccactgtacacactaataaaaggaaaaattgtaatattgggtaaattcatgtccttacacatgtagtagttatgagcccatgtccctagaatgagtaataatttatccctcccttggttgaatagtcaagaatgctgattttaattcttctaacagctttatccctcagaagggaaggcaagcaagttatatatgtagtttatttgtaagactgatatgaaattggaagatgaatctactattagctttaattatttttacatttaggaatattgcatcagtaactcataattttggttttctgttatcctgagttaacacaaattatccaaggagatggcggatcatctgctttgaggtgtttttttttgagaattttaatgtatctgaatataaaaggtaaaaatatgccaactagcaatttctgcccattccagaagtttggaaatattactcattactaggaattaaataaaatatggtttatctattgttatacctcttttaattcacatagctcatttttatcttttatttttgtttgttttttttgagatggagtcttgctctgtcaccaggcaggagtgcagtgatgcaaatctcggctcactctagccaccgactccctggttcaagcgattctcctgcctgagccttctgagtagctgggattacaggcaggcaccaccacgcccagctaatttttgtagagacaggatttcaccgtgttggccaggatggtctccatctcctgacctcatgatctgcctgcttcggcctcccaaagtgctgggattacaggtgggagccactacgcctggcccacatagctcatttttagactcacttccattaagtcttgtttggacccacgaacattgtctttttttttttaagatggagtttcacttttgttgcccagactgtagtgcaatggtgcaatctcagctcactgcaatctctgcctcctgggttctagcaattctcctgcctcagcctcccgagtagctggaattacaggcgcccgccaccacgcccagctaatttttgtgtttttagtagagacggggtttcaccatgttgggcaggccaggggtgatccgcccacctcagcctcccaaagtgctgggattacaggtgtgagccaccgcatctggccaacatgtcttttttttttttttcctttttaaccacaaagagacttaagcagtccttgtcacagatgatgaattgatgttgcaagtattgtcttagcttggattaattttcttgcttactgtaattttagataatatagctttgtaattagagattttatgtgtaaaccacaaaaatgtttacatgaaggccattattacagatgtgacgtgcataattattagtaatttgtatgtttacatgggtcagtctggcaaaaaattatgaagttttaaaaattaaaaaaaattataatgccagttttactggaaagtaaaattatttcagtaatcgattatagcaaaagtattgattttcattccagacaaaagtcagaatgaaaggtaatttctcaatactctttcagattaataaaagtacctgtagcgatttttatcattcacaagtatatcacaagtaagttagaatttgagaactgtgttctagatctctgaggagatgcagtcagatttctgaactgtctcagcaaatggtaagtaacttagagctagtaattaataacctgtcctttgatttctgattcagccaagaatggccatatttgggaaaggcagatctggagagtaaccacgttttcattcatttaccacttctaggcccctccagagctctcagatattttggggttgagcccttccccaaagccatacaggaccttttttttgtgatctgttctagccatttttatgttgggtgcttgttatggactgagcatttatgtcctcccacaccccccccataccttttttgaagtcctaacccccagtgtgatggtatttggagacagggcctttggaaggtaattacagttagaagaagtcgggagggttgggcccaggtctgattggattagtgcccttatatgaaaagacaccaggacgggcgcagtggctcacacctgtaatcccagcactttgggaggccaaggtgggtggatcacgaggtcaggagtttgagaccagcctggccaatgtagtgaaacaccatctctactaaaaatacaaaaattagctgggtgtggtagcgggctcctgtcatccaagctactcgggagggtgaggcatgagaatcacttgaacccgggagttggaggttgcagtgagcccagattgtgccactgtactccagcctgggtgacagagtgagactctgtctcaaaaaagaaaaaaaaaaaaaaagagacaccagagagcttgttagaagaggtcatgtgagcacacagttagaagaccttcaagccaaagaagaggcctgagattgaaacctaccttgcaggtaccttaattttggacttcccagcctccaaaactgtgagaaataagtttctgttaagtcactcagtctgtggtattttgttatggcagcctgagcaggtagttgttctttcagaaggtgttgataataaccacatgcaacaccaagtcacaaataataaaacagatgtaacttatattcatacagaaagttgggcactgccattgccttgttggtttacacggctgtgctagttcagtagcagaaaggtgctggtctcctttactcagtttacaatctaggcagtagaatgtaatcactgctttaaacttgatactgcttagggagagaatcattggtgctgggtaactttgggttctaggtttactttttgtgtatatataactgtttttggtaaatcacaagtttctgggcttgtcgaattagattttgttacagattatgagctttattatgctatacagttagttgtatgtatatatgcctttcccactagattttaagctttttttttttttttttttttgtgacggagtcttgctcttgtcgcccaggctgaagtggagtgcagtggcacaatctcggctcactgcagcctccacctcctaggttcaagcgattctcctgcctcggcctcccaagtaactgggactacaggcacgtgccaccacacccggctaatttttgtattttttgtagagacagggtttcgccatgttggctaggctggtcttgaacttctggcctcaggtgatccacccgcctcagcctcccaaagtgctgggatttacaggcatgagccaccacgcccagctatagctctttaagggttgtaaatttataatcattcttttactctcctgcaaattctgttgcacactgccttaatcaaggtagatgctgaatgcatttttgtataattgaatatgttgcaatccccaactctctccaactgttcctgtcaaagcagccactggattgttaactaatccatattagatggggttaattaatatcagatgggacaagtaagggctaataagattataggccaccaagtagatttctgtctagctcttatagagattgagtttattggacctgtttgataggaagttttggtgtttgggatgattaaaactgaagttcctatttattgaattatacctatttatattatttcatatcagtggtccacatgcaagtgaggcttctgagacagagtttgagttctctcttcaactaccataacacttaacctgtatctttttttttttttttttttttagacaggagtctcgctctgtcactcaggctggagtgtagtggtatgatctcggctcactgtaacctctgcctcctggattcaagcagttctccatgtctcagcctccctagtagctgggattacaggcctgtgccaccatgcctggctaattttttttttgtatttttagtagagacggggttttaccacgttggccaggctggtctcgaactcttgacctcgagcgatcaacttgccttggcctcccaaagtgctgggattacaggcatgagccacagcgcccagccgtctttttttttaaatagcaatttaacactgttcacagttactcatgtacatgtcatgccatctattacactgtaagttctgtgagggtagctgtatcaaatttatctaactctctctagtatgcatgacatagtaagtattcaataaatatttgcatattagtgataaggatacaggttctgaatagtgggtccttaccatttaagaattagtatttgatggccgggcggggtggctcacgcctgtaatcccagcactttgggaggctgaggcgggcggatcatgagatcaggagatcgagaccatcctggctaacatggtgaaatcccgtctttacaaaaaaaatacaaaagaattaaccaagtgtggtggtgggtgcctgtagtcccagctactgctttgtgaggctgaggcaggcagatcacctgaggtgggaaattcaagaccagcctgaccaacatggagaaaccccatctctactaaaaatacaaaattagccgggcgtggtggcgcatgtctgtaatcccagctactcgggaggctgaggcaggagaatggcgtgaacccgggaggcggagcttgcagtgagccaggatcgcgccactgcactccagcctgggcgacagagcgagactccgtctcaaaaaaaaaaaaaaaaaaaaaattagtatttgatatttgatcattaaatatgaattaagaggacttagactttttgttaaatgtcaagctgggaaaagttgtcatttaaatgaattgcctcttatttaatttcgtctgatgatacattttgtttttattttgtaaaaaattattttttttctttttggagacagggtcttgctctgttgcccaggctggtcacaaactcctgacctcaagcaatcctcctgccttagcctcccaaaatgctgggattacaggcgtgacgacctcgcccggccttgtattatgatacattttgaacaactacaagtagacttggtataatgaacctgcacgtacccattgccaagttctgacaactgtctgtctatagccaattatgcatttcttaaattagaacccccccaatatacccaaatatatatatatgtgtgcatatatatagtaagttgtaacaaagttgtgaattcatacctgaagtatctcaagtgatgcaagttttatgaatttttgtttatgccttttgggaagagttgtattgacaaattttttatgcttaaagtaaaccataaatcaaaaaaataaaatctaggatgcaataaaacaaaacaacttcttgacataagtatggtatgtaaatctgttttgattggaaatcaatttgttatattgccagaattcctgttttagaatacatctctgctgatctgtctgtattcttagactgcatatctgggatgaactctgggcagaattcacatgggcttcctttgaaataaacaagacttttcaaattcttagtcgatctgcagaacctgtagccaggcactgaaccattttgatagatgcagtaatcgttgcaagtgtatatttcaagggagttctggctgggtcctagtttatgcttgtggcagaagcagtgagtaactgggaggaagttggtgagtaagcttcaaggaagaagtcatttttagtactctggatcttcctgattttaaagcactacaaaatggtgcattttcattcttgtcaagtgataacagatatattctgatgagcctgaaatgaatatatattgtatcatttttataatatctagcaaggtttgtattttcctagaacttgaactaaatttcagttcataaaatttataaaatacttagttgttgtaaaatatttttggaatgttcacataggtgacacacaaatgtcccattttcattctttctatagtaaatatgttctgatatgtgaaggtttagcagatgcatcagcatttaatcctagaggatctggcataatcttttcccccaagaatagaaattttttctgcttatgaaagtagtacatgtttctttaaaaacaaatcaatattgacttctgcctgctgtatagcactatgcctccacctggccatgaccaggggcatgtcctggtccacctacctgaaaatgtttgcaaccagcctcctggccatgtgcacaggggctgaagttgtcccacaggtattacgggccaacctgacaatacatgaagttccaccaaagtctgagaactcagaactgagctttggggactgaaagacagcacaaacctcaaatttctcagcactggaaacctcaaaatataactgaattccataaataagattttaagtcttaaatatgtatttttaaatgtattaaaagtcaagctgcttgtatttaagcacctaatacaatgcttaggttgtaaaaggagatgctcaataggtactaactgatatattgagatttaattatggtttgaccaatatttattggaaaccgccaaagcttaaatcatcagcttcttgaatgtgatttgaaaggtaatttagtattgaatagcatgtgagctagagtatttcattctttctggtttatttcttcaaatagactttgaatataatggtgaatgggtattataaattaactaataaaaatgacattgaaaatgaaaaaatatatatattaaagtgtagaaagtgaccaggcgtggtggctcacacctgtaatccaagcaccttgggaggctgaggcaggaggatctcttgatcccaggagttcaagaccagcctgggcaacatagcgagacttcgtctctaaaaaaaaaaaagagagagaaaaaaattttttttatttaaaaaaagtgtagaaagtgtcaagaccccacttcttaccattatttggtatatttctctatacccacccacccttcctccttactccctccctcccttcccaatctttttatctttttgtattctgattttttgtttgtatattttgctttaatttaatgtatcctttaaaaatttcccatacattttatatgtatatataaaaacgcatgctgccaaagataatttataagaaagaccattgaatttttttaaaagtgatatatattcattgaaaaaaatttagaatatatagcaaagcaataaagaactaaataaaattgctgtaactcctctttcaaagataagtgcttttatgattttgttgtatttttttctgtatataggtacatatatagtatttataaagctgtactcatagtacattttcacatcacaggtaccatatcagtgttattaaatattttgtatgccaggggctagacataccaagacaaccaatatgtggttctacttaaataatattagagtatcttttatgatgacacttcatgagttgactataataatcttagacttctaagagtttgggttttcaaaagatcacttagcttttttgggtgatttttcccccttactgtgagatgagagaggctgtttggatttgggattggggtagcggggacagcaacttttcttttctttttcttttttattttgaggtagggtattgctgtgtcacccaggctggagtgcagtggtgtgatctcggctcactgcaacctccacctcccgggctcaggtgatcctcctgcttcagcctcccagtaactgggactacaggcgcgtgccacatgcctggctaattttgtatttttagtagagatggggtttcaccatgttggccaggctggtctctaactcctgacctcaggtgatacgcccacctgggcctcccaaaatactgggattacaggcatgagccgctgcatcagccagcagtttttcttgtggttttttttgtttgttttgttttgttttgtttttgagatagggtcttactctgttgtccacgctggagtgctgtggtatgatcgtagctcactgcagcctcaaactcctgggctcaagtgattccttctgcctccgcctcccgagtagctgggactacaggtatgcaccaccatacctggcaaatttttacaaagttttttgtagggacggggtcttgctacattccccatgtcggtcttgaactcctggcctcaagcaactctcctgtctcagcctcccaaagcactgggattacaagtgtgagccaccacaccatgccagtttttcctgttcagtgtgatattttatcttgttagactacagtgtgttaaaacttgttttactaaattttcaaacatactcaaaagtggagagaatagtataatgaatacccgtatgttcatcacccatgtttagaatattattaaatataaagattttgctgcgtttgtcttagctctttaaaatttttctttttctctttgtgacctaaaggaaattccatatcttatcactttacttctacattcttgactaagatgactaagacatatagttacatggttttttgttttgtttttgttttttaaagacgaaatctcgctcttgtcccccaggctggagtgcaatggtgccatctcagctcagtgcaacctctgccttctgggtacaagcgattctcctgcctcagcctcccaagtagctgggattacaggctcctgccaccacgcctggctaatttttgtatttttagtagagacggcggggggaggtttcaccatgttgacaaggctggtctggaactcctgacctcaggtgatccacccgcctcggcctcccaaagtgctgggattacaggcgtgagccaccgcgcccagcctgtttttttgtttgtgtgttttgttttttttgagacagagtcttgctctgtttcccaggctggagtgaagtggtgccatctcagctcagagacagagtcttgctctgtttcccaggctggagtgaagtggtgccatcttggctcactgcaaccttcacctcccaggttcaagtgattctcctgcctcagcctcccaagtagctgggactacaggcatgtgtcaccacacccggctaatttttttgtatttttagtagagacgggatttcaccgtgttgcccaggctggtctcgaactcctgagctcaggcagtctgcctgcctcagcctcccaaagtgctgggattacacgtgtgaaccaacccgcccggcctgttgttttcttacataattcattatcatacctacaaagttaacagttactaatatcatcttacacctaaatttctctgatagactaaggttattttttaacatcttaatccaatcaaatgtttgtatcctgtaatgctctcattgaaacagctatatttctttttcagattagtgatgatgaaccaggttatgaccttgatttattttgcatacctaatcattatgctgaggatttggaaagggtgtttattcctcatggactaattatggacaggtaagtaagatcttaaaatgaggttttttactttttcttgtgttaatttcaaacatcagcagctgttctgagtacttgctatttgaacataaactaggccaacttattaaataactgatgctttctaaaatcttctttattaaaaataaaagaggagggccttactaattacttagtatcagttgtggtatagtgggactctgtagggaccagaacaaagtaaacattgaagggagatggaagaaggaactctagccagagtcttgcatttctcagtcctaaacagggtaatggactggggctgaatcacatgaaggcaaggtcagatttttattattatgcacatctagcttgaaaattttctgttaagtcaattacagtgaaaaaccttacctggtattgaatgcttgcattgtatgtctggctattctgtgtttttattttaaaattataatatcaaaatatttgtgttataaaatattctaactatggaggccataaacaagaagactaaagttctctcctttcagccttctgtacacatttcttctcaagcactggcctatgcatgtatactatatgcaaaagtacatatatacatttatattttaacgtatgagtatagttttaaatgttattggacacttttaatattagtgtgtctagagctatctaatatattttaaaggttgcatagcattctgtcttatggagataccataactgatttaaccagtccactattgatagacactattttgttcttaccgactgtactagaagaaacattcttttacatgtttggtacttgttcagctttattcaagtggaatttctgggtcaaggggaaagagtttattgaatattttggtattgccaaattttcctctaagaagttgaatcattttatactcctgatgttatatgagagtacctttctcttcacaatttgtctcttttttttttttttttgagacaaggtctctgttgcccaggctggggtgcagtgcagcagaatgatcacagttcactgcagtctcaacctcctgggttcaagcgatccttccacctcagcctcctgagtagctgggactataggtgtgcgccaccactcccagctaatatttttattttgtagaaacagggttcgccatgttacccagcctcccaaagtgctgggattacaggcatgagccactggcccagtttctacagtctctcttaatattgtatattatccagaaaatttcatttaatcagaacctgccagtctgataggtgaaaatggtatcttgtttttatttgcatttaaaaaaaattatgatagtggtatgcttggtttttttgaaggtatcaaattttttaccttatgaaacatgagggcaaaggatgtgatacgtggaagatttaaaaaaaatttttaatgcatttttttgagacaaggtcttgctctattgtccaggctggagtgcagtggcacaatcacagttcactccagcctcaacatcctgcactaaagtgattttcccacctcacctctcaagtagctgggactacaggtacatgctaccatgcctggctaatttttttttttttgcaggcatggggtctcactatattgcccaggttggtgtggaagtttaatgactaagaggtgtttgttataaagtttaatgtatgaaactttctattaaattcctgattttatttctgtaggactgaacgtcttgctcgagatgtgatgaaggagatgggaggccatcacattgtagccctctgtgtgctcaaggggggctataaattctttgctgacctgctggattacatcaaagcactgaatagaaatagtgatagatccattcctatgactgtagattttatcagactgaagagctattgtgtgagtatatttaatatatgattctttttagtggcaacagtaggttttcttatattttctttgaatctctgcaaaccatacttgctttcatttcacttggttacagtgagatttttctaacatattcactagtactttacatcaaagccaatactgtttttttaaaactagtcaccttggaggatatatacttattttacaggtgtgtgtggttttttaaataaactccttttaggaattgctgttgggacttgggatacttttttcactatacatactggtgacagataccctctcttgagctacatcggtttgtggggagtcaaaagtcctttggagctaggtttgacaaataaggtgggttaacacttgtttcctagaaagcacatggagagctagagtattggcgaattgaagaaatccccctttttttttaacacacttaagaaaggggactgcaggtatactcaagagagtaagtcgcaccagaaaccacttttgatccacagtctgcctgtgtcacacaattgaaatgcatcacaacattgacactgtggatgaaacaaaatcagtgtgaattttagtagtgaatttcattcataatttgatcgtgcaaacgtttgatttttattactttagactattgtttctgattttatgttgggttggtatttcctgtgagttactgttttacctttaaaataggaatttttcatactcttcaaagattagaacaaatgtccagtttttgctgtttcatgaatgagtcctgtccatctttgtagaaactcgccttatgttcacatttttattgagaataagaccacttatctacatttaactatcaacctcatcctctccattaatcatctattttagtgacccaagtttttgaccttttccatgtttacatcaatcctgtaggtgattgggcagccatttaagtattattatagacattttcactatcccattaaaaccctttatgcccatacatcataacactacttcctacccataagctccttttaacttgttaaagtcttgcttgaattaaagacttgtttacggtatcgataagcttgatatcaaaacgccaactttgacccggaacgcggaaaacacctgagaaaaacacctgggcgagtctccacgtaaacggtcaaagtccccgcggccctagacaaatattacgcgctatgagtaacacaaaattattcagatttcacttcctcttattcagttttcccgcgaaaatggccaaatcttactcggttacgcccaaatttactacaacatccgcctaaaaccgcgcgaaaattgtcacttcctgtgtacaccggcgcacaccaaaaacgtcacttttgccacatccgtcgcttacatgtgttccgccacacttgcaacatcacacttccgccacactactacgtcacccgccccgttcccacgccccgcgccacgtcacaaactccaccccctcattatcatattggcttcaatccaaaataaggtatattattgatgatgttt

SEQ ID NO: 125 - DNA, 30122 bp, synthetic construct
  source 1..30122: mol_type = other DNA
aaacatcatcaataatataccttattttggattgaagccaatatgataatgagggggtggagtttgtgacgtggcgcggggcgtgggaacggggcgggtgacgtaggttttagggcggagtgatgccccccctcgaggttcgacggtatcgataagcttgatttaattaaggccggcccctaggggcgcgccgtcgacgcgacaactgtcttattaccctgttatccctaccttaattaacatttccataccacatttgtagaggttttacttgctttaaaaaacctcccacacctccccctgaacctgaaacataaaatgaatgcaattgttgttgttaacttgtttattgcagcttataatggttacaaataaagcaatagcatcacaaatttcacaaataaagcatttttttcactgcattctagttgtggtttgtccaaactcatcaatgtatcttatcatgtctggccagctagctagtcaagcgtaatcaggcacatcgtatggatagccggcataatctggcacgtcataagggtagccggcgtagtcgggcacatcataggggtagctgccccctccgcccttgccggggctcaggctcagggacttctgggtgtagtggttgtgcagggcctcgtgcatcacgctgcagctgaacacgttgccctgctgccaccggctcttgtccacggtcagcttggagtacaggaagaatgagccgtcgctgtccagcacagggggggtggtcttgtagttgttctcgggctggccgttgctctcccattccacggcgatatcgctggggtagaagcctttcaccaggcaggtcagggacacctggttcttggtcagctcgtcccggctggggggcagtgtgtacacctggggctcgcggggctggcccttggccttgctgatggttttctcgatgggggcaggcagagccttgttggacaccttgcacttgtactctttgccgttcagccagtcctggtgcagcacggtcagcacggacaccacccggtaggtgctgttgtactgttcctctctgggcttggtcttggcgttgtgcacttccacgccgtccacgtaccaattaaacttcacttcagggtcctcgtgggacacgtccaccaccacgcaggtcacttcgggggtccggctgatcatcagggtgtccttgggctttggggggaacaggaacacgctaggtccgcccagcagctcaggggcagggcaggggggacaggtgtgggtcttgtcgcagctcttggcctctctcttgatttccaccttggtgccctgtccgaaggtggcggggtggtacaggtactgctggcagtagtaggtggcgaagtcttcgggctgcagggagctgatggtcagggtgaagtcggtgccggagccgctgccgctgaatctgctgggcacgccgctgtacaggaagctggcgctgtagatcagcagcttgggggccttgccgggcttctgctgataccaagccacggcggtggacacgtcctggctggcccgacaggtgatggtcactctgtcgcccacgctggcgctcaggctgctggggctctgggtcatctggatgtcgctgcctccgccgcctgatcctccccctccggatccgcctccgccagcagacacagtcaccagtgtgccctggccccagtaatcgaagccgccaggccagtgccttctggcgcagtagtacacagcggtgtcctcggcccgcaggctgttcatctgcaggtaggcggtgttcttgctggtgtcggcgctgatggtgaaccggcccttcacgctgtcggcgtagtaggtgctgccgccgtaggggctgatccaggccacccattccagtcccttgccaggggcctggcgcacccagtggatccagctgtcgctgaaggtgaagccgctggcggcgcaagacagtctcaggctgccgccaggctgcaccagtccgccgccagattccaccagctgcacctcagagtgggcgcctgtggcggctccgaccaggaacaggatccgccagatccagtccatggtgccggcgctgaggacagtgctcagcggtccttcggcagtctccgggcccagcaacaggcttgtagtcccggagcgcgacggcgttccgaccgatctgagggcgacaggagcccccgatcaggcggagccacgagacgggctccgagttggcctggaaagggcaggccgcggcgcttacctctcggccccgcagaggcagacgctcccgtcgctgtggtctcggcccgtgtggagcgcgccgccgccgactcggcttatataccctccccccagccccgtcgtggaggcctccgattggcgaaggcgctcctcgttggaggacgctgattggtccatgccaccaagctggccgctgccgattcgaagcggcctcctccgcaacttacgtcactgctacgccccccgggctgactcattggctcttggtcactctcaacggccgccaatgaggggcagcatccgccctgtgcgccggtcctattggttcagcagctgcctgtccctcgggtgacctctcaacccgagaccgtttccgccggtaactagtcaaaacaaactcccattgacgtcaatggggtggagacttggaaatccccgtgagtcaaaccgctatccacgcccattgatgtactgccaaaaccgcatcatcatggtaatagcgatgactaatacgtagatgtactgccaagtaggaaagtcccataaggtcatgtactgggcataatgccaggcgggccatttaccgtcattgacgtcaatagggggcgtacttggcatatgatacacttgatgtactgccaagtgggcagtttaccgtaaatactccacccattgacgtcaatggaaagtccctattggcgttactatgggaacatacgtcattattgacgtcaatgggcgggggtcgttgggcggtcagccaggcgggccatttaccgtaagttatgtaacgcctgcaggcagctttctatgcaacccaaggactcagtttttggcctgttttagtgacaggcaatcagcaacatgctgcatttctctccagtgttgtaatcaaagaaaccctcccatagctttaaatgatattccttccccttccaattatgtggggggaaaacaaccctattctccacccagaagtgttaactcaagaattacattttcaagaagtttccagattcgtaaaaccagaattagatgtctttcacctaaatgtctcggtgttgaccaaaggaacacacaggtttctcatttaacttttttaatgggtctcaaaattctgtgacaaatttttggtcaagttgtttccattaaaaagtactgattttaaaaactaataacttaaaactgccacacgcaaaaaagaaaaccaaagtggtccacaaaacattctcctttccttctgaaggttttacgatgcattgttatcattaaccagtcttttactactaaacttaaatggccaattgaaacaaacagttctgagaccgttcttccaccactgattaagagtggggtggcaggtattagggataatcctaggttaggaagcattcagatagctcatcactctatcaatagtcactgcccgaattctgaaagcatgaagaagtatgcagagcttgattttagttttataaaaatccggttcttcaagggaggatttttgtggcacagtctcactgttgaaattcagggcctgcatcagctcatcaataactgccagcatgttttgatctagaaagatctgcctcttaggatccatcagcagctttgcattcatggtcttgaactccacctggtacatcttcaagtcttcataaatactactaaggcacagggccatcataaaagaggtctttctggaggccaggcaactcccattagttatgaaagaggtctctctggaatttaggcaactctcattcttggttaattccaatggtaaacaggcctccactgtgctggttttatcttttgtgatatcttcatgatcaatctcttcagaagtgcaagggtaaaattctagagtttgtctggccttctggagcatgttgctgacggccctcagcaggttttgggagtggtgaaggcatgggaacattcctgggtctggagtggccacggggaggtttctggcgcccaccccaggtacccctactccaggaacactgcagggcacagatgcccattcgctccaagatgagctatagtagcggtcctgggcccgcacgctaatgctggcatttttgcggcagatgaccgtggctgaggtcttgtccgtgaagactctatctttcttttctctcttgctcttgccctggacctgaacgcagaatgtcagggagaagtaggaatgtggagtactccaggtgtcagggtactcccagctgacctccacctgccgagaattctttaatggcttcagctgcaagttcttgggtgggtcaggtttgatgatgtccctgatgaagaagctgctggtgtagttttcatacttgagcttgtgaacggcatccaccatgacctcaatgggcagactctcctcagcagctgggcaggcactgtcctcctggcactccactgagtactcatactccttgttgtcccctctgactctctctgcagagagtgtagcagctccgcacgtcaccccttgggggtcagaagagcctctgctgcttttgacactgaatgtcaaatcagtactgattgtcgtcagccaccagcaggtgaaacgtccagaataattcttggcctcgcatcttagaaaggtcttatttttgggttctttctggtcctttaaaatatcagtggaccaaattccatcttcctttttgtgaagcagcaggagcgaatggcttagaacctcgcctcctttgtgacaggtgtactggccagcatctccaaactctttgacttggatggtcagggttttgccagagcctaagacctcactgctctggtccaaggtccaggtgataccatcttcttcaggggtgtcacaggtgaggaccaccatttctccaggggcatccggataccaatccaattctacgacataaacatctttcttcagttcccatatggccacgaggggagatgccagaaaaaccagggaaaaccaagagatgaccaactgctggtgacccatggtaagctttctagattcatgacgtgcgaccggtgagtctcaagtccccttcgatcgcaggagccgcctccaccccccacccctgggttcggatcctcacacctccagccgcgcggtccgcccactacaccccaagcaggtcgggccgcttttcacccccacttctcgcgggcgggggacgggaaacatgaacccaccaatcgcgccgcaccacgcacccacggcacccaatgaggattcgtgagggggggcggaagtccaccaatcggagctgtccaggtgcggtgaccgatgcccgaagcgtggctccttccgattggtcagggtttgcagcttttctccaatcaaatggctccgcgggcccctcacgcgtgggaccgcccctttgcctgggcggccttggcctctaagggaaaacgtccaatgaatgtaagcagagaacacatccatccttttagagaggtcgcggcggaactacttccggatcctagagagcgtttattccgtgaccggggaaacggtagccatgacaacgtgttcttcaccctttcccatctatgcctggggtttcgttggaagtgattccagcacgactttcgcggccagctttctcgtgtggcggcgcttctcggaaagaagaaacacacgagagaggttgcaaatcccctagaaccctttcagatggcgggggggcgggggggtggcggtggtgatgaaactagtgggactatggttgctgactaattgagatgcatgctttgcatacttctgcctgctggggagcctggggactttccacacctggttgctgactaattgagatgcatgctttgcatacttctgcctgctggggagcctggggactttccacaccctaactgacacacattccacagctggttctttcagcctcagaaggtacctaaccaagttcctctttcagaggttatttcaggccctgcaggttaattaagctagccgacgcgttggccaggagctcagatctccggatccaagcttatcgatttcgaacccaaatggatctaccacatttgtagaggttttacttgctttaaaaaacctcccacacctccccctgaacctgaaacataaaatgaatgcaattgttgttgttaacttgtttattgcagcttataatggttacaaataaagcaatagcatcacaaatttcacaaataaagcaatagcatcacaaatttcacaaataaagcatttttttcactgcattctagttgtggtttgtccaaactcatcaatgtatcttatcatgtcgagctagctagtcaggacttcagttccagctttgtgccggctccgaaggtcagcgggttgctagaccattgctgacagtaatatgtggcggcatcctcggcttccatagagctgattgtcaggctgtagctggtgccagatccagatccgctgaatctgtagggcacgccggaggccactttgcttgtgtcgtagatccaccgcttggggcttgtgccagacttctgctgataccagttcatgtaggacacgctgctgctggctctgcatgtcatggtcactttctcgcctggggaagcgctcatgatggcggggctttgtgtcagctgaatatcggagccaccaccaccgcttccaccaccacctgaaccgcctccgccactagaaactgtcagggttgtgccctggccccagtaatccagacagtagtggtcgtcgtagtaccgggcacaatagtacacagcgctatcttcagaggtcaggctggacagctgcatgtaggcggtagagctgctcttgtcggtggtcagtgtggccttgtccttgaacttctggttgtaattggtgtagccccggctggggttgatgtagccgatccattccagtccttggccaggcctctgcttgacccagtgcatggtgtaccgggtgaatgtgtagccgctggtcttgcaggacatcttcacagaggcgccaggtctagccagttcggcgccagactgttgcagcttgatatcggatccgccacctccgccagatgacactgtgaccagtgttcctctgccccagtagtcgaggccctgtctggcgcaataatacacggcggtgtcctcggctctcagggagttcatctgcaggtacaggctgttcttggcgttgtcccggctgatggtgaatctgcccttgatgctgtccaggtagtaggtgtagctgccgccgctgctgattgtggacacccattcaaggcctttgccaggagcctgtcggacccagctcatatcgtagctgctgaaggtgaagccggaagcggcacagctcagtctcagagagccgccaggtttcacaagtccgccgcctgattccaccagctgcacttcagatccaccaccgccactacctccgcctccgcttcctccgccgccagatcctccgccacctctcttgatttccaccttggtgcctccgccaaatgtcaggggattgctggaccactgcaggcagtagtacacggcgaagtcctcaggttccaggctgcttatggtcagggtgaaatcggtgccgctgccagagccagaaaatctggcaggcactccgctggccagattgctggtcaggtagatcaggattctaggggcctgtccgggcttctgctgcagccagtagatgtagttgatggagctgctggcgctacagctcagggtagctctctcgccagggctcagagacagtgtggctggagactgtgtcagcacgatctcgccggtggtatcaggcagccaaagcagcagcaggaacagcagctgagcaggggcttccatggtggccctccttcgccggtgatctcagctgtaggaaagagaagaaggttagtagtcgacgtgtccctctcgatgaatctaagtatcaattgtgagcgctcacaagtcaacactctttttgataaatctagtagatatcacttacgtaggcgccggtcacagcttggatctgtaacggcgcagaacagaaaacgaaacaaagacgtagagttgagcaagcagggtcaggcaaagcgtggagagccggctgagtctaggtaggctccaagggagcgccggacaaaggcccggtctcgacctgagctttaaacttacctagacggcggacgcagttcaggaggcaccacaggcgggaggcggcagaacgcgactcaaccggcgtggatggcggcctcaggtagggcggcgggcgcgtgaaggagagatgcgagcccctcgaagcttcagctgtgttctggcggcaaacccgttgcgaaaaagaacgttcacggcgactactgcacttatatacggttctcccccaccctcgggaaaaaggcggagccagtacacgacatcactttcccagtttaccccgcgccaccttctctaggcaccggttcaattgccgacccctccccccaacttctcggggactgtgggcgatgtgcgctctgcccactgacgggcaccggagcgatcgcagatccttcgatagagaaatgttctggcacctgcacttgcactggggacagcctattttgctagtttgttttgtttcgttttgttttgatggagagcgtatgttagttacgattcacacaaaaaaccaacacacagatgtaatgaaaataaagatattttattgcggccgctcgagtctagaggtatacatgccatggtccgcggtattaccctgttatccctaagacaactgtcctgcatgcgacgtcggcgcgccatcgaattcctgcagcccgggggatccctttgttgattttttccacatagattatttttgactgttttggcactttatataaatggaatcatatagtaaatatatacatgtatatatgtatatatacactatatatgtatatatatagtgtatatatatacatgtatatatgtatatttacatatatactgtatatatgtatatttacatatatactgtatatatgtatatatacacgtatatactgtatatatacagtatatactgtatatatatactgtatatatgtgtatatatatatacagtatatatacagtatacatatatatacatgtatatatacacagtatatatacatgtatatatacacagtatatatacatgtatatatacacagtatatatacatgtatatatacacagtatatatacactgtatatatgtatatatatactgtgtatatatatacagtatatatacagtatatatatacatgtatatgtatatatatactgtatatatgtgtatatatacgtatatatactgtatatatatatagacacttttgtgtctggcttcttgctctcatcataaagcacttgaaatccatccatgttgtagctggtatcagtagctagtttcttttcattgctgagaagtatcactttttattgatgagtagttttacattgtatgaacatgcccgagtttgtttatgcattctactaatagacacctgggctgtttgcagtttttggctattacaaagaaaatttctatatttttttccaacttttattttaggttcagcgggtacatgggcaggtttgttacatcggtaaattgcatgtcactggggtttggtgtacagattatttcaccacccaggtaataagcatagtacctgataggcaggtttttgatcctcaccctcctccctcaagtaggccccagtgtctattgttctattccttttttttttttttgagatggagtctcactctgttgcccaggctggagtgcagtggtgcgatctcggctcactgcaaggtccacctccagggttcaagcgattctactgccgcagcctcccgagtagctgggattacaggcacccaccaccacgcccggctaatttttgtatttttagtagagactgggtttcaccatgttggccaggatggtctcgaactcctcacctcaggtgatccgcccgcttcggcctcgcaaagtactgggattacaggcgtgagccacggtgcctggcctatggttccattctttgtgtacacgtgtactcagtgtttagcttccacttgtaagtgaaaacatgcagtatttggttttctgaaattcttgtcttcatctttttgtagacaatccactacttttatttttaaatattaggaacaatagcctctgtgtgtcctgaattgcaatgttttttctctgattttgctgctcatcttgtaacctgtatggtgtttttctgtgtgcaagctttttactttacgtgggcaattttatcattcttttcttttatggtttctgggtttcatgtcatgattggagaagcttgatctaccctgatactataaaaatatccaccttggcttttttttttttttttagatggattttcactcttgttgcccaggctggagtgcaatggcgtgatctcggctcaccacaacctctgcctcccaggttcaagtgattctcctgcctcggcctcctgagtagctgggattacaggcatgcgccaccacgctcagctaattttgtatttttagtagagacaggatttcaccatgttggtcaggctggtcttgaactccccacctcaggtgatctgtctgcctcggcctcccaaagtgctgggattacaggcgtgacccaccacacctggcccacgttgttttctgatagtgttttcacgtgttattttttctgtcttactctttgaatcatctaaatgtatcttaatgtcaggagtgaggtagaggacccagttgtttggtttaaatgactagccagttttcccaacaccaggtgttgaacatccctcactgatgtgagatgctgcctttttcacagtctcaatccccatgtgcatttctatttattttccttccactttattcacatctttttcagtatccacaaccatattgttttaaatagcttcatgatatgttttaatatttggtagagctagaaccctttcttggttctttttcttttcttcttctcctccttttcctcctccttctttctcctcctccttcttctttctttttagaaatttcctggctattcttgttttgtagtcttccagataaataattttgaatcactttgtcatgttccagaaaataatactgccagaatttttattgtgatcacagaagttttacagattcatctgggggaaaaaaacccatcttcccagaatacagaaagggtgagggaaagacaaacatcaaggacaagtctcaggttctggacttggagaccaagaggatttggggcatccgggagcagggcagggaggtgtgatggctgcctttcactgagtaggaggatgcccagacttgggggaactatggaaagtttggttcagactttctgagttggagatgtctatgcgcagtccacagggcgaagccctggaggtagaggccctccttactgcctccctcattcagtctgaggtccattctccacatggacactgaagtgactcaaggcttcccttgttggatcaggatagtctccagggccctgggtggtctgggcctgcccacctccccatcccctctcctgcctgccctcctcttgctcactggaccccacccaccagcctccttctattcctcctgacatttgcacttgctgttccgtctctgcttggaacatcctagctctttgcatggcttgctccttcccatcttttaatctaagctcaaatatcactccttcagatatgcctttcccaaatatcctagctaaagagaactgctccccacttcccacaagccctagcaaactgggactctccttcttgctttctttctctctgccccttctgtgttttttccatagaccttaacttgttactgttttatttgttgatgtgtttacatcatttgtccccctgtgatggttagttttatgtgtcaacttggctaggctgtaggggctgttcgtcaatcaaacactgatctatgtgtagctgtgaagggattttgtagctgtgattaatagttgactttaagtaaggaagattatcctggagaatgtgggggaaggggcagacctcagccaatcagttgaaaggccttaagaacaaagctgagatttccccgaggaagaagaaattctgcctgtggactgcagcatcagctcctgcttgagaggttccaggctgcccttcctgacagcctgtcctatgattttggacttgccttgccaggtttttcctctttcttgaccccccaaaaccatatatatctcctgctggtttgtttctctggtgtaatcctgagggatgaacactcctccctcccagttcactctgggagaggttggggatcatgtttgtctatttccccatgcctggcccatgcgtgtttattgaatcactgaacaaccacgcattaggaagccagtcatatgtgcttcttcagaacctcatgtccattgccagatctccctggcttttgtggctagaggacaagtgagagatagtagcttacccacagaccttggccctgaggcccccaggggcctgagcctgctgtaagggaggagggagcccctgaggtctcacacacctccctggggatctggcattttcccctggggctggcctcagagctgggcgggggcagattatggagtgggttgtagagggagcacctccccactagcaatcatggttttttctgcgcctctcatagggaggcctacaggcctccaccttcagctcttcaggagccacaggcagctgagtgacttctgcatcacagtcttctcagagacaaacttgcagtaagaaagaggggcccgtgagggaccccagagaaggctgttgtcaaagcaggatgagagtgaactcttccatgggggacacccagcgtctccaagctcttttatgctgtcttcaaggggtctagagagcttcagcccaacatgagacccagtccagcagcatttccctgcgaagtgaaagttaggaccctgactagatacaccacgctgacctcagccagaatatcaagatgctgaggcgctgagatgctgggatgctaaggtgctaaggtgctggggtgctggggtgctaggatgctgaggttttgtgatactgggtcgctgagatgctgggatactggggtgctgaagtgctggggtactggggtgttgccatgctgaaatgctggggtgttgggatgctgaggtgctgggttgctgggatgctgggatagtccttggatgctgcggtgctgagatgctggtctgctggtctgctggggtgttgggatgctgggattttgggatgctggagtgctgcagtgctgcagtgctgagatgctggagtgctggggtgctggaatactgtagtactggtgtgctggagcattgagatgctagggcactgggatgctaaggtgctgagatgctgcagtgctggggtgttgggatgccgaggtgttgggatgcttaagtgctggggtgttgggatgctggggtgctggaacactatggtgctggggtgctggagtgttgagatactgtagtggtgggatgcttaagtgctggggtgctgggtgttgggatgcctaggtgctggggtgccgagatgctggagtactagtgtgctgggatgctgaagtgctggggtcctgagatgctgcagtgctagggtgctgagattctgggctgctggagtgttggggtgctgggatgctggagtgctgagatgcttggacaatggggtgctggaatactatggtgctggggtgctggggtattgagatgctagggtactgggatgctgaagtgctgagatcctggagtgctgggctgctgggccacaggctcttgaatccattcgtctgcccaggggaagaaaccagaagataaagagctaatgaaggagctttggttgagagggaggaagtaatggaaggagcaacatcttgtggaggagcaggagagaatggacctcaggttgggagagagggccaggctacaggccagagaggcagaaggattccagcagagtgtgggctccaggagccaaggggaaacaggtttctgggaggagagagtccagtactgctgaagtggcaagtccgctgaggaccaggaagcttcatttggctttatgaccaggaggaatttggaactgtgactagagtacttagggggaaggaggcaagactggagccagattgctctgggttgaggggtgagtgggaggtgaagcagggcactgtcactcctttgaagggtggcagagagctggaattggtgctggatgggctgtggggtgacagggtcatgtggaaagcccctggggggcacctggaaaaggagaagctgacagtacagtgagaggacagctaagggaaagcggaatggcagaacacgcactgccaggaggaatgaggatagggtcaggagtgccaggggcagtgaggccagcctggggtcaggtggcaggacgtgtccaggaagctggtctgcactgcagcccacactggctcagccttgaggttccctgtgtggttggggtaggaagttgaaccctctgggaatggaagatggaaccagctctgcgagccaagctcagcttttatctatgggtctctgagggctggcagagctgagtggggacaactgtgatccgtgaggctctcaggttgaggtggcccctccgggagggcttcattttcccagcgggtaggttctaagcagcagtggctgggcaggtgggtccaacacagagccagagaagggtgaatgggcctcctggcaccccacccctgctgcccctgagctcagtgatggagggggacagcacagctgagcccaagtgctttggtgtggccctgagggaaagctgcagcctgcctggggcctggcatggatgggacacttgaggcagagggacaatagtgggcgctgcagtgaggctggctcttggagaggtttcctgaggagtgctgcctgagacgggcagggagaacagagacaaagttggtgacagggaatgaaagctgactgaaggactttacccagacctatgaggatatctctctcagcaggaagcaggaggggactgtgtgaggactggccaagagctggagtgttgggaaaatgactctttctccgacccctctgtcctagctctggcccctggactgcggaggtctgcttccacccccattggtcgatcgttgtcccttgtcacagccattgagaattttggcagggagcatgttcttagagcatttttaggctctgcgggacataacagctctgcctcagagcacatgcctttctcagctcctgaaagccactgatcaaattggaacattttgtaccttagggatgaggatatcaactctcccagccacttagagggataaatgtgatgatgcattcaattgtgactacatctgatcccaactgttgcttcagctgctctcctatagcacatggcgggaggcgtgcatcccagtagctacctccccacttttggggagatgtggttccatccatgaaacctgggtacccgcctaccaggtcctggcctatcaggtggcagggtctggtcaaagaagggcatgtgtggtcttcagcaagggagacaggacggtggtgcagagcgtctagaccctcagggcaagtctcccccacacctgctcccggggcagttgtctttgtgacctcccatccccctctgtttcatcctctataaaatgaggggctgagccccaaaataacaggcttctttgccatgatgcaaaactgctgaatctttctttctgacacacaaggcatcgagcagcctctgaaagaaccaaagccactagcaggcttcctgacttgggtttgtaggtactgaatactcccttgaaaaataaaaacatagaggcacttttctcctggctgtttattacagaacgaagaaaaaacacactggcttgaaacagacgccagatttcaaatgtagaggtgaaatacgaggtggcaattaaaatgtgattacagaaagtctggacactgagaaaagtttacaggacagtgggtgtgggttttctataacagacacttaaatatacatgacgataattgcagatagaaaccatcaaagacaaaccccaaatcaactaataatgtttacagatgttcccccccaaaccacagagccttacatcaaaacaaatactgaaaggctttaaaccaggaacagctcgccttaaccccacgagggtgcacacaagctgggctttttctctcggtctgaatggtaaagggaggaggatactctagctcctccaggtggattgctgagacagggctcggctcacacactgtctctgcgcctctcccaaatctggagaactctcccagcctcctggtaaagtgtctctgtggggcacttaacgataaaacagcttctgctgtaaagctcattaggaaagagctagcctgcaacctccacggagtgggaactacatcaggcattttgctaactgctgtatcctaggccaataaatgttgatcacatttatagctgccatggtagggtggggacccctgctatctatctgtggaggctctgggagcccctgacacaaactttctgaagcagagcctccccaaccccttttccattccctatacctgacagatggcccaggaacccattagaaatggaaggtcactgcagcagtatgtgaatgtgcgtgtgggagaagggcaggatcagagccctgggggtgtggcagcccccaagtgattctaatccagatcctagggttgtttccctgtcccattgaaatagctgctttaaggggcctgactcagggaaatcagtctcttgaattaagtggtgattttggagtcatttagaccaggccttcaattgggatccactagttctagagcggccgggcccagggaaccccgcaggcgggggcggccagtttcccgggttcggctttacgtcacgcgagggcggcagggaggacggaatggcggggtttggggtgggtccctcctcgggggagccctgggaaaagaggactgcgtgtgggaagagaaggtggaaatggcgttttggttgacatgtgccgcctgcgagcgtgctgcggggaggggccgagggcagattcgggaatgatggcgcggggtgggggcgtgggggctttctcgggagaggcccttccctggaagtttggggtgcgatggtgaggttctcggggcacctctggaggggcctcggcacggaaagcgaccacctgggagggcgtgtggggaccaggttttgcctttagttttgcacacactgtagttcatctttatggagatgctcatggcctcattgaagccccactacagctctggtagcggtaaccatgcgtatttgacacacgaaggaactagggaaaaggcattaggtcatttcaagccgaaattcacatgtgctagaatccagattccatgctgaccgatgccccaggatatagaaaatgagaatctggtccttaccttcaagaacattcttaaccgtaatcagcctctggtatcttagctccaccctcactggttttttcttgtttgttgaaccggccaagctgctggcctccctcctcaaccgttctgatcatgcttgctaaaatagtcaaaaccccggccagttaaatatgctttagcctgctttattatgattatttttgttgttttggcaatgacctggttacctgttgtttctcccactaaaactttttaagggcaggaatcaccgccgtaactctagcacttagcacagtacttggcttgtaagaggtcctcgatgatggtttgttgaatgaatacattaaataattaaccacttgaaccctaagaaagaagcgattctatttcatattaggcattgtaatgacttaaggtaaagagcagtgctattaacggagtctaactgggaatccagcttgtttgggctatttactagttgtgtggctgtgggcaacttacttcacctctctgggcttaagtcattttatgtatatctgaggtgctggctacctcttggagttattgagaggattataagacagtctatgtgaatcagcaacccttgcatggcccctggcggggaacagtaataatagccatcatcatgtttacttacatagtcctaattagtcttcaaaacagccctgtagcaatggtatgattattaccattttacagatgaggaacctttgaagcctcagagaggctaacagacataccctaggtcatacagttattaagagaaggagctctgtctcgaacctagctctctctctctcgagtaataccagttaaaaaataggctacaaataggtactcaaaaaaatggtagtggctgttgtttttattcagttgctgaggaaaaaatgttgatttttcatctctaaacatcaacttacttaattctgccaatttcttttttttgagacagggtctcactctgtcacctaggatggagtgcagtggcacaatcactgctcactgcagcctcgacttcccgggctcgggtgattctccccaggctcaggggattctcccacttcagcctcccaagtagctgggactacaggtgcgcaccaccatccctggctaatatttgtactttattttatttatttatttatttattttttgagatggagtttcgctcttgttgcccgggctggagtacagtggcatgatctcggctcagtgcaacctctgcctcccgggttcaagcgattctcctacctcatccccctgagtagctgggattacaggcgcctgccaccatgcctggctaattttttgtatttttaatagagacgaggtttcaccatgttggccaggctactctcgaactcctgatctcaggtgatccacccgccttggcctcccaaagtgctgggattacaggcgtgagccactgcgcccggcctaatatttgtattttttgtagagatggtgttttgccatgttgtccaggctggtcttgaactcctgagctcaagcgatctgcccgcctctgcttcccaaagtgctgggattacaggcatgagccaccgtgcctggcctaggtagacgcttttagctttggggtgtgatgcctgccccagtatatagtgaatttaattattgctagagctggctgtttgttagttttctttgaacataagatactcattgtttttagtttgcaaatccctcttcctttttaaaaaatttctttcccttaaattgtttgcatgttagcaataacaaatgcttaaatggtgctatgtgctagatactcttctaagccctgttatgtatattaactaattttttaaattacacaaatcagagaggttaagtaacttgcccaagattacccaacaatactaggatttgaacctaagtttgtctcaccccagattctgctcttaatctctaaacttttaagttagtagtgacaatagtaggtatttattgaatacttaactatgttttaggcgttgaagtaaatattttgcaggcattatctaatgtaaacaccctaaagttacataacaggtaccctttaggtaaataaacactagtatgaccttggaggcacagatagttgaagtaacttgcccaatatcacttacatgaaattggccctcaaatgtgtctgatacaacccatgctgcttgtaactatcgttttaaactgccagggtaaacttggacacacttgagctaagaaaaagcttttagatttttgcaaattaatgtgaaagatatgctttatgtggatataatatcttctaaatttcggggatggtagtcctagaaatgtaatcctgccctagccgagcttaccctgccaataattttttacagaattggtaaaacggagcaccttttttttgtccttggccacactgttatcaacagggtgtagattgacatcaatctgtaggtgtaaaccagaattactctttgtgaccaccaggaaatagagcagttcagttcaggggtttctttctgtgaatttagcactgtgacctgcatactacaagtctactttgttttctatccattgtttgtatctgggtattgcaaaaggtaggaaaaggaccaaccagatcagcagagaagagttgccttggagttttcttttagttttctgcagttcattagatagtaactaggccatgtcattttactcccttgtagtgaagatatgttgaagttgtactggtatactcttctacctttctgtaattttatattgtgtagacttgataaaatttatgtgtcaatcaccaccattaatatcaatattgagcctcaattcttatttttctgcccagtggctgccaaattactaacatttacaataattcactactactaagataatctactagttcgatcacatacttcaaattgttatggaactactgtcttcagcattgtgcttctgataactgataagtataattttttttttgtccagagtgaacatgtctattcttccactgtacacactaataaaaggaaaaattgtaatattgggtaaattcatgtccttacacatgtagtagttatgagcccatgtccctagaatgagtaataatttatccctcccttggttgaatagtcaagaatgctgattttaattcttctaacagctttatccctcagaagggaaggcaagcaagttatatatgtagtttatttgtaagactgatatgaaattggaagatgaatctactattagctttaattatttttacatttaggaatattgcatcagtaactcataattttggttttctgttatcctgagttaacacaaattatccaaggagatggcggatcatctgctttgaggtgtttttttttgagaattttaatgtatctgaatataaaaggtaaaaatatgccaactagcaatttctgcccattccagaagtttggaaatattactcattactaggaattaaataaaatatggtttatctattgttatacctcttttaattcacatagctcatttttatcttttatttttgtttgttttttttgagatggagtcttgctctgtcaccaggcaggagtgcagtgatgcaaatctcggctcactctagccaccgactccctggttcaagcgattctcctgcctgagccttctgagtagctgggattacaggcaggcaccaccacgcccagctaatttttgtagagacaggatttcaccgtgttggccaggatggtctccatctcctgacctcatgatctgcctgcttcggcctcccaaagtgctgggattacaggtgggagccactacgcctggcccacatagctcatttttagactcacttccattaagtcttgtttggacccacgaacattgtctttttttttttaagatggagtttcacttttgttgcccagactgtagtgcaatggtgcaatctcagctcactgcaatctctgcctcctgggttctagcaattctcctgcctcagcctcccgagtagctggaattacaggcgcccgccaccacgcccagctaatttttgtgtttttagtagagacggggtttcaccatgttgggcaggccaggggtgatccgcccacctcagcctcccaaagtgctgggattacaggtgtgagccaccgcatctggccaacatgtcttttttttttttttcctttttaaccacaaagagacttaagcagtccttgtcacagatgatgaattgatgttgcaagtattgtcttagcttggattaattttcttgcttactgtaattttagataatatagctttgtaattagagattttatgtgtaaaccacaaaaatgtttacatgaaggccattattacagatgtgacgtgcataattattagtaatttgtatgtttacatgggtcagtctggcaaaaaattatgaagttttaaaaattaaaaaaaattataatgccagttttactggaaagtaaaattatttcagtaatcgattatagcaaaagtattgattttcattccagacaactgtctgtctatagccaattatgcatttcttaaattagaacccccccaatatacccaaatatatatatatgtgtgcatatatatagtaagttgtaacaaagttgtgaattcatacctgaagtatctcaagtgatgcaagttttatgaatttttgtttatgccttttgggaagagttgtattgacaaattttttatgcttaaagtaaaccataaatcaaaaaaataaaatctaggatgcaataaaacaaaacaacttcttgacataagtatggtatgtaaatctgttttgattggaaatcaatttgttatattgccagaattcctgttttagaatacatctctgctgatctgtctgtattcttagactgcatatctgggatgaactctgggcagaattcacatgggcttcctttgaaataaacaagacttttcaaattcttagtcgatctgcagaacctgtagccaggcactgaaccattttgatagatgcagtaatcgttgcaagtgtatatttcaagggagttctggctgggtcctagtttatgcttgtggcagaagcagtgagtaactgggaggaagttggtgagtaagcttcaaggaagaagtcatttttagtactctggatcttcctgattttaaagcactacaaaatggtgcattttcattcttgtcaagtgataacagatatattctgatgagcctgaaatgaatatatattgtatcatttttataatatctagcaaggtttgtattttcctagaacttgaactaaatttcagttcataaaatttataaaatacttagttgttgtaaaatatttttggaatgttcacataggtgacacacaaatgtcccattttcattctttctatagtaaatatgttctgatatgtgaaggtttagcagatgcatcagcatttaatcctagaggatctggcataatcttttcccccaagaatagaaattttttctgcttatgaaagtagtacatgtttctttaaaaacaaatcaatattgacttctgcctgctgtatagcactatgcctccacctggccatgaccaggggcatgtcctggtccacctacctgaaaatgtttgcaaccagcctcctggccatgtgcacaggggctgaagttgtcccacaggtattacgggccaacctgacaatacatgaagttccaccaaagtctgagaactcagaactgagctttggggactgaaagacagcacaaacctcaaatttctcagcactggaaacctcaaaatataactgaattccataaataagattttaagtcttaaatatgtatttttaaatgtattaaaagtcaagctgcttgtatttaagcacctaatacaatgcttaggttgtaaaaggagatgctcaataggtactaactgatatattgagatttaattatggtttgaccaatatttattggaaaccgccaaagcttaaatcatcagcttcttgaatgtgatttgaaaggtaatttagtattgaatagcatgtgagctagagtatttcattctttctggtttatttcttcaaatagactttgaatataatggtgaatgggtattataaattaactaataaaaatgacattgaaaatgaaaaaatatatatattaaagtgtagaaagtgaccaggcgtggtggctcacacctgtaatccaagcaccttgggaggctgaggcaggaggatctcttgatcccaggagttcaagaccagcctgggcaacatagcgagacttcgtctctaaaaaaaaaaaagagagagaaaaaaattttttttatttaaaaaaagtgtagaaagtgtcaagaccccacttcttaccattatttggtatatttctctatacccacccacccttcctccttactccctccctcccttcccaatctttttatctttttgtattctgattttttgtttgtatattttgctttaatttaatgtatcctttaaaaatttcccatacattttatatgtatatataaaaacgcatgctgccaaagataatttataagaaagaccattgaatttttttaaaagtgatatatattcattgaaaaaaatttagaatatatagcaaagcaataaagaactaaataaaattgctgtaactcctctttcaaagataagtgcttttatgattttgttgtatttttttctgtatataggtacatatatagtatttataaagctgtactcatagtacattttcacatcacaggtaccatatcagtgttattaaatattttgtatgccaggggctagacataccaagacaaccaatatgtggttctacttaaataatattagagtatcttttatgatgacacttcatgagttgactataataatcttagacttctaagagtttgggttttcaaaagatcacttagcttttttgggtgatttttcccccttactgtgagatgagagaggctgtttggatttgggattggggtagcggggacagcaacttttcttttctttttcttttttattttgaggtagggtattgctgtgtcacccaggctggagtgcagtggtgtgatctcggctcactgcaacctccacctcccgggctcaggtgatcctcctgcttcagcctcccagtaactgggactacaggcgcgtgccacatgcctggctaattttgtatttttagtagagatggggtttcaccatgttggccaggctggtctctaactcctgacctcaggtgatacgcccacctgggcctcccaaaatactgggattacaggcatgagccgctgcatcagccagcagtttttcttgtggttttttttgtttgttttgttttgttttgtttttgagatagggtcttactctgttgtccacgctggagtgctgtggtatgatcgtagctcactgcagcctcaaactcctgggctcaagtgattccttctgcctccgcctcccgagtagctgggactacaggtatgcaccaccatacctggcaaatttttacaaagttttttgtagggacggggtcttgctacattccccatgtcggtcttgaactcctggcctcaagcaactctcctgtctcagcctcccaaagcactgggattacaagtgtgagccaccacaccatgccagtttttcctgttcagtgtgatattttatcttgttagactacagtgtgttaaaacttgttttactaaattttcaaacatactcaaaagtggagagaatagtataatgaatacccgtatgttcatcacccatgtttagaatattattaaatataaagattttgctgcgtttgtcttagctctttaaaatttttctttttctctttgtgacctaaaggaaattccatatcttatcactttacttctacattcttgactaagatgactaagacatatagttacatggttttttgttttgtttttgttttttaaagacgaaatctcgctcttgtcccccaggctggagtgcaatggtgccatctcagctcagtgcaacctctgccttctgggtacaagcgattctcctgcctcagcctcccaagtagctgggattacaggctcctgccaccacgcctggctaatttttgtatttttagtagagacggcggggggaggtttcaccatgttgacaaggctggtctggaactcctgacctcaggtgatccacccgcctcggcctcccaaagtgctgggattacaggcgtgagccaccgcgcccagcctgtttttttgtttgtgtgttttgttttttttgagacagagtcttgctctgtttcccaggctggagtgaagtggtgccatctcagctcagagacagagtcttgctctgtttcccaggctggagtgaagtggtgccatcttggctcactgcaaccttcacctcccaggttcaagtgattctcctgcctcagcctcccaagtagctgggactacaggcatgtgtcaccacacccggctaatttttttgtatttttagtagagacgggatttcaccgtgttgcccaggctggtctcgaactcctgagctcaggcagtctgcctgcctcagcctcccaaagtgctgggattacacgtgtgaaccaacccgcccggcctgttgttttcttacataattcattatcatacctacaaagttaacagttactaatatcatcttacacctaaatttctctgatagactaaggttattttttaacatcttaatccaatcaaatgtttgtatcctgtaatgctctcattgaaacagctatatttctttttcagattagtgatgatgaaccaggttatgaccttgatttattttgcatacctaatcattatgctgaggatttggaaagggtgtttattcctcatggactaattatggacaggtaagtaagatcttaaaatgaggttttttactttttcttgtgttaatttcaaacatcagcagctgttctgagtacttgctatttgaacataaactaggccaacttattaaataactgatgctttctaaaatcttctttattaaaaataaaagaggagggccttactaattacttagtatcagttgtggtatagtgggactctgtagggaccagaacaaagtaaacattgaagggagatggaagaaggaactctagccagagtcttgcatttctcagtcctaaacagggtaatggactggggctgaatcacatgaaggcaaggtcagatttttattattatgcacatctagcttgaaaattttctgttaagtcaattacagtgaaaaaccttacctggtattgaatgcttgcattgtatgtctggctattctgtgtttttattttaaaattataatatcaaaatatttgtgttataaaatattctaactatggaggccataaacaagaagactaaagttctctcctttcagccttctgtacacatttcttctcaagcactggcctatgcatgtatactatatgcaaaagtacatatatacatttatattttaacgtatgagtatagttttaaatgttattggacacttttaatattagtgtgtctagagctatctaatatattttaaaggttgcatagcattctgtcttatggagataccataactgatttaaccagtccactattgatagacactattttgttcttaccgactgtactagaagaaacattcttttacatgtttggtacttgttcagctttattcaagtggaatttctgggtcaaggggaaagagtttattgaatattttggtattgccaaattttcctctaagaagttgaatcattttatactcctgatgttatatgagagtacctttctcttcacaatttgtctcttttttttttttttttgagacaaggtctctgttgcccaggctggggtgcagtgcagcagaatgatcacagttcactgcagtctcaacctcctgggttcaagcgatccttccacctcagcctcctgagtagctgggactataggtgtgcgccaccactcccagctaatatttttattttgtagaaacagggttcgccatgttacccagcctcccaaagtgctgggattacaggcatgagccactggcccagtttctacagtctctcttaatattgtatattatccagaaaatttcatttaatcagaacctgccagtctgataggtgaaaatggtatcttgtttttatttgcatttaaaaaaaattatgatagtggtatgcttggtttttttgaaggtatcaaattttttaccttatgaaacatgagggcaaaggatgtgatacgtggaagatttaaaaaaaatttttaatgcatttttttgagacaaggtcttgctctattgtccaggctggagtgcagtggcacaatcacagttcactccagcctcaacatcctgcactaaagtgattttcccacctcacctctcaagtagctgggactacaggtacatgctaccatgcctggctaatttttttttttttgcaggcatggggtctcactatattgcccaggttggtgtggaagtttaatgactaagaggtgtttgttataaagtttaatgtatgaaactttctattaaattcctgattttatttctgtaggactgaacgtcttgctcgagatgtgatgaaggagatgggaggccatcacattgtagccctctgtgtgctcaaggggggctataaattctttgctgacctgctggattacatcaaagcactgaatagaaatagtgatagatccattcctatgactgtagattttatcagactgaagagctattgtgtgagtatatttaatatatgattctttttagtggcaacagtaggttttcttatattttctttgaatctctgcaaaccatacttgctttcatttcacttggttacagtgagatttttctaacatattcactagtactttacatcaaagccaatactgtttttttaaaactagtcaccttggaggatatatacttattttacaggtgtgtgtggttttttaaataaactccttttaggaattgctgttgggacttgggatacttttttcactatacatactggtgacagataccctctcttgagctacatcggtttgtggggagtcaaaagtcctttggagctaggtttgacaaataaggtgggttaacacttgtttcctagaaagcacatggagagctagagtattggcgaattgaagaaatccccctttttttttaacacacttaagaaaggggactgcaggtatactcaagagagtaagtcgcaccagaaaccacttttgatccacagtctgcctgtgtcacacaattgaaatgcatcacaacattgacactgtggatgaaacaaaatcagtgtgaattttagtagtgaatttcattcataatttgatcgtgcaaacgtttgatttttattactttagactattgtttctgattttatgttgggttggtatttcctgtgagttactgttttacctttaaaataggaatttttcatactcttcaaagattagaacaaatgtccagtttttgctgtttcatgaatgagtcctgtccatctttgtagaaactcgccttatgttcacatttttattgagaataagaccacttatctacatttaactatcaacctcatcctctccattaatcatctattttagtgacccaagtttttgaccttttccatgtttacatcaatcctgtaggtgattgggcagccatttaagtattattatagacattttcactatcccattaaaaccctttatgcccatacatcataacactacttcctacccataagctccttttaacttgttaaagtcttgcttgaattaaagacttgtttacggtatcgataagcttgatatcaaaacgccaactttgacccggaacgcggaaaacacctgagaaaaacacctgggcgagtctccacgtaaacggtcaaagtccccgcggccctagacaaatattacgcgctatgagtaacacaaaattattcagatttcacttcctcttattcagttttcccgcgaaaatggccaaatcttactcggttacgcccaaatttactacaacatccgcctaaaaccgcgcgaaaattgtcacttcctgtgtacaccggcgcacaccaaaaacgtcacttttgccacatccgtcgcttacatgtgttccgccacacttgcaacatcacacttccgccacactactacgtcacccgccccgttcccacgccccgcgccacgtcacaaactccaccccctcattatcatattggcttcaatccaaaataaggtatattattgatgatgttt

SEQ ID NO: 126 - DNA, 35010 bp, synthetic construct
  source 1..35010: mol_type = other DNA
taacatcatcaataatataccttattttggattgaagccaatatgataatgagggggtggagtttgtgacgtggcgcggggcgtgggaacggggcgggtgacgtagtagtgtggcggaagtgtgatgttgcaagtgtggcggaacacatgtaagcgacggatgtggcaaaagtgacgtttttggtgtgcgccggtgtacacaggaagtgacaattttcgcgcggttttaggcggatgttgtagtaaatttgggcgtaaccgagtaagatttggccattttcgcgggaaaactgaataagaggaagtgaaatctgaataattttgtgttactcatagcgcgtaatatttgtctagggccgcggggactttgaccgtttacgtggagactcgcccaggtgtttttctcaggtgttttccgcgttccgggtcaaagttggcgttttattattatagtcagctgacgtgtagtgtatttatacccggtgagttcctcaagaggccactcttgagtgccagcgagtagagttttctcctccgagccgctccgacaccgggactgaaaatgagacatattatctgccacggaggtgttattaccgaagaaatggccgccagtcttttggaccagctgatcgaagaggtactggctgataatcttccacctcctagccattttgaaccacctacccttcacgaactgtatgatttagacgtgacggcccccgaagatcccaacgaggaggcggtttcgcagatttttcccgagtctgtaatgttggcggtgcaggaagggattgacttattcacttttccgccggcgcccggttctccggagccgcctcacctttcccggcagcccgagcagccggagcagagagccttgggtccggtttctatgccaaaccttgtgccggaggtgatcgatccacccagtgacgacgaggatgaagagggtgaggagtttgtgttagattatgtggagcaccccgggcacggttgcaggtcttgtcattatcaccggaggaatacgggggacccagatattatgtgttcgctttgctatatgaggacctgtggcatgtttgtctacagtaagtgaaaattatgggcagtcggtgatagagtggtgggtttggtgtggtaatttttttttaatttttacagttttgtggtttaaagaattttgtattgtgattttttaaaaggtcctgtgtctgaacctgagcctgagcccgagccagaaccggagcctgcaagacctacccggcgtcctaaattggtgcctgctatcctgagacgcccgacatcacctgtgtctagagaatgcaatagtagtacggatagctgtgactccggtccttctaacacacctcctgagatacacccggtggtcccgctgtgccccattaaaccagttgccgtgagagttggtgggcgtcgccaggctgtggaatgtatcgaggacttgcttaacgagtctgggcaacctttggacttgagctgtaaacgccccaggccataaggtgtaaacctgtgattgcgtgtgtggttaacgcctttgtttgctgaatgagttgatgtaagtttaataaagggtgagataatgtttaacttgcatggcgtgttaaatggggcggggcttaaagggtatataatgcgccgtgggctaatcttggttacatctgacctcatggaggcttgggagtgtttggaagatttttctgctgtgcgtaacttgctggaacagagctctaacagtacctcttggttttggaggtttctgtggggctcatcccaggcaaagttagtctgcagaattaaggaggattacaagtgggaatttgaagagcttttgaaatcctgtggtgagctgtttgattctttgaatctgggtcaccaggcgcttttccaagagaaggtcatcaagactttggatttttccacaccggggcgcgctgcggctgctgttgcttttttgagttttataaaggataaatggagcgaagaaacccatctgagcggggggtacctgctggattttctggccatgcatctgtggagagcggttgtgagacacaagaatcgcctgctactgttgtcttccgtccgcccggcgataataccgacggaggagcagcagcagcagcaggaggaagccaggcggcggcggcaggagcagagcccatggaacccgagagccggcctggaccctcgggaatgaatgttgttcaggtggctgaactgtatccagaactgagacgcattttgacaattacagaggatgggcaggggctaaagggggtaaagagggagcggggggcttgtgaggctacagaggaggctaggaatctagcttttagcttaatgaccagacaccgtcctgagtgtattacttttcaacagatcaaggataattgcgctaatgagcttgatctgctggcgcagaagtattccatagagcagctgaccacttactggctgcagccaggggatgattttgaggaggctattagggtatatgcaaaggtggcacttaggccagattgcaagtacaagatcagcaaacttgtaaatatcaggaattgttgctacatttctgggaacggggccgaggtggagatagatacggaggatagggtggcctttagatgtagcatgataaatatgtggccgggggtgcttggcatggacggggtggttattatgaatgtaaggtttactggccccaattttagcggtacggttttcctggccaataccaaccttatcctacacggtgtaagcttctatgggtttaacaatacctgtgtggaagcctggaccgatgtaagggttcggggctgtgccttttactgctgctggaagggggtggtgtgtcgccccaaaagcagggcttcaattaagaaatgcctctttgaaaggtgtaccttgggtatcctgtctgagggtaactccagggtgcgccacaatgtggcctccgactgtggttgcttcatgctagtgaaaagcgtggctgtgattaagcataacatggtatgtggcaactgcgaggacagggcctctcagatgctgacctgctcggacggcaactgtcaccttctgaagaccattcacgtagccagccactctcgcaaggcctggccagtgtttgagcataacatactgacccgctgttccttgcatttgggtaacaggaggggggtgttcctaccttaccaatgcaatttgagtcacactaagatattgcttgagcccgagagcatgtccaaggtgaacctgaacggggtgtttgacatgaccatgaagatctggaaggtgctgaggtacgatgagacccgcaccaggtgcagaccctgcgagtgtggcggtaaacatattaggaaccagcctgtgatgctggatgtgaccgaggagctgaggcccgatcacttggtgctggcctgcacccgcgctgagtttggctctagcgatgaagatacagattgaggtactgaaatgtgtgggcgtggcttaagggtgggaaagaatatataaggtgggggtcttatgtagttttgtatctgttttgcagcagccgccgccgccatgagcaccaactcgtttgatggaagcattgtgagctcatatttgacaacgcgcatgcccccatgggccggggtgcgtcagaatgtgatgggctccagcattgatggtcgccccgtcctgcccgcaaactctactaccttgacctacgagaccgtgtctggaacgccgttggagactgcagcctccgccgccgcttcagccgctgcagccaccgcccgcgggattgtgactgactttgctttcctgagcccgcttgcaagcagtgcagcttcccgttcatccgcccgcgatgacaagttgacggctcttttggcacaattggattctttgacccgggaacttaatgtcgtttctcagcagctgttggatctgcgccagcaggtttctgccctgaaggcttcctcccctcccaatgcggtttaaaacataaataaaaaaccagactctgtttggatttggatcaagcaagtgtcttgctgtctttatttaggggttttgcgcgcgcggtaggcccgggaccagcggtctcggtcgttgagggtcctgtgtattttttccaggacgtggtaaaggtgactctggatgttcagatacatgggcataagcccgtctctggggtggaggtagcaccactgcagagcttcatgctgcggggtggtgttgtagatgatccagtcgtagcaggagcgctgggcgtggtgcctaaaaatgtctttcagtagcaagctgattgccaggggcaggcccttggtgtaagtgtttacaaagcggttaagctgggatgggtgcatacgtggggatatgagatgcatcttggactgtatttttaggttggctatgttcccagccatatccctccggggattcatgttgtgcagaaccaccagcacagtgtatccggtgcacttgggaaatttgtcatgtagcttagaaggaaatgcgtggaagaacttggagacgcccttgtgacctccaagattttccatgcattcgtccataatgatggcaatgggcccacgggcggcggcctgggcgaagatatttctgggatcactaacgtcatagttgtgttccaggatgagatcgtcataggccatttttacaaagcgcgggcggagggtgccagactgcggtataatggttccatccggcccaggggcgtagttaccctcacagatttgcatttcccacgctttgagttcagatggggggatcatgtctacctgcggggcgatgaagaaaacggtttccggggtaggggagatcagctgggaagaaagcaggttcctgagcagctgcgacttaccgcagccggtgggcccgtaaatcacacctattaccgggtgcaactggtagttaagagagctgcagctgccgtcatccctgagcaggggggccacttcgttaagcatgtccctgactcgcatgttttccctgaccaaatccgccagaaggcgctcgccgcccagcgatagcagttcttgcaaggaagcaaagtttttcaacggtttgagaccgtccgccgtaggcatgcttttgagcgtttgaccaagcagttccaggcggtcccacagctcggttacctgctctacggcatctcgatccagcatatctcctcgtttcgcgggttggggcggctttcgctgtacggcagtagtcggtgctcgtccagacgggccagggtcatgtctttccacgggcgcagggtcctcgtcagcgtagtctgggtcacggtgaaggggtgcgctccgggctgcgcgctggccagggtgcgcttgaggctggtcctgctggtgctgaagcgctgccggtcttcgccctgcgcgtcggccaggtagcatttgaccatggtgtcatagtccagcccctccgcggcgtggcccttggcgcgcagcttgcccttggaggaggcgccgcacgaggggcagtgcagacttttgagggcgtagagcttgggcgcgagaaataccgattccggggagtaggcatccgcgccgcaggccccgcagacggtctcgcattccacgagccaggtgagctctggccgttcggggtcaaaaaccaggtttcccccatgctttttgatgcgtttcttacctctggtttccatgagccggtgtccacgctcggtgacgaaaaggctgtccgtgtccccgtatacagacttgagaggcctgtcctcgagcggtgttccgcggtcctcctcgtatagaaactcggaccactctgagacaaaggctcgcgtccaggccagcacgaaggaggctaagtgggaggggtagcggtcgttgtccactagggggtccactcgctccagggtgtgaagacacatgtcgccctcttcggcatcaaggaaggtgattggtttgtaggtgtaggccacgtgaccgggtgttcctgaaggggggctataaaagggggtgggggcgcgttcgtcctcactctcttccgcatcgctgtctgcgagggccagctgttggggtgagtactccctctgaaaagcgggcatgacttctgcgctaagattgtcagtttccaaaaacgaggaggatttgatattcacctggcccgcggtgatgcctttgagggtggccgcatccatctggtcagaaaagacaatctttttgttgtcaagcttggtggcaaacgacccgtagagggcgttggacagcaacttggcgatggagcgcagggtttggtttttgtcgcgatcggcgcgctccttggccgcgatgtttagctgcacgtattcgcgcgcaacgcaccgccattcgggaaagacggtggtgcgctcgtcgggcaccaggtgcacgcgccaaccgcggttgtgcagggtgacaaggtcaacgctggtggctacctctccgcgtaggcgctcgttggtccagcagaggcggccgcccttgcgcgagcagaatggcggtagggggtctagctgcgtctcgtccggggggtctgcgtccacggtaaagaccccgggcagcaggcgcgcgtcgaagtagtctatcttgcatccttgcaagtctagcgcctgctgccatgcgcgggcggcaagcgcgcgctcgtatgggttgagtgggggaccccatggcatggggtgggtgagcgcggaggcgtacatgccgcaaatgtcgtaaacgtagaggggctctctgagtattccaagatatgtagggtagcatcttccaccgcggatgctggcgcgcacgtaatcgtatagttcgtgcgagggagcgaggaggtcgggaccgaggttgctacgggcgggctgctctgctcggaagactatctgcctgaagatggcatgtgagttggatgatatggttggacgctggaagacgttgaagctggcgtctgtgagacctaccgcgtcacgcacgaaggaggcgtaggagtcgcgcagcttgttgaccagctcggcggtgacctgcacgtctagggcgcagtagtccagggtttccttgatgatgtcatacttatcctgtcccttttttttccacagctcgcggttgaggacaaactcttcgcggtctttccagtactcttggatcggaaacccgtcggcctccgaacggtaagagcctagcatgtagaactggttgacggcctggtaggcgcagcatcccttttctacgggtagcgcgtatgcctgcgcggccttccggagcgaggtgtgggtgagcgcaaaggtgtccctgaccatgactttgaggtactggtatttgaagtcagtgtcgtcgcatccgccctgctcccagagcaaaaagtccgtgcgctttttggaacgcggatttggcagggcgaaggtgacatcgttgaagagtatctttcccgcgcgaggcataaagttgcgtgtgatgcggaagggtcccggcacctcggaacggttgttaattacctgggcggcgagcacgatctcgtcaaagccgttgatgttgtggcccacaatgtaaagttccaagaagcgcgggatgcccttgatggaaggcaattttttaagttcctcgtaggtgagctcttcaggggagctgagcccgtgctctgaaagggcccagtctgcaagatgagggttggaagcgacgaatgagctccacaggtcacgggccattagcatttgcaggtggtcgcgaaaggtcctaaactggcgacctatggccattttttctggggtgatgcagtagaaggtaagcgggtcttgttcccagcggtcccatccaaggttcgcggctaggtctcgcgcggcagtcactagaggctcatctccgccgaacttcatgaccagcatgaagggcacgagctgcttcccaaaggcccccatccaagtataggtctctacatcgtaggtgacaaagagacgctcggtgcgaggatgcgagccgatcgggaagaactggatctcccgccaccaattggaggagtggctattgatgtggtgaaagtagaagtccctgcgacgggccgaacactcgtgctggcttttgtaaaaacgtgcgcagtactggcagcggtgcacgggctgtacatcctgcacgaggttgacctgacgaccgcgcacaaggaagcagagtgggaatttgagcccctcgcctggcgggtttggctggtggtcttctacttcggctgcttgtccttgaccgtctggctgctcgaggggagttacggtggatcggaccaccacgccgcgcgagcccaaagtccagatgtccgcgcgcggcggtcggagcttgatgacaacatcgcgcagatgggagctgtccatggtctggagctcccgcggcgtcaggtcaggcgggagctcctgcaggtttacctcgcatagacgggtcagggcgcgggctagatccaggtgatacctaatttccaggggctggttggtggcggcgtcgatggcttgcaagaggccgcatccccgcggcgcgactacggtaccgcgcggcgggcggtgggccgcgggggtgtccttggatgatgcatctaaaagcggtgacgcgggcgagcccccggaggtagggggggctccggacccgccgggagagggggcaggggcacgtcggcgccgcgcgcgggcaggagctggtgctgcgcgcgtaggttgctggcgaacgcgacgacgcggcggttgatctcctgaatctggcgcctctgcgtgaagacgacgggcccggtgagcttgagcctgaaagagagttcgacagaatcaatttcggtgtcgttgacggcggcctggcgcaaaatctcctgcacgtctcctgagttgtcttgataggcgatctcggccatgaactgctcgatctcttcctcctggagatctccgcgtccggctcgctccacggtggcggcgaggtcgttggaaatgcgggccatgagctgcgagaaggcgttgaggcctccctcgttccagacgcggctgtagaccacgcccccttcggcatcgcgggcgcgcatgaccacctgcgcgagattgagctccacgtgccgggcgaagacggcgtagtttcgcaggcgctgaaagaggtagttgagggtggtggcggtgtgttctgccacgaagaagtacataacccagcgtcgcaacgtggattcgttgatatcccccaaggcctcaaggcgctccatggcctcgtagaagtccacggcgaagttgaaaaactgggagttgcgcgccgacacggttaactcctcctccagaagacggatgagctcggcgacagtgtcgcgcacctcgcgctcaaaggctacaggggcctcttcttcttcttcaatctcctcttccataagggcctccccttcttcttcttctggcggcggtgggggaggggggacacggcggcgacgacggcgcaccgggaggcggtcgacaaagcgctcgatcatctccccgcggcgacggcgcatggtctcggtgacggcgcggccgttctcgcgggggcgcagttggaagacgccgcccgtcatgtcccggttatgggttggcggggggctgccatgcggcagggatacggcgctaacgatgcatctcaacaattgttgtgtaggtactccgccgccgagggacctgagcgagtccgcatcgaccggatcggaaaacctctcgagaaaggcgtctaaccagtcacagtcgcaaggtaggctgagcaccgtggcgggcggcagcgggcggcggtcggggttgtttctggcggaggtgctgctgatgatgtaattaaagtaggcggtcttgagacggcggatggtcgacagaagcaccatgtccttgggtccggcctgctgaatgcgcaggcggtcggccatgccccaggcttcgttttgacatcggcgcaggtctttgtagtagtcttgcatgagcctttctaccggcacttcttcttctccttcctcttgtcctgcatctcttgcatctatcgctgcggcggcggcggagtttggccgtaggtggcgccctcttcctcccatgcgtgtgaccccgaagcccctcatcggctgaagcagggctaggtcggcgacaacgcgctcggctaatatggcctgctgcacctgcgtgagggtagactggaagtcatccatgtccacaaagcggtggtatgcgcccgtgttgatggtgtaagtgcagttggccataacggaccagttaacggtctggtgacccggctgcgagagctcggtgtacctgagacgcgagtaagccctcgagtcaaatacgtagtcgttgcaagtccgcaccaggtactggtatcccaccaaaaagtgcggcggcggctggcggtagaggggccagcgtagggtggccggggctccgggggcgagatcttccaacataaggcgatgatatccgtagatgtacctggacatccaggtgatgccggcggcggtggtggaggcgcgcggaaagtcgcggacgcggttccagatgttgcgcagcggcaaaaagtgctccatggtcgggacgctctggccggtcaggcgcgcgcaatcgttgacgctctagaccgtgcaaaaggagagcctgtaagcgggcactcttccgtggtctggtggataaattcgcaagggtatcatggcggacgaccggggttcgagccccgtatccggccgtccgccgtgatccatgcggttaccgcccgcgtgtcgaacccaggtgtgcgacgtcagacaacgggggagtgctccttttggcttccttccaggcgcggcggctgctgcgctagcttttttggccactggccgcgcgcagcgtaagcggttaggctggaaagcgaaagcattaagtggctcgctccctgtagccggagggttattttccaagggttgagtcgcgggacccccggttcgagtctcggaccggccggactgcggcgaacgggggtttgcctccccgtcatgcaagaccccgcttgcaaattcctccggaaacagggacgagccccttttttgcttttcccagatgcatccggtgctgcggcagatgcgcccccctcctcagcagcggcaagagcaagagcagcggcagacatgcagggcaccctcccctcctcctaccgcgtcaggaggggcgacatccgcggttgacgcggcagcagatggtgattacgaacccccgcggcgccgggcccggcactacctggacttggaggagggcgagggcctggcgcggctaggagcgccctctcctgagcggtacccaagggtgcagctgaagcgtgatacgcgtgaggcgtacgtgccgcggcagaacctgtttcgcgaccgcgagggagaggagcccgaggagatgcgggatcgaaagttccacgcagggcgcgagctgcggcatggcctgaatcgcgagcggttgctgcgcgaggaggactttgagcccgacgcgcgaaccgggattagtcccgcgcgcgcacacgtggcggccgccgacctggtaaccgcatacgagcagacggtgaaccaggagattaactttcaaaaaagctttaacaaccacgtgcgtacgcttgtggcgcgcgaggaggtggctataggactgatgcatctgtgggactttgtaagcgcgctggagcaaaacccaaatagcaagccgctcatggcgcagctgttccttatagtgcagcacagcagggacaacgaggcattcagggatgcgctgctaaacatagtagagcccgagggccgctggctgctcgatttgataaacatcctgcagagcatagtggtgcaggagcgcagcttgagcctggctgacaaggtggccgccatcaactattccatgcttagcctgggcaagttttacgcccgcaagatataccataccccttacgttcccatagacaaggaggtaaagatcgaggggttctacatgcgcatggcgctgaaggtgcttaccttgagcgacgacctgggcgtttatcgcaacgagcgcatccacaaggccgtgagcgtgagccggcggcgcgagctcagcgaccgcgagctgatgcacagcctgcaaagggccctggctggcacgggcagcggcgatagagaggccgagtcctactttgacgcgggcgctgacctgcgctgggccccaagccgacgcgccctggaggcagctggggccggacctgggctggcggtggcacccgcgcgcgctggcaacgtcggcggcgtggaggaatatgacgaggacgatgagtacgagccagaggacggcgagtactaagcggtgatgtttctgatcagatgatgcaagacgcaacggacccggcggtgcgggcggcgctgcagagccagccgtccggccttaactccacggacgactggcgccaggtcatggaccgcatcatgtcgctgactgcgcgcaatcctgacgcgttccggcagcagccgcaggccaaccggctctccgcaattctggaagcggtggtcccggcgcgcgcaaaccccacgcacgagaaggtgctggcgatcgtaaacgcgctggccgaaaacagggccatccggcccgacgaggccggcctggtctacgacgcgctgcttcagcgcgtggctcgttacaacagcggcaacgtgcagaccaacctggaccggctggtgggggatgtgcgcgaggccgtggcgcagcgtgagcgcgcgcagcagcagggcaacctgggctccatggttgcactaaacgccttcctgagtacacagcccgccaacgtgccgcggggacaggaggactacaccaactttgtgagcgcactgcggctaatggtgactgagacaccgcaaagtgaggtgtaccagtctgggccagactattttttccagaccagtagacaaggcctgcagaccgtaaacctgagccaggctttcaaaaacttgcaggggctgtggggggtgcgggctcccacaggcgaccgcgcgaccgtgtctagcttgctgacgcccaactcgcgcctgttgctgctgctaatagcgcccttcacggacagtggcagcgtgtcccgggacacatacctaggtcacttgctgacactgtaccgcgaggccataggtcaggcgcatgtggacgagcatactttccaggagattacaagtgtcagccgcgcgctggggcaggaggacacgggcagcctggaggcaaccctaaactacctgctgaccaaccggcggcagaagatcccctcgttgcacagtttaaacagcgaggaggagcgcattttgcgctacgtgcagcagagcgtgagccttaacctgatgcgcgacggggtaacgcccagcgtggcgctggacatgaccgcgcgcaacatggaaccgggcatgtatgcctcaaaccggccgtttatcaaccgcctaatggactacttgcatcgcgcggccgccgtgaaccccgagtatttcaccaatgccatcttgaacccgcactggctaccgccccctggtttctacaccgggggattcgaggtgcccgagggtaacgatggattcctctgggacgacatagacgacagcgtgttttccccgcaaccgcagaccctgctagagttgcaacagcgcgagcaggcagaggcggcgctgcgaaaggaaagcttccgcaggccaagcagcttgtccgatctaggcgctgcggccccgcggtcagatgctagtagcccatttccaagcttgatagggtctcttaccagcactcgcaccacccgcccgcgcctgctgggcgaggaggagtacctaaacaactcgctgctgcagccgcagcgcgaaaaaaacctgcctccggcatttcccaacaacgggatagagagcctagtggacaagatgagtagatggaagacgtacgcgcaggagcacagggacgtgccaggcccgcgcccgcccacccgtcgtcaaaggcacgaccgtcagcggggtctggtgtgggaggacgatgactcggcagacgacagcagcgtcctggatttgggagggagtggcaacccgtttgcgcaccttcgccccaggctggggagaatgttttaaaaaaaaaaaagcatgatgcaaaataaaaaactcaccaaggccatggcaccgagcgttggttttcttgtattccccttagtatgcggcgcgcggcgatgtatgaggaaggtcctcctccctcctacgagagtgtggtgagcgcggcgccagtggcggcggcgctgggttctcccttcgatgctcccctggacccgccgtttgtgcctccgcggtacctgcggcctaccggggggagaaacagcatccgttactctgagttggcacccctattcgacaccacccgtgtgtacctggtggacaacaagtcaacggatgtggcatccctgaactaccagaacgaccacagcaactttctgaccacggtcattcaaaacaatgactacagcccgggggaggcaagcacacagaccatcaatcttgacgaccggtcgcactggggcggcgacctgaaaaccatcctgcataccaacatgccaaatgtgaacgagttcatgtttaccaataagtttaaggcgcgggtgatggtgtcgcgcttgcctactaaggacaatcaggtggagctgaaatacgagtgggtggagttcacgctgcccgagggcaactactccgagaccatgaccatagaccttatgaacaacgcgatcgtggagcactacttgaaagtgggcagacagaacggggttctggaaagcgacatcggggtaaagtttgacacccgcaacttcagactggggtttgaccccgtcactggtcttgtcatgcctggggtatatacaaacgaagccttccatccagacatcattttgctgccaggatgcggggtggacttcacccacagccgcctgagcaacttgttgggcatccgcaagcggcaacccttccaggagggctttaggatcacctacgatgatctggagggtggtaacattcccgcactgttggatgtggacgcctaccaggcgagcttgaaagatgacaccgaacagggcgggggtggcgcaggcggcagcaacagcagtggcagcggcgcggaagagaactccaacgcggcagccgcggcaatgcagccggtggaggacatgaacgatcatgccattcgcggcgacacctttgccacacgggctgaggagaagcgcgctgaggccgaagcagcggccgaagctgccgcccccgctgcgcaacccgaggtcgagaagcctcagaagaaaccggtgatcaaacccctgacagaggacagcaagaaacgcagttacaacctaataagcaatgacagcaccttcacccagtaccgcagctggtaccttgcatacaactacggcgaccctcagaccggaatccgctcatggaccctgctttgcactcctgacgtaacctgcggctcggagcaggtctactggtcgttgccagacatgatgcaagaccccgtgaccttccgctccacgcgccagatcagcaactttccggtggtgggcgccgagctgttgcccgtgcactccaagagcttctacaacgaccaggccgtctactcccaactcatccgccagtttacctctctgacccacgtgttcaatcgctttcccgagaaccagattttggcgcgcccgccagcccccaccatcaccaccgtcagtgaaaacgttcctgctctcacagatcacgggacgctaccgctgcgcaacagcatcggaggagtccagcgagtgaccattactgacgccagacgccgcacctgcccctacgtttacaaggccctgggcatagtctcgccgcgcgtcctatcgagccgcactttttgagcaagcatgtccatccttatatcgcccagcaataacacaggctggggcctgcgcttcccaagcaagatgtttggcggggccaagaagcgctccgaccaacacccagtgcgcgtgcgcgggcactaccgcgcgccctggggcgcgcacaaacgcggccgcactgggcgcaccaccgtcgatgacgccatcgacgcggtggtggaggaggcgcgcaactacacgcccacgccgccaccagtgtccacagtggacgcggccattcagaccgtggtgcgcggagcccggcgctatgctaaaatgaagagacggcggaggcgcgtagcacgtcgccaccgccgccgacccggcactgccgcccaacgcgcggcggcggccctgcttaaccgcgcacgtcgcaccggccgacgggcggccatgcgggccgctcgaaggctggccgcgggtattgtcactgtgccccccaggtccaggcgacgagcggccgccgcagcagccgcggccattagtgctatgactcagggtcgcaggggcaacgtgtattgggtgcgcgactcggttagcggcctgcgcgtgcccgtgcgcacccgccccccgcgcaactagattgcaagaaaaaactacttagactcgtactgttgtatgtatccagcggcggcggcgcgcaacgaagctatgtccaagcgcaaaatcaaagaagagatgctccaggtcatcgcgccggagatctatggccccccgaagaaggaagagcaggattacaagccccgaaagctaaagcgggtcaaaaagaaaaagaaagatgatgatgatgaacttgacgacgaggtggaactgctgcacgctaccgcgcccaggcgacgggtacagtggaaaggtcgacgcgtaaaacgtgttttgcgacccggcaccaccgtagtctttacgcccggtgagcgctccacccgcacctacaagcgcgtgtatgatgaggtgtacggcgacgaggacctgcttgagcaggccaacgagcgcctcggggagtttgcctacggaaagcggcataaggacatgctggcgttgccgctggacgagggcaacccaacacctagcctaaagcccgtaacactgcagcaggtgctgcccgcgcttgcaccgtccgaagaaaagcgcggcctaaagcgcgagtctggtgacttggcacccaccgtgcagctgatggtacccaagcgccagcgactggaagatgtcttggaaaaaatgaccgtggaacctgggctggagcccgaggtccgcgtgcggccaatcaagcaggtggcgccgggactgggcgtgcagaccgtggacgttcagatacccactaccagtagcaccagtattgccaccgccacagagggcatggagacacaaacgtccccggttgcctcagcggtggcggatgccgcggtgcaggcggtcgctgcggccgcgtccaagacctctacggaggtgcaaacggacccgtggatgtttcgcgtttcagccccccggcgcccgcgcggttcgaggaagtacggcgccgccagcgcgctactgcccgaatatgccctacatccttccattgcgcctacccccggctatcgtggctacacctaccgccccagaagacgagcaactacccgacgccgaaccaccactggaacccgccgccgccgtcgccgtcgccagcccgtgctggccccgatttccgtgcgcagggtggctcgcgaaggaggcaggaccctggtgctgccaacagcgcgctaccaccccagcatcgtttaaaagccggtctttgtggttcttgcagatatggccctcacctgccgcctccgtttcccggtgccgggattccgaggaagaatgcaccgtaggaggggcatggccggccacggcctgacgggcggcatgcgtcgtgcgcaccaccggcggcggcgcgcgtcgcaccgtcgcatgcgcggcggtatcctgcccctccttattccactgatcgccgcggcgattggcgccgtgcccggaattgcatccgtggccttgcaggcgcagagacactgattaaaaacaagttgcatgtggaaaaatcaaaataaaaagtctggactctcacgctcgcttggtcctgtaactattttgtagaatggaagacatcaactttgcgtctctggccccgcgacacggctcgcgcccgttcatgggaaactggcaagatatcggcaccagcaatatgagcggtggcgccttcagctggggctcgctgtggagcggcattaaaaatttcggttccaccgttaagaactatggcagcaaggcctggaacagcagcacaggccagatgctgagggataagttgaaagagcaaaatttccaacaaaaggtggtagatggcctggcctctggcattagcggggtggtggacctggccaaccaggcagtgcaaaataagattaacagtaagcttgatccccgccctcccgtagaggagcctccaccggccgtggagacagtgtctccagaggggcgtggcgaaaagcgtccgcgccccgacagggaagaaactctggtgacgcaaatagacgagcctccctcgtacgaggaggcactaaagcaaggcctgcccaccacccgtcccatcgcgcccatggctaccggagtgctgggccagcacacacccgtaacgctggacctgcctccccccgccgacacccagcagaaacctgtgctgccaggcccgaccgccgttgttgtaacccgtcctagccgcgcgtccctgcgccgcgccgccagcggtccgcgatcgttgcggcccgtagccagtggcaactggcaaagcacactgaacagcatcgtgggtctgggggtgcaatccctgaagcgccgacgatgcttctgaatagctaacgtgtcgtatgtgtgtcatgtatgcgtccatgtcgccgccagaggagctgctgagccgccgcgcgcccgctttccaagatggctaccccttcgatgatgccgcagtggtcttacatgcacatctcgggccaggacgcctcggagtacctgagccccgggctggtgcagtttgcccgcgccaccgagacgtacttcagcctgaataacaagtttagaaaccccacggtggcgcctacgcacgacgtgaccacagaccggtcccagcgtttgacgctgcggttcatccctgtggaccgtgaggatactgcgtactcgtacaaggcgcggttcaccctagctgtgggtgataaccgtgtgctggacatggcttccacgtactttgacatccgcggcgtgctggacaggggccctacttttaagccctactctggcactgcctacaacgccctggctcccaagggtgccccaaatccttgcgaatgggatgaagctgctactgctcttgaaataaacctagaagaagaggacgatgacaacgaagacgaagtagacgagcaagctgagcagcaaaaaactcacgtatttgggcaggcgccttattctggtataaatattacaaaggagggtattcaaataggtgtcgaaggtcaaacacctaaatatgccgataaaacatttcaacctgaacctcaaataggagaatctcagtggtacgaaactgaaattaatcatgcagctgggagagtccttaaaaagactaccccaatgaaaccatgttacggttcatatgcaaaacccacaaatgaaaatggagggcaaggcattcttgtaaagcaacaaaatggaaagctagaaagtcaagtggaaatgcaatttttctcaactactgaggcgaccgcaggcaatggtgataacttgactcctaaagtggtattgtacagtgaagatgtagatatagaaaccccagacactcatatttcttacatgcccactattaaggaaggtaactcacgagaactaatgggccaacaatctatgcccaacaggcctaattacattgcttttagggacaattttattggtctaatgtattacaacagcacgggtaatatgggtgttctggcgggccaagcatcgcagttgaatgctgttgtagatttgcaagacagaaacacagagctttcataccagcttttgcttgattccattggtgatagaaccaggtacttttctatgtggaatcaggctgttgacagctatgatccagatgttagaattattgaaaatcatggaactgaagatgaacttccaaattactgctttccactgggaggtgtgattaatacagagactcttaccaaggtaaaacctaaaacaggtcaggaaaatggatgggaaaaagatgctacagaattttcagataaaaatgaaataagagttggaaataattttgccatggaaatcaatctaaatgccaacctgtggagaaatttcctgtactccaacatagcgctgtatttgcccgacaagctaaagtacagtccttccaacgtaaaaatttctgataacccaaacacctacgactacatgaacaagcgagtggtggctcccgggttagtggactgctacattaaccttggagcacgctggtcccttgactatatggacaacgtcaacccatttaaccaccaccgcaatgctggcctgcgctaccgctcaatgttgctgggcaatggtcgctatgtgcccttccacatccaggtgcctcagaagttctttgccattaaaaacctccttctcctgccgggctcatacacctacgagtggaacttcaggaaggatgttaacatggttctgcagagctccctaggaaatgacctaagggttgacggagccagcattaagtttgatagcatttgcctttacgccaccttcttccccatggcccacaacaccgcctccacgcttgaggccatgcttagaaacgacaccaacgaccagtcctttaacgactatctctccgccgccaacatgctctaccctatacccgccaacgctaccaacgtgcccatatccatcccctcccgcaactgggcggctttccgcggctgggccttcacgcgccttaagactaaggaaaccccatcactgggctcgggctacgacccttattacacctactctggctctataccctacctagatggaaccttttacctcaaccacacctttaagaaggtggccattacctttgactcttctgtcagctggcctggcaatgaccgcctgcttacccccaacgagtttgaaattaagcgctcagttgacggggagggttacaacgttgcccagtgtaacatgaccaaagactggttcctggtacaaatgctagctaactacaacattggctaccagggcttctatatcccagagagctacaaggaccgcatgtactccttctttagaaacttccagcccatgagccgtcaggtggtggatgatactaaatacaaggactaccaacaggtgggcatcctacaccaacacaacaactctggatttgttggctaccttgcccccaccatgcgcgaaggacaggcctaccctgctaacttcccctatccgcttataggcaagaccgcagttgacagcattacccagaaaaagtttctttgcgatcgcaccctttggcgcatcccattctccagtaactttatgtccatgggcgcactcacagacctgggccaaaaccttctctacgccaactccgcccacgcgctagacatgacttttgaggtggatcccatggacgagcccacccttctttatgttttgtttgaagtctttgacgtggtccgtgtgcaccggccgcaccgcggcgtcatcgaaaccgtgtacctgcgcacgcccttctcggccggcaacgccacaacataaagaagcaagcaacatcaacaacagctgccgccatgggctccagtgagcaggaactgaaagccattgtcaaagatcttggttgtgggccatattttttgggcacctatgacaagcgctttccaggctttgtttctccacacaagctcgcctgcgccatagtcaatacggccggtcgcgagactgggggcgtacactggatggcctttgcctggaacccgcactcaaaaacatgctacctctttgagccctttggcttttctgaccagcgactcaagcaggtttaccagtttgagtacgagtcactcctgcgccgtagcgccattgcttcttcccccgaccgctgtataacgctggaaaagtccacccaaagcgtacaggggcccaactcggccgcctgtggactattctgctgcatgtttctccacgcctttgccaactggccccaaactcccatggatcacaaccccaccatgaaccttattaccggggtacccaactccatgctcaacagtccccaggtacagcccaccctgcgtcgcaaccaggaacagctctacagcttcctggagcgccactcgccctacttccgcagccacagtgcgcagattaggagcgccacttctttttgtcacttgaaaaacatgtaaaaataatgtactagagacactttcaataaaggcaaatgcttttatttgtacactctcgggtgattatttacccccacccttgccgtctgcgccgtttaaaaatcaaaggggttctgccgcgcatcgctatgcgccactggcagggacacgttgcgatactggtgtttagtgctccacttaaactcaggcacaaccatccgcggcagctcggtgaagttttcactccacaggctgcgcaccatcaccaacgcgtttagcaggtcgggcgccgatatcttgaagtcgcagttggggcctccgccctgcgcgcgcgagttgcgatacacagggttgcagcactggaacactatcagcgccgggtggtgcacgctggccagcacgctcttgtcggagatcagatccgcgtccaggtcctccgcgttgctcagggcgaacggagtcaactttggtagctgccttcccaaaaagggcgcgtgcccaggctttgagttgcactcgcaccgtagtggcatcaaaaggtgaccgtgcccggtctgggcgttaggatacagcgcctgcataaaagccttgatctgcttaaaagccacctgagcctttgcgccttcagagaagaacatgccgcaagacttgccggaaaactgattggccggacaggccgcgtcgtgcacgcagcaccttgcgtcggtgttggagatctgcaccacatttcggccccaccggttcttcacgatcttggccttgctagactgctccttcagcgcgcgctgcccgttttcgctcgtcacatccatttcaatcacgtgctccttatttatcataatgcttccgtgtagacacttaagctcgccttcgatctcagcgcagcggtgcagccacaacgcgcagcccgtgggctcgtgatgcttgtaggtcacctctgcaaacgactgcaggtacgcctgcaggaatcgccccatcatcgtcacaaaggtcttgttgctggtgaaggtcagctgcaacccgcggtgctcctcgttcagccaggtcttgcatacggccgccagagcttccacttggtcaggcagtagtttgaagttcgcctttagatcgttatccacgtggtacttgtccatcagcgcgcgcgcagcctccatgcccttctcccacgcagacacgatcggcacactcagcgggttcatcaccgtaatttcactttccgcttcgctgggctcttcctcttcctcttgcgtccgcataccacgcgccactgggtcgtcttcattcagccgccgcactgtgcgcttacctcctttgccatgcttgattagcaccggtgggttgctgaaacccaccatttgtagcgccacatcttctctttcttcctcgctgtccacgattacctctggtgatggcgggcgctcgggcttgggagaagggcgcttctttttcttcttgggcgcaatggccaaatccgccgccgaggtcgatggccgcgggctgggtgtgcgcggcaccagcgcgtcttgtgatgagtcttcctcgtcctcggactcgatacgccgcctcatccgcttttttgggggcgcccggggaggcggcggcgacggggacggggacgacacgtcctccatggttgggggacgtcgcgccgcaccgcgtccgcgctcgggggtggtttcgcgctgctcctcttcccgactggccatttccttctcctataggcagaaaaagatcatggagtcagtcgagaagaaggacagcctaaccgccccctctgagttcgccaccaccgcctccaccgatgccgccaacgcgcctaccaccttccccgtcgaggcacccccgcttgaggaggaggaagtgattatcgagcaggacccaggttttgtaagcgaagacgacgaggaccgctcagtaccaacagaggataaaaagcaagaccaggacaacgcagaggcaaacgaggaacaagtcgggcggggggacgaaaggcatggcgactacctagatgtgggagacgacgtgctgttgaagcatctgcagcgccagtgcgccattatctgcgacgcgttgcaagagcgcagcgatgtgcccctcgccatagcggatgtcagccttgcctacgaacgccacctattctcaccgcgcgtaccccccaaacgccaagaaaacggcacatgcgagcccaacccgcgcctcaacttctaccccgtatttgccgtgccagaggtgcttgccacctatcacatctttttccaaaactgcaagatacccctatcctgccgtgccaaccgcagccgagcggacaagcagctggccttgcggcagggcgctgtcatacctgatatcgcctcgctcaacgaagtgccaaaaatctttgagggtcttggacgcgacgagaagcgcgcggcaaacgctctgcaacaggaaaacagcgaaaatgaaagtcactctggagtgttggtggaactcgagggtgacaacgcgcgcctagccgtactaaaacgcagcatcgaggtcacccactttgcctacccggcacttaacctaccccccaaggtcatgagcacagtcatgagtgagctgatcgtgcgccgtgcgcagcccctggagagggatgcaaatttgcaagaacaaacagaggagggcctacccgcagttggcgacgagcagctagcgcgctggcttcaaacgcgcgagcctgccgacttggaggagcgacgcaaactaatgatggccgcagtgctcgttaccgtggagcttgagtgcatgcagcggttctttgctgacccggagatgcagcgcaagctagaggaaacattgcactacacctttcgacagggctacgtacgccaggcctgcaagatctccaacgtggagctctgcaacctggtctcctaccttggaattttgcacgaaaaccgccttgggcaaaacgtgcttcattccacgctcaagggcgaggcgcgccgcgactacgtccgcgactgcgtttacttatttctatgctacacctggcagacggccatgggcgtttggcagcagtgcttggaggagtgcaacctcaaggagctgcagaaactgctaaagcaaaacttgaaggacctatggacggccttcaacgagcgctccgtggccgcgcacctggcggacatcattttccccgaacgcctgcttaaaaccctgcaacagggtctgccagacttcaccagtcaaagcatgttgcagaactttaggaactttatcctagagcgctcaggaatcttgcccgccacctgctgtgcacttcctagcgactttgtgcccattaagtaccgcgaatgccctccgccgctttggggccactgctaccttctgcagctagccaactaccttgcctaccactctgacataatggaagacgtgagcggtgacggtctactggagtgtcactgtcgctgcaacctatgcaccccgcaccgctccctggtttgcaattcgcagctgcttaacgaaagtcaaattatcggtacctttgagctgcagggtccctcgcctgacgaaaagtccgcggctccggggttgaaactcactccggggctgtggacgtcggcttaccttcgcaaatttgtacctgaggactaccacgcccacgagattaggttctacgaagaccaatcccgcccgccaaatgcggagcttaccgcctgcgtcattacccagggccacattcttggccaattgcaagccatcaacaaagcccgccaagagtttctgctacgaaagggacggggggtttacttggacccccagtccggcgaggagctcaacccaatccccccgccgccgcagccctatcagcagcagccgcgggcccttgcttcccaggatggcacccaaaaagaagctgcagctgccgccgccacccacggacgaggaggaatactgggacagtcaggcagaggaggttttggacgaggaggaggaggacatgatggaagactgggagagcctagacgaggaagcttccgaggtcgaagaggtgtcagacgaaacaccgtcaccctcggtcgcattcccctcgccggcgccccagaaatcggcaaccggttccagcatggctacaacctccgctcctcaggcgccgccggcactgcccgttcgccgacccaaccgtagatgggacaccactggaaccagggccggtaagtccaagcagccgccgccgttagcccaagagcaacaacagcgccaaggctaccgctcatggcgcgggcacaagaacgccatagttgcttgcttgcaagactgtgggggcaacatctccttcgcccgccgctttcttctctaccatcacggcgtggccttcccccgtaacatcctgcattactaccgtcatctctacagcccatactgcaccggcggcagcggcagcggcagcaacagcagcggccacacagaagcaaaggcgaccggatagcaagactctgacaaagcccaagaaatccacagcggcggcagcagcaggaggaggagcgctgcgtctggcgcccaacgaacccgtatcgacccgcgagcttagaaacaggatttttcccactctgtatgctatatttcaacagagcaggggccaagaacaagagctgaaaataaaaaacaggtctctgcgatccctcacccgcagctgcctgtatcacaaaagcgaagatcagcttcggcgcacgctggaagacgcggaggctctcttcagtaaatactgcgcgctgactcttaaggactagtttcgcgccctttctcaaatttaagcgcgaaaactacgtcatctccagcggccacacccggcgccagcacctgtcgtcagcgccattatgagcaaggaaattcccacgccctacatgtggagttaccagccacaaatgggacttgcggctggagctgcccaagactactcaacccgaataaactacatgagcgcgggaccccacatgatatcccgggtcaacggaatccgcgcccaccgaaaccgaattctcttggaacaggcggctattaccaccacacctcgtaataaccttaatccccgtagttggcccgctgccctggtgtaccaggaaagtcccgctcccaccactgtggtacttcccagagacgcccaggccgaagttcagatgactaactcaggggcgcagcttgcgggcggctttcgtcacagggtgcggtcgcccgggcagggtataactcacctgacaatcagagggcgaggtattcagctcaacgacgagtcggtgagctcctcgcttggtctccgtccggacgggacatttcagatcggcggcgccggccgctcttcattcacgcctcgtcaggcaatcctaactctgcagacctcgtcctctgagccgcgctctggaggcattggaactctgcaatttattgaggagtttgtgccatcggtctactttaaccccttctcgggacctcccggccactatccggatcaatttattcctaactttgacgcggtaaaggactcggcggatggctacgactgaatgttaagtggagaggcagagcaactgcgcctgaaacacctggtccactgtcgccgccacaagtgctttgcccgcgactccggtgagttttgctactttgaattgcccgaggatcatatcgagggcccggcgcacggcgtccggcttaccgcccagggagagcttgcccgtagcctgattcgggagtttacccagcgccccctgctagttgagcgggacaggggaccctgtgttctcactgtgatttgcaactgtcctaaccctggattacatcaagatctttgttgccatctctgtgctgagtataataaatacagaaattaaaatatactggggctcctatcgccatcctgtaaacgccaccgtcttcacccgcccaagcaaaccaaggcgaaccttacctggtacttttaacatctctccctctgtgatttacaacagtttcaacccagacggagtgagtctacgagagaacctctccgagctcagctactccatcagaaaaaacaccaccctccttacctgccgggaacgtacgacctagggataacagggtaataagcaattgactctatgtgggatatgctccagcgctacaaccttgaagtcaggcttcctggatgtcagcatctgactttggccagcacctgtcccgcggatttgttccagtccaactacagcgacccaccctaacagagatgaccaacacaaccaacgcggccgccgctaccggacttacatctaccacaaatacaccccaagtttctgcctttgtcaataactgggataacttgggcatgtggtggttctccatagcgcttatgtttgtatgccttattattatgtggctcatctgctgcctaaagcgcaaacgcgcccgaccacccatctatagtcccatcattgtgctacacccaaacaatgatggaatccatagattggacggactgaaacacatgttcttttctcttacagtatgattaaatgagacatgattcctcgagtttttatattactgacccttgttgcgcttttttgtgcgtgctccacattggctgcggtttctcacatcgaagtagactgcattccagccttcacagtctatttgctttacggatttgtcaccctcacgctcatctgcagcctcatcactgtggtcatcgcctttatccagtgcattgactgggtctgtgtgcgctttgcatatctcagacaccatccccagtacagggacaggactatagctgagcttcttagaattctttaattatgaaatttactgtgacttttctgctgattatttgcaccctatctgcgttttgttccccgacctccaagcctcaaagacatatatcatgcagattcactcgtatatggaatattccaagttgctacaatgaaaaaagcgatctttccgaagcctggttatatgcaatcatctctgttatggtgttctgcagtaccatcttagccctagctatatatccctaccttgacattggctggaaacgaatagatgccatgaaccacccaactttccccgcgcccgctatgcttccactgcaacaagttgttgccggcggctttgtcccagccaatcagcctcgccccacttctcccacccccactgaaatcagctactttaatctaacaggaggagatgactgacaccctagatctagaaatggacggaattattacagagcagcgcctgctagaaagacgcagggcagcggccgagcaacagcgcatgaatcaagagctccaagacatggttaacttgcaccagtgcaaaaggggtatcttttgtctggtaaagcaggccaaagtcacctacgacagtaataccaccggacaccgccttagctacaagttgccaaccaagcgtcagaaattggtggtcatggtgggagaaaagcccattaccataactcagcactcggtagaaaccgaaggctgcattcactcaccttgtcaaggacctgaggatctctgcacccttattaagaccctgtgcggtctcaaagatcttattccctttaactaataaaaaaaaataataaagcatcacttacttaaaatcagttagcaaatttctgtccagtttattcagcagcacctccttgccctcctcccagctctggtattgcagcttcctcctggctgcaaactttctccacaatctaaatggaatgtcagtttcctcctgttcctgtccatccgcacccactatcttcatgttgttgcagatgaagcgcgcaagaccgtctgaagataccttcaaccccgtgtatccatatgacacggaaaccggtcctccaactgtgccttttcttactcctccctttgtatcccccaatgggtttcaagagagtccccctggggtactctctttgcgcctatccgaacctctagttacctccaatggcatgcttgcgctcaaaatgggcaacggcctctctctggacgaggccggcaaccttacctcccaaaatgtaaccactgtgagcccacctctcaaaaaaaccaagtcaaacataaacctggaaatatctgcacccctcacagttacctcagaagccctaactgtggctgccgccgcacctctaatggtcgcgggcaacacactcaccatgcaatcacaggccccgctaaccgtgcacgactccaaacttagcattgccacccaaggacccctcacagtgtcagaaggaaagctagccctgcaaacatcaggccccctcaccaccaccgatagcagtacccttactatcactgcctcaccccctctaactactgccactggtagcttgggcattgacttgaaagagcccatttatacacaaaatggaaaactaggactaaagtacggggctcctttgcatgtaacagacgacctaaacactttgaccgtagcaactggtccaggtgtgactattaataatacttccttgcaaactaaagttactggagccttgggttttgattcacaaggcaatatgcaacttaatgtagcaggaggactaaggattgattctcaaaacagacgccttatacttgatgttagttatccgtttgatgctcaaaaccaactaaatctaagactaggacagggccctctttttataaactcagcccacaacttggatattaactacaacaaaggcctttacttgtttacagcttcaaacaattccaaaaagcttgaggttaacctaagcactgccaaggggttgatgtttgacgctacagccatagccattaatgcaggagatgggcttgaatttggttcacctaatgcaccaaacacaaatcccctcaaaacaaaaattggccatggcctagaatttgattcaaacaaggctatggttcctaaactaggaactggccttagttttgacagcacaggtgccattacagtaggaaacaaaaataatgataagctaaccctatggacaggtccaaaaccagaagccaactgcataattgaatacgggaaacaaaacccagatagcaaactaactttaatccttgtaaaaaatggaggaattgttaatggatatgtaacgctaatgggagcctcagactacgttaacaccttatttaaaaacaaaaatgtctccattaatgtagaactatactttgatgccactggtcatatattaccagactcatcttctcttaaaacagatctagaactaaaatacaagcaaaccgctgactttagtgcaagaggttttatgccaagtactacagcgtatccatttgtccttcctaatgcgggaacacataatgaaaattatatttttggtcaatgctactacaaagcaagcgatggtgccctttttccgttggaagttactgttatgcttaataaacgcctgccagatagtcgcacatcctatgttatgacttttttatggtccttgaatgctggtctagctccagaaactactcaggcaaccctcataacctccccatttaccttttcctatattagagaagatgactaataaactctaaagaatcgtttgtgttatgtttcaacgtgtttatttttcaattgcagaaaatttcaagtcatttttcattcagtagtatagccccaccaccacatagcttatacagatcaccgtaccttaatcaaactcacagaaccctagtattcaacctgccacctccctcccaacacacagagtacacagtcctttctccccggctggccttaaaaagcatcatatcatgggtaacagacatattcttaggtgttatattccacacggtttcctgtcgagccaaacgctcatcagtgatattaataaactccccgggcagctcacttaagttcatgtcgctgtccagctgctgagccacaggctgctgtccaacttgcggttgcttaacgggcggcgaaggagaagtccacgcctacatgggggtagagtcataatcgtgcatcaggatagggcggtggtgctgcagcagcgcgcgaataaactgctgccgccgccgctccgtcctgcaggaatacaacatggcagtggtctcctcagcgatgattcgcaccgcccgcagcataaggcgccttgtcctccgggcacagcagcgcaccctgatctcacttaaatcagcacagtaactgcagcacagcaccacaatattgttcaaaatcccacagtgcaaggcgctgtatccaaagctcatggcggggaccacagaacccacgtggccatcataccacaagcgcaggtagattaagtggcgacccctcataaacacgctggacataaacattacctcttttggcatgttgtaattcaccacctcccggtaccatataaacctctgattaaacatggcgccatccaccaccatcctaaaccagctggccaaaacctgcccgccggctatacactgcagggaaccgggactggaacaatgacagtggagagcccaggactcgtaaccatggatcatcatgctcgtcatgatatcaatgttggcacaacacaggcacacgtgcatacacttcctcaggattacaagctcctcccgcgttagaaccatatcccagggaacaacccattcctgaatcagcgtaaatcccacactgcagggaagacctcgcacgtaactcacgttgtgcattgtcaaagtgttacattcgggcagcagcggatgatcctccagtatggtagcgcgggtttctgtctcaaaaggaggtagacgatccctactgtacggagtgcgccgagacaaccgagatcgtgttggtcgtagtgtcatgccaaatggaacgccggacgtagtcatatttcctgaagcaaaaccaggtgcgggcgtgacaaacagatctgcgtctccggtctcgccgcttagatcgctctgtgtagtagttgtagtatatccactctctcaaagcatccaggcgccccctggcttcgggttctatgtaaactccttcatgcgccgctgccctgataacatccaccaccgcagaataagccacacccagccaacctacacattcgttctgcgagtcacacacgggaggagcgggaagagctggaagaaccatgtttttttttttattccaaaagattatccaaaacctcaaaatgaagatctattaagtgaacgcgctcccctccggtggcgtggtcaaactctacagccaaagaacagataatggcatttgtaagatgttgcacaatggcttccaaaaggcaaacggccctcacgtccaagtggacgtaaaggctaaacccttcagggtgaatctcctctataaacattccagcaccttcaaccatgcccaaataattctcatctcgccaccttctcaatatatctctaagcaaatcccgaatattaagtccggccattgtaaaaatctgctccagagcgccctccaccttcagcctcaagcagcgaatcatgattgcaaaaattcaggttcctcacagacctgtataagattcaaaagcggaacattaacaaaaataccgcgatcccgtaggtcccttcgcagggccagctgaacataatcgtgcaggtctgcacggaccagcgcggccacttccccgccaggaaccttgacaaaagaacccacactgattatgacacgcatactcggagctatgctaaccagcgtagccccgatgtaagctttgttgcatgggcggcgatataaaatgcaaggtgctgctcaaaaaatcaggcaaagcctcgcgcaaaaaagaaagcacatcgtagtcatgctcatgcagataaaggcaggtaagctccggaaccaccacagaaaaagacaccatttttctctcaaacatgtctgcgggtttctgcataaacacaaaataaaataacaaaaaaacatttaaacattagaagcctgtcttacaacaggaaaaacaacccttataagcataagacggactacggccatgccggcgtgaccgtaaaaaaactggtcaccgtgattaaaaagcaccaccgacagctcctcggtcatgtccggagtcataatgtaagactcggtaaacacatcaggttgattcatcggtcagtgctaaaaagcgaccgaaatagcccgggggaatacatacccgcaggcgtagagacaacattacagcccccataggaggtataacaaaattaataggagagaaaaacacataaacacctgaaaaaccctcctgcctaggcaaaatagcaccctcccgctccagaacaacatacagcgcttcacagcggcagcctaacagtcagccttaccagtaaaaaagaaaacctattaaaaaaacaccactcgacacggcaccagctcaatcagtcacagtgtaaaaaagggccaagtgcagagcgagtatatataggactaaaaaatgacgtaacggttaaagtccacaaaaaacacccagaaaaccgcacgcgaacctacgcccagaaacgaaagccaaaaaacccacaacttcctcaaatcgtcacttccgttttcccacgttacgtaacttcccattttaagaaaactacaattcccaacacatacaagttactccgccctaaaacctacgtcacccgccccgttcccacgccccgcgccacgtcacaaactccaccccctcattatcatattggcttcaatccaaaataaggtatattattgatgatgttaat

SEQ ID NO: 127 - DNA, 39752 bp, synthetic construct
  source 1..39752: mol_type = other DNA
taacatcatcaattataccttccattttggattgaagccaatatgataatgagggggtggagtttgtgacgtggcgcggggcgtgggaacggggcgggtgacgtagtagtgtggcggaagtgtgatgttgcaagtgtggcggaacacatgtaagcgacggatgtggcaaaagtgacgtttttggtgtgcgccggtgtacacaggaagtgacaattttcgcgcggttttaggcggatgttgtagtaaatttgggcgtaaccgagtaagatttggccattttcgcgggaaaactgaataagaggaagtgaaatctgaataattttgtgttactcatagcgcgtaatatttgtctagggccgcggggactttgaccgtttacgtggagactcgcccaggtgtttttctcaggtgttttccgcgtacgtcggcggctcgtggctcttccgggaaaaggattctcggaaagtggttcgagtacgtcggcggctcgtggctcttccgggaaaaggattctcggaaagtggttcgaagtacgtcgaccacaaaccccgcccagcgtcttgtcattggcgtcgacgctgtacggggtcaaagttggcgttttattattatagtcagctgacgtgtagtgtatttatacccggtgagttcctcaagaggccactcttgagtgccagcgagtagagttttctcctccgagccgctccgacaccgggactgaaaatgagacatattatctgccacggaggtgttattaccgaagaaatggccgccagtcttttggaccagctgatcgaagaggtactggctgataatcttccacctcctagccattttgaaccacctacccttcacgaactgtatgatttagacgtgacggcccccgaagatcccaacgaggaggcggtttcgcagatttttcccgactctgtaatgttggcggtgcaggaagggattgacttactcacttttccgccggcgcccggttctccggagccgcctcacctttcccggcagcccgagcagccggagcagagagccttgggtccggtttctatgccaaaccttgtaccggaggtgatcgatccacccagtgacgacgaggatgaagagggtgaggagtttgtgttagattatgtggagcaccccgggcacggttgcaggtcttgtcattatcaccggaggaatacgggggacccagatattatgtgttcgctttgctatatgaggacctgtggcatgtttgtctacagtaagtgaaaattatgggcagtgggtgatagagtggtgggtttggtgtggtaattttttttttaatttttacagttttgtggtttaaagaattttgtattgtgatttttttaaaaggtcctgtgtctgaacctgagcctgagcccgagccagaaccggagcctgcaagacctacccgccgtcctaaaatggcgcctgctatcctgagacgcccgacatcacctgtgtctagagaatgcaatagtagtacggatagctgtgactccggtccttctaacacacctcctgagatacacccggtggtcccgctgtgccccattaaaccagttgccgtgagagttggtgggcgtcgccaggctgtggaatgtatcgaggacttgcttaacgagcctgggcaacctttggacttgagctgtaaacgccccaggccataaggtgtaaacctgtgattgcgtgtgtggttaacgcctttgtttgctgaatgagttgatgtaagtttaataaagggtgagataatgtttaacttgcatggcgtgttaaatggggcggggcttaaagggtatataatgcgccgtgggctaatcttggttacatctgacctcatggaggcttgggagtgtttggaagatttttctgctgtgcgtaacttgctggaacagagctctaacagtacctcttggttttggaggtttctgtggggctcatcccaggcaaagttagtctgcagaattaaggaggattacaagtgggaatttgaagagcttttgaaatcctgtggtgagctgtttgattctttgaatctgggtcaccaggcgcttttccaagagaaggtcatcaagactttggatttttccacaccggggcgcgctgcggctgctgttgcttttttgagttttataaaggataaatggagcgaagaaacccatctgagcggggggtacctgctggattttctggccatgcatctgtggagagcggttgtgagacacaagaatcgcctgctactgttgtcttccgtccgcccggcgataataccgacggaggagcagcagcagcagcaggaggaagccaggcggcggcggcaggagcagagcccatggaacccgagagccggcctggaccctcgggaatgaatgttgtacaggtggctgaactgtatccagaactgagacgcattttgacaattacagaggatgggcaggggctaaagggggtaaagagggagcggggggcttgtgaggctacagaggaggctaggaatctagcttttagcttaatgaccagacaccgtcctgagtgtattacttttcaacagatcaaggataattgcgctaatgagcttgatctgctggcgcagaagtattccatagagcagctgaccacttactggctgcagccaggggatgattttgaggaggctattagggtatatgcaaaggtggcacttaggccagattgcaagtacaagatcagcaaacttgtaaatatcaggaattgttgctacatttctgggaacggggccgaggtggagatagatacggaggatagggtggcctttagatgtagcatgataaatatgtggccgggggtgcttggcatggacggggtggttattatgaatgtaaggtttactggccccaattttagcggtacggttttcctggccaataccaaccttatcctacacggtgtaagcttctatgggtttaacaatacctgtgtggaagcctggaccgatgtaagggttcggggctgtgccttttactgctgctggaagggggtggtgtgtcgccccaaaagcagggcttcaattaagaaatgcctctttgaaaggtgtaccttgggtatcctgtctgagggtaactccagggtgcgccacaatgtggcctccgactgtggttgcttcatgctagtgaaaagcgtggctgtgattaagcataacatggtatgtggcaactgcgaggacagggcctctcagatgctgacctgctcggacggcaactgtcacctgctgaagaccattcacgtagccagccactctcgcaaggcctggccagtgtttgagcataacatactgacccgctgttccttgcatttgggtaacaggaggggggtgttcctaccttaccaatgcaatttgagtcacactaagatattgcttgagcccgagagcatgtccaaggtgaacctgaacggggtgtttgacatgaccatgaagatctggaaggtgctgaggtacgatgagacccgcaccaggtgcagaccctgcgagtgtggcggtaaacatattaggaaccagcctgtgatgctggatgtgaccgaggagctgaggcccgatcacttggtgctggcctgcacccgcgctgagtttggctctagcgatgaagatacagattgaggtactgaaatgtgtgggcgtggcttaagggtgggaaagaatatataaggtgggggtcttatgtagttttgtatctgttttgcagcagccgccgccgccatgagcaccaactcgtttgatggaagcattgtgagctcatatttgacaacgcgcatgcccccatgggccggggtgcgtcagaatgtgatgggctccagcattgatggtcgccccgtcctgcccgcaaactctactaccttgacctacgagaccgtgtctggaacgccgttggagactgcagcctccgccgccgcttcagccgctgcagccaccgcccgcgggattgtgactgactttgctttcctgagcccgcttgcaagcagtgcagcttcccgttcatccgcccgcgatgacaagttgacggctcttttggcacaattggattctttgacccgggaacttaatgtcgtttctcagcagctgttggatctgcgccagcaggtttctgccctgaaggcttcctcccctcccaatgcggtttaaaacataaataaaaaaccagactctgtttggatttggatcaagcaagtgtcttgctgtctttatttaggggttttgcgcgcgcggtaggcccgggaccagcggtctcggtcgttgagggtcctgtgtattttttccaggacgtggtaaaggtgactctggatgttcagatacatgggcataagcccgtctctggggtggaggtagcaccactgcagagcttcatgctgcggggtggtgttgtagatgatccagtcgtagcaggagcgctgggcgtggtgcctaaaaatgtctttcagtagcaagctgattgccaggggcaggcccttggtgtaagtgtttacaaagcggttaagctgggatgggtgcatacgtggggatatgagatgcatcttggactgtatttttaggttggctatgttcccagccatatccctccggggattcatgttgtgcagaaccaccagcacagtgtatccggtgcacttgggaaatttgtcatgtagcttagaaggaaatgcgtggaagaacttggagacgcccttgtgacctccaagattttccatgcattcgtccataatgatggcaatgggcccacgggcggcggcctgggcgaagatatttctgggatcactaacgtcatagttgtgttccaggatgagatcgtcataggccatttttacaaagcgcgggcggagggtgccagactgcggtataatggttccatccggcccaggggcgtagttaccctcacagatttgcatttcccacgctttgagttcagatggggggatcatgtctacctgcggggcgatgaagaaaacggtttccggggtaggggagatcagctgggaagaaagcaggttcctgagcagctgcgacttaccgcagccggtgggcccgtaaatcacacctattaccgggtgcaactggtagttaagagagctgcagctgccgtcatccctgagcaggggggccacttcgttaagcatgtccctgactcgcatgttttccctgaccaaatccgccagaaggcgctcgccgcccagcgatagcagttcttgcaaggaagcaaagtttttcaacggtttgagaccgtccgccgtaggcatgcttttgagcgtttgaccaagcagttccaggcggtcccacagctcggtcacctgctctacggcatctcgatccagcatatctcctcgtttcgcgggttggggcggctttcgctgtacggcagtagtcggtgctcgtccagacgggccagggtcatgtctttccacgggcgcagggtcctcgtcagcgtagtctgggtcacggtgaaggggtgcgctccgggctgcgcgctggccagggtgcgcttgaggctggtcctgctggtgctgaagcgctgccggtcttcgccctgcgcgtcggccaggtagcatttgaccatggtgtcatagtccagcccctccgcggcgtggcccttggcgcgcagcttgcccttggaggaggcgccgcacgaggggcagtgcagacttttgagggcgtagagcttgggcgcgagaaataccgattccggggagtaggcatccgcgccgcaggccccgcagacggtctcgcattccacgagccaggtgagctctggccgttcggggtcaaaaaccaggtttcccccatgctttttgatgcgtttcttacctctggtttccatgagccggtgtccacgctcggtgacgaaaaggctgtccgtgtccccgtatacagactnnngttttgagaggcctgtcctcgagcggtgttccgcggtcctcctcgtatagaaactcggaccactctgagacaaaggctcgcgtccaggccagcacgaaggaggctaagtgggaggggtagcggtcgttgtccactagggggtccactcgctccagggtgtgaagacacatgtcgccctcttcggcatcaaggaaggtgattggtttgtaggtgtaggccacgtgaccgggtgttcctgaaggggggctataaaagggggtgggggcgcgttcgtcctcactctcttccgcatcgctgtctgcgagggccagctgttggggtgagtactccctctgaaaagcgggcatgacttctgcgctaagattgtcagtttccaaaaacgaggaggatttgatattcacctggcccgcggtgatgcctttgagggtggccgcatccatctggtcagaaaagacaatctttttgttgtcaagcttggtggcaaacgacccgtagagggcgttggacagcaacttggcgatggagcgcagggtttggtttttgtcgcgatcggcgcgctccttggccgcgatgtttagctgcacgtattcgcgcgcaacgcaccgccattcgggaaagacggtggtgcgctcgtcgggcaccaggtgcacgcgccaaccgcggttgtgcagggtgacaaggtcaacgctggtggctacctctccgcgtaggcgctcgttggtccagcagaggcggccgcccttgcgcgagcagaatggcggtagggggtctagctgcgtctcgtccggggggtctgcgtccacggtaaagaccccgggcagcaggcgcgcgtcgaagtagtctatcttgcatccttgcaagtctagcgcctgctgccatgcgcgggcggcaagcgcgcgctcgtatgggttgagtgggggaccccatggcatggggtgggtgagcgcggaggcgtacatgccgcaaatgtcgtaaacgtagaggggctctctgagtattccaagatatgtagggtagcatcttccaccgcggatgctggcgcgcacgtaatcgtatagttcgtgcgagggagcgaggaggtcgggaccgaggttgctacgggcgggctgctctgctcggaagactatctgcctgaagatggcatgtgagttggatgatatggttggacgctggaagacgttgaagctggcgtctgtgagacctaccgcgtcacgcacgaaggaggcgtaggagtcgcgcagcttgttgaccagctcggcggtgacctgcacgtctagggcgcagtagtccagggtttccttgatgatgtcatacttatcctgtcccttttttttccacagctcgcggttgaggacaaactcttcgcggtctttccagtactcttggatcggaaacccgtcggcctccgaacggtaagagcctagcatgtagaactggttgacggcctggtaggcgcagcatcccttttctacgggtagcgcgtatgcctgcgcggccttccggagcgaggtgtgggtgagcgcaaaggtgtccctgaccatgactttgaggtactggtatttgaagtcagtgtcgtcgcatccgccctgctcccagagcaaaaagtccgtgcgctttttggaacgcggatttggcagggcgaaggtgacatcgttgaagagtatctttcccgcgcgaggcataaagttgcgtgtgatgcggaagggtcccggcacctcggaacggttgttaattacctgggcggcgagcacgatctcgtcaaagccgttgatgttgtggcccacaatgtaaagttccaagaagcgcgggatgcccttgatggaaggcaattttttaagttcctcgtaggtgagctcttcaggggagctgagcccgtgctctgaaagggcccagtctgcaagatgagggttggaagcgacgaatgagctccacaggtcacgggccattagcatttgcaggtggtcgcgaaaggtcctaaactggcgacctatggccattttttctggggtgatgcagtagaaggtaagcgggtcttgttcccagcggtcccatccaaggttcgcggctaggtctcgcgcggcagtcactagaggctcatctccgccgaacttcatgaccagcatgaagggcacgagctgcttcccaaaggcccccatccaagtataggtctctacatcgtaggtgacaaagagacgctcggtgcgaggatgcgagccgatcgggaagaactggatctcccgccaccaattggaggagtggctattgatgtggtgaaagtagaagtccctgcgacgggccgaacactcgtgctggcttttgtaaaaacgtgcgcagtactggcagcggtgcacgggctgtacatcctgcacgaggttgacctgacgaccgcgcacaaggaagcagagtgggaatttgagcccctcgcctggcgggtttggctggtggtcttctacttcggctgcttgtccttgaccgtctggctgctcgaggggagttacggtggatcggaccaccacgccgcgcgagcccaaagtccagatgtccgcgcgcggcggtcggagcttgatgacaacatcgcgcagatgggagctgtccatggtctggagctcccgcggcgtcaggtcaggcgggagctcctgcaggtttacctcgcatagacgggtcagggcgcgggctagatccaggtgatacctaatttccaggggctggttggtggcggcgtcgatggcttgcaagaggccgcatccccgcggcgcgactacggtaccgcgcggcgggcggtgggccgcgggggtgtccttggatgatgcatctaaaagcggtgacgcgggcgagcccccggaggtagggggggctccggacccgccgggagagggggcaggggcacgtcggcgccgcgcgcgggcaggagctggtgctgcgcgcgtaggttgctggcgaacgcgacgacgcggcggttgatctcctgaatctggcgcctctgcgtgaagacgacgggcccggtgagcttgagcctgaaagagagttcgacagaatcaatttcggtgtcgttgacggcggcctggcgcaaaatctcctgcacgtctcctgagttgtcttgataggcgatctcggccatgaactgctcgatctcttcctcctggagatctccgcgtccggctcgctccacggtggcggcgaggtcgttggaaatgcgggccatgagctgcgagaaggcgttgaggcctccctcgttccagacgcggctgtagaccacgcccccttcggcatcgcgggcgcgcatgaccacctgcgcgagattgagctccacgtgccgggcgaagacggcgtagtttcgcaggcgctgaaagaggtagttgagggtggtggcggtgtgttctgccacgaagaagtacataacccagcgtcgcaacgtggattcgttgatatcccccaaggcctcaaggcgctccatggcctcgtagaagtccacggcgaagttgaaaaactgggagttgcgcgccgacacggttaactcctcctccagaagacggatgagctcggcgacagtgtcgcgcacctcgcgctcaaaggctacaggggcctcttcttcttcttcaatctcctcttccataagggcctccccttcttcttcttctggcggcggtgggggaggggggacacggcggcgacgacggcgcaccgggaggcggtcgacaaagcgctcgatcatctccccgcggcgacggcgcatggtctcggtgacggcgcggccgttctcgcgggggcgcagttggaagacgccgcccgtcatgtcccggttatgggttggcggggggctgccatgcggcagggatacggcgctaacgatgcatctcaacaattgttgtgtaggtactccgccgccgagggacctgagcgagtccgcatcgaccggatcggaaaacctctcgagaaaggcgtctaaccagtcacagtcgcaaggtaggctgagcaccgtggcgggcggcagcgggcggcggtcggggttgtttctggcggaggtgctgctgatgatgtaattaaagtaggcggtcttgagacggcggatggtcgacagaagcaccatgtccttgggtccggcctgctgaatgcgcaggcggtcggccatgccccaggcttcgttttgacatcggcgcaggtctttgtagtagtcttgcatgagcctttctaccggcacttcttcttctccttcctcttgtcctgcatctcttgcatctatcgctgcggcggcggcggagtttggccgtaggtggcgccctcttcctcccatgcgtgtgaccccgaagcccctcatcggctgaagcagggctaggtcggcgacaacgcgctcggctaatatggcctgctgcacctgcgtgagggtagactggaagtcatccatgtccacaaagcggtggtatgcgcccgtgttgatggtgtaagtgcagttggccataacggaccagttaacggtctggtgacccggctgcgagagctcggtgtacctgagacgcgagtaagccctcgagtcaaatacgtagtcgttgcaagtccgcaccaggtactggtatcccaccaaaaagtgcggcggcggctggcggtagaggggccagcgtagggtggccggggctccgggggcgagatcttccaacataaggcgatgatatccgtagatgtacctggacatccaggtgatgccggcggcggtggtggaggcgcgcggaaagtcgcggacgcggttccagatgttgcgcagcggcaaaaagtgctccatggtcgggacgctctggccggtcaggcgcgcgcaatcgttgacgctctaccgtgcaaaaggagagcctgtaagcgggcactcttccgtggtctggtggataaattcgcaagggtatcatggcggacgaccggggttcgagccccgtatccggccgtccgccgtgatccatgcggttaccgcccgcgtgtcgaacccaggtgtgcgacgtcagacaacgggggagtgctccttttggcttccttccaggcgcggcggctgctgcgctagcttttttggccactggccgcgcgcagcgtaagcggttaggctggaaagcgaaagcattaagtggctcgctccctgtagccggagggttattttccaagggttgagtcgcgggacccccggttcgagtctcggaccggccggactgcggcgaacgggggtttgcctccccgtcatgcaagaccccgcttgcaaattcctccggaaacagggacgagccccttttttgcttttcccagatgcatccggtgctgcggcagatgcgcccccctcctcagcagcggcaagagcaagagcagcggcagacatgcagggcaccctcccctcctcctaccgcgtcaggaggggcgacatccgcggttgacgcggcagcagatggtgattacgaacccccgcggcgccgggcccggcactacctggacttggaggagggcgagggcctggcgcggctaggagcgccctctcctgagcggtacccaagggtgcagctgaagcgtgatacgcgtgaggcgtacgtgccgcggcagaacctgtttcgcgaccgcgagggagaggagcccgaggagatgcgggatcgaaagttccacgcagggcgcgagctgcggcatggcctgaatcgcgagcggttgctgcgcgaggaggactttgagcccgacgcgcgaaccgggattagtcccgcgcgcgcacacgtggcggccgccgacctggtaaccgcatacgagcagacggtgaaccaggagattaactttcaaaaaagctttaacaaccacgtgcgtacgcttgtggcgcgcgaggaggtggctataggactgatgcatctgtgggactttgtaagcgcgctggagcaaaacccaaatagcaagccgctcatggcgcagctgttccttatagtgcagcacagcagggacaacgaggcattcagggatgcgctgctaaacatagtagagcccgagggccgctggctgctcgatttgataaacatcctgcagagcatagtggtgcaggagcgcagcttgagcctggctgacaaggtggccgccatcaactattccatgcttagcctgggcaagttttacgcccgcaagatataccataccccttacgttcccatagacaaggaggtaaagatcgaggggttctacatgcgcatggcgctgaaggtgcttaccttgagcgacgacctgggcgtttatcgcaacgagcgcatccacaaggccgtgagcgtgagccggcggcgcgagctcagcgaccgcgagctgatgcacagcctgcaaagggccctggctggcacgggcagcggcgatagagaggccgagtcctactttgacgcgggcgctgacctgcgctgggccccaagccgacgcgccctggaggcagctggggccggacctgggctggcggtggcacccgcgcgcgctggcaacgtcggcggcgtggaggaatatgacgaggacgatgagtacgagccagaggacggcgagtactaagcggtgatgtttctgatcagatgatgcaagacgcaacggacccggcggtgcgggcggcgctgcagagccagccgtccggccttaactccacggacgactggcgccaggtcatggaccgcatcatgtcgctgactgcgcgcaatcctgacgcgttccggcagcagccgcaggccaaccggctctccgcaattctggaagcggtggtcccggcgcgcgcaaaccccacgcacgagaaggtgctggcgatcgtaaacgcgctggccgaaaacagggccatccggcccgacgaggccggcctggtctacgacgcgctgcttcagcgcgtggctcgttacaacagcggcaacgtgcagaccaacctggaccggctggtgggggatgtgcgcgaggccgtggcgcagcgtgagcgcgcgcagcagcagggcaacctgggctccatggttgcactaaacgccttcctgagtacacagcccgccaacgtgccgcggggacaggaggactacaccaactttgtgagcgcactgcggctaatggtgactgagacaccgcaaagtgaggtgtaccagtctgggccagactattttttccagaccagtagacaaggcctgcagaccgtaaacctgagccaggctttcaaaaacttgcaggggctgtggggggtgcgggctcccacaggcgaccgcgcgaccgtgtctagcttgctgacgcccaactcgcgcctgttgctgctgctaatagcgcccttcacggacagtggcagcgtgtcccgggacacatacctaggtcacttgctgacactgtaccgcgaggccataggtcaggcgcatgtggacgagcatactttccaggagattacaagtgtcagccgcgcgctggggcaggaggacacgggcagcctggaggcaaccctaaactacctgctgaccaaccggcggcagaagatcccctcgttgcacagtttaaacagcgaggaggagcgcattttgcgctacgtgcagcagagcgtgagccttaacctgatgcgcgacggggtaacgcccagcgtggcgctggacatgaccgcgcgcaacatggaaccgggcatgtatgcctcaaaccggccgtttatcaaccgcctaatggactacttgcatcgcgcggccgccgtgaaccccgagtatttcaccaatgccatcttgaacccgcactggctaccgccccctggtttctacaccgggggattcgaggtgcccgagggtaacgatggattcctctgggacgacatagacgacagcgtgttttccccgcaaccgcagaccctgctagagttgcaacagcgcgagcaggcagaggcggcgctgcgaaaggaaagcttccgcaggccaagcagcttgtccgatctaggcgctgcggccccgcggtcagatgctagtagcccatttccaagcttgatagggtctcttaccagcactcgcaccacccgcccgcgcctgctgggcgaggaggagtacctaaacaactcgctgctgcagccgcagcgcgaaaaaaacctgcctccggcatttcccaacaacgggatagagagcctagtggacaagatgagtagatggaagacgtacgcgcaggagcacagggacgtgccaggcccgcgcccgcccacccgtcgtcaaaggcacgaccgtcagcggggtctggtgtgggaggacgatgactcggcagacgacagcagcgtcctggatttgggagggagtggcaacccgtttgcgcaccttcgccccaggctggggagaatgttttaaaaaaaaaaaagcatgatgcaaaataaaaaactcaccaaggccatggcaccgagcgttggttttcttgtattccccttagtatgcggcgcgcggcgatgtatgaggaaggtcctcctccctcctacgagagtgtggtgagcgcggcgccagtggcggcggcgctgggttctcccttcgatgctcccctggacccgccgtttgtgcctccgcggtacctgcggcctaccggggggagaaacagcatccgttactctgagttggcacccctattcgacaccacccgtgtgtacctggtggacaacaagtcaacggatgtggcatccctgaactaccagaacgaccacagcaactttctgaccacggtcattcaaaacaatgactacagcccgggggaggcaagcacacagaccatcaatcttgacgaccggtcgcactggggcggcgacctgaaaaccatcctgcataccaacatgccaaatgtgaacgagttcatgtttaccaataagtttaaggcgcgggtgatggtgtcgcgcttgcctactaaggacaatcaggtggagctgaaatacgagtgggtggagttcacgctgcccgagggcaactactccgagaccatgaccatagaccttatgaacaacgcgatcgtggagcactacttgaaagtgggcagacagaacggggttctggaaagcgacatcggggtaaagtttgacacccgcaacttcagactggggtttgaccccgtcactggtcttgtcatgcctggggtatatacaaacgaagccttccatccagacatcattttgctgccaggatgcggggtggacttcacccacagccgcctgagcaacttgttgggcatccgcaagcggcaacccttccaggagggctttaggatcacctacgatgatctggagggtggtaacattcccgcactgttggatgtggacgcctaccaggcgagcttgaaagatgacaccgaacagggcgggggtggcgcaggcggcagcaacagcagtggcagcggcgcggaagagaactccaacgcggcagccgcggcaatgcagccggtggaggacatgaacgatcatgccattcgcggcgacacctttgccacacgggctgaggagaagcgcgctgaggccgaagcagcggccgaagctgccgcccccgctgcgcaacccgaggtcgagaagcctcagaagaaaccggtgatcaaacccctgacagaggacagcaagaaacgcagttacaacctaataagcaatgacagcaccttcacccagtaccgcagctggtaccttgcatacaactacggcgaccctcagaccggaatccgctcatggaccctgctttgcactcctgacgtaacctgcggctcggagcaggtctactggtcgttgccagacatgatgcaagaccccgtgaccttccgctccacgcgccagatcagcaactttccggtggtgggcgccgagctgttgcccgtgcactccaagagcttctacaacgaccaggccgtctactcccaactcatccgccagtttacctctctgacccacgtgttcaatcgctttcccgagaaccagattttggcgcgcccgccagcccccaccatcaccaccgtcagtgaaaacgttcctgctctcacagatcacgggacgctaccgctgcgcaacagcatcggaggagtccagcgagtgaccattactgacgccagacgccgcacctgcccctacgtttacaaggccctgggcatagtctcgccgcgcgtcctatcgagccgcactttttgagcaagcatgtccatccttatatcgcccagcaataacacaggctggggcctgcgcttcccaagcaagatgtttggcggggccaagaagcgctccgaccaacacccagtgcgcgtgcgcgggcactaccgcgcgccctggggcgcgcacaaacgcggccgcactgggcgcaccaccgtcgatgacgccatcgacgcggtggtggaggaggcgcgcaactacacgcccacgccgccaccagtgtccacagtggacgcggccattcagaccgtggtgcgcggagcccggcgctatgctaaaatgaagagacggcggaggcgcgtagcacgtcgccaccgccgccgacccggcactgccgcccaacgcgcggcggcggccctgcttaaccgcgcacgtcgcaccggccgacgggcggccatgcgggccgctcgaaggctggccgcgggtattgtcactgtgccccccaggtccaggcgacgagcggccgccgcagcagccgcggccattagtgctatgactcagggtcgcaggggcaacgtgtattgggtgcgcgactcggttagcggcctgcgcgtgcccgtgcgcacccgccccccgcgcaactagattgcaagaaaaaactacttagactcgtactgttgtatgtatccagcggcggcggcgcgcaacgaagctatgtccaagcgcaaaatcaaagaagagatgctccaggtcatcgcgccggagatctatggccccccgaagaaggaagagcaggattacaagccccgaaagctaaagcgggtcaaaaagaaaaagaaagatgatgatgatgaacttgacgacgaggtggaactgctgcacgctaccgcgcccaggcgacgggtacagtggaaaggtcgacgcgtaaaacgtgttttgcgacccggcaccaccgtagtctttacgcccggtgagcgctccacccgcacctacaagcgcgtgtatgatgaggtgtacggcgacgaggacctgcttgagcaggccaacgagcgcctcggggagtttgcctacggaaagcggcataaggacatgctggcgttgccgctggacgagggcaacccaacacctagcctaaagcccgtaacactgcagcaggtgctgcccgcgcttgcaccgtccgaagaaaagcgcggcctaaagcgcgagtctggtgacttggcacccaccgtgcagctgatggtacccaagcgccagcgactggaagatgtcttggaaaaaatgaccgtggaacctgggctggagcccgaggtccgcgtgcggccaatcaagcaggtggcgccgggactgggcgtgcagaccgtggacgttcagatacccactaccagtagcaccagtattgccaccgccacagagggcatggagacacaaacgtccccggttgcctcagcggtggcggatgccgcggtgcaggcggtcgctgcggccgcgtccaagacctctacggaggtgcaaacggacccgtggatgtttcgcgtttcagccccccggcgcccgcgcggttcgaggaagtacggcgccgccagcgcgctactgcccgaatatgccctacatccttccattgcgcctacccccggctatcgtggctacacctaccgccccagaagacgagcaactacccgacgccgaaccaccactggaacccgccgccgccgtcgccgtcgccagcccgtgctggccccgatttccgtgcgcagggtggctcgcgaaggaggcaggaccctggtgctgccaacagcgcgctaccaccccagcatcgtttaaaagccggtctttgtggttcttgcagatatggccctcacctgccgcctccgtttcccggtgccgggattccgaggaagaatgcaccgtaggaggggcatggccggccacggcctgacgggcggcatgcgtcgtgcgcaccaccggcggcggcgcgcgtcgcaccgtcgcatgcgcggcggtatcctgcccctccttattccactgatcgccgcggcgattggcgccgtgcccggaattgcatccgtggccttgcaggcgcagagacactgattaaaaacaagttgcatgtggaaaaatcaaaataaaaagtctggactctcacgctcgcttggtcctgtaactattttgtagaatggaagacatcaactttgcgtctctggccccgcgacacggctcgcgcccgttcatgggaaactggcaagatatcggcaccagcaatatgagcggtggcgccttcagctggggctcgctgtggagcggcattaaaaatttcggttccaccgttaagaactatggcagcaaggcctggaacagcagcacaggccagatgctgagggataagttgaaagagcaaaatttccaacaaaaggtggtagatggcctggcctctggcattagcggggtggtggacctggccaaccaggcagtgcaaaataagattaacagtaagcttgatccccgccctcccgtagaggagcctccaccggccgtggagacagtgtctccagaggggcgtggcgaaaagcgtccgcgccccgacagggaagaaactctggtgacgcaaatagacgagcctccctcgtacgaggaggcactaaagcaaggcctgcccaccacccgtcccatcgcgcccatggctaccggagtgctgggccagcacacacccgtaacgctggacctgcctccccccgccgacacccagcagaaacctgtgctgccaggcccgaccgccgttgttgtaacccgtcctagccgcgcgtccctgcgccgcgccgccagcggtccgcgatcgttgcggcccgtagccagtggcaactggcaaagcacactgaacagcatcgtgggtctgggggtgcaatccctgaagcgccgacgatgcttctgaatagctaacgtgtcgtatgtgtgtcatgtatgcgtccatgtcgccgccagaggagctgctgagccgccgcgcgcccgctttccaagatggctaccccttcgatgatgccgcagtggtcttacatgcacatctcgggccaggacgcctcggagtacctgagccccgggctggtgcagtttgcccgcgccaccgagacgtacttcagcctgaataacaagtttagaaaccccacggtggcgcctacgcacgacgtgaccacagaccggtcccagcgtttgacgctgcggttcatccctgtggaccgtgaggatactgcgtactcgtacaaggcgcggttcaccctagctgtgggtgataaccgtgtgctggacatggcttccacgtactttgacatccgcggcgtgctggacaggggccctacttttaagccctactctggcactgcctacaacgccctggctcccaagggtgccccaaatccttgcgaatgggatgaagctgctactgctcttgaaataaacctagaagaagaggacgatgacaacgaagacgaagtagacgagcaagctgagcagcaaaaaactcacgtatttgggcaggcgccttattctggtataaatattacaaaggagggtattcaaataggtgtcgaaggtcaaacacctaaatatgccgataaaacatttcaacctgaacctcaaataggagaatctcagtggtacgaaactgaaattaatcatgcagctgggagagtccttaaaaagactaccccaatgaaaccatgttacggttcatatgcaaaacccacaaatgaaaatggagggcaaggcattcttgtaaagcaacaaaatggaaagctagaaagtcaagtggaaatgcaatttttctcaactactgaggcgaccgcaggcaatggtgataacttgactcctaaagtggtattgtacagtgaagatgtagatatagaaaccccagacactcatatttcttacatgcccactattaaggaaggtaactcacgagaactaatgggccaacaatctatgcccaacaggcctaattacattgcttttagggacaattttattggtctaatgtattacaacagcacgggtaatatgggtgttctggcgggccaagcatcgcagttgaatgctgttgtagatttgcaagacagaaacacagagctttcataccagcttttgcttgattccattggtgatagaaccaggtacttttctatgtggaatcaggctgttgacagctatgatccagatgttagaattattgaaaatcatggaactgaagatgaacttccaaattactgctttccactgggaggtgtgattaatacagagactcttaccaaggtaaaacctaaaacaggtcaggaaaatggatgggaaaaagatgctacagaattttcagataaaaatgaaataagagttggaaataattttgccatggaaatcaatctaaatgccaacctgtggagaaatttcctgtactccaacatagcgctgtatttgcccgacaagctaaagtacagtccttccaacgtaaaaatttctgataacccaaacacctacgactacatgaacaagcgagtggtggctcccgggttagtggactgctacattaaccttggagcacgctggtcccttgactatatggacaacgtcaacccatttaaccaccaccgcaatgctggcctgcgctaccgctcaatgttgctgggcaatggtcgctatgtgcccttccacatccaggtgcctcagaagttctttgccattaaaaacctccttctcctgccgggctcatacacctacgagtggaacttcaggaaggatgttaacatggttctgcagagctccctaggaaatgacctaagggttgacggagccagcattaagtttgatagcatttgcctttacgccaccttcttccccatggcccacaacaccgcctccacgcttgaggccatgcttagaaacgacaccaacgaccagtcctttaacgactatctctccgccgccaacatgctctaccctatacccgccaacgctaccaacgtgcccatatccatcccctcccgcaactgggcggctttccgcggctgggccttcacgcgccttaagactaaggaaaccccatcactgggctcgggctacgacccttattacacctactctggctctataccctacctagatggaaccttttacctcaaccacacctttaagaaggtggccattacctttgactcttctgtcagctggcctggcaatgaccgcctgcttacccccaacgagtttgaaattaagcgctcagttgacggggagggttacaacgttgcccagtgtaacatgaccaaagactggttcctggtacaaatgctagctaactacaacattggctaccagggcttctatatcccagagagctacaaggaccgcatgtactccttctttagaaacttccagcccatgagccgtcaggtggtggatgatactaaatacaaggactaccaacaggtgggcatcctacaccaacacaacaactctggatttgttggctaccttgcccccaccatgcgcgaaggacaggcctaccctgctaacttcccctatccgcttataggcaagaccgcagttgacagcattacccagaaaaagtttctttgcgatcgcaccctttggcgcatcccattctccagtaactttatgtccatgggcgcactcacagacctgggccaaaaccttctctacgccaactccgcccacgcgctagacatgacttttgaggtggatcccatggacgagcccacccttctttatgttttgtttgaagtctttgacgtggtccgtgtgcaccggccgcaccgcggcgtcatcgaaaccgtgtacctgcgcacgcccttctcggccggcaacgccacaacataaagaagcaagcaacatcaacaacagctgccgccatgggctccagtgagcaggaactgaaagccattgtcaaagatcttggttgtgggccatattttttgggcacctatgacaagcgctttccaggctttgtttctccacacaagctcgcctgcgccatagtcaatacggccggtcgcgagactgggggcgtacactggatggcctttgcctggaacccgcactcaaaaacatgctacctctttgagccctttggcttttctgaccagcgactcaagcaggtttaccagtttgagtacgagtcactcctgcgccgtagcgccattgcttcttcccccgaccgctgtataacgctggaaaagtccacccaaagcgtacaggggcccaactcggccgcctgtggactattctgctgcatgtttctccacgcctttgccaactggccccaaactcccatggatcacaaccccaccatgaaccttattaccggggtacccaactccatgctcaacagtccccaggtacagcccaccctgcgtcgcaaccaggaacagctctacagcttcctggagcgccactcgccctacttccgcagccacagtgcgcagattaggagcgccacttctttttgtcacttgaaaaacatgtaaaaataatgtactagagacactttcaataaaggcaaatgcttttatttgtacactctcgggtgattatttacccccacccttgccgtctgcgccgtttaaaaatcaaaggggttctgccgcgcatcgctatgcgccactggcagggacacgttgcgatactggtgtttagtgctccacttaaactcaggcacaaccatccgcggcagctcggtgaagttttcactccacaggctgcgcaccatcaccaacgcgtttagcaggtcgggcgccgatatcttgaagtcgcagttggggcctccgccctgcgcgcgcgagttgcgatacacagggttgcagcactggaacactatcagcgccgggtggtgcacgctggccagcacgctcttgtcggagatcagatccgcgtccaggtcctccgcgttgctcagggcgaacggagtcaactttggtagctgccttcccaaaaagggcgcgtgcccaggctttgagttgcactcgcaccgtagtggcatcaaaaggtgaccgtgcccggtctgggcgttaggatacagcgcctgcataaaagccttgatctgcttaaaagccacctgagcctttgcgccttcagagaagaacatgccgcaagacttgccggaaaactgattggccggacaggccgcgtcgtgcacgcagcaccttgcgtcggtgttggagatctgcaccacatttcggccccaccggttcttcacgatcttggccttgctagactgctccttcagcgcgcgctgcccgttttcgctcgtcacatccatttcaatcacgtgctccttatttatcataatgcttccgtgtagacacttaagctcgccttcgatctcagcgcagcggtgcagccacaacgcgcagcccgtgggctcgtgatgcttgtaggtcacctctgcaaacgactgcaggtacgcctgcaggaatcgccccatcatcgtcacaaaggtcttgttgctggtgaaggtcagctgcaacccgcggtgctcctcgttcagccaggtcttgcatacggccgccagagcttccacttggtcaggcagtagtttgaagttcgcctttagatcgttatccacgtggtacttgtccatcagcgcgcgcgcagcctccatgcccttctcccacgcagacacgatcggcacactcagcgggttcatcaccgtaatttcactttccgcttcgctgggctcttcctcttcctcttgcgtccgcataccacgcgccactgggtcgtcttcattcagccgccgcactgtgcgcttacctcctttgccatgcttgattagcaccggtgggttgctgaaacccaccatttgtagcgccacatcttctctttcttcctcgctgtccacgattacctctggtgatggcgggcgctcgggcttgggagaagggcgcttctttttcttcttgggcgcaatggccaaatccgccgccgaggtcgatggccgcgggctgggtgtgcgcggcaccagcgcgtcttgtgatgagtcttcctcgtcctcggactcgatacgccgcctcatccgcttttttgggggcgcccggggaggcggcggcgacggggacggggacgacacgtcctccatggttgggggacgtcgcgccgcaccgcgtccgcgctcgggggtggtttcgcgctgctcctcttcccgactggccatttccttctcctataggcagaaaaagatcatggagtcagtcgagaagaaggacagcctaaccgccccctctgagttcgccaccaccgcctccaccgatgccgccaacgcgcctaccaccttccccgtcgaggcacccccgcttgaggaggaggaagtgattatcgagcaggacccaggttttgtaagcgaagacgacgaggaccgctcagtaccaacagaggataaaaagcaagaccaggacaacgcagaggcaaacgaggaacaagtcgggcggggggacgaaaggcatggcgactacctagatgtgggagacgacgtgctgttgaagcatctgcagcgccagtgcgccattatctgcgacgcgttgcaagagcgcagcgatgtgcccctcgccatagcggatgtcagccttgcctacgaacgccacctattctcaccgcgcgtaccccccaaacgccaagaaaacggcacatgcgagcccaacccgcgcctcaacttctaccccgtatttgccgtgccagaggtgcttgccacctatcacatctttttccaaaactgcaagatacccctatcctgccgtgccaaccgcagccgagcggacaagcagctggccttgcggcagggcgctgtcatacctgatatcgcctcgctcaacgaagtgccaaaaatctttgagggtcttggacgcgacgagaagcgcgcggcaaacgctctgcaacaggaaaacagcgaaaatgaaagtcactctggagtgttggtggaactcgagggtgacaacgcgcgcctagccgtactaaaacgcagcatcgaggtcacccactttgcctacccggcacttaacctaccccccaaggtcatgagcacagtcatgagtgagctgatcgtgcgccgtgcgcagcccctggagagggatgcaaatttgcaagaacaaacagaggagggcctacccgcagttggcgacgagcagctagcgcgctggcttcaaacgcgcgagcctgccgacttggaggagcgacgcaaactaatgatggccgcagtgctcgttaccgtggagcttgagtgcatgcagcggttctttgctgacccggagatgcagcgcaagctagaggaaacattgcactacacctttcgacagggctacgtacgccaggcctgcaagatctccaacgtggagctctgcaacctggtctcctaccttggaattttgcacgaaaaccgccttgggcaaaacgtgcttcattccacgctcaagggcgaggcgcgccgcgactacgtccgcgactgcgtttacttatttctatgctacacctggcagacggccatgggcgtttggcagcagtgcttggaggagtgcaacctcaaggagctgcagaaactgctaaagcaaaacttgaaggacctatggacggccttcaacgagcgctccgtggccgcgcacctggcggacatcattttccccgaacgcctgcttaaaaccctgcaacagggtctgccagacttcaccagtcaaagcatgttgcagaactttaggaactttatcctagagcgctcaggaatcttgcccgccacctgctgtgcacttcctagcgactttgtgcccattaagtaccgcgaatgccctccgccgctttggggccactgctaccttctgcagctagccaactaccttgcctaccactctgacataatggaagacgtgagcggtgacggtctactggagtgtcactgtcgctgcaacctatgcaccccgcaccgctccctggtttgcaattcgcagctgcttaacgaaagtcaaattatcggtacctttgagctgcagggtccctcgcctgacgaaaagtccgcggctccggggttgaaactcactccggggctgtggacgtcggcttaccttcgcaaatttgtacctgaggactaccacgcccacgagattaggttctacgaagaccaatcccgcccgccaaatgcggagcttaccgcctgcgtcattacccagggccacattcttggccaattgcaagccatcaacaaagcccgccaagagtttctgctacgaaagggacggggggtttacttggacccccagtccggcgaggagctcaacccaatccccccgccgccgcagccctatcagcagcagccgcgggcccttgcttcccaggatggcacccaaaaagaagctgcagctgccgccgccacccacggacgaggaggaatactgggacagtcaggcagaggaggttttggacgaggaggaggaggacatgatggaagactgggagagcctagacgaggaagcttccgaggtcgaagaggtgtcagacgaaacaccgtcaccctcggtcgcattcccctcgccggcgccccagaaatcggcaaccggttccagcatggctacaacctccgctcctcaggcgccgccggcactgcccgttcgccgacccaaccgtagatgggacaccactggaaccagggccggtaagtccaagcagccgccgccgttagcccaagagcaacaacagcgccaaggctaccgctcatggcgcgggcacaagaacgccatagttgcttgcttgcaagactgtgggggcaacatctccttcgcccgccgctttcttctctaccatcacggcgtggccttcccccgtaacatcctgcattactaccgtcatctctacagcccatactgcaccggcggcagcggcagcggcagcaacagcagcggccacacagaagcaaaggcgaccggatagcaagactctgacaaagcccaagaaatccacagcggcggcagcagcaggaggaggagcgctgcgtctggcgcccaacgaacccgtatcgacccgcgagcttagaaacaggatttttcccactctgtatgctatatttcaacagagcaggggccaagaacaagagctgaaaataaaaaacaggtctctgcgatccctcacccgcagctgcctgtatcacaaaagcgaagatcagcttcggcgcacgctggaagacgcggaggctctcttcagtaaatactgcgcgctgactcttaaggactagtttcgcgccctttctcaaatttaagcgcgaaaactacgtcatctccagcggccacacccggcgccagcacctgtcgtcagcgccattatgagcaaggaaattcccacgccctacatgtggagttaccagccacaaatgggacttgcggctggagctgcccaagactactcaacccgaataaactacatgagcgcgggaccccacatgatatcccgggtcaacggaatccgcgcccaccgaaaccgaattctcttggaacaggcggctattaccaccacacctcgtaataaccttaatccccgtagttggcccgctgccctggtgtaccaggaaagtcccgctcccaccactgtggtacttcccagagacgcccaggccgaagttcagatgactaactcaggggcgcagcttgcgggcggctttcgtcacagggtgcggtcgcccgggcagggtataactcacctgacaatcagagggcgaggtattcagctcaacgacgagtcggtgagctcctcgcttggtctccgtccggacgggacatttcagatcggcggcgccggccgctcttcattcacgcctcgtcaggcaatcctaactctgcagacctcgtcctctgagccgcgctctggaggcattggaactctgcaatttattgaggagtttgtgccatcggtctactttaaccccttctcgggacctcccggccactatccggatcaatttattcctaactttgacgcggtaaaggactcggcggatggctacgactgaatgttaagtggagaggcagagcaactgcgcctgaaacacctggtccactgtcgccgccacaagtgctttgcccgcgactccggtgagttttgctactttgaattgcccgaggatcatatcgagggcccggcgcacggcgtccggcttaccgcccagggagagcttgcccgtagcctgattcgggagtttacccagcgccccctgctagttgagcgggacaggggaccctgtgttctcactgtgatttgcaactgtcctaaccctggattacatcaagatctttgttgccatctctgtgctgagtataataaatacagaaattaaaatatactggggctcctatcgccatcctgtaaacgccaccgtcttcacccgcccaagcaaaccaaggcgaaccttacctggtacttttaacatctctccctctgtgatttacaacagtttcaacccagacggagtgagtctacgagagaacctctccgagctcagctactccatcagaaaaaacaccaccctccttacctgccgggaacgtacgacctagggataacagggtaataagcaattgactctatgtgggatatgctccagcgctacaaccttgaagtcaggcttcctggatgtcagcatctgactttggccagcacctgtcccgcggatttgttccagtccaactacagcgacccaccctaacagagatgaccaacacaaccaacgcggccgccgctaccggacttacatctaccacaaatacaccccaagtttctgcctttgtcaataactgggataacttgggcatgtggtggttctccatagcgcttatgtttgtatgccttattattatgtggctcatctgctgcctaaagcgcaaacgcgcccgaccacccatctatagtcccatcattgtgctacacccaaacaatgatggaatccatagattggacggactgaaacacatgttcttttctcttacagtatgattaaatgagacatgattcctcgagtttttatattactgacccttgttgcgcttttttgtgcgtgctccacattggctgcggtttctcacatcgaagtagactgcattccagccttcacagtctatttgctttacggatttgtcaccctcacgctcatctgcagcctcatcactgtggtcatcgcctttatccagtgcattgactgggtctgtgtgcgctttgcatatctcagacaccatccccagtacagggacaggactatagctgagcttcttagaattctttaattatgaaatttactgtgacttttctgctgattatttgcaccctatctgcgttttgttccccgacctccaagcctcaaagacatatatcatgcagattcactcgtatatggaatattccaagttgctacaatgaaaaaagcgatctttccgaagcctggttatatgcaatcatctctgttatggtgttctgcagtaccatcttagccctagctatatatccctaccttgacattggctggaaacgaatagatgccatgaaccacccaactttccccgcgcccgctatgcttccactgcaacaagttgttgccggcggctttgtcccagccaatcagcctcgccccacttctcccacccccactgaaatcagctactttaatctaacaggaggagatgactgacaccctagatctagaaatggacggaattattacagagcagcgcctgctagaaagacgcagggcagcggccgagcaacagcgcatgaatcaagagctccaagacatggttaacttgcaccagtgcaaaaggggtatcttttgtctggtaaagcaggccaaagtcacctacgacagtaataccaccggacaccgccttagctacaagttgccaaccaagcgtcagaaattggtggtcatggtgggagaaaagcccattaccataactcagcactcggtagaaaccgaaggctgcattcactcaccttgtcaaggacctgaggatctctgcacccttattaagaccctgtgcggtctcaaagatcttattccctttaactaataaaaaaaaataataaagcatcacttacttaaaatcagttagcaaatttctgtccagtttattcagcagcacctccttgccctcctcccagctctggtattgcagcttcctcctggctgcaaactttctccacaatctaaatggaatgtcagtttcctcctgttcctgtccatccgcacccactatcttcatgttgttgcagatgaagcgcgcaagaccgtctgaagataccttcaaccccgtgtatccatatgacacggaaaccggtcctccaactgtgccttttcttactcctccctttgtatcccccaatgggtttcaagagagtccccctggggtactctctttgcgcctatccgaacctctagttacctccaatggcatgcttgcgctcaaaatgggcaacggcctctctctggacgaggccggcaaccttacctcccaaaatgtaaccactgtgagcccacctctcaaaaaaaccaagtcaaacataaacctggaaatatctgcacccctcacagttacctcagaagccctaactgtggctgccgccgcacctctaatggtcgcgggcaacacactcaccatgcaatcacaggccccgctaaccgtgcacgactccaaacttagcattgccacccaaggacccctcacagtgtcagaaggaaagctagccctgcaaacatcaggccccctcaccaccaccgatagcagtacccttactatcactgcctcaccccctctaactactgccactggtagcttgggcattgacttgaaagagcccatttatacacaaaatggaaaactaggactaaagtacggggctcctttgcatgtaacagacgacctaaacactttgaccgtagcaactggtccaggtgtgactattaataatacttccttgcaaactaaagttactggagccttgggttttgattcacaaggcaatatgcaacttaatgtagcaggaggactaaggattgattctcaaaacagacgccttatacttgatgttagttatccgtttgatgctcaaaaccaactaaatctaagactaggacagggccctctttttataaactcagcccacaacttggatattaactacaacaaaggcctttacttgtttacagcttcaaacaattccaaaaagcttgaggttaacctaagcactgccaaggggttgatgtttgacgctacagccatagccattaatgcaggagatgggcttgaatttggttcacctaatgcaccaaacacaaatcccctcaaaacaaaaattggccatggcctagaatttgattcaaacaaggctatggttcctaaactaggaactggccttagttttgacagcacaggtgccattacagtaggaaacaaaaataatgataagctaaccctatggacaggtccaaaaccagaagccaactgcataattgaatacgggaaacaaaacccagatagcaaactaactttaatccttgtaaaaaatggaggaattgttaatggatatgtaacgctaatgggagcctcagactacgttaacaccttatttaaaaacaaaaatgtctccattaatgtagaactatactttgatgccactggtcatatattaccagactcatcttctcttaaaacagatctagaactaaaatacaagcaaaccgctgactttagtgcaagaggttttatgccaagtactacagcgtatccatttgtccttcctaatgcgggaacacataatgaaaattatatttttggtcaatgctactacaaagcaagcgatggtgccctttttccgttggaagttactgttatgcttaataaacgcctgccagatagtcgcacatcctatgttatgacttttttatggtccttgaatgctggtctagctccagaaactactcaggcaaccctcataacctccccatttaccttttcctatattagagaagatgactaataaactctaaagaatcgtttgtgttatgtttcaacgtgtttatttttcaattgcagaaaatttcaagtcatttttcattcagtagtatagccccaccaccacatagcttatacagatcaccgtaccttaatcaaactcacagaaccctagtattcaacctgccacctccctcccaacacacagagtacacagtcctttctccccggctggccttaaaaagcatcatatcatgggtaacagacatattcttaggtgttatattccacacggtttcctgtcgagccaaacgctcatcaagtgatattaataaactccccgggcagctcacttaagttcatgtcgctgtccagctgctgagccacaggctgctgtccaacttgcggttgcttaacgggcggcgaaggagaagtccacgcctacatggggggagagtcataatcgtgcatcaggatagggcggtggtgctgcagcagcgcgcgaataaactgctgccgccgccgctccgtcctgcaggaatacaacatggcagtggtctcctcagcgatgattcgcaccgcccgcagcataaggcgcttgtcctccgggcacagcagcgcaccctgatctcacttaaatcagcacagtaactgcagcacagcaccacaatattgttcaaaatcccacagtgcaaggcgctgtatccaaagctcatggcggggaccacagaacccacgtggccatcataccacaagcgcaggtagattaagtggcgacccctcataaacacgctggacataaacattacctcttttggcatgttgtaattcaccacctcccggtaccatataaacctctgattaaacatggcgccatccaccaccatcctaaaccagctggccaaaacctgccccgccgggntatacactgcagggaaccgggacttggacaatgacaagtgggagagcccaggactcgtaaccatggatcatcatgctcgtcatgatatcaatgttggcacaacacaggcacacgtgcatacacttcctcaggattacaagctcctcccgcgttagaaccatatcccagggaacaacccattcctgaatcagcgtaaatcccacactgcagggaagacctcgcacgtaactcacgttgtgcattgtcaaagtgttacattcgggcagcagcggatgatcctccagtatggtagcgcgggtttctgtctcaaaaggaggtagacgatccctactgtacggagtgcgccgagacaaccgagatcgtgttggtcgtagtgtcatgccaaatggaacgccggacgtagtcatatttcctgaagcaaaaccaggtgcgggcgtgacaaacagatctgcgtctccggtctcgccgcttagatcgctctgtgtagtagttgtagtatatccactctctcaaagcatccaggcgccccctggcttcgggttctatgtaaactccttcatgcgccgctgccctgataacatccaccaccgcagaataagccacacccagccaacctacacattcgttctgcgagtcacacacgggaggagcgggaagagctggaagaaccatgtttttttttttattccaaaagattatccaaaacctcaaaatgaagatctattaagtgaacgcgctcccctccggtggcgtggtcaaactctacagccaaagaacagataatggcatttgtaagatgttgcacaatggcttccaaaaggcaaacggccctcacgtccaagtggacgtaaaggctaaacccttcagggtgaatctcctctataaacattccagcaccttcaaccatgcccaaataattctcatctcgccaccttctcaatatatctctaagcaaatcccgaatatttaagtccgggccattgtaaaaaatttggctccagagcgccctccaccttcagcctcaagcagcgaatcatgattgcaaaaattcaggttcctcacagacctgtataagattcaaaagcggaacattaacaaaaataccgcgatcccgtaggtcccttcgcagggccagctgaacataatcgtgcaggtctgcacggaccagcgcggccacttccccgccaggaaccatgacaaaagaacccacactgattatgacacgcatactcggagctatgctaaccagcgtagccccgatgtaagcttgttgcatgggcggcgatataaaatgcaaggtgctgctcaaaaaatcaggcaaagcctcgcgcaaaaaagaaagcacatcgtagtcatgctcatgcagataaaggcaggtaagctccggaaccaccacagaaaaagacaccatttttctctcaaacatgtctgcgggtttctgcataaacacaaaataaaataacaaaaaaacatttaaacattagaagcctgtcttacaacaggaaaaacaacccttataagcataagacggactacggccatgccggcgtgaccgtaaaaaaactggtcaccgtgattaaaaagcaccaccgacagctcctcggtcagtccggagtcataatgtaagactcggtaaacacatcaggttgattcacatcggtcagtgttaaaaagcgaccgaaatagccngggggaatacaatacccgcaggcgtagagacaacattacagcccccataggaggtataacaaaattaataggagagaaaaacacataaacacctgaaaaaccctcctgcctaggcaaaatagcaccctcccgctccagaacaacatacagcgcttccacagcggcagccataacagtcagccttaccagtaaaaaagaaaacctattaaaaaaacaccactcgacacggcaccagctcaatcagtcacagtgtaaaaaagggccaagtgcagagcgagtatatataggactaaaaaatgacggtaacggttaaagtccacaaaaaacacccagaaaaccgcacgcgaacctacgcccagaaacgaaagccaaaaaacccacaacttcctcaaatcgtcacttccgttttcccacgttacgtcacttcccattttaagaaaactacaattcccaacacatacaagttactccgccctaaaacctacgtcacccgccccgttcccacgccccgcgccacgtcacaaactccaccccctcattatcatattggcttcaatccaaaataaggtatattattgatgatgttaattaacatgcatggatcctcgtctcgacgatgcccttgagagccttcaacccagtcagctccttccggtgggcgcggggcatgactatcgtcgccgcacttatgactgtcttctttatcatgcaactcgtaggacaggtgccggcagcgctctgggtcattttcggcgaggaccgctttcgctggagcgcgacgatgatcggcctgtcgcttgcggtattcggaatcttgcacgccctcgctcaagccttcgtcactggtcccgccaccaaacgtttcggcgagaagcaggccattatcgccggcatggcggccgacgcgctgggctacgtcttgctggcgttcgcgacgcgaggctggatggccttccccattatgattcttctcgcttccggcggcatcgggatgcccgcgttgcaggccatgctgtccaggcaggtagatgacgaccatcagggacagcttcaaggatcgctcgcggctcttaccagcctaacttcgatcactggaccgctgatcgtcacggcgatttatgccgcctcggcgagcacatggaacgggttggcatggattgtaggcgccgccctataccttgtctgcctccccgcgttgcgtcgcggtgcatggagccgggccacctcgacctgaatggaagccggcggcacctcgctaacggattcaccactccaagaattggagccaatcaattcttgcggagaactgtgaatgcgcaaaccaacccttggcagaacatatccatcgcgtccgccatctccagcagccgcacgcggcgcatctcgggcagcgttgggtcctggccacgggtgcgcatgatcgtgctcctgtcgttgaggacccggctaggctggcggggttgccttactggttagcagaatgaatcaccgatacgcgagcgaacgtgaagcgactgctgctgcaaaacgtctgcgacctgagcaacaacatgaatggtcttcggtttccgtgtttcgtaaagtctggaaacgcggaagtcagcgccctgcaccattatgttccggatctgcatcgcaggatgctgctggctaccctgtggaacacctacatctgtattaacgaagcgctggcattgaccctgagtgatttttctctggtcccgccgcatccataccgccagttgtttaccctcacaacgttccagtaaccgggcatgttcatcatcagtaacccgtatcgtgagcatcctctctcgtttcatcggtatcattacccccatgaacagaaattcccccttacacggaggcatcaagtgaccaaacaggaaaaaaccgcccttaacatggcccgctttatcagaagccagacattaacgcttctggagaaactcaacgagctggacgcggatgaacaggcagacatctgtgaatcgcttcacgaccacgctgatgagctttaccgcagctgcctcgcgcgtttcggtgatgacggtgaaaacctctgacacatgcagctcccggagacggtcacagcttgtctgtaagcggatgccgggagcagacaagcccgtcagggcgcgtcagcgggtgttggcgggtgtcggggcgcagccatgacccagtcacgtagcgatagcggagtgtatactggcttaactatgcggcatcagagcagattgtactgagagtgcaccatatgcggtgtgaaataccgcacagatgcgtaaggagaaaataccgcatcaggcgctcttccgcttcctcgctcactgactcgctgcgctcggtcgttcggctgcggcgagcggtatcagctcactcaaaggcggtaatacggttatccacagaatcaggggataacgcaggaaagaacatgtgagcaaaaggccagcaaaaggccaggaaccgtaaaaaggccgcgttgctggcgtttttccataggctccgcccccctgacgagcatcacaaaaatcgacgctcaagtcagaggtggcgaaacccgacaggactataaagataccaggcgtttccccctggaagctccctcgtgcgctctcctgttccgaccctgccgcttaccggatacctgtccgcctttctcccttcgggaagcgtggcgctttctcaatgctcacgctgtaggtatctcagttcggtgtaggtcgttcgctccaagctgggctgtgtgcacgaaccccccgttcagcccgaccgctgcgccttatccggtaactatcgtcttgagtccaacccggtaagacacgacttatcgccactggcagcagccactggtaacaggattagcagagcgaggtatgtaggcggtgctacagagttcttgaagtggtggcctaactacggctacactagaaggacagtatttggtatctgcgctctgctgaagccagttaccttcggaaaaagagttggtagctcttgatccggcaaacaaaccaccgctggtagcggtggtttttttgtttgcaagcagcagattacgcgcagaaaaaaaggatctcaagaagatcctttgatcttttctacggggtctgacgctcagtggaacgaaaactcacgttaagggattttggtcatgagattatcaaaaaggatcttcacctagatccttttaaattaaaaatgaagttttaaatcaatctaaagtatatatgagtaaacttggtctgacagttaccaatgcttaatcagtgaggcacctatctcagcgatctgtctatttcgttcatccatagttgcctgactccccgtcgtgtagataactacgatacgggagggcttaccatctggccccagtgctgcaatgataccgcgagacccacgctcaccggctccagatttatcagcaataaaccagccagccggaagggccgagcgcagaagtggtcctgcaactttatccgcctccatccagtctattaattgttgccgggaagctagagtaagtagttcgccagttaatagtttgcgcaacgttggttgnnnnnnaaaaaggatcttcacctagatccttttcacgtagaaagccagtccgcagaaacggtgctgaccccggatgaatgtcagctactgggctatctggacaagggaaaacgcaagcgcaaagagaaagcaggtagcttgcagtgggcttacatggcgatagctagactgggcggttttatggacagcaagcgaaccggaattgccagctggggcgccctctggtaaggttgggaagccctgcaaagtaaactggatggctttctcgccgccaaggatctgatggcgcaggggatcaagctctgatcaagagacaggatgaggatcgtttcgcatgattgaacaagatggattgcacgcaggttctccggccgcttgggtggagaggctattcggctatgactgggcacaacagacaatcggctgctctgatgccgccgtgttccggctgtcagcgcaggggcgcccggttctttttgtcaagaccgacctgtccggtgccctgaatgaactgcaagacgaggcagcgcggctatcgtggctggccacgacgggcgttccttgcgcagctgtgctcgacgttgtcactgaagcgggaagggactggctgctattgggcgaagtgccggggcaggatctcctgtcatctcaccttgctcctgccgagaaagtatccatcatggctgatgcaatgcggcggctgcatacgcttgatccggctacctgcccattcgaccaccaagcgaaacatcgcatcgagcgagcacgtactcggatggaagccggtcttgtcgatcaggatgatctggacgaagagcatcaggggctcgcgccagccgaactgttcgccaggctcaaggcgagcatgcccgacggcgaggatctcgtcgtgacccatggcgatgcctgcttgccgaatatcatggtggaaaatggccgcttttctggattcatcgactgtggccggctgggtgtggcggaccgctatcaggacatagcgttggctacccgtgatattgctgaagagcttggcggcgaatgggctgaccgcttcctcgtgctttacggtatcgccgctcccgattcgcagcgcatcgccttctatcgccttcttgacgagttcttctgaattttgttaaaatttttgttaaatcagctcattttttaaccaataggccgaaatcggcaacatcccttataaatcaaaagaatagaccgcgatagggttgagtgttgttccagtttggaacaagagtccactattaaagaacgtggactccaacgtcaaagggcgaaaaaccgtctatcagggcgatggcccactacgtgaaccatcacccaaatcaagttttttgcggtcgaggtgccgtaaagctctaaatcggaaccctaaagggagcccccgatttagagcttgacggggaaagccggcgaacgtggcgagaaaggaagggaagaaagcgaaaggagcgggcgctagggcgctggcaagtgtagcggtcacgctgcgcgtaaccaccacacccgcgcgcttaatgcgccgctacagggcgcgtccattcgccattcaggatcgaattaattcttaat

SEQ ID NO: 128-129 - skipped (2 entries)

SEQ ID NO: 130 - protein, 580 aa, Homo sapiens CD44v6
MDKFWWHAAWGLCLVPLSLAQIDLNITCRFAGVFHVEKNGRYSISRTEAADLCKAFNSTLPTMAQMEKALSIGFETCRYGFIEGHVVIPRIHPNSICAANNTGVYILTSNTSQYDTYCFNASAPPEEDCTSVTDLPNAFDGPITITIVNRDGTRYVQKGEYRTNPEDIYPSNPTDDDVSSGSSSERSSTSGGYIFYTFSTVHPIPDEDSPWITDSTDRIPATIQATPSSTTEETATQKEQWFGNRWHEGYRQTPKEDSHSTTGTAAASAHTSHPMQGRTTPSPEDSSWTDFFNPISHPMGRGHQAGRRMDMDSSHSITLQPTANPNTGLVEDLDRTGPLSMTTQQSNSQSFSTSHEGLEEDKDHPTTSTLTSSNRNDVTGGRRDPNHSEGSTTLLEGYTSHYPHTKESRTFIPVTSAKTGSFGVTAVTVGDSNSNVNRSLSGDQDTFHPSGGSHTTHGSESDGHSHGSQEGGANTTSGPIRTPQIPEWLIILASLLALALILAVCIAVNSRRRCGQKKKLVINSGNGAVEDRKPSGLNGEASKSQEMVHLVNKESSETPDQFMTADETRNLQNVDMKIGV

SEQ ID NO: 131 - protein, 436 aa, synthetic construct
EVQLQQSGPELKKPGETVKISCKASGYPFTNYGMNWVKQAPGQGLKWMGWINTSTGESTFADDFKGRFDFSLETSANTAYLQINNLKSEDMATYFCARWEVYHGYVPYWGQGTTVTVSSGGGGSGGGGSGGGGSDIQLTQSHKFLSTSVGDRVSITCKASQDVYNAVAWYQQKPGQSPKLLIYSASSRYTGVPSRFTGSGSGPDFTFTISSVQAEDLAVYFCQQHFRTPFTFGSGTKLEIKEPKSCDKTHTCPTRFWVLVVVGGVLACYSLLVTVAFIIFWVRSKRSRLLHSDYMNMTPRRPGPTRKHYQPYAPPRDFAAYRSRVKFSRSADAPAYQQGQNQLYNELNLGRREEYDVLDKRRGRDPEMGGKPQRRKNPQEGLYNELQKDKMAEAYSEIGMKGERRRGKGHDGLYQGLSTATKDTYDALHMQALPPR